European Patent Application EP 4 560 019 A1, published May 28, 2025. Title: siRNA and compositions for prophylactic and therapeutic treatment of ocular retinal conditions. Applicant: Sylentis S.A.U. The sequence listing filed with the application follows.

SEQUENCE LISTING (1436 sequences)

SEQ ID NO: 1 - DNA, 19 bp, synthetic construct
  source 1..19: mol_type = other DNA
cggaattagtgactggatc

SEQ ID NO: 2 - DNA, 19 bp, synthetic construct
  source 1..19: mol_type = other DNA
gtgccaaaatctctctgga

SEQ ID NO: 3 - DNA, 19 bp, synthetic construct
  source 1..19: mol_type = other DNA
tggagcatgtgcgaattca

SEQ ID NO: 4 - DNA, 19 bp, synthetic construct
  source 1..19: mol_type = other DNA
agtgtgccaaaatctctct

SEQ ID NO: 5 - DNA, 19 bp, synthetic construct
  source 1..19: mol_type = other DNA
gagtgtgccaaaatctctc

SEQ ID NO: 6 - DNA, 19 bp, synthetic construct
  source 1..19: mol_type = other DNA
gtgtgccaaaatctctctg

SEQ ID NO: 7 - DNA, 19 bp, synthetic construct
  source 1..19: mol_type = other DNA
gtgactggatccaaggacc

SEQ ID NO: 8 - DNA, 19 bp, synthetic construct
  source 1..19: mol_type = other DNA
gatggagcatgtgcgaatt

SEQ ID NO: 9 - DNA, 19 bp, synthetic construct
  source 1..19: mol_type = other DNA
gaccctcgaaggtggaaga

SEQ ID NO: 10 - DNA, 19 bp, synthetic construct
  source 1..19: mol_type = other DNA
ccggaattagtgactggat

SEQ ID NO: 11 - DNA, 19 bp, synthetic construct
  source 1..19: mol_type = other DNA
ggactacaatgagactcat

SEQ ID NO: 12 - DNA, 19 bp, synthetic construct
  source 1..19: mol_type = other DNA
gccaatgatggagcatgtg

SEQ ID NO: 13 - DNA, 19 bp, synthetic construct
  source 1..19: mol_type = other DNA
ggaattagtgactggatcc

SEQ ID NO: 14 - DNA, 19 bp, synthetic construct
  source 1..19: mol_type = other DNA
acttttgaagaagtggtca

SEQ ID NO: 15 - DNA, 19 bp, synthetic construct
  source 1..19: mol_type = other DNA
tgtgccaaaatctctctgg

SEQ ID NO: 16 - DNA, 19 bp, synthetic construct
  source 1..19: mol_type = other DNA
ttagtgactggatccaagg

SEQ ID NO: 17 - DNA, 19 bp, synthetic construct
  source 1..19: mol_type = other DNA
attagtgactggatccaag

SEQ ID NO: 18 - DNA, 19 bp, synthetic construct
  source 1..19: mol_type = other DNA
ggccaagaaagaccacctt

SEQ ID NO: 19 - DNA, 19 bp, synthetic construct
  source 1..19: mol_type = other DNA
gcaagcctttactcccata

SEQ ID NO: 20 - DNA, 19 bp, synthetic construct
  source 1..19: mol_type = other DNA
accaaagcaagcctttact

SEQ ID NO: 21 - DNA, 19 bp, synthetic construct
  source 1..19: mol_type = other DNA
aagcctttactcccataga

SEQ ID NO: 22 - DNA, 19 bp, synthetic construct
  source 1..19: mol_type = other DNA
agcagatggagttcttgaa

SEQ ID NO: 23 - DNA, 19 bp, synthetic construct
  source 1..19: mol_type = other DNA
catggactacaatgagact

SEQ ID NO: 24 - DNA, 19 bp, synthetic construct
  source 1..19: mol_type = other DNA
gaattagtgactggatcca

SEQ ID NO: 25 - DNA, 19 bp, synthetic construct
  source 1..19: mol_type = other DNA
aattagtgactggatccaa

SEQ ID NO: 26 - DNA, 19 bp, synthetic construct
  source 1..19: mol_type = other DNA
tagtgactggatccaagga

SEQ ID NO: 27 - DNA, 19 bp, synthetic construct
  source 1..19: mol_type = other DNA
agtgactggatccaaggac

SEQ ID NO: 28 - DNA, 19 bp, synthetic construct
  source 1..19: mol_type = other DNA
tgactggatccaaggacca

SEQ ID NO: 29 - DNA, 19 bp, synthetic construct
  source 1..19: mol_type = other DNA
ccaatgatggagcatgtgc

SEQ ID NO: 30 - DNA, 19 bp, synthetic construct
  source 1..19: mol_type = other DNA
caatgatggagcatgtgcg

SEQ ID NO: 31 - DNA, 19 bp, synthetic construct
  source 1..19: mol_type = other DNA
aatgatggagcatgtgcga

SEQ ID NO: 32 - DNA, 19 bp, synthetic construct
  source 1..19: mol_type = other DNA
atgatggagcatgtgcgaa

SEQ ID NO: 33 - DNA, 19 bp, synthetic construct
  source 1..19: mol_type = other DNA
tgatggagcatgtgcgaat

SEQ ID NO: 34 - DNA, 19 bp, synthetic construct
  source 1..19: mol_type = other DNA
atggagcatgtgcgaattc

SEQ ID NO: 35 - DNA, 19 bp, synthetic construct
  source 1..19: mol_type = other DNA
gaactggaccctcgaaggt

SEQ ID NO: 36 - DNA, 19 bp, synthetic construct
  source 1..19: mol_type = other DNA
aactggaccctcgaaggtg

SEQ ID NO: 37 - DNA, 19 bp, synthetic construct
  source 1..19: mol_type = other DNA
actggaccctcgaaggtgg

SEQ ID NO: 38 - DNA, 19 bp, synthetic construct
  source 1..19: mol_type = other DNA
ctggaccctcgaaggtgga

SEQ ID NO: 39 - DNA, 19 bp, synthetic construct
  source 1..19: mol_type = other DNA
tggaccctcgaaggtggaa

SEQ ID NO: 40 - DNA, 19 bp, synthetic construct
  source 1..19: mol_type = other DNA
ggaccctcgaaggtggaag

SEQ ID NO: 41 - DNA, 19 bp, synthetic construct
  source 1..19: mol_type = other DNA
caagcttgtcactgtgacr

SEQ ID NO: 42 - DNA, 19 bp, synthetic construct
  source 1..19: mol_type = other DNA
accaaaacctggctggttg

SEQ ID NO: 43 - DNA, 19 bp, synthetic construct
  source 1..19: mol_type = other DNA
acaccagctggctgatgag

SEQ ID NO: 44 - DNA, 19 bp, synthetic construct
  source 1..19: mol_type = other DNA
ctgcagtgcaggaaagaca

SEQ ID NO: 45 - DNA, 19 bp, synthetic construct
  source 1..19: mol_type = other DNA
gtcatagccatgtggttca

SEQ ID NO: 46 - DNA, 19 bp, synthetic construct
  source 1..19: mol_type = other DNA
accagctggctgatgagcy

SEQ ID NO: 47 - DNA, 19 bp, synthetic construct
  source 1..19: mol_type = other DNA
acaagcttgtcactgtgac

SEQ ID NO: 48 - DNA, 19 bp, synthetic construct
  source 1..19: mol_type = other DNA
caaaacctggctggttggr

SEQ ID NO: 49 - DNA, 19 bp, synthetic construct
  source 1..19: mol_type = other DNA
acaccaacccctccaagtt

SEQ ID NO: 50 - DNA, 19 bp, synthetic construct
  source 1..19: mol_type = other DNA
gcatcaaggtgctggacgt

SEQ ID NO: 51 - DNA, 19 bp, synthetic construct
  source 1..19: mol_type = other DNA
tgcagtgcaggaaagacat

SEQ ID NO: 52 - DNA, 19 bp, synthetic construct
  source 1..19: mol_type = other DNA
tcatcaacaggcagttcta

SEQ ID NO: 53 - DNA, 19 bp, synthetic construct
  source 1..19: mol_type = other DNA
caccagctggctgatgagc

SEQ ID NO: 54 - DNA, 19 bp, synthetic construct
  source 1..19: mol_type = other DNA
ggaccaaaacctggctggt

SEQ ID NO: 55 - DNA, 19 bp, synthetic construct
  source 1..19: mol_type = other DNA
gaccaaaacctggctggtt

SEQ ID NO: 56 - DNA, 19 bp, synthetic construct
  source 1..19: mol_type = other DNA
ccaaaacctggctggttgg

SEQ ID NO: 57 - DNA, 19 bp, synthetic construct
  source 1..19: mol_type = other DNA
aggctgggcagcaggtgtc

SEQ ID NO: 58 - DNA, 19 bp, synthetic construct
  source 1..19: mol_type = other DNA
agttcacctactgctggca

SEQ ID NO: 59 - DNA, 19 bp, synthetic construct
  source 1..19: mol_type = other DNA
gttcacctactgctggcat

SEQ ID NO: 60 - DNA, 19 bp, synthetic construct
  source 1..19: mol_type = other DNA
ccctgatgcccaccaagga

SEQ ID NO: 61 - DNA, 19 bp, synthetic construct
  source 1..19: mol_type = other DNA
cctgatgcccaccaaggat

SEQ ID NO: 62 - DNA, 19 bp, synthetic construct
  source 1..19: mol_type = other DNA
cctactccctgctcttccg

SEQ ID NO: 63 - DNA, 19 bp, synthetic construct
  source 1..19: mol_type = other DNA
ctactccctgctcttccgt

SEQ ID NO: 64 - DNA, 19 bp, synthetic construct
  source 1..19: mol_type = other DNA
ggagaacccgctcagcccc

SEQ ID NO: 65 - RNA, 19 nt, synthetic construct
  source 1..19: mol_type = other RNA
gatccagtcactaattccg

SEQ ID NO: 66 - RNA, 19 nt, synthetic construct
  source 1..19: mol_type = other RNA
tccagagagattttggcac

SEQ ID NO: 67 - RNA, 19 nt, synthetic construct
  source 1..19: mol_type = other RNA
tgaattcgcacatgctcca

SEQ ID NO: 68 - RNA, 19 nt, synthetic construct
  source 1..19: mol_type = other RNA
agagagattttggcacact

SEQ ID NO: 69 - RNA, 19 nt, synthetic construct
  source 1..19: mol_type = other RNA
gagagattttggcacactc

SEQ ID NO: 70 - RNA, 19 nt, synthetic construct
  source 1..19: mol_type = other RNA
cagagagattttggcacac

SEQ ID NO: 71 - RNA, 19 nt, synthetic construct
  source 1..19: mol_type = other RNA
ggtccttggatccagtcac

SEQ ID NO: 72 - RNA, 19 nt, synthetic construct
  source 1..19: mol_type = other RNA
aattcgcacatgctccatc

SEQ ID NO: 73 - RNA, 19 nt, synthetic construct
  source 1..19: mol_type = other RNA
tcttccaccttcgagggtc

SEQ ID NO: 74 - RNA, 19 nt, synthetic construct
  source 1..19: mol_type = other RNA
atccagtcactaattccgg

SEQ ID NO: 75 - RNA, 19 nt, synthetic construct
  source 1..19: mol_type = other RNA
atgagtctcattgtagtcc

SEQ ID NO: 76 - RNA, 19 nt, synthetic construct
  source 1..19: mol_type = other RNA
cacatgctccatcattggc

SEQ ID NO: 77 - RNA, 19 nt, synthetic construct
  source 1..19: mol_type = other RNA
ggatccagtcactaattcc

SEQ ID NO: 78 - RNA, 19 nt, synthetic construct
  source 1..19: mol_type = other RNA
tgaccacttcttcaaaagt

SEQ ID NO: 79 - RNA, 19 nt, synthetic construct
  source 1..19: mol_type = other RNA
ccagagagattttggcaca

SEQ ID NO: 80 - RNA, 19 nt, synthetic construct
  source 1..19: mol_type = other RNA
ccttggatccagtcactaa

SEQ ID NO: 81 - RNA, 19 nt, synthetic construct
  source 1..19: mol_type = other RNA
cttggatccagtcactaat

SEQ ID NO: 82 - RNA, 19 nt, synthetic construct
  source 1..19: mol_type = other RNA
aaggtggtctttcttggcc

SEQ ID NO: 83 - RNA, 19 nt, synthetic construct
  source 1..19: mol_type = other RNA
tatgggagtaaaggcttgc

SEQ ID NO: 84 - RNA, 19 nt, synthetic construct
  source 1..19: mol_type = other RNA
agtaaaggcttgctttggt

SEQ ID NO: 85 - RNA, 19 nt, synthetic construct
  source 1..19: mol_type = other RNA
tctatgggagtaaaggctt

SEQ ID NO: 86 - RNA, 19 nt, synthetic construct
  source 1..19: mol_type = other RNA
ttcaagaactccatctgct

SEQ ID NO: 87 - RNA, 19 nt, synthetic construct
  source 1..19: mol_type = other RNA
agtctcattgtagtccatg

SEQ ID NO: 88 - RNA, 19 nt, synthetic construct
  source 1..19: mol_type = other RNA
tggatccagtcactaattc

SEQ ID NO: 89 - RNA, 19 nt, synthetic construct
  source 1..19: mol_type = other RNA
ttggatccagtcactaatt

SEQ ID NO: 90 - RNA, 19 nt, synthetic construct
  source 1..19: mol_type = other RNA
tccttggatccagtcacta

SEQ ID NO: 91 - RNA, 19 nt, synthetic construct
  source 1..19: mol_type = other RNA
gtccttggatccagtcact

SEQ ID NO: 92 - RNA, 19 nt, synthetic construct
  source 1..19: mol_type = other RNA
tggtccttggatccagtca

SEQ ID NO: 93 - RNA, 19 nt, synthetic construct
  source 1..19: mol_type = other RNA
gcacatgctccatcattgg

SEQ ID NO: 94 - RNA, 19 nt, synthetic construct
  source 1..19: mol_type = other RNA
cgcacatgctccatcattg

SEQ ID NO: 95 - RNA, 19 nt, synthetic construct
  source 1..19: mol_type = other RNA
tcgcacatgctccatcatt

SEQ ID NO: 96 - RNA, 19 nt, synthetic construct
  source 1..19: mol_type = other RNA
ttcgcacatgctccatcat

SEQ ID NO: 97 - RNA, 19 nt, synthetic construct
  source 1..19: mol_type = other RNA
attcgcacatgctccatca

SEQ ID NO: 98 - RNA, 19 nt, synthetic construct
  source 1..19: mol_type = other RNA
gaattcgcacatgctccat

SEQ ID NO: 99 - RNA, 19 nt, synthetic construct
  source 1..19: mol_type = other RNA
accttcgagggtccagttc

SEQ ID NO: 100 - RNA, 19 nt, synthetic construct
  source 1..19: mol_type = other RNA
caccttcgagggtccagtt

SEQ ID NO: 101 - RNA, 19 nt, synthetic construct
  source 1..19: mol_type = other RNA
ccaccttcgagggtccagt

SEQ ID NO: 102 - RNA, 19 nt, synthetic construct
  source 1..19: mol_type = other RNA
tccaccttcgagggtccag

SEQ ID NO: 103 - RNA, 19 nt, synthetic construct
  source 1..19: mol_type = other RNA
ttccaccttcgagggtcca

SEQ ID NO: 104 - RNA, 19 nt, synthetic construct
  source 1..19: mol_type = other RNA
cttccaccttcgagggtcc

SEQ ID NO: 105 - RNA, 19 nt, synthetic construct
  source 1..19: mol_type = other RNA
tgtcacagtgacaagcttg

SEQ ID NO: 106 - RNA, 19 nt, synthetic construct
  source 1..19: mol_type = other RNA
caaccagccaggttttggt

SEQ ID NO: 107 - RNA, 19 nt, synthetic construct
  source 1..19: mol_type = other RNA
ctcatcagccagctggtgt

SEQ ID NO: 108 - RNA, 19 nt, synthetic construct
  source 1..19: mol_type = other RNA
tgtctttcctgcactgcag

SEQ ID NO: 109 - RNA, 19 nt, synthetic construct
  source 1..19: mol_type = other RNA
tgaaccacatggctatgac

SEQ ID NO: 110 - RNA, 19 nt, synthetic construct
  source 1..19: mol_type = other RNA
agctcatcagccagctggt

SEQ ID NO: 111 - RNA, 19 nt, synthetic construct
  source 1..19: mol_type = other RNA
gtcacagtgacaagcttgt

SEQ ID NO: 112 - RNA, 19 nt, synthetic construct
  source 1..19: mol_type = other RNA
tccaaccagccaggttttg

SEQ ID NO: 113 - RNA, 19 nt, synthetic construct
  source 1..19: mol_type = other RNA
aacttggaggggttggtgt

SEQ ID NO: 114 - RNA, 19 nt, synthetic construct
  source 1..19: mol_type = other RNA
acgtccagcaccttgatgc

SEQ ID NO: 115 - RNA, 19 nt, synthetic construct
  source 1..19: mol_type = other RNA
atgtctttcctgcactgca

SEQ ID NO: 116 - RNA, 19 nt, synthetic construct
  source 1..19: mol_type = other RNA
tagaactgcctgttgatga

SEQ ID NO: 117 - RNA, 19 nt, synthetic construct
  source 1..19: mol_type = other RNA
gctcatcagccagctggtg

SEQ ID NO: 118 - RNA, 19 nt, synthetic construct
  source 1..19: mol_type = other RNA
accagccaggttttggtcc

SEQ ID NO: 119 - RNA, 19 nt, synthetic construct
  source 1..19: mol_type = other RNA
aaccagccaggttttggtc

SEQ ID NO: 120 - RNA, 19 nt, synthetic construct
  source 1..19: mol_type = other RNA
ccaaccagccaggttttgg

SEQ ID NO: 121 - RNA, 19 nt, synthetic construct
  source 1..19: mol_type = other RNA
gacacctgctgcccagcct

SEQ ID NO: 122 - RNA, 19 nt, synthetic construct
  source 1..19: mol_type = other RNA
tgccagcagtaggtgaact

SEQ ID NO: 123 - RNA, 19 nt, synthetic construct
  source 1..19: mol_type = other RNA
atgccagcagtaggtgaac

SEQ ID NO: 124 - RNA, 19 nt, synthetic construct
  source 1..19: mol_type = other RNA
tccttggtgggcatcaggg

SEQ ID NO: 125 - RNA, 19 nt, synthetic construct
  source 1..19: mol_type = other RNA
atccttggtgggcatcagg

SEQ ID NO: 126 - RNA, 19 nt, synthetic construct
  source 1..19: mol_type = other RNA
cggaagagcagggagtagg

SEQ ID NO: 127 - RNA, 19 nt, synthetic construct
  source 1..19: mol_type = other RNA
acggaagagcagggagtag

SEQ ID NO: 128 - RNA, 19 nt, synthetic construct
  source 1..19: mol_type = other RNA
ggggctgagcgggttctcc

SEQ ID NO: 129 - RNA, 19 nt, synthetic construct
  source 1..19: mol_type = other RNA
cggaattagtgactggatc

SEQ ID NO: 130 - RNA, 19 nt, synthetic construct
  source 1..19: mol_type = other RNA
gtgccaaaatctctctgga

SEQ ID NO: 131 - RNA, 19 nt, synthetic construct
  source 1..19: mol_type = other RNA
tggagcatgtgcgaattca

SEQ ID NO: 132 - RNA, 19 nt, synthetic construct
  source 1..19: mol_type = other RNA
agtgtgccaaaatctctct

SEQ ID NO: 133 - RNA, 19 nt, synthetic construct
  source 1..19: mol_type = other RNA
gagtgtgccaaaatctctc

SEQ ID NO: 134 - RNA, 19 nt, synthetic construct
  source 1..19: mol_type = other RNA
gtgtgccaaaatctctctg

SEQ ID NO: 135 - RNA, 19 nt, synthetic construct
  source 1..19: mol_type = other RNA
gtgactggatccaaggacc

SEQ ID NO: 136 - RNA, 19 nt, synthetic construct
  source 1..19: mol_type = other RNA
gatggagcatgtgcgaatt

SEQ ID NO: 137 - RNA, 19 nt, synthetic construct
  source 1..19: mol_type = other RNA
gaccctcgaaggtggaaga

SEQ ID NO: 138 - RNA, 19 nt, synthetic construct
  source 1..19: mol_type = other RNA
ccggaattagtgactggat

SEQ ID NO: 139 - RNA, 19 nt, synthetic construct
  source 1..19: mol_type = other RNA
ggactacaatgagactcat

SEQ ID NO: 140 - RNA, 19 nt, synthetic construct
  source 1..19: mol_type = other RNA
gccaatgatggagcatgtg

SEQ ID NO: 141 - RNA, 19 nt, synthetic construct
  source 1..19: mol_type = other RNA
ggaattagtgactggatcc

SEQ ID NO: 142 - RNA, 19 nt, synthetic construct
  source 1..19: mol_type = other RNA
acttttgaagaagtggtca

SEQ ID NO: 143 - RNA, 19 nt, synthetic construct
  source 1..19: mol_type = other RNA
tgtgccaaaatctctctgg

SEQ ID NO: 144 - RNA, 19 nt, synthetic construct
  source 1..19: mol_type = other RNA
ttagtgactggatccaagg

SEQ ID NO: 145 - RNA, 19 nt, synthetic construct
  source 1..19: mol_type = other RNA
attagtgactggatccaag

SEQ ID NO: 146 - RNA, 19 nt, synthetic construct
  source 1..19: mol_type = other RNA
ggccaagaaagaccacctt

SEQ ID NO: 147 - RNA, 19 nt, synthetic construct
  source 1..19: mol_type = other RNA
gcaagcctttactcccata

SEQ ID NO: 148 - RNA, 19 nt, synthetic construct
  source 1..19: mol_type = other RNA
accaaagcaagcctttact

SEQ ID NO: 149 - RNA, 19 nt, synthetic construct
  source 1..19: mol_type = other RNA
aagcctttactcccataga

SEQ ID NO: 150 - RNA, 19 nt, synthetic construct
  source 1..19: mol_type = other RNA
agcagatggagttcttgaa

SEQ ID NO: 151 - RNA, 19 nt, synthetic construct
  source 1..19: mol_type = other RNA
catggactacaatgagact

SEQ ID NO: 152 - RNA, 19 nt, synthetic construct
  source 1..19: mol_type = other RNA
gaattagtgactggatcca

SEQ ID NO: 153 - RNA, 19 nt, synthetic construct
  source 1..19: mol_type = other RNA
aattagtgactggatccaa

SEQ ID NO: 154 - RNA, 19 nt, synthetic construct
  source 1..19: mol_type = other RNA
tagtgactggatccaagga

SEQ ID NO: 155 - RNA, 19 nt, synthetic construct
  source 1..19: mol_type = other RNA
agtgactggatccaaggac

SEQ ID NO: 156 - RNA, 19 nt, synthetic construct
  source 1..19: mol_type = other RNA
tgactggatccaaggacca

SEQ ID NO: 157 - RNA, 19 nt, synthetic construct
  source 1..19: mol_type = other RNA
ccaatgatggagcatgtgc

SEQ ID NO: 158 - RNA, 19 nt, synthetic construct
  source 1..19: mol_type = other RNA
caatgatggagcatgtgcg

SEQ ID NO: 159 - RNA, 19 nt, synthetic construct
  source 1..19: mol_type = other RNA
aatgatggagcatgtgcga

SEQ ID NO: 160 - RNA, 19 nt, synthetic construct
  source 1..19: mol_type = other RNA
atgatggagcatgtgcgaa

SEQ ID NO: 161 - RNA, 19 nt, synthetic construct
  source 1..19: mol_type = other RNA
tgatggagcatgtgcgaat

SEQ ID NO: 162 - RNA, 19 nt, synthetic construct
  source 1..19: mol_type = other RNA
atggagcatgtgcgaattc

SEQ ID NO: 163 - RNA, 19 nt, synthetic construct
  source 1..19: mol_type = other RNA
gaactggaccctcgaaggt

SEQ ID NO: 164 - RNA, 19 nt, synthetic construct
  source 1..19: mol_type = other RNA
aactggaccctcgaaggtg

SEQ ID NO: 165 - RNA, 19 nt, synthetic construct
  source 1..19: mol_type = other RNA
actggaccctcgaaggtgg

SEQ ID NO: 166 - RNA, 19 nt, synthetic construct
  source 1..19: mol_type = other RNA
ctggaccctcgaaggtgga

SEQ ID NO: 167 - RNA, 19 nt, synthetic construct
  source 1..19: mol_type = other RNA
tggaccctcgaaggtggaa

SEQ ID NO: 168 - RNA, 19 nt, synthetic construct
  source 1..19: mol_type = other RNA
ggaccctcgaaggtggaag

SEQ ID NO: 169 - RNA, 19 nt, synthetic construct
  source 1..19: mol_type = other RNA
caagcttgtcactgtgaca

SEQ ID NO: 170 - RNA, 19 nt, synthetic construct
  source 1..19: mol_type = other RNA
accaaaacctggctggttg

SEQ ID NO: 171 - RNA, 19 nt, synthetic construct
  source 1..19: mol_type = other RNA
acaccagctggctgatgag

SEQ ID NO: 172 - RNA, 19 nt, synthetic construct
  source 1..19: mol_type = other RNA
ctgcagtgcaggaaagaca

SEQ ID NO: 173 - RNA, 19 nt, synthetic construct
  source 1..19: mol_type = other RNA
gtcatagccatgtggttca

SEQ ID NO: 174 - RNA, 19 nt, synthetic construct
  source 1..19: mol_type = other RNA
accagctggctgatgagct

SEQ ID NO: 175 - RNA, 19 nt, synthetic construct
  source 1..19: mol_type = other RNA
acaagcttgtcactgtgac

SEQ ID NO: 176 - RNA, 19 nt, synthetic construct
  source 1..19: mol_type = other RNA
caaaacctggctggttgga

SEQ ID NO: 177 - RNA, 19 nt, synthetic construct
  source 1..19: mol_type = other RNA
acaccaacccctccaagtt

SEQ ID NO: 178 - RNA, 19 nt, synthetic construct
  source 1..19: mol_type = other RNA
gcatcaaggtgctggacgt

SEQ ID NO: 179 - RNA, 19 nt, synthetic construct
  source 1..19: mol_type = other RNA
tgcagtgcaggaaagacat

SEQ ID NO: 180 - RNA, 19 nt, synthetic construct
  source 1..19: mol_type = other RNA
tcatcaacaggcagttcta

SEQ ID NO: 181 - RNA, 19 nt, synthetic construct
  source 1..19: mol_type = other RNA
caccagctggctgatgagc

SEQ ID NO: 182 - RNA, 19 nt, synthetic construct
  source 1..19: mol_type = other RNA
ggaccaaaacctggctggt

SEQ ID NO: 183 - RNA, 19 nt, synthetic construct
  source 1..19: mol_type = other RNA
gaccaaaacctggctggtt

SEQ ID NO: 184 - RNA, 19 nt, synthetic construct
  source 1..19: mol_type = other RNA
ccaaaacctggctggttgg

SEQ ID NO: 185 - RNA, 19 nt, synthetic construct
  source 1..19: mol_type = other RNA
aggctgggcagcaggtgtc

SEQ ID NO: 186 - RNA, 19 nt, synthetic construct
  source 1..19: mol_type = other RNA
agttcacctactgctggca

SEQ ID NO: 187 - RNA, 19 nt, synthetic construct
  source 1..19: mol_type = other RNA
gttcacctactgctggcat

SEQ ID NO: 188 - RNA, 19 nt, synthetic construct
  source 1..19: mol_type = other RNA
ccctgatgcccaccaagga

SEQ ID NO: 189 - RNA, 19 nt, synthetic construct
  source 1..19: mol_type = other RNA
cctgatgcccaccaaggat

SEQ ID NO: 190 - RNA, 19 nt, synthetic construct
  source 1..19: mol_type = other RNA
cctactccctgctcttccg

SEQ ID NO: 191 - RNA, 19 nt, synthetic construct
  source 1..19: mol_type = other RNA
ctactccctgctcttccgt

SEQ ID NO: 192 - RNA, 19 nt, synthetic construct
  source 1..19: mol_type = other RNA
ggagaacccgctcagcccc

SEQ ID NO: 193 - RNA, 21 nt, synthetic construct
  source 1..21: mol_type = other RNA
tccagagagattttggcactt

SEQ ID NO: 194 - DNA, 21 bp, synthetic construct
  source 1..21: mol_type = other DNA
  misc_feature 1..19: note = RNA
  misc_feature 20..21: note = DNA
tccagagagattttggcactt

SEQ ID NO: 195 - RNA, 21 nt, synthetic construct
  source 1..21: mol_type = other RNA
tccagagagattttggcactt

SEQ ID NO: 196 - DNA, 21 bp, synthetic construct
  source 1..21: mol_type = other DNA
  misc_feature 1..19: note = RNA
  misc_feature 20..21: note = DNA
tccagagagattttggcactt

SEQ ID NO: 197 - RNA, 21 nt, synthetic construct
  source 1..21: mol_type = other RNA
tccagagagattttggcactt

SEQ ID NO: 198 - DNA, 21 bp, synthetic construct
  source 1..21: mol_type = other DNA
  misc_feature 1..19: note = RNA
  misc_feature 20..21: note = DNA
tccagagagattttggcactt

SEQ ID NO: 199 - RNA, 21 nt, synthetic construct
  source 1..21: mol_type = other RNA
tccagagagattttggcactt

SEQ ID NO: 200 - DNA, 21 bp, synthetic construct
  source 1..21: mol_type = other DNA
  misc_feature 1..19: note = RNA
  misc_feature 20..21: note = DNA
tccagagagattttggcactt

SEQ ID NO: 201 - RNA, 21 nt, synthetic construct
  source 1..21: mol_type = other RNA
tgaattcgcacatgctccatt

SEQ ID NO: 202 - DNA, 21 bp, synthetic construct
  source 1..21: mol_type = other DNA
  misc_feature 1..19: note = RNA
  misc_feature 20..21: note = DNA
tgaattcgcacatgctccatt

SEQ ID NO: 203 - RNA, 21 nt, synthetic construct
  source 1..21: mol_type = other RNA
tgaattcgcacatgctccatt

SEQ ID NO: 204 - DNA, 21 bp, synthetic construct
  source 1..21: mol_type = other DNA
  misc_feature 1..19: note = RNA
  misc_feature 20..21: note = DNA
tgaattcgcacatgctccatt

SEQ ID NO: 205 - RNA, 21 nt, synthetic construct
  source 1..21: mol_type = other RNA
tgaattcgcacatgctccatt

SEQ ID NO: 206 - DNA, 21 bp, synthetic construct
  source 1..21: mol_type = other DNA
  misc_feature 1..19: note = RNA
  misc_feature 20..21: note = DNA
tgaattcgcacatgctccatt

SEQ ID NO: 207 - RNA, 21 nt, synthetic construct
  source 1..21: mol_type = other RNA
tgaattcgcacatgctccatt

SEQ ID NO: 208 - DNA, 21 bp, synthetic construct
  source 1..21: mol_type = other DNA
  misc_feature 1..19: note = RNA
  misc_feature 20..21: note = DNA
tgaattcgcacatgctccatt

SEQ ID NO: 209 - RNA, 21 nt, synthetic construct
  source 1..21: mol_type = other RNA
cagagagattttggcacactt

SEQ ID NO: 210 - DNA, 21 bp, synthetic construct
  source 1..21: mol_type = other DNA
  misc_feature 1..19: note = RNA
  misc_feature 20..21: note = DNA
cagagagattttggcacactt

SEQ ID NO: 211 - RNA, 21 nt, synthetic construct
  source 1..21: mol_type = other RNA
cagagagattttggcacactt

SEQ ID NO: 212 - DNA, 21 bp, synthetic construct
  source 1..21: mol_type = other DNA
  misc_feature 1..19: note = RNA
  misc_feature 20..21: note = DNA
cagagagattttggcacactt

SEQ ID NO: 213 - RNA, 21 nt, synthetic construct
  source 1..21: mol_type = other RNA
cagagagattttggcacactt

SEQ ID NO: 214 - DNA, 21 bp, synthetic construct
  source 1..21: mol_type = other DNA
  misc_feature 1..19: note = RNA
  misc_feature 20..21: note = DNA
cagagagattttggcacactt

SEQ ID NO: 215 - RNA, 21 nt, synthetic construct
  source 1..21: mol_type = other RNA
cagagagattttggcacactt

SEQ ID NO: 216 - DNA, 21 bp, synthetic construct
  source 1..21: mol_type = other DNA
  misc_feature 1..19: note = RNA
  misc_feature 20..21: note = DNA
cagagagattttggcacactt

SEQ ID NO: 217 - RNA, 21 nt, synthetic construct
  source 1..21: mol_type = other RNA
ggtccttggatccagtcactt

SEQ ID NO: 218 - DNA, 21 bp, synthetic construct
  source 1..21: mol_type = other DNA
  misc_feature 1..19: note = RNA
  misc_feature 20..21: note = DNA
ggtccttggatccagtcactt

SEQ ID NO: 219 - RNA, 21 nt, synthetic construct
  source 1..21: mol_type = other RNA
ggtccttggatccagtcactt

SEQ ID NO: 220 - DNA, 21 bp, synthetic construct
  source 1..21: mol_type = other DNA
  misc_feature 1..19: note = RNA
  misc_feature 20..21: note = DNA
ggtccttggatccagtcactt

SEQ ID NO: 221 - RNA, 21 nt, synthetic construct
  source 1..21: mol_type = other RNA
ggtccttggatccagtcactt

SEQ ID NO: 222 - DNA, 21 bp, synthetic construct
  source 1..21: mol_type = other DNA
  misc_feature 1..19: note = RNA
  misc_feature 20..21: note = DNA
ggtccttggatccagtcactt

SEQ ID NO: 223 - RNA, 21 nt, synthetic construct
  source 1..21: mol_type = other RNA
ggtccttggatccagtcactt

SEQ ID NO: 224 - DNA, 21 bp, synthetic construct
  source 1..21: mol_type = other DNA
  misc_feature 1..19: note = RNA
  misc_feature 20..21: note = DNA
ggtccttggatccagtcactt

SEQ ID NO: 225 - RNA, 21 nt, synthetic construct
  source 1..21: mol_type = other RNA
aattcgcacatgctccatctt

SEQ ID NO: 226 - DNA, 21 bp, synthetic construct
  source 1..21: mol_type = other DNA
  misc_feature 1..19: note = RNA
  misc_feature 20..21: note = DNA
aattcgcacatgctccatctt

SEQ ID NO: 227 - RNA, 21 nt, synthetic construct
  source 1..21: mol_type = other RNA
aattcgcacatgctccatctt

SEQ ID NO: 228 - DNA, 21 bp, synthetic construct
  source 1..21: mol_type = other DNA
  misc_feature 1..19: note = RNA
  misc_feature 20..21: note = DNA
aattcgcacatgctccatctt

SEQ ID NO: 229 - RNA, 21 nt, synthetic construct
  source 1..21: mol_type = other RNA
aattcgcacatgctccatctt

SEQ ID NO: 230 - DNA, 21 bp, synthetic construct
  source 1..21: mol_type = other DNA
  misc_feature 1..19: note = RNA
  misc_feature 20..21: note = DNA
aattcgcacatgctccatctt

SEQ ID NO: 231 - RNA, 21 nt, synthetic construct
  source 1..21: mol_type = other RNA
aattcgcacatgctccatctt

SEQ ID NO: 232 - DNA, 21 bp, synthetic construct
  source 1..21: mol_type = other DNA
  misc_feature 1..19: note = RNA
  misc_feature 20..21: note = DNA
aattcgcacatgctccatctt

SEQ ID NO: 233 - RNA, 21 nt, synthetic construct
  source 1..21: mol_type = other RNA
tcttccaccttcgagggtctt

SEQ ID NO: 234 - DNA, 21 bp, synthetic construct
  source 1..21: mol_type = other DNA
  misc_feature 1..19: note = RNA
  misc_feature 20..21: note = DNA
tcttccaccttcgagggtctt

SEQ ID NO: 235 - RNA, 21 nt, synthetic construct
  source 1..21: mol_type = other RNA
tcttccaccttcgagggtctt

SEQ ID NO: 236 - DNA, 21 bp, synthetic construct
  source 1..21: mol_type = other DNA
  misc_feature 1..19: note = RNA
  misc_feature 20..21: note = DNA
tcttccaccttcgagggtctt

SEQ ID NO: 237 - RNA, 21 nt, synthetic construct
  source 1..21: mol_type = other RNA
tcttccaccttcgagggtctt

SEQ ID NO: 238 - DNA, 21 bp, synthetic construct
  source 1..21: mol_type = other DNA
  misc_feature 1..19: note = RNA
  misc_feature 20..21: note = DNA
tcttccaccttcgagggtctt

SEQ ID NO: 239 - RNA, 21 nt, synthetic construct
  source 1..21: mol_type = other RNA
tcttccaccttcgagggtctt

SEQ ID NO: 240 - DNA, 21 bp, synthetic construct
  source 1..21: mol_type = other DNA
  misc_feature 1..19: note = RNA
  misc_feature 20..21: note = DNA
tcttccaccttcgagggtctt

SEQ ID NO: 241 - RNA, 21 nt, synthetic construct
  source 1..21: mol_type = other RNA
ggatccagtcactaattcctt

SEQ ID NO: 242 - DNA, 21 bp, synthetic construct
  source 1..21: mol_type = other DNA
  misc_feature 1..19: note = RNA
  misc_feature 20..21: note = DNA
ggatccagtcactaattcctt

SEQ ID NO: 243 - RNA, 21 nt, synthetic construct
  source 1..21: mol_type = other RNA
ggatccagtcactaattcctt

SEQ ID NO: 244 - DNA, 21 bp, synthetic construct
  source 1..21: mol_type = other DNA
  misc_feature 1..19: note = RNA
  misc_feature 20..21: note = DNA
ggatccagtcactaattcctt

SEQ ID NO: 245 - RNA, 21 nt, synthetic construct
  source 1..21: mol_type = other RNA
ggatccagtcactaattcctt

SEQ ID NO: 246 - DNA, 21 bp, synthetic construct
  source 1..21: mol_type = other DNA
  misc_feature 1..19: note = RNA
  misc_feature 20..21: note = DNA
ggatccagtcactaattcctt

SEQ ID NO: 247 - RNA, 21 nt, synthetic construct
  source 1..21: mol_type = other RNA
ggatccagtcactaattcctt

SEQ ID NO: 248 - DNA, 21 bp, synthetic construct
  source 1..21: mol_type = other DNA
  misc_feature 1..19: note = RNA
  misc_feature 20..21: note = DNA
ggatccagtcactaattcctt

SEQ ID NO: 249 - RNA, 21 nt, synthetic construct
  source 1..21: mol_type = other RNA
ccagagagattttggcacatt

SEQ ID NO: 250 - DNA, 21 bp, synthetic construct
  source 1..21: mol_type = other DNA
  misc_feature 1..19: note = RNA
  misc_feature 20..21: note = DNA
ccagagagattttggcacatt

SEQ ID NO: 251 - RNA, 21 nt, synthetic construct
  source 1..21: mol_type = other RNA
ccagagagattttggcacatt

SEQ ID NO: 252 - DNA, 21 bp, synthetic construct
  source 1..21: mol_type = other DNA
  misc_feature 1..19: note = RNA
  misc_feature 20..21: note = DNA
ccagagagattttggcacatt

SEQ ID NO: 253 - RNA, 21 nt, synthetic construct
  source 1..21: mol_type = other RNA
ccagagagattttggcacatt

SEQ ID NO: 254 - DNA, 21 bp, synthetic construct
  source 1..21: mol_type = other DNA
  misc_feature 1..19: note = RNA
  misc_feature 20..21: note = DNA
ccagagagattttggcacatt

SEQ ID NO: 255 - RNA, 21 nt, synthetic construct
  source 1..21: mol_type = other RNA
ccagagagattttggcacatt

SEQ ID NO: 256 - DNA, 21 bp, synthetic construct
  source 1..21: mol_type = other DNA
  misc_feature 1..19: note = RNA
  misc_feature 20..21: note = DNA
ccagagagattttggcacatt

SEQ ID NO: 257 - RNA, 21 nt, synthetic construct
  source 1..21: mol_type = other RNA
ccttggatccagtcactaatt

SEQ ID NO: 258 - DNA, 21 bp, synthetic construct
  source 1..21: mol_type = other DNA
  misc_feature 1..19: note = RNA
  misc_feature 20..21: note = DNA
ccttggatccagtcactaatt

SEQ ID NO: 259 - RNA, 21 nt, synthetic construct
  source 1..21: mol_type = other RNA
ccttggatccagtcactaatt

SEQ ID NO: 260 - DNA, 21 bp, synthetic construct
  source 1..21: mol_type = other DNA
  misc_feature 1..19: note = RNA
  misc_feature 20..21: note = DNA
ccttggatccagtcactaatt

SEQ ID NO: 261 - RNA, 21 nt, synthetic construct
  source 1..21: mol_type = other RNA
ccttggatccagtcactaatt

SEQ ID NO: 262 - DNA, 21 bp, synthetic construct
  source 1..21: mol_type = other DNA
  misc_feature 1..19: note = RNA
  misc_feature 20..21: note = DNA
ccttggatccagtcactaatt

SEQ ID NO: 263 - RNA, 21 nt, synthetic construct
  source 1..21: mol_type = other RNA
ccttggatccagtcactaatt

SEQ ID NO: 264 - DNA, 21 bp, synthetic construct
  source 1..21: mol_type = other DNA
  misc_feature 1..19: note = RNA
  misc_feature 20..21: note = DNA
ccttggatccagtcactaatt

SEQ ID NO: 265 - RNA, 21 nt, synthetic construct
  source 1..21: mol_type = other RNA
cttggatccagtcactaattt

SEQ ID NO: 266 - DNA, 21 bp, synthetic construct
  source 1..21: mol_type = other DNA
  misc_feature 1..19: note = RNA
  misc_feature 20..21: note = DNA
cttggatccagtcactaattt

SEQ ID NO: 267 - RNA, 21 nt, synthetic construct
  source 1..21: mol_type = other RNA
cttggatccagtcactaattt

SEQ ID NO: 268 - DNA, 21 bp, synthetic construct
  source 1..21: mol_type = other DNA
  misc_feature 1..19: note = RNA
  misc_feature 20..21: note = DNA
cttggatccagtcactaattt

SEQ ID NO: 269 - RNA, 21 nt, synthetic construct
  source 1..21: mol_type = other RNA
cttggatccagtcactaattt

SEQ ID NO: 270 - DNA, 21 bp, synthetic construct
  source 1..21: mol_type = other DNA
  misc_feature 1..19: note = RNA
  misc_feature 20..21: note = DNA
cttggatccagtcactaattt

SEQ ID NO: 271 - RNA, 21 nt, synthetic construct
  source 1..21: mol_type = other RNA
cttggatccagtcactaattt

SEQ ID NO: 272 - DNA, 21 bp, synthetic construct
  source 1..21: mol_type = other DNA
  misc_feature 1..19: note = RNA
  misc_feature 20..21: note = DNA
cttggatccagtcactaattt

SEQ ID NO: 273 - RNA, 21 nt, synthetic construct
  source 1..21: mol_type = other RNA
tggatccagtcactaattctt

SEQ ID NO: 274 - DNA, 21 bp, synthetic construct
  source 1..21: mol_type = other DNA
  misc_feature 1..19: note = RNA
  misc_feature 20..21: note = DNA
tggatccagtcactaattctt

SEQ ID NO: 275 - RNA, 21 nt, synthetic construct
  source 1..21: mol_type = other RNA
tggatccagtcactaattctt

SEQ ID NO: 276 - DNA, 21 bp, synthetic construct
  source 1..21: mol_type = other DNA
  misc_feature 1..19: note = RNA
  misc_feature 20..21: note = DNA
tggatccagtcactaattctt

SEQ ID NO: 277 - RNA, 21 nt, synthetic construct
  source 1..21: mol_type = other RNA
tggatccagtcactaattctt

SEQ ID NO: 278 - DNA, 21 bp, synthetic construct
  source 1..21: mol_type = other DNA
  misc_feature 1..19: note = RNA
  misc_feature 20..21: note = DNA
tggatccagtcactaattctt

SEQ ID NO: 279 - RNA, 21 nt, synthetic construct
  source 1..21: mol_type = other RNA
tggatccagtcactaattctt

SEQ ID NO: 280 - DNA, 21 bp, synthetic construct
  source 1..21: mol_type = other DNA
  misc_feature 1..19: note = RNA
  misc_feature 20..21: note = DNA
tggatccagtcactaattctt

SEQ ID NO: 281 - RNA, 21 nt, synthetic construct
  source 1..21: mol_type = other RNA
ttggatccagtcactaatttt

SEQ ID NO: 282 - DNA, 21 bp, synthetic construct
  source 1..21: mol_type = other DNA
  misc_feature 1..19: note = RNA
  misc_feature 20..21: note = DNA
ttggatccagtcactaatttt

SEQ ID NO: 283 - RNA, 21 nt, synthetic construct
  source 1..21: mol_type = other RNA
ttggatccagtcactaatttt

SEQ ID NO: 284 - DNA, 21 bp, synthetic construct
  source 1..21: mol_type = other DNA
  misc_feature 1..19: note = RNA
  misc_feature 20..21: note = DNA
ttggatccagtcactaatttt

SEQ ID NO: 285 - RNA, 21 nt, synthetic construct
  source 1..21: mol_type = other RNA
ttggatccagtcactaatttt

SEQ ID NO: 286 - DNA, 21 bp, synthetic construct
  source 1..21: mol_type = other DNA
  misc_feature 1..19: note = RNA
  misc_feature 20..21: note = DNA
ttggatccagtcactaatttt

SEQ ID NO: 287 - RNA, 21 nt, synthetic construct
  source 1..21: mol_type = other RNA
ttggatccagtcactaatttt

SEQ ID NO: 288 - DNA, 21 bp, synthetic construct
  source 1..21: mol_type = other DNA
  misc_feature 1..19: note = RNA
  misc_feature 20..21: note = DNA
ttggatccagtcactaatttt

SEQ ID NO: 289 - RNA, 21 nt, synthetic construct
  source 1..21: mol_type = other RNA
tccttggatccagtcactatt

SEQ ID NO: 290 - DNA, 21 bp, synthetic construct
  source 1..21: mol_type = other DNA
  misc_feature 1..19: note = RNA
  misc_feature 20..21: note = DNA
tccttggatccagtcactatt

SEQ ID NO: 291 - RNA, 21 nt, synthetic construct
  source 1..21: mol_type = other RNA
tccttggatccagtcactatt

SEQ ID NO: 292 - DNA, 21 bp, synthetic construct
  source 1..21: mol_type = other DNA
  misc_feature 1..19: note = RNA
  misc_feature 20..21: note = DNA
tccttggatccagtcactatt

SEQ ID NO: 293 - RNA, 21 nt, synthetic construct
  source 1..21: mol_type = other RNA
tccttggatccagtcactatt

SEQ ID NO: 294 - DNA, 21 bp, synthetic construct
  source 1..21: mol_type = other DNA
  misc_feature 1..19: note = RNA
  misc_feature 20..21: note = DNA
tccttggatccagtcactatt

SEQ ID NO: 295 - RNA, 21 nt, synthetic construct
  source 1..21: mol_type = other RNA
tccttggatccagtcactatt

SEQ ID NO: 296 - DNA, 21 bp, synthetic construct
  source 1..21: mol_type = other DNA
  misc_feature 1..19: note = RNA
  misc_feature 20..21: note = DNA
tccttggatccagtcactatt

SEQ ID NO: 297 - RNA, 21 nt, synthetic construct
  source 1..21: mol_type = other RNA
gtccttggatccagtcacttt

SEQ ID NO: 298 - DNA, 21 bp, synthetic construct
  source 1..21: mol_type = other DNA
  misc_feature 1..19: note = RNA
  misc_feature 20..21: note = DNA
gtccttggatccagtcacttt

SEQ ID NO: 299 - RNA, 21 nt, synthetic construct
  source 1..21: mol_type = other RNA
gtccttggatccagtcacttt

SEQ ID NO: 300 - DNA, 21 bp, synthetic construct
  source 1..21: mol_type = other DNA
  misc_feature 1..19: note = RNA
  misc_feature 20..21: note = DNA
gtccttggatccagtcacttt

SEQ ID NO: 301 - RNA, 21 nt, synthetic construct
  source 1..21: mol_type = other RNA
gtccttggatccagtcacttt

SEQ ID NO: 302 - DNA, 21 bp, synthetic construct
  source 1..21: mol_type = other DNA
  misc_feature 1..19: note = RNA
  misc_feature 20..21: note = DNA
gtccttggatccagtcacttt

SEQ ID NO: 303 - RNA, 21 nt, synthetic construct
  source 1..21: mol_type = other RNA
gtccttggatccagtcacttt

SEQ ID NO: 304 - DNA, 21 bp, synthetic construct
  source 1..21: mol_type = other DNA
  misc_feature 1..19: note = RNA
  misc_feature 20..21: note = DNA
gtccttggatccagtcacttt

SEQ ID NO: 305 - RNA, 21 nt, synthetic construct
  source 1..21: mol_type = other RNA
tggtccttggatccagtcatt

SEQ ID NO: 306 - DNA, 21 bp, synthetic construct
  source 1..21: mol_type = other DNA
  misc_feature 1..19: note = RNA
  misc_feature 20..21: note = DNA
tggtccttggatccagtcatt

SEQ ID NO: 307 - RNA, 21 nt, synthetic construct
  source 1..21: mol_type = other RNA
tggtccttggatccagtcatt

SEQ ID NO: 308 - DNA, 21 bp, synthetic construct
  source 1..21: mol_type = other DNA
  misc_feature 1..19: note = RNA
  misc_feature 20..21: note = DNA
tggtccttggatccagtcatt

SEQ ID NO: 309 - RNA, 21 nt, synthetic construct
  source 1..21: mol_type = other RNA
tggtccttggatccagtcatt

SEQ ID NO: 310 - DNA, 21 bp, synthetic construct
  source 1..21: mol_type = other DNA
  misc_feature 1..19: note = RNA
  misc_feature 20..21: note = DNA
tggtccttggatccagtcatt

SEQ ID NO: 311 - RNA, 21 nt, synthetic construct
  source 1..21: mol_type = other RNA
tggtccttggatccagtcatt

SEQ ID NO: 312 - DNA, 21 bp, synthetic construct
  source 1..21: mol_type = other DNA
  misc_feature 1..19: note = RNA
  misc_feature 20..21: note = DNA
tggtccttggatccagtcatt

SEQ ID NO: 313 - RNA, 21 nt, synthetic construct
  source 1..21: mol_type = other RNA
cgcacatgctccatcattgtt

SEQ ID NO: 314 - DNA, 21 bp, synthetic construct
  source 1..21: mol_type = other DNA
  misc_feature 1..19: note = RNA
  misc_feature 20..21: note = DNA
cgcacatgctccatcattgtt

SEQ ID NO: 315 - RNA, 21 nt, synthetic construct
  source 1..21: mol_type = other RNA
cgcacatgctccatcattgtt

SEQ ID NO: 316 - DNA, 21 bp, synthetic construct
  source 1..21: mol_type = other DNA
  misc_feature 1..19: note = RNA
  misc_feature 20..21: note = DNA
cgcacatgctccatcattgtt

SEQ ID NO: 317 - RNA, 21 nt, synthetic construct
  source 1..21: mol_type = other RNA
cgcacatgctccatcattgtt

SEQ ID NO: 318 - DNA, 21 bp, synthetic construct
  source 1..21: mol_type = other DNA
  misc_feature 1..19: note = RNA
  misc_feature 20..21: note = DNA
cgcacatgctccatcattgtt

SEQ ID NO: 319 - RNA, 21 nt, synthetic construct
  source 1..21: mol_type = other RNA
cgcacatgctccatcattgtt

SEQ ID NO: 320 - DNA, 21 bp, synthetic construct
  source 1..21: mol_type = other DNA
  misc_feature 1..19: note = RNA
  misc_feature 20..21: note = DNA
cgcacatgctccatcattgtt

SEQ ID NO: 321 - RNA, 21 nt, synthetic construct
  source 1..21: mol_type = other RNA
tcgcacatgctccatcatttt

SEQ ID NO: 322 - DNA, 21 bp, synthetic construct
  source 1..21: mol_type = other DNA
  misc_feature 1..19: note = RNA
  misc_feature 20..21: note = DNA
tcgcacatgctccatcatttt

SEQ ID NO: 323 - RNA, 21 nt, synthetic construct
  source 1..21: mol_type = other RNA
tcgcacatgctccatcatttt

SEQ ID NO: 324 - DNA, 21 bp, synthetic construct
  source 1..21: mol_type = other DNA
  misc_feature 1..19: note = RNA
  misc_feature 20..21: note = DNA
tcgcacatgctccatcatttt

SEQ ID NO: 325 - RNA, 21 nt, synthetic construct
  source 1..21: mol_type = other RNA
tcgcacatgctccatcatttt

SEQ ID NO: 326 - DNA, 21 bp, synthetic construct
  source 1..21: mol_type = other DNA
  misc_feature 1..19: note = RNA
  misc_feature 20..21: note = DNA
tcgcacatgctccatcatttt

SEQ ID NO: 327 - RNA, 21 nt, synthetic construct
  source 1..21: mol_type = other RNA
tcgcacatgctccatcatttt

SEQ ID NO: 328 - DNA, 21 bp, synthetic construct
  source 1..21: mol_type = other DNA
  misc_feature 1..19: note = RNA
  misc_feature 20..21: note = DNA
tcgcacatgctccatcatttt

SEQ ID NO: 329 - RNA, 21 nt, synthetic construct
  source 1..21: mol_type = other RNA
ttcgcacatgctccatcattt

SEQ ID NO: 330 - DNA, 21 bp, synthetic construct
  source 1..21: mol_type = other DNA
  misc_feature 1..19: note = RNA
  misc_feature 20..21: note = DNA
ttcgcacatgctccatcattt

SEQ ID NO: 331 - RNA, 21 nt, synthetic construct
  source 1..21: mol_type = other RNA
ttcgcacatgctccatcattt

SEQ ID NO: 332 - DNA, 21 bp, synthetic construct
  source 1..21: mol_type = other DNA
  misc_feature 1..19: note = RNA
  misc_feature 20..21: note = DNA
ttcgcacatgctccatcattt

SEQ ID NO: 333 - RNA, 21 nt, synthetic construct
  source 1..21: mol_type = other RNA
ttcgcacatgctccatcattt

SEQ ID NO: 334 - DNA, 21 bp, synthetic construct
  source 1..21: mol_type = other DNA
  misc_feature 1..19: note = RNA
  misc_feature 20..21: note = DNA
ttcgcacatgctccatcattt

SEQ ID NO: 335 - RNA, 21 nt, synthetic construct
  source 1..21: mol_type = other RNA
ttcgcacatgctccatcattt

SEQ ID NO: 336 - DNA, 21 bp, synthetic construct
  source 1..21: mol_type = other DNA
  misc_feature 1..19: note = RNA
  misc_feature 20..21: note = DNA
ttcgcacatgctccatcattt

SEQ ID NO: 337 - RNA, 21 nt, synthetic construct
  source 1..21: mol_type = other RNA
attcgcacatgctccatcatt

SEQ ID NO: 338 - DNA, 21 bp, synthetic construct
  source 1..21: mol_type = other DNA
  misc_feature 1..19: note = RNA
  misc_feature 20..21: note = DNA
attcgcacatgctccatcatt

SEQ ID NO: 339 - RNA, 21 nt, synthetic construct
  source 1..21: mol_type = other RNA
attcgcacatgctccatcatt

SEQ ID NO: 340 - DNA, 21 bp, synthetic construct
  source 1..21: mol_type = other DNA
  misc_feature 1..19: note = RNA
  misc_feature 20..21: note = DNA
attcgcacatgctccatcatt

SEQ ID NO: 341 - RNA, 21 nt, synthetic construct
  source 1..21: mol_type = other RNA
attcgcacatgctccatcatt

SEQ ID NO: 342 - DNA, 21 bp, synthetic construct
  source 1..21: mol_type = other DNA
  misc_feature 1..19: note = RNA
  misc_feature 20..21: note = DNA
attcgcacatgctccatcatt

SEQ ID NO: 343 - RNA, 21 nt, synthetic construct
  source 1..21: mol_type = other RNA
attcgcacatgctccatcatt

SEQ ID NO: 344 - DNA, 21 bp, synthetic construct
  source 1..21: mol_type = other DNA
  misc_feature 1..19: note = RNA
  misc_feature 20..21: note = DNA
attcgcacatgctccatcatt

SEQ ID NO: 345 - RNA, 21 nt, synthetic construct
  source 1..21: mol_type = other RNA
gaattcgcacatgctccattt

SEQ ID NO: 346 - DNA, 21 bp, synthetic construct
  source 1..21: mol_type = other DNA
  misc_feature 1..19: note = RNA
  misc_feature 20..21: note = DNA
gaattcgcacatgctccattt

SEQ ID NO: 347 - RNA, 21 nt, synthetic construct
  source 1..21: mol_type = other RNA
gaattcgcacatgctccattt

SEQ ID NO: 348 - DNA, 21 bp, synthetic construct
  source 1..21: mol_type = other DNA
  misc_feature 1..19: note = RNA
  misc_feature 20..21: note = DNA
gaattcgcacatgctccattt

SEQ ID NO: 349 - RNA, 21 nt, synthetic construct
  source 1..21: mol_type = other RNA
gaattcgcacatgctccattt

SEQ ID NO: 350 - DNA, 21 bp, synthetic construct
  source 1..21: mol_type = other DNA
  misc_feature 1..19: note = RNA
  misc_feature 20..21: note = DNA
gaattcgcacatgctccattt

SEQ ID NO: 351 - RNA, 21 nt, synthetic construct
  source 1..21: mol_type = other RNA
gaattcgcacatgctccattt

SEQ ID NO: 352 - DNA, 21 bp, synthetic construct
  source 1..21: mol_type = other DNA
  misc_feature 1..19: note = RNA
  misc_feature 20..21: note = DNA
gaattcgcacatgctccattt

SEQ ID NO: 353 - RNA, 21 nt, synthetic construct
  source 1..21: mol_type = other RNA
ccaccttcgagggtccagttt

SEQ ID NO: 354 - DNA, 21 bp, synthetic construct
  source 1..21: mol_type = other DNA
  misc_feature 1..19: note = RNA
  misc_feature 20..21: note = DNA
ccaccttcgagggtccagttt

SEQ ID NO: 355 - RNA, 21 nt, synthetic construct
  source 1..21: mol_type = other RNA
ccaccttcgagggtccagttt

SEQ ID NO: 356 - DNA, 21 bp, synthetic construct
  source 1..21: mol_type = other DNA
  misc_feature 1..19: note = RNA
  misc_feature 20..21: note = DNA
ccaccttcgagggtccagttt

SEQ ID NO: 357 - RNA, 21 nt, synthetic construct
  source 1..21: mol_type = other RNA
ccaccttcgagggtccagttt

SEQ ID NO: 358 - DNA, 21 bp, synthetic construct
  source 1..21: mol_type = other DNA
  misc_feature 1..19: note = RNA
  misc_feature 20..21: note = DNA
ccaccttcgagggtccagttt

SEQ ID NO: 359 - RNA, 21 nt, synthetic construct
  source 1..21: mol_type = other RNA
ccaccttcgagggtccagttt

SEQ ID NO: 360 - DNA, 21 bp, synthetic construct
  source 1..21: mol_type = other DNA
  misc_feature 1..19: note = RNA
  misc_feature 20..21: note = DNA
ccaccttcgagggtccagttt

SEQ ID NO: 361 - RNA, 21 nt, synthetic construct
  source 1..21: mol_type = other RNA
tccaccttcgagggtccagtt

SEQ ID NO: 362 - DNA, 21 bp, synthetic construct
  source 1..21: mol_type = other DNA
  misc_feature 1..19: note = RNA
  misc_feature 20..21: note = DNA
tccaccttcgagggtccagtt

SEQ ID NO: 363 - RNA, 21 nt, synthetic construct
  source 1..21: mol_type = other RNA
tccaccttcgagggtccagtt

SEQ ID NO: 364 - DNA, 21 bp, synthetic construct
  source 1..21: mol_type = other DNA
  misc_feature 1..19: note = RNA
  misc_feature 20..21: note = DNA
tccaccttcgagggtccagtt

SEQ ID NO: 365 - RNA, 21 nt, synthetic construct
  source 1..21: mol_type = other RNA
tccaccttcgagggtccagtt

SEQ ID NO: 366 - DNA, 21 bp, synthetic construct
  source 1..21: mol_type = other DNA
  misc_feature 1..19: note = RNA
  misc_feature 20..21: note = DNA
tccaccttcgagggtccagtt

SEQ ID NO: 367 - RNA, 21 nt, synthetic construct
  source 1..21: mol_type = other RNA
tccaccttcgagggtccagtt

SEQ ID NO: 368 - DNA, 21 bp, synthetic construct
  source 1..21: mol_type = other DNA
  misc_feature 1..19: note = RNA
  misc_feature 20..21: note = DNA
tccaccttcgagggtccagtt

SEQ ID NO: 369 - RNA, 21 nt, synthetic construct
  source 1..21: mol_type = other RNA
ttccaccttcgagggtccatt

SEQ ID NO: 370 - DNA, 21 bp, synthetic construct
  source 1..21: mol_type = other DNA
  misc_feature 1..19: note = RNA
  misc_feature 20..21: note = DNA
ttccaccttcgagggtccatt

SEQ ID NO: 371 - RNA, 21 nt, synthetic construct
  source 1..21: mol_type = other RNA
ttccaccttcgagggtccatt

SEQ ID NO: 372 - DNA, 21 bp, synthetic construct
  source 1..21: mol_type = other DNA
  misc_feature 1..19: note = RNA
  misc_feature 20..21: note = DNA
ttccaccttcgagggtccatt

SEQ ID NO: 373 - RNA, 21 nt, synthetic construct
  source 1..21: mol_type = other RNA
ttccaccttcgagggtccatt

SEQ ID NO: 374 - DNA, 21 bp, synthetic construct
  source 1..21: mol_type = other DNA
  misc_feature 1..19: note = RNA
  misc_feature 20..21: note = DNA
ttccaccttcgagggtccatt

SEQ ID NO: 375 - RNA, 21 nt, synthetic construct
  source 1..21: mol_type = other RNA
ttccaccttcgagggtccatt

SEQ ID NO: 376 - DNA, 21 bp, synthetic construct
  source 1..21: mol_type = other DNA
  misc_feature 1..19: note = RNA
  misc_feature 20..21: note = DNA
ttccaccttcgagggtccatt

SEQ ID NO: 377 - RNA, 21 nt, synthetic construct
  source 1..21: mol_type = other RNA
cttccaccttcgagggtcctt

SEQ ID NO: 378 - DNA, 21 bp, synthetic construct
  source 1..21: mol_type = other DNA
  misc_feature 1..19: note = RNA
  misc_feature 20..21: note = DNA
cttccaccttcgagggtcctt

SEQ ID NO: 379 - RNA, 21 nt, synthetic construct
  source 1..21: mol_type = other RNA
cttccaccttcgagggtcctt

SEQ ID NO: 380 - DNA, 21 bp, synthetic construct
  source 1..21: mol_type = other DNA
  misc_feature 1..19: note = RNA
  misc_feature 20..21: note = DNA
cttccaccttcgagggtcctt

SEQ ID NO: 381 - RNA, 21 nt, synthetic construct
  source 1..21: mol_type = other RNA
cttccaccttcgagggtcctt

SEQ ID NO: 382 - DNA, 21 bp, synthetic construct
  source 1..21: mol_type = other DNA
  misc_feature 1..19: note = RNA
  misc_feature 20..21: note = DNA
cttccaccttcgagggtcctt

SEQ ID NO: 383 - RNA, 21 nt, synthetic construct
  source 1..21: mol_type = other RNA
cttccaccttcgagggtcctt

SEQ ID NO: 384 - DNA, 21 bp, synthetic construct
  source 1..21: mol_type = other DNA
  misc_feature 1..19: note = RNA
  misc_feature 20..21: note = DNA
cttccaccttcgagggtcctt

SEQ ID NO: 385 - RNA, 21 nt, synthetic construct
  source 1..21: mol_type = other RNA
caaccagccaggttttggttt

SEQ ID NO: 386 - RNA, 21 nt, synthetic construct
  source 1..21: mol_type = other RNA
caaccagccaggttttggttt

SEQ ID NO: 387 - DNA, 21 bp, synthetic construct
  source 1..21: mol_type = other DNA
  misc_feature 1..19: note = RNA
  misc_feature 20..21: note = DNA
caaccagccaggttttggttt

SEQ ID NO: 388 - RNA, 21 nt, synthetic construct
  source 1..21: mol_type = other RNA
caaccagccaggttttggttt

SEQ ID NO: 389 - DNA, 21 bp, synthetic construct
  source 1..21: mol_type = other DNA
  misc_feature 1..19: note = RNA
  misc_feature 20..21: note = DNA
caaccagccaggttttggttt

SEQ ID NO: 390 - DNA, 21 bp, synthetic construct
  source 1..21: mol_type = other DNA
  misc_feature 1..19: note = RNA
  misc_feature 20..21: note = DNA
caaccagccaggttttggttt

SEQ ID NO: 391 - RNA, 21 nt, synthetic construct
  source 1..21: mol_type = other RNA
caaccagccaggttttggttt

SEQ ID NO: 392 - DNA, 21 bp, synthetic construct
  source 1..21: mol_type = other DNA
  misc_feature 1..19: note = RNA
  misc_feature 20..21: note = DNA
caaccagccaggttttggttt

SEQ ID NO: 393 - RNA, 21 nt, synthetic construct
  source 1..21: mol_type = other RNA
agctcatcagccagctggttt

SEQ ID NO: 394 - DNA, 21 bp, synthetic construct
  source 1..21: mol_type = other DNA
  misc_feature 1..19: note = RNA
  misc_feature 20..21: note = DNA
agctcatcagccagctggttt

SEQ ID NO: 395 - RNA, 21 nt, synthetic construct
  source 1..21: mol_type = other RNA
agctcatcagccagctggttt

SEQ ID NO: 396 - DNA, 21 bp, synthetic construct
  source 1..21: mol_type = other DNA
  misc_feature 1..19: note = RNA
  misc_feature 20..21: note = DNA
agctcatcagccagctggttt

SEQ ID NO: 397 - RNA, 21 nt, synthetic construct
  source 1..21: mol_type = other RNA
agctcatcagccagctggttt

SEQ ID NO: 398 - DNA, 21 bp, synthetic construct
  source 1..21: mol_type = other DNA
  misc_feature 1..19: note = RNA
  misc_feature 20..21: note = DNA
agctcatcagccagctggttt

SEQ ID NO: 399 - RNA, 21 nt, synthetic construct
  source 1..21: mol_type = other RNA
agctcatcagccagctggttt

SEQ ID NO: 400 - DNA, 21 bp, synthetic construct
  source 1..21: mol_type = other DNA
  misc_feature 1..19: note = RNA
  misc_feature 20..21: note = DNA
agctcatcagccagctggttt

SEQ ID NO: 401 - RNA, 21 nt, synthetic construct
  source 1..21: mol_type = other RNA
tccaaccagccaggttttgtt

SEQ ID NO: 402 - RNA, 21 nt, synthetic construct
  source 1..21: mol_type = other RNA
tccaaccagccaggttttgtt

SEQ ID NO: 403 - RNA, 21 nt, synthetic construct
  source 1..21: mol_type = other RNA
tccaaccagccaggttttgtt

SEQ ID NO: 404 - DNA, 21 bp, synthetic construct
  source 1..21: mol_type = other DNA
  misc_feature 1..19: note = RNA
  misc_feature 20..21: note = DNA
tccaaccagccaggttttgtt

SEQ ID NO: 405 - DNA, 21 bp, synthetic construct
  source 1..21: mol_type = other DNA
  misc_feature 1..19: note = RNA
  misc_feature 20..21: note = DNA
tccaaccagccaggttttgtt

SEQ ID NO: 406 - DNA, 21 bp, synthetic construct
  source 1..21: mol_type = other DNA
  misc_feature 1..19: note = RNA
  misc_feature 20..21: note = DNA
tccaaccagccaggttttgtt

SEQ ID NO: 407 - RNA, 21 nt, synthetic construct
  source 1..21: mol_type = other RNA
tccaaccagccaggttttgtt

SEQ ID NO: 408 - DNA, 21 bp, synthetic construct
  source 1..21: mol_type = other DNA
  misc_feature 1..19: note = RNA
  misc_feature 20..21: note = DNA
tccaaccagccaggttttgtt

SEQ ID NO: 409 - RNA, 21 nt, synthetic construct
  source 1..21: mol_type = other RNA
ccaaccagccaggttttggtt

SEQ ID NO: 410 - DNA, 21 bp, synthetic construct
  source 1..21: mol_type = other DNA
  misc_feature 1..19: note = RNA
  misc_feature 20..21: note = DNA
ccaaccagccaggttttggtt

SEQ ID NO: 411 - RNA, 21 nt, synthetic construct
  source 1..21: mol_type = other RNA
ccaaccagccaggttttggtt

SEQ ID NO: 412 - DNA, 21 bp, synthetic construct
  source 1..21: mol_type = other DNA
  misc_feature 1..19: note = RNA
  misc_feature 20..21: note = DNA
ccaaccagccaggttttggtt

SEQ ID NO: 413 - RNA, 21 nt, synthetic construct
  source 1..21: mol_type = other RNA
ccaaccagccaggttttggtt

SEQ ID NO: 414 - DNA, 21 bp, synthetic construct
  source 1..21: mol_type = other DNA
  misc_feature 1..19: note = RNA
  misc_feature 20..21: note = DNA
ccaaccagccaggttttggtt

SEQ ID NO: 415 - RNA, 21 nt, synthetic construct
  source 1..21: mol_type = other RNA
ccaaccagccaggttttggtt

SEQ ID NO: 416 - DNA, 21 bp, synthetic construct
  source 1..21: mol_type = other DNA
  misc_feature 1..19: note = RNA
  misc_feature 20..21: note = DNA
ccaaccagccaggttttggtt

SEQ ID NO: 417 - RNA, 19 nt, synthetic construct
  source 1..19: mol_type = other RNA
gtgccaaaatctctcacct

SEQ ID NO: 418 - RNA, 19 nt, synthetic construct
  source 1..19: mol_type = other RNA
gtgccaaaatctctcacct

SEQ ID NO: 419 - RNA, 19 nt, synthetic construct
  source 1..19: mol_type = other RNA
gtgccaaaatctctctcct

SEQ ID NO: 420 - RNA, 19 nt, synthetic construct
  source 1..19: mol_type = other RNA
gtgccaaaatctctctcct

SEQ ID NO: 421 - RNA, 19 nt, synthetic construct
  source 1..19: mol_type = other RNA
gtgccaaaatctctctgct

SEQ ID NO: 422 - RNA, 19 nt, synthetic construct
  source 1..19: mol_type = other RNA
gtgccaaaatctctctgct

SEQ ID NO: 423 - RNA, 19 nt, synthetic construct
  source 1..19: mol_type = other RNA
gtgccaaaatctctctggt

SEQ ID NO: 424 - RNA, 19 nt, synthetic construct
  source 1..19: mol_type = other RNA
gtgccaaaatctctctggt

SEQ ID NO: 425 - RNA, 19 nt, synthetic construct
  source 1..19: mol_type = other RNA
tggagcatgtgcgaaaagt

SEQ ID NO: 426 - RNA, 19 nt, synthetic construct
  source 1..19: mol_type = other RNA
tggagcatgtgcgaaaagt

SEQ ID NO: 427 - RNA, 19 nt, synthetic construct
  source 1..19: mol_type = other RNA
tggagcatgtgcgaatagt

SEQ ID NO: 428 - RNA, 19 nt, synthetic construct
  source 1..19: mol_type = other RNA
tggagcatgtgcgaatagt

SEQ ID NO: 429 - RNA, 19 nt, synthetic construct
  source 1..19: mol_type = other RNA
tggagcatgtgcgaattct

SEQ ID NO: 430 - RNA, 19 nt, synthetic construct
  source 1..19: mol_type = other RNA
tggagcatgtgcgaattct

SEQ ID NO: 431 - RNA, 19 nt, synthetic construct
  source 1..19: mol_type = other RNA
tggagcatgtgcgaattgt

SEQ ID NO: 432 - RNA, 19 nt, synthetic construct
  source 1..19: mol_type = other RNA
tggagcatgtgcgaattgt

SEQ ID NO: 433 - RNA, 19 nt, synthetic construct
  source 1..19: mol_type = other RNA
gtgtgccaaaatctctcac

SEQ ID NO: 434 - RNA, 19 nt, synthetic construct
  source 1..19: mol_type = other RNA
gtgtgccaaaatctctcac

SEQ ID NO: 435 - RNA, 19 nt, synthetic construct
  source 1..19: mol_type = other RNA
gtgtgccaaaatctcagac

SEQ ID NO: 436 - RNA, 19 nt, synthetic construct
  source 1..19: mol_type = other RNA
gtgtgccaaaatctcagac

SEQ ID NO: 437 - RNA, 19 nt, synthetic construct
  source 1..19: mol_type = other RNA
gtgtgccaaaatctctctc

SEQ ID NO: 438 - RNA, 19 nt, synthetic construct
  source 1..19: mol_type = other RNA
gtgtgccaaaatctctctc

SEQ ID NO: 439 - RNA, 19 nt, synthetic construct
  source 1..19: mol_type = other RNA
gtgtgccaaaatctctgac

SEQ ID NO: 440 - RNA, 19 nt, synthetic construct
  source 1..19: mol_type = other RNA
gtgtgccaaaatctctgac

SEQ ID NO: 441 - RNA, 19 nt, synthetic construct
  source 1..19: mol_type = other RNA
gtgactggatccaagctgg

SEQ ID NO: 442 - RNA, 19 nt, synthetic construct
  source 1..19: mol_type = other RNA
gtgactggatccaagctgg

SEQ ID NO: 443 - RNA, 19 nt, synthetic construct
  source 1..19: mol_type = other RNA
gtgactggatccaaggacg

SEQ ID NO: 444 - RNA, 19 nt, synthetic construct
  source 1..19: mol_type = other RNA
gtgactggatccaaggacg

SEQ ID NO: 445 - RNA, 19 nt, synthetic construct
  source 1..19: mol_type = other RNA
gtgactggatccaaggagg

SEQ ID NO: 446 - RNA, 19 nt, synthetic construct
  source 1..19: mol_type = other RNA
gtgactggatccaaggagg

SEQ ID NO: 447 - RNA, 19 nt, synthetic construct
  source 1..19: mol_type = other RNA
gtgactggatccaaggtgg

SEQ ID NO: 448 - RNA, 19 nt, synthetic construct
  source 1..19: mol_type = other RNA
gtgactggatccaaggtgg

SEQ ID NO: 449 - RNA, 19 nt, synthetic construct
  source 1..19: mol_type = other RNA
gatggagcatgtgcgaaaa

SEQ ID NO: 450 - RNA, 19 nt, synthetic construct
  source 1..19: mol_type = other RNA
gatggagcatgtgcgaaaa

SEQ ID NO: 451 - RNA, 19 nt, synthetic construct
  source 1..19: mol_type = other RNA
gatggagcatgtgcgaata

SEQ ID NO: 452 - RNA, 19 nt, synthetic construct
  source 1..19: mol_type = other RNA
gatggagcatgtgcgaata

SEQ ID NO: 453 - RNA, 19 nt, synthetic construct
  source 1..19: mol_type = other RNA
gatggagcatgtgcgataa

SEQ ID NO: 454 - RNA, 19 nt, synthetic construct
  source 1..19: mol_type = other RNA
gatggagcatgtgcgataa

SEQ ID NO: 455 - RNA, 19 nt, synthetic construct
  source 1..19: mol_type = other RNA
gatggagcatgtgcgttaa

SEQ ID NO: 456 - RNA, 19 nt, synthetic construct
  source 1..19: mol_type = other RNA
gatggagcatgtgcgttaa

SEQ ID NO: 457 - RNA, 19 nt, synthetic construct
  source 1..19: mol_type = other RNA
gaccctcgaaggtggaact

SEQ ID NO: 458 - RNA, 19 nt, synthetic construct
  source 1..19: mol_type = other RNA
gaccctcgaaggtggaact

SEQ ID NO: 459 - RNA, 19 nt, synthetic construct
  source 1..19: mol_type = other RNA
gaccctcgaaggtggaagt

SEQ ID NO: 460 - RNA, 19 nt, synthetic construct
  source 1..19: mol_type = other RNA
gaccctcgaaggtggaagt

SEQ ID NO: 461 - RNA, 19 nt, synthetic construct
  source 1..19: mol_type = other RNA
gaccctcgaaggtggatct

SEQ ID NO: 462 - RNA, 19 nt, synthetic construct
  source 1..19: mol_type = other RNA
gaccctcgaaggtggatct

SEQ ID NO: 463 - RNA, 19 nt, synthetic construct
  source 1..19: mol_type = other RNA
gaccctcgaaggtggttct

SEQ ID NO: 464 - RNA, 19 nt, synthetic construct
  source 1..19: mol_type = other RNA
gaccctcgaaggtggttct

SEQ ID NO: 465 - RNA, 19 nt, synthetic construct
  source 1..19: mol_type = other RNA
ggaattagtgactggaagg

SEQ ID NO: 466 - RNA, 19 nt, synthetic construct
  source 1..19: mol_type = other RNA
ggaattagtgactggaagg

SEQ ID NO: 467 - RNA, 19 nt, synthetic construct
  source 1..19: mol_type = other RNA
ggaattagtgactggatcg

SEQ ID NO: 468 - RNA, 19 nt, synthetic construct
  source 1..19: mol_type = other RNA
ggaattagtgactggatcg

SEQ ID NO: 469 - RNA, 19 nt, synthetic construct
  source 1..19: mol_type = other RNA
ggaattagtgactggatgg

SEQ ID NO: 470 - RNA, 19 nt, synthetic construct
  source 1..19: mol_type = other RNA
ggaattagtgactggatgg

SEQ ID NO: 471 - RNA, 19 nt, synthetic construct
  source 1..19: mol_type = other RNA
ggaattagtgactggtagg

SEQ ID NO: 472 - RNA, 19 nt, synthetic construct
  source 1..19: mol_type = other RNA
ggaattagtgactggtagg

SEQ ID NO: 473 - RNA, 19 nt, synthetic construct
  source 1..19: mol_type = other RNA
tgtgccaaaatctctcacc

SEQ ID NO: 474 - RNA, 19 nt, synthetic construct
  source 1..19: mol_type = other RNA
tgtgccaaaatctctcacc

SEQ ID NO: 475 - RNA, 19 nt, synthetic construct
  source 1..19: mol_type = other RNA
tgtgccaaaatctctctcc

SEQ ID NO: 476 - RNA, 19 nt, synthetic construct
  source 1..19: mol_type = other RNA
tgtgccaaaatctctctcc

SEQ ID NO: 477 - RNA, 19 nt, synthetic construct
  source 1..19: mol_type = other RNA
tgtgccaaaatctctctgc

SEQ ID NO: 478 - RNA, 19 nt, synthetic construct
  source 1..19: mol_type = other RNA
tgtgccaaaatctctctgc

SEQ ID NO: 479 - RNA, 19 nt, synthetic construct
  source 1..19: mol_type = other RNA
tgtgccaaaatctctgacc

SEQ ID NO: 480 - RNA, 19 nt, synthetic construct
  source 1..19: mol_type = other RNA
tgtgccaaaatctctgacc

SEQ ID NO: 481 - RNA, 19 nt, synthetic construct
  source 1..19: mol_type = other RNA
ttagtgactggatccaacc

SEQ ID NO: 482 - RNA, 19 nt, synthetic construct
  source 1..19: mol_type = other RNA
ttagtgactggatccaacc

SEQ ID NO: 483 - RNA, 19 nt, synthetic construct
  source 1..19: mol_type = other RNA
ttagtgactggatccaagc

SEQ ID NO: 484 - RNA, 19 nt, synthetic construct
  source 1..19: mol_type = other RNA
ttagtgactggatccaagc

SEQ ID NO: 485 - RNA, 19 nt, synthetic construct
  source 1..19: mol_type = other RNA
ttagtgactggatccatcc

SEQ ID NO: 486 - RNA, 19 nt, synthetic construct
  source 1..19: mol_type = other RNA
ttagtgactggatccatcc

SEQ ID NO: 487 - RNA, 19 nt, synthetic construct
  source 1..19: mol_type = other RNA
ttagtgactggatccttcc

SEQ ID NO: 488 - RNA, 19 nt, synthetic construct
  source 1..19: mol_type = other RNA
ttagtgactggatccttcc

SEQ ID NO: 489 - RNA, 19 nt, synthetic construct
  source 1..19: mol_type = other RNA
attagtgactggatccaac

SEQ ID NO: 490 - RNA, 19 nt, synthetic construct
  source 1..19: mol_type = other RNA
attagtgactggatccaac

SEQ ID NO: 491 - RNA, 19 nt, synthetic construct
  source 1..19: mol_type = other RNA
attagtgactggatccatc

SEQ ID NO: 492 - RNA, 19 nt, synthetic construct
  source 1..19: mol_type = other RNA
attagtgactggatccatc

SEQ ID NO: 493 - RNA, 19 nt, synthetic construct
  source 1..19: mol_type = other RNA
attagtgactggatccttc

SEQ ID NO: 494 - RNA, 19 nt, synthetic construct
  source 1..19: mol_type = other RNA
attagtgactggatccttc

SEQ ID NO: 495 - RNA, 19 nt, synthetic construct
  source 1..19: mol_type = other RNA
attagtgactggatcgttc

SEQ ID NO: 496 - RNA, 19 nt, synthetic construct
  source 1..19: mol_type = other RNA
attagtgactggatcgttc

SEQ ID NO: 497 - RNA, 19 nt, synthetic construct
  source 1..19: mol_type = other RNA
gaattagtgactggaaggt

SEQ ID NO: 498 - RNA, 19 nt, synthetic construct
  source 1..19: mol_type = other RNA
gaattagtgactggaaggt

SEQ ID NO: 499 - RNA, 19 nt, synthetic construct
  source 1..19: mol_type = other RNA
gaattagtgactggatcct

SEQ ID NO: 500 - RNA, 19 nt, synthetic construct
  source 1..19: mol_type = other RNA
gaattagtgactggatcct

SEQ ID NO: 501 - RNA, 19 nt, synthetic construct
  source 1..19: mol_type = other RNA
gaattagtgactggatcgt

SEQ ID NO: 502 - RNA, 19 nt, synthetic construct
  source 1..19: mol_type = other RNA
gaattagtgactggatcgt

SEQ ID NO: 503 - RNA, 19 nt, synthetic construct
  source 1..19: mol_type = other RNA
gaattagtgactggatggt

SEQ ID NO: 504 - RNA, 19 nt, synthetic construct
  source 1..19: mol_type = other RNA
gaattagtgactggatggt

SEQ ID NO: 505 - RNA, 19 nt, synthetic construct
  source 1..19: mol_type = other RNA
aattagtgactggatccat

SEQ ID NO: 506 - RNA, 19 nt, synthetic construct
  source 1..19: mol_type = other RNA
aattagtgactggatccat

SEQ ID NO: 507 - RNA, 19 nt, synthetic construct
  source 1..19: mol_type = other RNA
aattagtgactggatcctt

SEQ ID NO: 508 - RNA, 19 nt, synthetic construct
  source 1..19: mol_type = other RNA
aattagtgactggatcctt

SEQ ID NO: 509 - RNA, 19 nt, synthetic construct
  source 1..19: mol_type = other RNA
aattagtgactggatcgtt

SEQ ID NO: 510 - RNA, 19 nt, synthetic construct
  source 1..19: mol_type = other RNA
aattagtgactggatcgtt

SEQ ID NO: 511 - RNA, 19 nt, synthetic construct
  source 1..19: mol_type = other RNA
aattagtgactggatggtt

SEQ ID NO: 512 - RNA, 19 nt, synthetic construct
  source 1..19: mol_type = other RNA
aattagtgactggatggtt

SEQ ID NO: 513 - RNA, 19 nt, synthetic construct
  source 1..19: mol_type = other RNA
tagtgactggatccaacct

SEQ ID NO: 514 - RNA, 19 nt, synthetic construct
  source 1..19: mol_type = other RNA
tagtgactggatccaacct

SEQ ID NO: 515 - RNA, 19 nt, synthetic construct
  source 1..19: mol_type = other RNA
tagtgactggatccaagct

SEQ ID NO: 516 - RNA, 19 nt, synthetic construct
  source 1..19: mol_type = other RNA
tagtgactggatccaagct

SEQ ID NO: 517 - RNA, 19 nt, synthetic construct
  source 1..19: mol_type = other RNA
tagtgactggatccaaggt

SEQ ID NO: 518 - RNA, 19 nt, synthetic construct
  source 1..19: mol_type = other RNA
tagtgactggatccaaggt

SEQ ID NO: 519 - RNA, 19 nt, synthetic construct
  source 1..19: mol_type = other RNA
tagtgactggatccatcct

SEQ ID NO: 520 - RNA, 19 nt, synthetic construct
  source 1..19: mol_type = other RNA
tagtgactggatccatcct

SEQ ID NO: 521 - RNA, 19 nt, synthetic construct
  source 1..19: mol_type = other RNA
agtgactggatccaacctg

SEQ ID NO: 522 - RNA, 19 nt, synthetic construct
  source 1..19: mol_type = other RNA
agtgactggatccaacctg

SEQ ID NO: 523 - RNA, 19 nt, synthetic construct
  source 1..19: mol_type = other RNA
agtgactggatccaagctg

SEQ ID NO: 524 - RNA, 19 nt, synthetic construct
  source 1..19: mol_type = other RNA
agtgactggatccaagctg

SEQ ID NO: 525 - RNA, 19 nt, synthetic construct
  source 1..19: mol_type = other RNA
agtgactggatccaaggag

SEQ ID NO: 526 - RNA, 19 nt, synthetic construct
  source 1..19: mol_type = other RNA
agtgactggatccaaggag

SEQ ID NO: 527 - RNA, 19 nt, synthetic construct
  source 1..19: mol_type = other RNA
agtgactggatccaaggtg

SEQ ID NO: 528 - RNA, 19 nt, synthetic construct
  source 1..19: mol_type = other RNA
agtgactggatccaaggtg

SEQ ID NO: 529 - RNA, 19 nt, synthetic construct
  source 1..19: mol_type = other RNA
tgactggatccaaggacct

SEQ ID NO: 530 - RNA, 19 nt, synthetic construct
  source 1..19: mol_type = other RNA
tgactggatccaaggacct

SEQ ID NO: 531 - RNA, 19 nt, synthetic construct
  source 1..19: mol_type = other RNA
tgactggatccaaggacgt

SEQ ID NO: 532 - RNA, 19 nt, synthetic construct
  source 1..19: mol_type = other RNA
tgactggatccaaggacgt

SEQ ID NO: 533 - RNA, 19 nt, synthetic construct
  source 1..19: mol_type = other RNA
tgactggatccaaggaggt

SEQ ID NO: 534 - RNA, 19 nt, synthetic construct
  source 1..19: mol_type = other RNA
tgactggatccaaggaggt

SEQ ID NO: 535 - RNA, 19 nt, synthetic construct
  source 1..19: mol_type = other RNA
tgactggatccaaggtggt

SEQ ID NO: 536 - RNA, 19 nt, synthetic construct
  source 1..19: mol_type = other RNA
tgactggatccaaggtggt

SEQ ID NO: 537 - RNA, 19 nt, synthetic construct
  source 1..19: mol_type = other RNA
caatgatggagcatgacgc

SEQ ID NO: 538 - RNA, 19 nt, synthetic construct
  source 1..19: mol_type = other RNA
caatgatggagcatgacgc

SEQ ID NO: 539 - RNA, 19 nt, synthetic construct
  source 1..19: mol_type = other RNA
caatgatggagcatgtcgc

SEQ ID NO: 540 - RNA, 19 nt, synthetic construct
  source 1..19: mol_type = other RNA
caatgatggagcatgtcgc

SEQ ID NO: 541 - RNA, 19 nt, synthetic construct
  source 1..19: mol_type = other RNA
caatgatggagcatgtgcc

SEQ ID NO: 542 - RNA, 19 nt, synthetic construct
  source 1..19: mol_type = other RNA
caatgatggagcatgtgcc

SEQ ID NO: 543 - RNA, 19 nt, synthetic construct
  source 1..19: mol_type = other RNA
caatgatggagcatgtggc

SEQ ID NO: 544 - RNA, 19 nt, synthetic construct
  source 1..19: mol_type = other RNA
caatgatggagcatgtggc

SEQ ID NO: 545 - RNA, 19 nt, synthetic construct
  source 1..19: mol_type = other RNA
aatgatggagcatgtcgct

SEQ ID NO: 546 - RNA, 19 nt, synthetic construct
  source 1..19: mol_type = other RNA
aatgatggagcatgtcgct

SEQ ID NO: 547 - RNA, 19 nt, synthetic construct
  source 1..19: mol_type = other RNA
aatgatggagcatgtgcct

SEQ ID NO: 548 - RNA, 19 nt, synthetic construct
  source 1..19: mol_type = other RNA
aatgatggagcatgtgcct

SEQ ID NO: 549 - RNA, 19 nt, synthetic construct
  source 1..19: mol_type = other RNA
aatgatggagcatgtgcgt

SEQ ID NO: 550 - RNA, 19 nt, synthetic construct
  source 1..19: mol_type = other RNA
aatgatggagcatgtgcgt

SEQ ID NO: 551 - RNA, 19 nt, synthetic construct
  source 1..19: mol_type = other RNA
aatgatggagcatgtggct

SEQ ID NO: 552 - RNA, 19 nt, synthetic construct
  source 1..19: mol_type = other RNA
aatgatggagcatgtggct

SEQ ID NO: 553 - RNA, 19 nt, synthetic construct
  source 1..19: mol_type = other RNA
atgatggagcatgtgcctt

SEQ ID NO: 554 - RNA, 19 nt, synthetic construct
  source 1..19: mol_type = other RNA
atgatggagcatgtgcctt

SEQ ID NO: 555 - RNA, 19 nt, synthetic construct
  source 1..19: mol_type = other RNA
atgatggagcatgtgcgat

SEQ ID NO: 556 - RNA, 19 nt, synthetic construct
  source 1..19: mol_type = other RNA
atgatggagcatgtgcgat

SEQ ID NO: 557 - RNA, 19 nt, synthetic construct
  source 1..19: mol_type = other RNA
atgatggagcatgtgcgtt

SEQ ID NO: 558 - RNA, 19 nt, synthetic construct
  source 1..19: mol_type = other RNA
atgatggagcatgtgcgtt

SEQ ID NO: 559 - RNA, 19 nt, synthetic construct
  source 1..19: mol_type = other RNA
atgatggagcatgtggctt

SEQ ID NO: 560 - RNA, 19 nt, synthetic construct
  source 1..19: mol_type = other RNA
atgatggagcatgtggctt

SEQ ID NO: 561 - RNA, 19 nt, synthetic construct
  source 1..19: mol_type = other RNA
tgatggagcatgtgcctta

SEQ ID NO: 562 - RNA, 19 nt, synthetic construct
  source 1..19: mol_type = other RNA
tgatggagcatgtgcctta

SEQ ID NO: 563 - RNA, 19 nt, synthetic construct
  source 1..19: mol_type = other RNA
tgatggagcatgtgcgaaa

SEQ ID NO: 564 - RNA, 19 nt, synthetic construct
  source 1..19: mol_type = other RNA
tgatggagcatgtgcgaaa

SEQ ID NO: 565 - RNA, 19 nt, synthetic construct
  source 1..19: mol_type = other RNA
tgatggagcatgtgcgata

SEQ ID NO: 566 - RNA, 19 nt, synthetic construct
  source 1..19: mol_type = other RNA
tgatggagcatgtgcgata

SEQ ID NO: 567 - RNA, 19 nt, synthetic construct
  source 1..19: mol_type = other RNA
tgatggagcatgtgcgtta

SEQ ID NO: 568 - RNA, 19 nt, synthetic construct
  source 1..19: mol_type = other RNA
tgatggagcatgtgcgtta

SEQ ID NO: 569 - RNA, 19 nt, synthetic construct
  source 1..19: mol_type = other RNA
atggagcatgtgcgaaaag

SEQ ID NO: 570 - RNA, 19 nt, synthetic construct
  source 1..19: mol_type = other RNA
atggagcatgtgcgaaaag

SEQ ID NO: 571 - RNA, 19 nt, synthetic construct
  source 1..19: mol_type = other RNA
atggagcatgtgcgaatag

SEQ ID NO: 572 - RNA, 19 nt, synthetic construct
  source 1..19: mol_type = other RNA
atggagcatgtgcgaatag

SEQ ID NO: 573 - RNA, 19 nt, synthetic construct
  source 1..19: mol_type = other RNA
atggagcatgtgcgaattg

SEQ ID NO: 574 - RNA, 19 nt, synthetic construct
  source 1..19: mol_type = other RNA
atggagcatgtgcgaattg

SEQ ID NO: 575 - RNA, 19 nt, synthetic construct
  source 1..19: mol_type = other RNA
atggagcatgtgcgataag

SEQ ID NO: 576 - RNA, 19 nt, synthetic construct
  source 1..19: mol_type = other RNA
atggagcatgtgcgataag

SEQ ID NO: 577 - RNA, 19 nt, synthetic construct
  source 1..19: mol_type = other RNA
actggaccctcgaagcacc

SEQ ID NO: 578 - RNA, 19 nt, synthetic construct
  source 1..19: mol_type = other RNA
actggaccctcgaagcacc

SEQ ID NO: 579 - RNA, 19 nt, synthetic construct
  source 1..19: mol_type = other RNA
actggaccctcgaaggacc

SEQ ID NO: 580 - RNA, 19 nt, synthetic construct
  source 1..19: mol_type = other RNA
actggaccctcgaaggacc

SEQ ID NO: 581 - RNA, 19 nt, synthetic construct
  source 1..19: mol_type = other RNA
actggaccctcgaaggtcc

SEQ ID NO: 582 - RNA, 19 nt, synthetic construct
  source 1..19: mol_type = other RNA
actggaccctcgaaggtcc

SEQ ID NO: 583 - RNA, 19 nt, synthetic construct
  source 1..19: mol_type = other RNA
actggaccctcgaaggtgc

SEQ ID NO: 584 - RNA, 19 nt, synthetic construct
  source 1..19: mol_type = other RNA
actggaccctcgaaggtgc

SEQ ID NO: 585 - RNA, 19 nt, synthetic construct
  source 1..19: mol_type = other RNA
ctggaccctcgaaggacct

SEQ ID NO: 586 - RNA, 19 nt, synthetic construct
  source 1..19: mol_type = other RNA
ctggaccctcgaaggacct

SEQ ID NO: 587 - RNA, 19 nt, synthetic construct
  source 1..19: mol_type = other RNA
ctggaccctcgaaggtcct

SEQ ID NO: 588 - RNA, 19 nt, synthetic construct
  source 1..19: mol_type = other RNA
ctggaccctcgaaggtcct

SEQ ID NO: 589 - RNA, 19 nt, synthetic construct
  source 1..19: mol_type = other RNA
ctggaccctcgaaggtgct

SEQ ID NO: 590 - RNA, 19 nt, synthetic construct
  source 1..19: mol_type = other RNA
ctggaccctcgaaggtgct

SEQ ID NO: 591 - RNA, 19 nt, synthetic construct
  source 1..19: mol_type = other RNA
ctggaccctcgaaggtggt

SEQ ID NO: 592 - RNA, 19 nt, synthetic construct
  source 1..19: mol_type = other RNA
ctggaccctcgaaggtggt

SEQ ID NO: 593 - RNA, 19 nt, synthetic construct
  source 1..19: mol_type = other RNA
tggaccctcgaaggtcctt

SEQ ID NO: 594 - RNA, 19 nt, synthetic construct
  source 1..19: mol_type = other RNA
tggaccctcgaaggtcctt

SEQ ID NO: 595 - RNA, 19 nt, synthetic construct
  source 1..19: mol_type = other RNA
tggaccctcgaaggtgctt

SEQ ID NO: 596 - RNA, 19 nt, synthetic construct
  source 1..19: mol_type = other RNA
tggaccctcgaaggtgctt

SEQ ID NO: 597 - RNA, 19 nt, synthetic construct
  source 1..19: mol_type = other RNA
tggaccctcgaaggtggat

SEQ ID NO: 598 - RNA, 19 nt, synthetic construct
  source 1..19: mol_type = other RNA
tggaccctcgaaggtggat

SEQ ID NO: 599 - RNA, 19 nt, synthetic construct
  source 1..19: mol_type = other RNA
tggaccctcgaaggtggtt

SEQ ID NO: 600 - RNA, 19 nt, synthetic construct
  source 1..19: mol_type = other RNA
tggaccctcgaaggtggtt

SEQ ID NO: 601 - RNA, 19 nt, synthetic construct
  source 1..19: mol_type = other RNA
ggaccctcgaaggtgcttc

SEQ ID NO: 602 - RNA, 19 nt, synthetic construct
  source 1..19: mol_type = other RNA
ggaccctcgaaggtgcttc

SEQ ID NO: 603 - RNA, 19 nt, synthetic construct
  source 1..19: mol_type = other RNA
ggaccctcgaaggtggaac

SEQ ID NO: 604 - RNA, 19 nt, synthetic construct
  source 1..19: mol_type = other RNA
ggaccctcgaaggtggaac

SEQ ID NO: 605 - RNA, 19 nt, synthetic construct
  source 1..19: mol_type = other RNA
ggaccctcgaaggtggatc

SEQ ID NO: 606 - RNA, 19 nt, synthetic construct
  source 1..19: mol_type = other RNA
ggaccctcgaaggtggatc

SEQ ID NO: 607 - RNA, 19 nt, synthetic construct
  source 1..19: mol_type = other RNA
ggaccctcgaaggtggttc

SEQ ID NO: 608 - RNA, 19 nt, synthetic construct
  source 1..19: mol_type = other RNA
ggaccctcgaaggtggttc

SEQ ID NO: 609 - RNA, 19 nt, synthetic construct
  source 1..19: mol_type = other RNA
accaaaacctggctgcaac

SEQ ID NO: 610 - RNA, 19 nt, synthetic construct
  source 1..19: mol_type = other RNA
accaaaacctggctggtac

SEQ ID NO: 611 - RNA, 19 nt, synthetic construct
  source 1..19: mol_type = other RNA
accaaaacctggctgcaac

SEQ ID NO: 612 - RNA, 19 nt, synthetic construct
  source 1..19: mol_type = other RNA
accaaaacctggctggaac

SEQ ID NO: 613 - RNA, 19 nt, synthetic construct
  source 1..19: mol_type = other RNA
accaaaacctggctggaac

SEQ ID NO: 614 - RNA, 19 nt, synthetic construct
  source 1..19: mol_type = other RNA
accaaaacctggctggtac

SEQ ID NO: 615 - RNA, 19 nt, synthetic construct
  source 1..19: mol_type = other RNA
accaaaacctggctggttc

SEQ ID NO: 616 - RNA, 19 nt, synthetic construct
  source 1..19: mol_type = other RNA
accaaaacctggctggttc

SEQ ID NO: 617 - RNA, 19 nt, synthetic construct
  source 1..19: mol_type = other RNA
accagctggctgatgacga

SEQ ID NO: 618 - RNA, 19 nt, synthetic construct
  source 1..19: mol_type = other RNA
accagctggctgatgacga

SEQ ID NO: 619 - RNA, 19 nt, synthetic construct
  source 1..19: mol_type = other RNA
accagctggctgatgagca

SEQ ID NO: 620 - RNA, 19 nt, synthetic construct
  source 1..19: mol_type = other RNA
accagctggctgatgagca

SEQ ID NO: 621 - RNA, 19 nt, synthetic construct
  source 1..19: mol_type = other RNA
accagctggctgatgagga

SEQ ID NO: 622 - RNA, 19 nt, synthetic construct
  source 1..19: mol_type = other RNA
accagctggctgatgagga

SEQ ID NO: 623 - RNA, 19 nt, synthetic construct
  source 1..19: mol_type = other RNA
accagctggctgatgtcga

SEQ ID NO: 624 - RNA, 19 nt, synthetic construct
  source 1..19: mol_type = other RNA
accagctggctgatgtcga

SEQ ID NO: 625 - RNA, 19 nt, synthetic construct
  source 1..19: mol_type = other RNA
caaaacctggctggttgct

SEQ ID NO: 626 - RNA, 19 nt, synthetic construct
  source 1..19: mol_type = other RNA
caaaacctggctggttcct

SEQ ID NO: 627 - RNA, 19 nt, synthetic construct
  source 1..19: mol_type = other RNA
caaaacctggctggtacct

SEQ ID NO: 628 - RNA, 19 nt, synthetic construct
  source 1..19: mol_type = other RNA
caaaacctggctggtacct

SEQ ID NO: 629 - RNA, 19 nt, synthetic construct
  source 1..19: mol_type = other RNA
caaaacctggctggttcct

SEQ ID NO: 630 - RNA, 19 nt, synthetic construct
  source 1..19: mol_type = other RNA
caaaacctggctggttgct

SEQ ID NO: 631 - RNA, 19 nt, synthetic construct
  source 1..19: mol_type = other RNA
caaaacctggctggttggt

SEQ ID NO: 632 - RNA, 19 nt, synthetic construct
  source 1..19: mol_type = other RNA
caaaacctggctggttggt

SEQ ID NO: 633 - RNA, 19 nt, synthetic construct
  source 1..19: mol_type = other RNA
ccaaaacctggctggaacc

SEQ ID NO: 634 - RNA, 19 nt, synthetic construct
  source 1..19: mol_type = other RNA
ccaaaacctggctggaacc

SEQ ID NO: 635 - RNA, 19 nt, synthetic construct
  source 1..19: mol_type = other RNA
ccaaaacctggctggtacc

SEQ ID NO: 636 - RNA, 19 nt, synthetic construct
  source 1..19: mol_type = other RNA
ccaaaacctggctggtacc

SEQ ID NO: 637 - RNA, 19 nt, synthetic construct
  source 1..19: mol_type = other RNA
ccaaaacctggctggttcc

SEQ ID NO: 638 - RNA, 19 nt, synthetic construct
  source 1..19: mol_type = other RNA
ccaaaacctggctggttcc

SEQ ID NO: 639 - RNA, 19 nt, synthetic construct
  source 1..19: mol_type = other RNA
ccaaaacctggctggttgc

SEQ ID NO: 640 - RNA, 19 nt, synthetic construct
  source 1..19: mol_type = other RNA
ccaaaacctggctggttgc

SEQ ID NO: 641 - RNA, 20 nt, synthetic construct
  source 1..20: mol_type = other RNA
gatccagtcactaattccgg

SEQ ID NO: 642 - DNA, 20 bp, synthetic construct
  source 1..20: mol_type = other DNA
  misc_feature 1..19: note = RNA
  misc_feature 20: note = DNA
gatccagtcactaattccgt

SEQ ID NO: 643 - DNA, 20 bp, synthetic construct
  source 1..20: mol_type = other DNA
  misc_feature 1..19: note = RNA
  misc_feature 20: note = DNA
agagagattttggcacactt

SEQ ID NO: 644 - RNA, 20 nt, synthetic construct
  source 1..20: mol_type = other RNA
agagagattttggcacactc

SEQ ID NO: 645 - RNA, 20 nt, synthetic construct
  source 1..20: mol_type = other RNA
cagagagattttggcacact

SEQ ID NO: 646 - DNA, 20 bp, synthetic construct
  source 1..20: mol_type = other DNA
  misc_feature 1..19: note = RNA
  misc_feature 20: note = DNA
cagagagattttggcacact

SEQ ID NO: 647 - RNA, 21 nt, synthetic construct
  source 1..21: mol_type = other RNA
cagagagattttggcacactc

SEQ ID NO: 648 - RNA, 21 nt, synthetic construct
  source 1..21: mol_type = other RNA
cagagagattttggcacactt

SEQ ID NO: 649 - DNA, 21 bp, synthetic construct
  source 1..21: mol_type = other DNA
  misc_feature 1..19: note = RNA
  misc_feature 20..21: note = DNA
cagagagattttggcacactt

SEQ ID NO: 650 - RNA, 20 nt, synthetic construct
  source 1..20: mol_type = other RNA
ggtccttggatccagtcact

SEQ ID NO: 651 - DNA, 20 bp, synthetic construct
  source 1..20: mol_type = other DNA
  misc_feature 1..19: note = RNA
  misc_feature 20: note = DNA
ggtccttggatccagtcact

SEQ ID NO: 652 - RNA, 20 nt, synthetic construct
  source 1..20: mol_type = other RNA
aattcgcacatgctccatca

SEQ ID NO: 653 - DNA, 20 bp, synthetic construct
  source 1..20: mol_type = other DNA
  misc_feature 1..19: note = RNA
  misc_feature 20: note = DNA
aattcgcacatgctccatct

SEQ ID NO: 654 - RNA, 21 nt, synthetic construct
  source 1..21: mol_type = other RNA
aattcgcacatgctccatcat

SEQ ID NO: 655 - RNA, 21 nt, synthetic construct
  source 1..21: mol_type = other RNA
aattcgcacatgctccatctt

SEQ ID NO: 656 - DNA, 21 bp, synthetic construct
  source 1..21: mol_type = other DNA
  misc_feature 1..19: note = RNA
  misc_feature 20..21: note = DNA
aattcgcacatgctccatctt

SEQ ID NO: 657 - RNA, 20 nt, synthetic construct
  source 1..20: mol_type = other RNA
ggatccagtcactaattccg

SEQ ID NO: 658 - DNA, 20 bp, synthetic construct
  source 1..20: mol_type = other DNA
  misc_feature 1..19: note = RNA
  misc_feature 20: note = DNA
ggatccagtcactaattcct

SEQ ID NO: 659 - RNA, 21 nt, synthetic construct
  source 1..21: mol_type = other RNA
ggatccagtcactaattccgg

SEQ ID NO: 660 - RNA, 21 nt, synthetic construct
  source 1..21: mol_type = other RNA
ggatccagtcactaattcctt

SEQ ID NO: 661 - DNA, 21 bp, synthetic construct
  source 1..21: mol_type = other DNA
  misc_feature 1..19: note = RNA
  misc_feature 20..21: note = DNA
ggatccagtcactaattcctt

SEQ ID NO: 662 - RNA, 20 nt, synthetic construct
  source 1..20: mol_type = other RNA
ccagagagattttggcacac

SEQ ID NO: 663 - DNA, 20 bp, synthetic construct
  source 1..20: mol_type = other DNA
  misc_feature 1..19: note = RNA
  misc_feature 20: note = DNA
ccagagagattttggcacat

SEQ ID NO: 664 - RNA, 20 nt, synthetic construct
  source 1..20: mol_type = other RNA
ccttggatccagtcactaat

SEQ ID NO: 665 - DNA, 20 bp, synthetic construct
  source 1..20: mol_type = other DNA
  misc_feature 1..19: note = RNA
  misc_feature 20: note = DNA
ccttggatccagtcactaat

SEQ ID NO: 666 - RNA, 21 nt, synthetic construct
  source 1..21: mol_type = other RNA
ccttggatccagtcactaatt

SEQ ID NO: 667 - RNA, 21 nt, synthetic construct
  source 1..21: mol_type = other RNA
ccttggatccagtcactaatt

SEQ ID NO: 668 - DNA, 21 bp, synthetic construct
  source 1..21: mol_type = other DNA
  misc_feature 1..19: note = RNA
  misc_feature 20..21: note = DNA
ccttggatccagtcactaatt

SEQ ID NO: 669 - RNA, 20 nt, synthetic construct
  source 1..20: mol_type = other RNA
cttggatccagtcactaatt

SEQ ID NO: 670 - DNA, 20 bp, synthetic construct
  source 1..20: mol_type = other DNA
  misc_feature 1..19: note = RNA
  misc_feature 20: note = DNA
cttggatccagtcactaatt

SEQ ID NO: 671 - RNA, 21 nt, synthetic construct
  source 1..21: mol_type = other RNA
cttggatccagtcactaattc

SEQ ID NO: 672 - RNA, 21 nt, synthetic construct
  source 1..21: mol_type = other RNA
cttggatccagtcactaattt

SEQ ID NO: 673 - DNA, 21 bp, synthetic construct
  source 1..21: mol_type = other DNA
  misc_feature 1..19: note = RNA
  misc_feature 20..21: note = DNA
cttggatccagtcactaattt

SEQ ID NO: 674 - RNA, 20 nt, synthetic construct
  source 1..20: mol_type = other RNA
tggatccagtcactaattcc

SEQ ID NO: 675 - DNA, 20 bp, synthetic construct
  source 1..20: mol_type = other DNA
  misc_feature 1..19: note = RNA
  misc_feature 20: note = DNA
tggatccagtcactaattct

SEQ ID NO: 676 - RNA, 21 nt, synthetic construct
  source 1..21: mol_type = other RNA
tggatccagtcactaattccg

SEQ ID NO: 677 - RNA, 21 nt, synthetic construct
  source 1..21: mol_type = other RNA
tggatccagtcactaattctt

SEQ ID NO: 678 - DNA, 21 bp, synthetic construct
  source 1..21: mol_type = other DNA
  misc_feature 1..19: note = RNA
  misc_feature 20..21: note = DNA
tggatccagtcactaattctt

SEQ ID NO: 679 - RNA, 20 nt, synthetic construct
  source 1..20: mol_type = other RNA
ttggatccagtcactaattc

SEQ ID NO: 680 - DNA, 20 bp, synthetic construct
  source 1..20: mol_type = other DNA
  misc_feature 1..19: note = RNA
  misc_feature 20: note = DNA
ttggatccagtcactaattt

SEQ ID NO: 681 - RNA, 21 nt, synthetic construct
  source 1..21: mol_type = other RNA
ttggatccagtcactaattcc

SEQ ID NO: 682 - RNA, 21 nt, synthetic construct
  source 1..21: mol_type = other RNA
ttggatccagtcactaatttt

SEQ ID NO: 683 - DNA, 21 bp, synthetic construct
  source 1..21: mol_type = other DNA
  misc_feature 1..19: note = RNA
  misc_feature 20..21: note = DNA
ttggatccagtcactaatttt

SEQ ID NO: 684 - RNA, 20 nt, synthetic construct
  source 1..20: mol_type = other RNA
tccttggatccagtcactaa

SEQ ID NO: 685 - DNA, 20 bp, synthetic construct
  source 1..20: mol_type = other DNA
  misc_feature 1..19: note = RNA
  misc_feature 20: note = DNA
tccttggatccagtcactat

SEQ ID NO: 686 - RNA, 21 nt, synthetic construct
  source 1..21: mol_type = other RNA
tccttggatccagtcactaat

SEQ ID NO: 687 - RNA, 21 nt, synthetic construct
  source 1..21: mol_type = other RNA
tccttggatccagtcactatt

SEQ ID NO: 688 - DNA, 21 bp, synthetic construct
  source 1..21: mol_type = other DNA
  misc_feature 1..19: note = RNA
  misc_feature 20..21: note = DNA
tccttggatccagtcactatt

SEQ ID NO: 689 - RNA, 20 nt, synthetic construct
  source 1..20: mol_type = other RNA
gtccttggatccagtcacta

SEQ ID NO: 690 - DNA, 20 bp, synthetic construct
  source 1..20: mol_type = other DNA
  misc_feature 1..19: note = RNA
  misc_feature 20: note = DNA
gtccttggatccagtcactt

SEQ ID NO: 691 - RNA, 21 nt, synthetic construct
  source 1..21: mol_type = other RNA
gtccttggatccagtcactaa

SEQ ID NO: 692 - RNA, 21 nt, synthetic construct
  source 1..21: mol_type = other RNA
gtccttggatccagtcacttt

SEQ ID NO: 693 - DNA, 21 bp, synthetic construct
  source 1..21: mol_type = other DNA
  misc_feature 1..19: note = RNA
  misc_feature 20..21: note = DNA
gtccttggatccagtcacttt

SEQ ID NO: 694 - RNA, 20 nt, synthetic construct
  source 1..20: mol_type = other RNA
gcacatgctccatcattggc

SEQ ID NO: 695 - DNA, 20 bp, synthetic construct
  source 1..20: mol_type = other DNA
  misc_feature 1..19: note = RNA
  misc_feature 20: note = DNA
gcacatgctccatcattggt

SEQ ID NO: 696 - RNA, 20 nt, synthetic construct
  source 1..20: mol_type = other RNA
cgcacatgctccatcattgg

SEQ ID NO: 697 - DNA, 20 bp, synthetic construct
  source 1..20: mol_type = other DNA
  misc_feature 1..19: note = RNA
  misc_feature 20: note = DNA
cgcacatgctccatcattgt

SEQ ID NO: 698 - RNA, 21 nt, synthetic construct
  source 1..21: mol_type = other RNA
cgcacatgctccatcattggc

SEQ ID NO: 699 - RNA, 21 nt, synthetic construct
  source 1..21: mol_type = other RNA
cgcacatgctccatcattgtt

SEQ ID NO: 700 - DNA, 21 bp, synthetic construct
  source 1..21: mol_type = other DNA
  misc_feature 1..19: note = RNA
  misc_feature 20..21: note = DNA
cgcacatgctccatcattgtt

SEQ ID NO: 701 - RNA, 20 nt, synthetic construct
  source 1..20: mol_type = other RNA
tcgcacatgctccatcattg

SEQ ID NO: 702 - DNA, 20 bp, synthetic construct
  source 1..20: mol_type = other DNA
  misc_feature 1..19: note = RNA
  misc_feature 20: note = DNA
tcgcacatgctccatcattt

SEQ ID NO: 703 - RNA, 21 nt, synthetic construct
  source 1..21: mol_type = other RNA
tcgcacatgctccatcattgg

SEQ ID NO: 704 - RNA, 21 nt, synthetic construct
  source 1..21: mol_type = other RNA
tcgcacatgctccatcatttt

SEQ ID NO: 705 - DNA, 21 bp, synthetic construct
  source 1..21: mol_type = other DNA
  misc_feature 1..19: note = RNA
  misc_feature 20..21: note = DNA
tcgcacatgctccatcatttt

SEQ ID NO: 706 - RNA, 20 nt, synthetic construct
  source 1..20: mol_type = other RNA
ttcgcacatgctccatcatt

SEQ ID NO: 707 - DNA, 20 bp, synthetic construct
  source 1..20: mol_type = other DNA
  misc_feature 1..19: note = RNA
  misc_feature 20: note = DNA
ttcgcacatgctccatcatt

SEQ ID NO: 708 - RNA, 21 nt, synthetic construct
  source 1..21: mol_type = other RNA
ttcgcacatgctccatcattg

SEQ ID NO: 709 - RNA, 21 nt, synthetic construct
  source 1..21: mol_type = other RNA
ttcgcacatgctccatcattt

SEQ ID NO: 710 - DNA, 21 bp, synthetic construct
  source 1..21: mol_type = other DNA
  misc_feature 1..19: note = RNA
  misc_feature 20..21: note = DNA
ttcgcacatgctccatcattt

SEQ ID NO: 711 - RNA, 20 nt, synthetic construct
  source 1..20: mol_type = other RNA
attcgcacatgctccatcat

SEQ ID NO: 712 - DNA, 20 bp, synthetic construct
  source 1..20: mol_type = other DNA
  misc_feature 1..19: note = RNA
  misc_feature 20: note = DNA
attcgcacatgctccatcat

SEQ ID NO: 713 - RNA, 21 nt, synthetic construct
  source 1..21: mol_type = other RNA
attcgcacatgctccatcatt

SEQ ID NO: 714 - RNA, 21 nt, synthetic construct
  source 1..21: mol_type = other RNA
attcgcacatgctccatcatt

SEQ ID NO: 715 - DNA, 21 bp, synthetic construct
  source 1..21: mol_type = other DNA
  misc_feature 1..19: note = RNA
  misc_feature 20..21: note = DNA
attcgcacatgctccatcatt

SEQ ID NO: 716 - RNA, 20 nt, synthetic construct
  source 1..20: mol_type = other RNA
gaattcgcacatgctccatc

SEQ ID NO: 717 - DNA, 20 bp, synthetic construct
  source 1..20: mol_type = other DNA
  misc_feature 1..19: note = RNA
  misc_feature 20: note = DNA
gaattcgcacatgctccatt

SEQ ID NO: 718 - RNA, 20 nt, synthetic construct
  source 1..20: mol_type = other RNA
caccttcgagggtccagttc

SEQ ID NO: 719 - DNA, 20 bp, synthetic construct
  source 1..20: mol_type = other DNA
  misc_feature 1..19: note = RNA
  misc_feature 20: note = DNA
caccttcgagggtccagttt

SEQ ID NO: 720 - RNA, 20 nt, synthetic construct
  source 1..20: mol_type = other RNA
ccaccttcgagggtccagtt

SEQ ID NO: 721 - DNA, 20 bp, synthetic construct
  source 1..20: mol_type = other DNA
  misc_feature 1..19: note = RNA
  misc_feature 20: note = DNA
ccaccttcgagggtccagtt

SEQ ID NO: 722 - RNA, 21 nt, synthetic construct
  source 1..21: mol_type = other RNA
ccaccttcgagggtccagttc

SEQ ID NO: 723 - RNA, 21 nt, synthetic construct
  source 1..21: mol_type = other RNA
ccaccttcgagggtccagttt

SEQ ID NO: 724 - DNA, 21 bp, synthetic construct
  source 1..21: mol_type = other DNA
  misc_feature 1..19: note = RNA
  misc_feature 20..21: note = DNA
ccaccttcgagggtccagttt

SEQ ID NO: 725 - RNA, 20 nt, synthetic construct
  source 1..20: mol_type = other RNA
tccaccttcgagggtccagt

SEQ ID NO: 726 - DNA, 20 bp, synthetic construct
  source 1..20: mol_type = other DNA
  misc_feature 1..19: note = RNA
  misc_feature 20: note = DNA
tccaccttcgagggtccagt

SEQ ID NO: 727 - RNA, 21 nt, synthetic construct
  source 1..21: mol_type = other RNA
tccaccttcgagggtccagtt

SEQ ID NO: 728 - RNA, 21 nt, synthetic construct
  source 1..21: mol_type = other RNA
tccaccttcgagggtccagtt

SEQ ID NO: 729 - DNA, 21 bp, synthetic construct
  source 1..21: mol_type = other DNA
  misc_feature 1..19: note = RNA
  misc_feature 20..21: note = DNA
tccaccttcgagggtccagtt

SEQ ID NO: 730 - RNA, 20 nt, synthetic construct
  source 1..20: mol_type = other RNA
ttccaccttcgagggtccag

SEQ ID NO: 731 - DNA, 20 bp, synthetic construct
  source 1..20: mol_type = other DNA
  misc_feature 1..19: note = RNA
  misc_feature 20: note = DNA
ttccaccttcgagggtccat

SEQ ID NO: 732 - RNA, 21 nt, synthetic construct
  source 1..21: mol_type = other RNA
ttccaccttcgagggtccagt

SEQ ID NO: 733 - RNA, 21 nt, synthetic construct
  source 1..21: mol_type = other RNA
ttccaccttcgagggtccatt

SEQ ID NO: 734 - DNA, 21 bp, synthetic construct
  source 1..21: mol_type = other DNA
  misc_feature 1..19: note = RNA
  misc_feature 20..21: note = DNA
ttccaccttcgagggtccatt

SEQ ID NO: 735 - RNA, 20 nt, synthetic construct
  source 1..20: mol_type = other RNA
cttccaccttcgagggtcca

SEQ ID NO: 736 - DNA, 20 bp, synthetic construct
  source 1..20: mol_type = other DNA
  misc_feature 1..19: note = RNA
  misc_feature 20: note = DNA
cttccaccttcgagggtcct

SEQ ID NO: 737 - RNA, 21 nt, synthetic construct
  source 1..21: mol_type = other RNA
caaccagccaggttttggtcc

SEQ ID NO: 738 - RNA, 20 nt, synthetic construct
  source 1..20: mol_type = other RNA
caaccagccaggttttggtc

SEQ ID NO: 739 - DNA, 20 bp, synthetic construct
  source 1..20: mol_type = other DNA
  misc_feature 1..19: note = RNA
  misc_feature 20: note = DNA
caaccagccaggttttggtt

SEQ ID NO: 740 - RNA, 21 nt, synthetic construct
  source 1..21: mol_type = other RNA
caaccagccaggttttggttt

SEQ ID NO: 741 - DNA, 21 bp, synthetic construct
  source 1..21: mol_type = other DNA
  misc_feature 1..19: note = RNA
  misc_feature 20..21: note = DNA
caaccagccaggttttggttt

SEQ ID NO: 742 - RNA, 20 nt, synthetic construct
  source 1..20: mol_type = other RNA
gctcatcagccagctggtgt

SEQ ID NO: 743 - DNA, 20 bp, synthetic construct
  source 1..20: mol_type = other DNA
  misc_feature 1..19: note = RNA
  misc_feature 20: note = DNA
gctcatcagccagctggtgt

SEQ ID NO: 744 - RNA, 20 nt, synthetic construct
  source 1..20: mol_type = other RNA
aaccagccaggttttggtcc

SEQ ID NO: 745 - DNA, 20 bp, synthetic construct
  source 1..20: mol_type = other DNA
  misc_feature 1..19: note = RNA
  misc_feature 20: note = DNA
aaccagccaggttttggtct

SEQ ID NO: 746 - RNA, 20 nt, synthetic construct
  source 1..20: mol_type = other RNA
ccaaccagccaggttttggt

SEQ ID NO: 747 - DNA, 20 bp, synthetic construct
  source 1..20: mol_type = other DNA
  misc_feature 1..19: note = RNA
  misc_feature 20: note = DNA
ccaaccagccaggttttggt

SEQ ID NO: 748 - RNA, 20 nt, synthetic construct
  source 1..20: mol_type = other RNA
cggaattagtgactggatcc

SEQ ID NO: 749 - DNA, 20 bp, synthetic construct
  source 1..20: mol_type = other DNA
  misc_feature 1..19: note = RNA
  misc_feature 20: note = DNA
cggaattagtgactggatct

SEQ ID NO: 750 - DNA, 20 bp, synthetic construct
  source 1..20: mol_type = other DNA
  misc_feature 1..19: note = RNA
  misc_feature 20: note = DNA
agtgtgccaaaatctctctt

SEQ ID NO: 751 - RNA, 20 nt, synthetic construct
  source 1..20: mol_type = other RNA
agtgtgccaaaatctctctg

SEQ ID NO: 752 - RNA, 20 nt, synthetic construct
  source 1..20: mol_type = other RNA
gtgtgccaaaatctctctgg

SEQ ID NO: 753 - DNA, 20 bp, synthetic construct
  source 1..20: mol_type = other DNA
  misc_feature 1..19: note = RNA
  misc_feature 20: note = DNA
gtgtgccaaaatctctctgt

SEQ ID NO: 754 - RNA, 21 nt, synthetic construct
  source 1..21: mol_type = other RNA
gtgtgccaaaatctctctgga

SEQ ID NO: 755 - RNA, 21 nt, synthetic construct
  source 1..21: mol_type = other RNA
gtgtgccaaaatctctctgtt

SEQ ID NO: 756 - DNA, 21 bp, synthetic construct
  source 1..21: mol_type = other DNA
  misc_feature 1..19: note = RNA
  misc_feature 20..21: note = DNA
gtgtgccaaaatctctctgtt

SEQ ID NO: 757 - RNA, 20 nt, synthetic construct
  source 1..20: mol_type = other RNA
gtgactggatccaaggacca

SEQ ID NO: 758 - DNA, 20 bp, synthetic construct
  source 1..20: mol_type = other DNA
  misc_feature 1..19: note = RNA
  misc_feature 20: note = DNA
gtgactggatccaaggacct

SEQ ID NO: 759 - RNA, 20 nt, synthetic construct
  source 1..20: mol_type = other RNA
gatggagcatgtgcgaattc

SEQ ID NO: 760 - DNA, 20 bp, synthetic construct
  source 1..20: mol_type = other DNA
  misc_feature 1..19: note = RNA
  misc_feature 20: note = DNA
gatggagcatgtgcgaattt

SEQ ID NO: 761 - RNA, 21 nt, synthetic construct
  source 1..21: mol_type = other RNA
gatggagcatgtgcgaattca

SEQ ID NO: 762 - RNA, 21 nt, synthetic construct
  source 1..21: mol_type = other RNA
gatggagcatgtgcgaatttt

SEQ ID NO: 763 - DNA, 21 bp, synthetic construct
  source 1..21: mol_type = other DNA
  misc_feature 1..19: note = RNA
  misc_feature 20..21: note = DNA
gatggagcatgtgcgaatttt

SEQ ID NO: 764 - RNA, 20 nt, synthetic construct
  source 1..20: mol_type = other RNA
ggaattagtgactggatcca

SEQ ID NO: 765 - DNA, 20 bp, synthetic construct
  source 1..20: mol_type = other DNA
  misc_feature 1..19: note = RNA
  misc_feature 20: note = DNA
ggaattagtgactggatcct

SEQ ID NO: 766 - RNA, 21 nt, synthetic construct
  source 1..21: mol_type = other RNA
ggaattagtgactggatccaa

SEQ ID NO: 767 - RNA, 21 nt, synthetic construct
  source 1..21: mol_type = other RNA
ggaattagtgactggatcctt

SEQ ID NO: 768 - DNA, 21 bp, synthetic construct
  source 1..21: mol_type = other DNA
  misc_feature 1..19: note = RNA
  misc_feature 20..21: note = DNA
ggaattagtgactggatcctt

SEQ ID NO: 769 - RNA, 20 nt, synthetic construct
  source 1..20: mol_type = other RNA
tgtgccaaaatctctctgga

SEQ ID NO: 770 - DNA, 20 bp, synthetic construct
  source 1..20: mol_type = other DNA
  misc_feature 1..19: note = RNA
  misc_feature 20: note = DNA
tgtgccaaaatctctctggt

SEQ ID NO: 771 - RNA, 20 nt, synthetic construct
  source 1..20: mol_type = other RNA
ttagtgactggatccaagga

SEQ ID NO: 772 - DNA, 20 bp, synthetic construct
  source 1..20: mol_type = other DNA
  misc_feature 1..19: note = RNA
  misc_feature 20: note = DNA
ttagtgactggatccaaggt

SEQ ID NO: 773 - RNA, 21 nt, synthetic construct
  source 1..21: mol_type = other RNA
ttagtgactggatccaaggac

SEQ ID NO: 774 - RNA, 21 nt, synthetic construct
  source 1..21: mol_type = other RNA
ttagtgactggatccaaggtt

SEQ ID NO: 775 - DNA, 21 bp, synthetic construct
  source 1..21: mol_type = other DNA
  misc_feature 1..19: note = RNA
  misc_feature 20..21: note = DNA
ttagtgactggatccaaggtt

SEQ ID NO: 776 - RNA, 20 nt, synthetic construct
  source 1..20: mol_type = other RNA
attagtgactggatccaagg

SEQ ID NO: 777 - DNA, 20 bp, synthetic construct
  source 1..20: mol_type = other DNA
  misc_feature 1..19: note = RNA
  misc_feature 20: note = DNA
attagtgactggatccaagt

SEQ ID NO: 778 - RNA, 21 nt, synthetic construct
  source 1..21: mol_type = other RNA
attagtgactggatccaagga

SEQ ID NO: 779 - RNA, 21 nt, synthetic construct
  source 1..21: mol_type = other RNA
attagtgactggatccaagtt

SEQ ID NO: 780 - DNA, 21 bp, synthetic construct
  source 1..21: mol_type = other DNA
  misc_feature 1..19: note = RNA
  misc_feature 20..21: note = DNA
attagtgactggatccaagtt

SEQ ID NO: 781 - RNA, 20 nt, synthetic construct
  source 1..20: mol_type = other RNA
gaattagtgactggatccaa

SEQ ID NO: 782 - DNA, 20 bp, synthetic construct
  source 1..20: mol_type = other DNA
  misc_feature 1..19: note = RNA
  misc_feature 20: note = DNA
gaattagtgactggatccat

SEQ ID NO: 783 - RNA, 21 nt, synthetic construct
  source 1..21: mol_type = other RNA
gaattagtgactggatccaag

SEQ ID NO: 784 - RNA, 21 nt, synthetic construct
  source 1..21: mol_type = other RNA
gaattagtgactggatccatt

SEQ ID NO: 785 - DNA, 21 bp, synthetic construct
  source 1..21: mol_type = other DNA
  misc_feature 1..19: note = RNA
  misc_feature 20..21: note = DNA
gaattagtgactggatccatt

SEQ ID NO: 786 - RNA, 20 nt, synthetic construct
  source 1..20: mol_type = other RNA
aattagtgactggatccaag

SEQ ID NO: 787 - DNA, 20 bp, synthetic construct
  source 1..20: mol_type = other DNA
  misc_feature 1..19: note = RNA
  misc_feature 20: note = DNA
aattagtgactggatccaat

SEQ ID NO: 788 - RNA, 21 nt, synthetic construct
  source 1..21: mol_type = other RNA
aattagtgactggatccaagg

SEQ ID NO: 789 - RNA, 21 nt, synthetic construct
  source 1..21: mol_type = other RNA
aattagtgactggatccaatt

SEQ ID NO: 790 - DNA, 21 bp, synthetic construct
  source 1..21: mol_type = other DNA
  misc_feature 1..19: note = RNA
  misc_feature 20..21: note = DNA
aattagtgactggatccaatt

SEQ ID NO: 791 - RNA, 20 nt, synthetic construct
  source 1..20: mol_type = other RNA
tagtgactggatccaaggac

SEQ ID NO: 792 - DNA, 20 bp, synthetic construct
  source 1..20: mol_type = other DNA
  misc_feature 1..19: note = RNA
  misc_feature 20: note = DNA
tagtgactggatccaaggat

SEQ ID NO: 793 - RNA, 21 nt, synthetic construct
  source 1..21: mol_type = other RNA
tagtgactggatccaaggacc

SEQ ID NO: 794 - RNA, 21 nt, synthetic construct
  source 1..21: mol_type = other RNA
tagtgactggatccaaggatt

SEQ ID NO: 795 - DNA, 21 bp, synthetic construct
  source 1..21: mol_type = other DNA
  misc_feature 1..19: note = RNA
  misc_feature 20..21: note = DNA
tagtgactggatccaaggatt

SEQ ID NO: 796 - RNA, 20 nt, synthetic construct
  source 1..20: mol_type = other RNA
agtgactggatccaaggacc

SEQ ID NO: 797 - DNA, 20 bp, synthetic construct
  source 1..20: mol_type = other DNA
  misc_feature 1..19: note = RNA
  misc_feature 20: note = DNA
agtgactggatccaaggact

SEQ ID NO: 798 - RNA, 21 nt, synthetic construct
  source 1..21: mol_type = other RNA
agtgactggatccaaggacca

SEQ ID NO: 799 - RNA, 21 nt, synthetic construct
  source 1..21: mol_type = other RNA
agtgactggatccaaggactt

SEQ ID NO: 800 - DNA, 21 bp, synthetic construct
  source 1..21: mol_type = other DNA
  misc_feature 1..19: note = RNA
  misc_feature 20..21: note = DNA
agtgactggatccaaggactt

SEQ ID NO: 801 - RNA, 20 nt, synthetic construct
  source 1..20: mol_type = other RNA
ccaatgatggagcatgtgcg

SEQ ID NO: 802 - DNA, 20 bp, synthetic construct
  source 1..20: mol_type = other DNA
  misc_feature 1..19: note = RNA
  misc_feature 20: note = DNA
ccaatgatggagcatgtgct

SEQ ID NO: 803 - RNA, 20 nt, synthetic construct
  source 1..20: mol_type = other RNA
caatgatggagcatgtgcga

SEQ ID NO: 804 - DNA, 20 bp, synthetic construct
  source 1..20: mol_type = other DNA
  misc_feature 1..19: note = RNA
  misc_feature 20: note = DNA
caatgatggagcatgtgcgt

SEQ ID NO: 805 - RNA, 21 nt, synthetic construct
  source 1..21: mol_type = other RNA
caatgatggagcatgtgcgaa

SEQ ID NO: 806 - RNA, 21 nt, synthetic construct
  source 1..21: mol_type = other RNA
caatgatggagcatgtgcgtt

SEQ ID NO: 807 - DNA, 21 bp, synthetic construct
  source 1..21: mol_type = other DNA
  misc_feature 1..19: note = RNA
  misc_feature 20..21: note = DNA
caatgatggagcatgtgcgtt

SEQ ID NO: 808 - RNA, 20 nt, synthetic construct
  source 1..20: mol_type = other RNA
aatgatggagcatgtgcgaa

SEQ ID NO: 809 - DNA, 20 bp, synthetic construct
  source 1..20: mol_type = other DNA
  misc_feature 1..19: note = RNA
  misc_feature 20: note = DNA
aatgatggagcatgtgcgat

SEQ ID NO: 810 - RNA, 21 nt, synthetic construct
  source 1..21: mol_type = other RNA
aatgatggagcatgtgcgaat

SEQ ID NO: 811 - RNA, 21 nt, synthetic construct
  source 1..21: mol_type = other RNA
aatgatggagcatgtgcgatt

SEQ ID NO: 812 - DNA, 21 bp, synthetic construct
  source 1..21: mol_type = other DNA
  misc_feature 1..19: note = RNA
  misc_feature 20..21: note = DNA
aatgatggagcatgtgcgatt

SEQ ID NO: 813 - RNA, 20 nt, synthetic construct
  source 1..20: mol_type = other RNA
atgatggagcatgtgcgaat

SEQ ID NO: 814 - DNA, 20 bp, synthetic construct
  source 1..20: mol_type = other DNA
  misc_feature 1..19: note = RNA
  misc_feature 20: note = DNA
atgatggagcatgtgcgaat

SEQ ID NO: 815 - RNA, 21 nt, synthetic construct
  source 1..21: mol_type = other RNA
atgatggagcatgtgcgaatt

SEQ ID NO: 816 - RNA, 21 nt, synthetic construct
  source 1..21: mol_type = other RNA
atgatggagcatgtgcgaatt

SEQ ID NO: 817 - DNA, 21 bp, synthetic construct
  source 1..21: mol_type = other DNA
  misc_feature 1..19: note = RNA
  misc_feature 20..21: note = DNA
atgatggagcatgtgcgaatt

SEQ ID NO: 818 - RNA, 20 nt, synthetic construct
  source 1..20: mol_type = other RNA
tgatggagcatgtgcgaatt

SEQ ID NO: 819 - DNA, 20 bp, synthetic construct
  source 1..20: mol_type = other DNA
  misc_feature 1..19: note = RNA
  misc_feature 20: note = DNA
tgatggagcatgtgcgaatt

SEQ ID NO: 820 - RNA, 21 nt, synthetic construct
  source 1..21: mol_type = other RNA
tgatggagcatgtgcgaattc

SEQ ID NO: 821 - RNA, 21 nt, synthetic construct
  source 1..21: mol_type = other RNA
tgatggagcatgtgcgaattt

SEQ ID NO: 822 - DNA, 21 bp, synthetic construct
  source 1..21: mol_type = other DNA
  misc_feature 1..19: note = RNA
  misc_feature 20..21: note = DNA
tgatggagcatgtgcgaattt

SEQ ID NO: 823 - RNA, 20 nt, synthetic construct
  source 1..20: mol_type = other RNA
atggagcatgtgcgaattca

SEQ ID NO: 824 - DNA, 20 bp, synthetic construct
  source 1..20: mol_type = other DNA
  misc_feature 1..19: note = RNA
  misc_feature 20: note = DNA
atggagcatgtgcgaattct

SEQ ID NO: 825 - RNA, 20 nt, synthetic construct
  source 1..20: mol_type = other RNA
aactggaccctcgaaggtgg

SEQ ID NO: 826 - DNA, 20 bp, synthetic construct
  source 1..20: mol_type = other DNA
  misc_feature 1..19: note = RNA
  misc_feature 20: note = DNA
aactggaccctcgaaggtgt

SEQ ID NO: 827 - RNA, 20 nt, synthetic construct
  source 1..20: mol_type = other RNA
actggaccctcgaaggtgga

SEQ ID NO: 828 - DNA, 20 bp, synthetic construct
  source 1..20: mol_type = other DNA
  misc_feature 1..19: note = RNA
  misc_feature 20: note = DNA
actggaccctcgaaggtggt

SEQ ID NO: 829 - RNA, 21 nt, synthetic construct
  source 1..21: mol_type = other RNA
actggaccctcgaaggtggaa

SEQ ID NO: 830 - RNA, 21 nt, synthetic construct
  source 1..21: mol_type = other RNA
actggaccctcgaaggtggtt

SEQ ID NO: 831 - DNA, 21 bp, synthetic construct
  source 1..21: mol_type = other DNA
  misc_feature 1..19: note = RNA
  misc_feature 20..21: note = DNA
actggaccctcgaaggtggtt

SEQ ID NO: 832 - RNA, 20 nt, synthetic construct
  source 1..20: mol_type = other RNA
ctggaccctcgaaggtggaa

SEQ ID NO: 833 - DNA, 20 bp, synthetic construct
  source 1..20: mol_type = other DNA
  misc_feature 1..19: note = RNA
  misc_feature 20: note = DNA
ctggaccctcgaaggtggat

SEQ ID NO: 834 - RNA, 21 nt, synthetic construct
  source 1..21: mol_type = other RNA
ctggaccctcgaaggtggaag

SEQ ID NO: 835 - RNA, 21 nt, synthetic construct
  source 1..21: mol_type = other RNA
ctggaccctcgaaggtggatt

SEQ ID NO: 836 - DNA, 21 bp, synthetic construct
  source 1..21: mol_type = other DNA
  misc_feature 1..19: note = RNA
  misc_feature 20..21: note = DNA
ctggaccctcgaaggtggatt

SEQ ID NO: 837 - RNA, 20 nt, synthetic construct
  source 1..20: mol_type = other RNA
tggaccctcgaaggtggaag

SEQ ID NO: 838 - DNA, 20 bp, synthetic construct
  source 1..20: mol_type = other DNA
  misc_feature 1..19: note = RNA
  misc_feature 20: note = DNA
tggaccctcgaaggtggaat

SEQ ID NO: 839 - RNA, 21 nt, synthetic construct
  source 1..21: mol_type = other RNA
tggaccctcgaaggtggaaga

SEQ ID NO: 840 - RNA, 21 nt, synthetic construct
  source 1..21: mol_type = other RNA
tggaccctcgaaggtggaatt

SEQ ID NO: 841 - DNA, 21 bp, synthetic construct
  source 1..21: mol_type = other DNA
  misc_feature 1..19: note = RNA
  misc_feature 20..21: note = DNA
tggaccctcgaaggtggaatt

SEQ ID NO: 842 - RNA, 20 nt, synthetic construct
  source 1..20: mol_type = other RNA
ggaccctcgaaggtggaaga

SEQ ID NO: 843 - DNA, 20 bp, synthetic construct
  source 1..20: mol_type = other DNA
  misc_feature 1..19: note = RNA
  misc_feature 20: note = DNA
ggaccctcgaaggtggaagt

SEQ ID NO: 844 - RNA, 21 nt, synthetic construct
  source 1..21: mol_type = other RNA
accaaaacctggctggttgga

SEQ ID NO: 845 - RNA, 20 nt, synthetic construct
  source 1..20: mol_type = other RNA
accaaaacctggctggttgg

SEQ ID NO: 846 - DNA, 20 bp, synthetic construct
  source 1..20: mol_type = other DNA
  misc_feature 1..19: note = RNA
  misc_feature 20: note = DNA
accaaaacctggctggttgt

SEQ ID NO: 847 - RNA, 21 nt, synthetic construct
  source 1..21: mol_type = other RNA
accaaaacctggctggttgtt

SEQ ID NO: 848 - DNA, 21 bp, synthetic construct
  source 1..21: mol_type = other DNA
  misc_feature 1..19: note = RNA
  misc_feature 20..21: note = DNA
accaaaacctggctggttgtt

SEQ ID NO: 849 - RNA, 20 nt, synthetic construct
  source 1..20: mol_type = other RNA
caccagctggctgatgagct

SEQ ID NO: 850 - DNA, 20 bp, synthetic construct
  source 1..20: mol_type = other DNA
  misc_feature 1..19: note = RNA
  misc_feature 20: note = DNA
caccagctggctgatgagct

SEQ ID NO: 851 - RNA, 20 nt, synthetic construct
  source 1..20: mol_type = other RNA
gaccaaaacctggctggttg

SEQ ID NO: 852 - DNA, 20 bp, synthetic construct
  source 1..20: mol_type = other DNA
  misc_feature 1..19: note = RNA
  misc_feature 20: note = DNA
gaccaaaacctggctggttt

SEQ ID NO: 853 - RNA, 20 nt, synthetic construct
  source 1..20: mol_type = other RNA
ccaaaacctggctggttgga

SEQ ID NO: 854 - DNA, 20 bp, synthetic construct
  source 1..20: mol_type = other DNA
  misc_feature 1..19: note = RNA
  misc_feature 20: note = DNA
ccaaaacctggctggttggt

SEQ ID NO: 855 - RNA, 19 nt, synthetic construct
  source 1..19: mol_type = other RNA
gatccagtcactaattccg

SEQ ID NO: 856 - RNA, 19 nt, synthetic construct
  source 1..19: mol_type = other RNA
tccagagagattttggcac

SEQ ID NO: 857 - RNA, 19 nt, synthetic construct
  source 1..19: mol_type = other RNA
tgaattcgcacatgctcca

SEQ ID NO: 858 - RNA, 19 nt, synthetic construct
  source 1..19: mol_type = other RNA
ggtccttggatccagtcac

SEQ ID NO: 859 - RNA, 19 nt, synthetic construct
  source 1..19: mol_type = other RNA
aattcgcacatgctccatc

SEQ ID NO: 860 - RNA, 19 nt, synthetic construct
  source 1..19: mol_type = other RNA
gatccagtcactaattccg

SEQ ID NO: 861 - RNA, 19 nt, synthetic construct
  source 1..19: mol_type = other RNA
tccagagagattttggcac

SEQ ID NO: 862 - RNA, 19 nt, synthetic construct
  source 1..19: mol_type = other RNA
tgaattcgcacatgctcca

SEQ ID NO: 863 - RNA, 19 nt, synthetic construct
  source 1..19: mol_type = other RNA
ggtccttggatccagtcac

SEQ ID NO: 864 - RNA, 19 nt, synthetic construct
  source 1..19: mol_type = other RNA
aattcgcacatgctccatc

SEQ ID NO: 865 - RNA, 19 nt, synthetic construct
  source 1..19: mol_type = other RNA
gatccagtcactaattccg

SEQ ID NO: 866 - RNA, 19 nt, synthetic construct
  source 1..19: mol_type = other RNA
tccagagagattttggcac

SEQ ID NO: 867 - RNA, 19 nt, synthetic construct
  source 1..19: mol_type = other RNA
tgaattcgcacatgctcca

SEQ ID NO: 868 - RNA, 19 nt, synthetic construct
  source 1..19: mol_type = other RNA
ggtccttggatccagtcac

SEQ ID NO: 869 - RNA, 19 nt, synthetic construct
  source 1..19: mol_type = other RNA
aattcgcacatgctccatc

SEQ ID NO: 870 - RNA, 19 nt, synthetic construct
  source 1..19: mol_type = other RNA
gatccagtcactaattccg

SEQ ID NO: 871 - RNA, 19 nt, synthetic construct
  source 1..19: mol_type = other RNA
gatccagtcactaattccg

SEQ ID NO: 872 - RNA, 19 nt, synthetic construct
  source 1..19: mol_type = other RNA
tccagagagattttggcac

SEQ ID NO: 873 - RNA, 19 nt, synthetic construct
  source 1..19: mol_type = other RNA
tccagagagattttggcac

SEQ ID NO: 874 - RNA, 19 nt, synthetic construct
  source 1..19: mol_type = other RNA
tgaattcgcacatgctcca

SEQ ID NO: 875 - RNA, 19 nt, synthetic construct
  source 1..19: mol_type = other RNA
tgaattcgcacatgctcca

SEQ ID NO: 876 - RNA, 19 nt, synthetic construct
  source 1..19: mol_type = other RNA
ggtccttggatccagtcac

SEQ ID NO: 877 - RNA, 19 nt, synthetic construct
  source 1..19: mol_type = other RNA
ggtccttggatccagtcac

SEQ ID NO: 878 - RNA, 19 nt, synthetic construct
  source 1..19: mol_type = other RNA
aattcgcacatgctccatc

SEQ ID NO: 879 - RNA, 19 nt, synthetic construct
  source 1..19: mol_type = other RNA
aattcgcacatgctccatc

SEQ ID NO: 880 - RNA, 19 nt, synthetic construct
  source 1..19: mol_type = other RNA
tgtcacagtgacaagcttg

SEQ ID NO: 881 - RNA, 19 nt, synthetic construct
  source 1..19: mol_type = other RNA
caaccagccaggttttggt

SEQ ID NO: 882 - RNA, 19 nt, synthetic construct
  source 1..19: mol_type = other RNA
tgtctttcctgcactgcag

SEQ ID NO: 883 - RNA, 19 nt, synthetic construct
  source 1..19: mol_type = other RNA
tgaaccacatggctatgac

SEQ ID NO: 884 - RNA, 19 nt, synthetic construct
  source 1..19: mol_type = other RNA
tgtcacagtgacaagcttg

SEQ ID NO: 885 - RNA, 19 nt, synthetic construct
  source 1..19: mol_type = other RNA
caaccagccaggttttggt

SEQ ID NO: 886 - RNA, 19 nt, synthetic construct
  source 1..19: mol_type = other RNA
tgtctttcctgcactgcag

SEQ ID NO: 887 - RNA, 19 nt, synthetic construct
  source 1..19: mol_type = other RNA
tgaaccacatggctatgac

SEQ ID NO: 888 - RNA, 19 nt, synthetic construct
  source 1..19: mol_type = other RNA
tgtcacagtgacaagcttg

SEQ ID NO: 889 - RNA, 19 nt, synthetic construct
  source 1..19: mol_type = other RNA
caaccagccaggttttggt

SEQ ID NO: 890 - RNA, 19 nt, synthetic construct
  source 1..19: mol_type = other RNA
tgtctttcctgcactgcag

SEQ ID NO: 891 - RNA, 19 nt, synthetic construct
  source 1..19: mol_type = other RNA
tgaaccacatggctatgac

SEQ ID NO: 892 - RNA, 19 nt, synthetic construct
  source 1..19: mol_type = other RNA
tgtcacagtgacaagcttg

SEQ ID NO: 893 - RNA, 19 nt, synthetic construct
  source 1..19: mol_type = other RNA
tgtcacagtgacaagcttg

SEQ ID NO: 894 - RNA, 19 nt, synthetic construct
  source 1..19: mol_type = other RNA
tgtcacagtgacaagcttg

SEQ ID NO: 895 - RNA, 19 nt, synthetic construct
  source 1..19: mol_type = other RNA
caaccagccaggttttggt

SEQ ID NO: 896 - RNA, 19 nt, synthetic construct
  source 1..19: mol_type = other RNA
tgtcacagtgacaagcttg

SEQ ID NO: 897 - RNA, 19 nt, synthetic construct
  source 1..19: mol_type = other RNA
caaccagccaggttttggt

SEQ ID NO: 898 - RNA, 19 nt, synthetic construct
  source 1..19: mol_type = other RNA
caaccagccaggttttggt

SEQ ID NO: 899 - RNA, 21 nt, synthetic construct
  source 1..21: mol_type = other RNA
caaccagccaggttttggtcc

SEQ ID NO: 900 - RNA, 21 nt, synthetic construct
  source 1..21: mol_type = other RNA
caaccagccaggttttggtcc

SEQ ID NO: 901 - RNA, 21 nt, synthetic construct
  source 1..21: mol_type = other RNA
caaccagccaggttttggtcc

SEQ ID NO: 902 - RNA, 21 nt, synthetic construct
  source 1..21: mol_type = other RNA
caaccagccaggttttggtcc

SEQ ID NO: 903 - RNA, 21 nt, synthetic construct
  source 1..21: mol_type = other RNA
caaccagccaggttttggtcc

SEQ ID NO: 904 - RNA, 19 nt, synthetic construct
  source 1..19: mol_type = other RNA
tgtctttcctgcactgcag

SEQ ID NO: 905 - RNA, 19 nt, synthetic construct
  source 1..19: mol_type = other RNA
tgaaccacatggctatgac

SEQ ID NO: 906 - RNA, 19 nt, synthetic construct
  source 1..19: mol_type = other RNA
tgtctttcctgcactgcag

SEQ ID NO: 907 - RNA, 19 nt, synthetic construct
  source 1..19: mol_type = other RNA
tgaaccacatggctatgac

SEQ ID NO: 908 - RNA, 17 nt, synthetic construct
  source 1..17: mol_type = other RNA
gaattagtgactggatc

SEQ ID NO: 909 - RNA, 17 nt, synthetic construct
  source 1..17: mol_type = other RNA
gccaaaatctctctgga

SEQ ID NO: 910 - RNA, 17 nt, synthetic construct
  source 1..17: mol_type = other RNA
gagcatgtgcgaattca

SEQ ID NO: 911 - RNA, 17 nt, synthetic construct
  source 1..17: mol_type = other RNA
gactggatccaaggacc

SEQ ID NO: 912 - RNA, 17 nt, synthetic construct
  source 1..17: mol_type = other RNA
tggagcatgtgcgaatt

SEQ ID NO: 913 - RNA, 15 nt, synthetic construct
  source 1..15: mol_type = other RNA
attagtgactggatc

SEQ ID NO: 914 - RNA, 15 nt, synthetic construct
  source 1..15: mol_type = other RNA
caaaatctctctgga

SEQ ID NO: 915 - RNA, 15 nt, synthetic construct
  source 1..15: mol_type = other RNA
gcatgtgcgaattca

SEQ ID NO: 916 - RNA, 15 nt, synthetic construct
  source 1..15: mol_type = other RNA
ctggatccaaggacc

SEQ ID NO: 917 - RNA, 15 nt, synthetic construct
  source 1..15: mol_type = other RNA
gagcatgtgcgaatt

SEQ ID NO: 918 - RNA, 14 nt, synthetic construct
  source 1..14: mol_type = other RNA
ttagtgactggatc

SEQ ID NO: 919 - RNA, 14 nt, synthetic construct
  source 1..14: mol_type = other RNA
aaaatctctctgga

SEQ ID NO: 920 - RNA, 14 nt, synthetic construct
  source 1..14: mol_type = other RNA
catgtgcgaattca

SEQ ID NO: 921 - RNA, 14 nt, synthetic construct
  source 1..14: mol_type = other RNA
tggatccaaggacc

SEQ ID NO: 922 - RNA, 14 nt, synthetic construct
  source 1..14: mol_type = other RNA
agcatgtgcgaatt

SEQ ID NO: 923 - RNA, 17 nt, synthetic construct
  source 1..17: mol_type = other RNA
cggaattagtgactgga

SEQ ID NO: 924 - RNA, 15 nt, synthetic construct
  source 1..15: mol_type = other RNA
cggaattagtgactg

SEQ ID NO: 925 - RNA, 16 nt, synthetic construct
  source 1..16: mol_type = other RNA
gtgccaaaatctctct

SEQ ID NO: 926 - RNA, 15 nt, synthetic construct
  source 1..15: mol_type = other RNA
gtgccaaaatctctc

SEQ ID NO: 927 - RNA, 17 nt, synthetic construct
  source 1..17: mol_type = other RNA
tggagcatgtgcgaatt

SEQ ID NO: 928 - RNA, 15 nt, synthetic construct
  source 1..15: mol_type = other RNA
tggagcatgtgcgaa

SEQ ID NO: 929 - RNA, 17 nt, synthetic construct
  source 1..17: mol_type = other RNA
gtgactggatccaagga

SEQ ID NO: 930 - RNA, 15 nt, synthetic construct
  source 1..15: mol_type = other RNA
gtgactggatccaag

SEQ ID NO: 931 - RNA, 17 nt, synthetic construct
  source 1..17: mol_type = other RNA
gatggagcatgtgcgaa

SEQ ID NO: 932 - RNA, 15 nt, synthetic construct
  source 1..15: mol_type = other RNA
gatggagcatgtgcg

SEQ ID NO: 933 - RNA, 17 nt, synthetic construct
  source 1..17: mol_type = other RNA
agcttgtcactgtgaca

SEQ ID NO: 934 - RNA, 17 nt, synthetic construct
  source 1..17: mol_type = other RNA
caaaacctggctggttg

SEQ ID NO: 935 - RNA, 17 nt, synthetic construct
  source 1..17: mol_type = other RNA
gcagtgcaggaaagaca

SEQ ID NO: 936 - RNA, 17 nt, synthetic construct
  source 1..17: mol_type = other RNA
catagccatgtggttca

SEQ ID NO: 937 - RNA, 15 nt, synthetic construct
  source 1..15: mol_type = other RNA
cttgtcactgtgaca

SEQ ID NO: 938 - RNA, 15 nt, synthetic construct
  source 1..15: mol_type = other RNA
aaacctggctggttg

SEQ ID NO: 939 - RNA, 15 nt, synthetic construct
  source 1..15: mol_type = other RNA
agtgcaggaaagaca

SEQ ID NO: 940 - RNA, 15 nt, synthetic construct
  source 1..15: mol_type = other RNA
tagccatgtggttca

SEQ ID NO: 941 - RNA, 14 nt, synthetic construct
  source 1..14: mol_type = other RNA
ttgtcactgtgaca

SEQ ID NO: 942 - RNA, 14 nt, synthetic construct
  source 1..14: mol_type = other RNA
aacctggctggttg

SEQ ID NO: 943 - RNA, 14 nt, synthetic construct
  source 1..14: mol_type = other RNA
gtgcaggaaagaca

SEQ ID NO: 944 - RNA, 14 nt, synthetic construct
  source 1..14: mol_type = other RNA
agccatgtggttca

SEQ ID NO: 945 - RNA, 17 nt, synthetic construct
  source 1..17: mol_type = other RNA
cacttgtcactgtgaca

SEQ ID NO: 946 - RNA, 15 nt, synthetic construct
  source 1..15: mol_type = other RNA
cacttgtcactgtga

SEQ ID NO: 947 - RNA, 17 nt, synthetic construct
  source 1..17: mol_type = other RNA
caagcttgtcactgtga

SEQ ID NO: 948 - RNA, 17 nt, synthetic construct
  source 1..17: mol_type = other RNA
accaaaacctggctggt

SEQ ID NO: 949 - RNA, 15 nt, synthetic construct
  source 1..15: mol_type = other RNA
caagcttgtcactgt

SEQ ID NO: 950 - RNA, 15 nt, synthetic construct
  source 1..15: mol_type = other RNA
accaaaacctggctg

SEQ ID NO: 951 - RNA, 14 nt, synthetic construct
  source 1..14: mol_type = other RNA
accaaaacctggct

SEQ ID NO: 952 - RNA, 19 nt, synthetic construct
  source 1..19: mol_type = other RNA
caaaacctggctggttgga

SEQ ID NO: 953 - RNA, 17 nt, synthetic construct
  source 1..17: mol_type = other RNA
aaacctggctggttgga

SEQ ID NO: 954 - RNA, 16 nt, synthetic construct
  source 1..16: mol_type = other RNA
aacctggctggttgga

SEQ ID NO: 955 - RNA, 19 nt, synthetic construct
  source 1..19: mol_type = other RNA
accaaaacctggctggtga

SEQ ID NO: 956 - RNA, 17 nt, synthetic construct
  source 1..17: mol_type = other RNA
accaaaacctggctgga

SEQ ID NO: 957 - RNA, 17 nt, synthetic construct
  source 1..17: mol_type = other RNA
ctgcagtgcaggaaaga

SEQ ID NO: 958 - RNA, 17 nt, synthetic construct
  source 1..17: mol_type = other RNA
gtcatagccatgtggtt

SEQ ID NO: 959 - RNA, 15 nt, synthetic construct
  source 1..15: mol_type = other RNA
ctgcagtgcaggaaa

SEQ ID NO: 960 - RNA, 15 nt, synthetic construct
  source 1..15: mol_type = other RNA
gtcatagccatgtgg

SEQ ID NO: 961 - RNA, 19 nt, synthetic construct
  source 1..19: mol_type = other RNA
  modified_base 1: mod_base = OTHER; note = 2'-deoxy-2'-fluoroguanosine
  modified_base 2: mod_base = OTHER; note = 2'-deoxy-2'-fluoroadenosine
  modified_base 3: mod_base = OTHER; note = um
  modified_base 4: mod_base = OTHER; note = 2'-deoxy-2'-fluorocytidine
  modified_base 5: mod_base = OTHER; note = cm
  modified_base 6: mod_base = OTHER; note = 2'-deoxy-2'-fluoroadenosine
  modified_base 7: mod_base = OTHER; note = gm
  modified_base 8: mod_base = OTHER; note = 2'-deoxy-2'-fluorouridine
  modified_base 9: mod_base = OTHER; note = cm
  modified_base 10: mod_base = OTHER; note = 2'-deoxy-2'-fluoroadenosine
  modified_base 11: mod_base = OTHER; note = cm
  modified_base 12: mod_base = OTHER; note = 2'-deoxy-2'-fluorouridine
  modified_base 13: mod_base = OTHER; note = 2'-O-methyladenosine
  modified_base 14: mod_base = OTHER; note = 2'-deoxy-2'-fluoroadenosine
  modified_base 15: mod_base = OTHER; note = um
  modified_base 16: mod_base = OTHER; note = 2'-deoxy-2'-fluorouridine
  modified_base 17: mod_base = OTHER; note = cm
  modified_base 18: mod_base = OTHER; note = 2'-deoxy-2'-fluorocytidine
  modified_base 19: mod_base = OTHER; note = gm
gatccagtcactaattccg

SEQ ID NO: 962 - RNA, 19 nt, synthetic construct
  source 1..19: mol_type = other RNA
  modified_base 1: mod_base = OTHER; note = 2'-deoxy-2'-fluoroguanosine
  modified_base 2: mod_base = OTHER; note = 2'-deoxy-2'-fluoroadenosine
  modified_base 3: mod_base = OTHER; note = um
  modified_base 4: mod_base = OTHER; note = 2'-deoxy-2'-fluorocytidine
  modified_base 5: mod_base = OTHER; note = cm
  modified_base 6: mod_base = OTHER; note = 2'-deoxy-2'-fluoroadenosine
  modified_base 7: mod_base = OTHER; note = gm
  modified_base 8: mod_base = OTHER; note = 2'-deoxy-2'-fluorouridine
  modified_base 9: mod_base = OTHER; note = cm
  modified_base 10: mod_base = OTHER; note = 2'-deoxy-2'-fluoroadenosine
  modified_base 11: mod_base = OTHER; note = cm
  modified_base 12: mod_base = OTHER; note = 2'-deoxy-2'-fluorouridine
  modified_base 13: mod_base = OTHER; note = 2'-O-methyladenosine
  modified_base 14: mod_base = OTHER; note = 2'-deoxy-2'-fluoroadenosine
  modified_base 15: mod_base = OTHER; note = um
  modified_base 16: mod_base = OTHER; note = 2'-deoxy-2'-fluorouridine
  modified_base 17: mod_base = OTHER; note = cm
  modified_base 18: mod_base = OTHER; note = 2'-deoxy-2'-fluorocytidine
  modified_base 19: mod_base = OTHER; note = gm
  modified_base 1..3: mod_base = OTHER; note = phosphorothioate bond between nucleotides
  modified_base 17..19: mod_base = OTHER; note = phosphorothioate bond between nucleotides
gatccagtcactaattccg

SEQ ID NO: 963 - RNA, 19 nt, synthetic construct
  source 1..19: mol_type = other RNA
  modified_base 1: mod_base = OTHER; note = 2'-deoxy-2'-fluoroguanosine
  modified_base 2: mod_base = OTHER; note = 2'-deoxy-2'-fluoroadenosine
  modified_base 3: mod_base = OTHER; note = um
  modified_base 4: mod_base = OTHER; note = 2'-deoxy-2'-fluorocytidine
  modified_base 5: mod_base = OTHER; note = cm
  modified_base 6: mod_base = OTHER; note = 2'-deoxy-2'-fluoroadenosine
  modified_base 7: mod_base = OTHER; note = gm
  modified_base 8: mod_base = OTHER; note = 2'-deoxy-2'-fluorouridine
  modified_base 9: mod_base = OTHER; note = cm
  modified_base 10: mod_base = OTHER; note = 2'-deoxy-2'-fluoroadenosine
  modified_base 11: mod_base = OTHER; note = cm
  modified_base 12: mod_base = OTHER; note = 2'-deoxy-2'-fluorouridine
  modified_base 13: mod_base = OTHER; note = 2'-O-methyladenosine
  modified_base 14: mod_base = OTHER; note = 2'-deoxy-2'-fluoroadenosine
  modified_base 15: mod_base = OTHER; note = um
  modified_base 16: mod_base = OTHER; note = 2'-deoxy-2'-fluorouridine
  modified_base 17: mod_base = OTHER; note = cm
  modified_base 18: mod_base = OTHER; note = 2'-deoxy-2'-fluorocytidine
  modified_base 19: mod_base = OTHER; note = gm
  modified_base 1^2: mod_base = OTHER; note = phosphorothioate bond between nucleotides
  modified_base 18^19: mod_base = OTHER; note = phosphorothioate bond between nucleotides
gatccagtcactaattccg

SEQ ID NO: 964 - RNA, 19 nt, synthetic construct
  source 1..19: mol_type = other RNA
  modified_base 5: mod_base = OTHER; note = cm
  modified_base 7: mod_base = OTHER; note = gm
  modified_base 9: mod_base = OTHER; note = cm
  modified_base 12: mod_base = OTHER; note = um
  modified_base 1^2: mod_base = OTHER; note = phosphorothioate bond between nucleotides
  modified_base 18^19: mod_base = OTHER; note = phosphorothioate bond between nucleotides
gatccagtcactaattccg

SEQ ID NO: 965 - RNA, 19 nt, synthetic construct
  source 1..19: mol_type = other RNA
  modified_base 1: mod_base = OTHER; note = 5'-E-vinylphosphonate-2'-O-methyl-guanosine
  modified_base 2: mod_base = OTHER; note = 2'-deoxy-2'-fluoroadenosine
  modified_base 5: mod_base = OTHER; note = cm
  modified_base 7: mod_base = OTHER; note = gm
  modified_base 9: mod_base = OTHER; note = cm
  modified_base 12: mod_base = OTHER; note = um
  modified_base 1..3: mod_base = OTHER; note = phosphorothioate bond between nucleotides
  modified_base 17..19: mod_base = OTHER; note = phosphorothioate bond between nucleotides
gatccagtcactaattccg

SEQ ID NO: 966 - RNA, 19 nt, synthetic construct
  source 1..19: mol_type = other RNA
  modified_base 1: mod_base = OTHER; note = 5'-E-vinylphosphonate-2'-O-methyl-guanosine
  modified_base 2: mod_base = OTHER; note = 2'-deoxy-2'-fluoroadenosine
  modified_base 5: mod_base = OTHER; note = cm
  modified_base 7: mod_base = OTHER; note = gm
  modified_base 9: mod_base = OTHER; note = cm
  modified_base 12: mod_base = OTHER; note = um
  modified_base 1^2: mod_base = OTHER; note = phosphorothioate bond between nucleotides
  modified_base 18^19: mod_base = OTHER; note = phosphorothioate bond between nucleotides
gatccagtcactaattccg

SEQ ID NO: 967 - RNA, 19 nt, synthetic construct
  source 1..19: mol_type = other RNA
  modified_base 1: mod_base = OTHER; note = 5'-E-vinylphosphonate-2'-O-methyl-guanosine
  modified_base 2: mod_base = OTHER; note = 2'-deoxy-2'-fluoroadenosine
  modified_base 5: mod_base = OTHER; note = cm
  modified_base 7: mod_base = OTHER; note = gm
  modified_base 9: mod_base = OTHER; note = cm
  modified_base 12: mod_base = OTHER; note = um
  modified_base 1^2: mod_base = OTHER; note = phosphorothioate bond between nucleotides
  modified_base 18^19: mod_base = OTHER; note = phosphorothioate bond between nucleotides
gatccagtcactaattccg

SEQ ID NO: 968 - RNA, 19 nt, synthetic construct
  source 1..19: mol_type = other RNA
  modified_base 1: mod_base = OTHER; note = 5'-E-vinylphosphonate-2'-O-methyl-guanosine
  modified_base 2: mod_base = OTHER; note = 2'-deoxy-2'-fluoroadenosine
  modified_base 5: mod_base = OTHER; note = cm
  modified_base 7: mod_base = OTHER; note = gm
  modified_base 9: mod_base = OTHER; note = cm
  modified_base 12: mod_base = OTHER; note = um
  modified_base 1^2: mod_base = OTHER; note = phosphorothioate bond between nucleotides
  modified_base 18^19: mod_base = OTHER; note = phosphorothioate bond between nucleotides
gatccagtcactaattccg

SEQ ID NO: 969 - RNA, 19 nt, synthetic construct
  source 1..19: mol_type = other RNA
  modified_base 1: mod_base = OTHER; note = 5'-E-vinylphosphonate-2'-O-methyl-guanosine
  modified_base 2: mod_base = OTHER; note = 2'-deoxy-2'-fluoroadenosine
  modified_base 5: mod_base = OTHER; note = cm
  modified_base 7: mod_base = OTHER; note = gm
  modified_base 9: mod_base = OTHER; note = cm
  modified_base 12: mod_base = OTHER; note = um
  modified_base 1^2: mod_base = OTHER; note = phosphorothioate bond between nucleotides
  modified_base 18^19: mod_base = OTHER; note = phosphorothioate bond between nucleotides
gatccagtcactaattccg

SEQ ID NO: 970 - RNA, 19 nt, synthetic construct
  source 1..19: mol_type = other RNA
  modified_base 1: mod_base = OTHER; note = 5'-E-vinylphosphonate-2'-O-methyl-guanosine
  modified_base 2: mod_base = OTHER; note = 2'-deoxy-2'-fluoroadenosine
  modified_base 5: mod_base = OTHER; note = cm
  modified_base 7: mod_base = OTHER; note = gm
  modified_base 9: mod_base = OTHER; note = cm
  modified_base 12: mod_base = OTHER; note = um
  modified_base 1^2: mod_base = OTHER; note = phosphorothioate bond between nucleotides
  modified_base 18^19: mod_base = OTHER; note = phosphorothioate bond between nucleotides
gatccagtcactaattccg

SEQ ID NO: 971 - RNA, 19 nt, synthetic construct
  source 1..19: mol_type = other RNA
  modified_base 1: mod_base = OTHER; note = gm
  modified_base 2: mod_base = OTHER; note = 2'-deoxy-2'-fluoroadenosine
  modified_base 3: mod_base = OTHER; note = um
  modified_base 4: mod_base = OTHER; note = 2'-deoxy-2'-fluorocytidine
  modified_base 5: mod_base = OTHER; note = cm
  modified_base 6: mod_base = OTHER; note = 2'-deoxy-2'-fluoroadenosine
  modified_base 7: mod_base = OTHER; note = gm
  modified_base 1^2: mod_base = OTHER; note = phosphorothioate bond between nucleotides
  modified_base 18^19: mod_base = OTHER; note = phosphorothioate bond between nucleotides
gatccagtcactaattccg

SEQ ID NO: 972 - RNA, 19 nt, synthetic construct
  source 1..19: mol_type = other RNA
  modified_base 2: mod_base = OTHER; note = 2'-O-methyladenosine
  modified_base 4: mod_base = OTHER; note = cm
  modified_base 6: mod_base = OTHER; note = 2'-O-methyladenosine
  modified_base 8: mod_base = OTHER; note = um
  modified_base 10: mod_base = OTHER; note = 2'-O-methyladenosine
  modified_base 12: mod_base = OTHER; note = um
  modified_base 16: mod_base = OTHER; note = um
  modified_base 18: mod_base = OTHER; note = cm
  modified_base 1^2: mod_base = OTHER; note = phosphorothioate bond between nucleotides
  modified_base 18^19: mod_base = OTHER; note = phosphorothioate bond between nucleotides
gatccagtcactaattccg

SEQ ID NO: 973 - RNA, 19 nt, synthetic construct
  source 1..19: mol_type = other RNA
  modified_base 2: mod_base = OTHER; note = 2'-deoxy-2'-fluoroadenosine
  modified_base 4: mod_base = OTHER; note = 2'-deoxy-2'-fluorocytidine
  modified_base 6: mod_base = OTHER; note = 2'-deoxy-2'-fluoroadenosine
  modified_base 8: mod_base = OTHER; note = 2'-deoxy-2'-fluorouridine
  modified_base 10: mod_base = OTHER; note = 2'-deoxy-2'-fluoroadenosine
  modified_base 12: mod_base = OTHER; note = 2'-deoxy-2'-fluorouridine
  modified_base 16: mod_base = OTHER; note = 2'-deoxy-2'-fluorouridine
  modified_base 18: mod_base = OTHER; note = 2'-deoxy-2'-fluorocytidine
  modified_base 1^2: mod_base = OTHER; note = phosphorothioate bond between nucleotides
  modified_base 18^19: mod_base = OTHER; note = phosphorothioate bond between nucleotides
gatccagtcactaattccg

SEQ ID NO: 974 - RNA, 19 nt, synthetic construct
  source 1..19: mol_type = other RNA
  modified_base 6: mod_base = OTHER; note = 2'-O-methyladenosine
  modified_base 7: mod_base = OTHER; note = 2'-deoxy-2'-fluoroguanosine
  modified_base 8: mod_base = OTHER; note = 2'-deoxy-2'-fluorouridine
  modified_base 12: mod_base = OTHER; note = 2'-deoxy-2'-fluorouridine
  modified_base 13: mod_base = OTHER; note = 2'-O-methyladenosine
  modified_base 18^19: mod_base = OTHER; note = phosphorothioate bond between nucleotides
gatccagtcactaattcct

SEQ ID NO: 975 - RNA, 19 nt, synthetic construct
  source 1..19: mol_type = other RNA
  modified_base 3: mod_base = OTHER; note = 2'-deoxy-2'-fluorouridine
  modified_base 4: mod_base = OTHER; note = 2'-deoxy-2'-fluorocytidine
  modified_base 5: mod_base = OTHER; note = 2'-deoxy-2'-fluorocytidine
  modified_base 7: mod_base = OTHER; note = 2'-deoxy-2'-fluoroguanosine
  modified_base 8: mod_base = OTHER; note = 2'-deoxy-2'-fluorouridine
  modified_base 11: mod_base = OTHER; note = 2'-deoxy-2'-fluorocytidine
  modified_base 12: mod_base = OTHER; note = 2'-deoxy-2'-fluorouridine
  modified_base 15: mod_base = OTHER; note = 2'-deoxy-2'-fluorouridine
  modified_base 16: mod_base = OTHER; note = 2'-deoxy-2'-fluorouridine
  modified_base 17: mod_base = OTHER; note = 2'-deoxy-2'-fluorocytidine
  modified_base 18: mod_base = OTHER; note = 2'-deoxy-2'-fluorocytidine
  modified_base 18^19: mod_base = OTHER; note = phosphorothioate bond between nucleotides
gatccagtcactaattccg

SEQ ID NO: 976 - RNA, 19 nt, synthetic construct
  source 1..19: mol_type = other RNA
  modified_base 3: mod_base = OTHER; note = um
  modified_base 4: mod_base = OTHER; note = cm
  modified_base 5: mod_base = OTHER; note = cm
  modified_base 8: mod_base = OTHER; note = um
  modified_base 9: mod_base = OTHER; note = cm
  modified_base 11: mod_base = OTHER; note = cm
  modified_base 12: mod_base = OTHER; note = um
  modified_base 15: mod_base = OTHER; note = um
  modified_base 16: mod_base = OTHER; note = um
  modified_base 17: mod_base = OTHER; note = cm
  modified_base 18: mod_base = OTHER; note = cm
  modified_base 17..19: mod_base = OTHER; note = phosphorothioate bond between nucleotides
gatccagtcactaattccg

SEQ ID NO: 977 - RNA, 19 nt, synthetic construct
  source 1..19: mol_type = other RNA
  modified_base 1^2: mod_base = OTHER; note = phosphorothioate bond between nucleotides
  modified_base 18^19: mod_base = OTHER; note = phosphorothioate bond between nucleotides
gatccagtcactaattccg

SEQ ID NO: 978 - RNA, 19 nt, synthetic construct
  source 1..19: mol_type = other RNA
  modified_base 1: mod_base = OTHER; note = 5'-E-vinylphosphonate-2'-O-methyl-guanosine
  modified_base 3: mod_base = OTHER; note = m5u
  modified_base 4: mod_base = m5c
  modified_base 5: mod_base = m5c
  modified_base 8: mod_base = OTHER; note = m5u
  modified_base 18^19: mod_base = OTHER; note = phosphorothioate bond between nucleotides
gatccagtcactaattccg

SEQ ID NO: 979 - RNA, 19 nt, synthetic construct
  source 1..19: mol_type = other RNA
  modified_base 1: mod_base = OTHER; note = 5'-E-vinylphosphonate-2'-O-methyl-guanosine
  modified_base 11: mod_base = m5c
  modified_base 12: mod_base = OTHER; note = m5u
  modified_base 15: mod_base = OTHER; note = m5u
  modified_base 16: mod_base = OTHER; note = m5u
  modified_base 17: mod_base = m5c
  modified_base 18: mod_base = m5c
  modified_base 18^19: mod_base = OTHER; note = phosphorothioate bond between nucleotides
gatccagtcactaattccg

SEQ ID NO: 980 - RNA, 19 nt, synthetic construct
  source 1..19: mol_type = other RNA
  modified_base 1: mod_base = OTHER; note = 2'-deoxy-2'-fluorouridine
  modified_base 2: mod_base = OTHER; note = 2'-deoxy-2'-fluorocytidine
  modified_base 3: mod_base = OTHER; note = cm
  modified_base 4: mod_base = OTHER; note = 2'-deoxy-2'-fluoroadenosine
  modified_base 5: mod_base = OTHER; note = gm
  modified_base 6: mod_base = OTHER; note = 2'-deoxy-2'-fluoroadenosine
  modified_base 7: mod_base = OTHER; note = gm
  modified_base 8: mod_base = OTHER; note = 2'-deoxy-2'-fluoroadenosine
  modified_base 9: mod_base = OTHER; note = gm
  modified_base 10: mod_base = OTHER; note = 2'-deoxy-2'-fluoroadenosine
  modified_base 11: mod_base = OTHER; note = um
  modified_base 12: mod_base = OTHER; note = 2'-deoxy-2'-fluorouridine
  modified_base 13: mod_base = OTHER; note = um
  modified_base 14: mod_base = OTHER; note = 2'-deoxy-2'-fluorouridine
  modified_base 15: mod_base = OTHER; note = gm
  modified_base 16: mod_base = OTHER; note = 2'-deoxy-2'-fluoroguanosine
  modified_base 17: mod_base = OTHER; note = cm
  modified_base 18: mod_base = OTHER; note = 2'-deoxy-2'-fluoroadenosine
  modified_base 19: mod_base = OTHER; note = cm
tccagagagattttggcac

SEQ ID NO: 981 - RNA, 19 nt, synthetic construct
  source 1..19: mol_type = other RNA
  modified_base 1: mod_base = OTHER; note = 2'-deoxy-2'-fluorouridine
  modified_base 2: mod_base = OTHER; note = 2'-deoxy-2'-fluorocytidine
  modified_base 3: mod_base = OTHER; note = cm
  modified_base 4: mod_base = OTHER; note = 2'-deoxy-2'-fluoroadenosine
  modified_base 5: mod_base = OTHER; note = gm
  modified_base 6: mod_base = OTHER; note = 2'-deoxy-2'-fluoroadenosine
  modified_base 7: mod_base = OTHER; note = gm
  modified_base 8: mod_base = OTHER; note = 2'-deoxy-2'-fluoroadenosine
  modified_base 9: mod_base = OTHER; note = gm
  modified_base 10: mod_base = OTHER; note = 2'-deoxy-2'-fluoroadenosine
  modified_base 11: mod_base = OTHER; note = um
  modified_base 12: mod_base = OTHER; note = 2'-deoxy-2'-fluorouridine
  modified_base 13: mod_base = OTHER; note = um
  modified_base 14: mod_base = OTHER; note = 2'-deoxy-2'-fluorouridine
  modified_base 15: mod_base = OTHER; note = gm
  modified_base 16: mod_base = OTHER; note = 2'-deoxy-2'-fluoroguanosine
  modified_base 17: mod_base = OTHER; note = cm
  modified_base 18: mod_base = OTHER; note = 2'-deoxy-2'-fluoroadenosine
  modified_base 19: mod_base = OTHER; note = cm
  modified_base 1..3: mod_base = OTHER; note = phosphorothioate bond between nucleotides
  modified_base 17..19: mod_base = OTHER; note = phosphorothioate bond between nucleotides
tccagagagattttggcac

SEQ ID NO: 982 - RNA, 19 nt, synthetic construct
  source 1..19: mol_type = other RNA
  modified_base 1: mod_base = OTHER; note = 2'-deoxy-2'-fluorouridine
  modified_base 2: mod_base = OTHER; note = 2'-deoxy-2'-fluorocytidine
  modified_base 3: mod_base = OTHER; note = cm
  modified_base 4: mod_base = OTHER; note = 2'-deoxy-2'-fluoroadenosine
  modified_base 5: mod_base = OTHER; note = gm
  modified_base 6: mod_base = OTHER; note = 2'-deoxy-2'-fluoroadenosine
  modified_base 7: mod_base = OTHER; note = gm
  modified_base 8: mod_base = OTHER; note = 2'-deoxy-2'-fluoroadenosine
  modified_base 9: mod_base = OTHER; note = gm
  modified_base 10: mod_base = OTHER; note = 2'-deoxy-2'-fluoroadenosine
  modified_base 11: mod_base = OTHER; note = um
  modified_base 12: mod_base = OTHER; note = 2'-deoxy-2'-fluorouridine
  modified_base 13: mod_base = OTHER; note = um
  modified_base 14: mod_base = OTHER; note = 2'-deoxy-2'-fluorouridine
  modified_base 15: mod_base = OTHER; note = gm
  modified_base 16: mod_base = OTHER; note = 2'-deoxy-2'-fluoroguanosine
  modified_base 17: mod_base = OTHER; note = cm
  modified_base 18: mod_base = OTHER; note = 2'-deoxy-2'-fluoroadenosine
  modified_base 19: mod_base = OTHER; note = cm
  modified_base 1..3: mod_base = OTHER; note = phosphorothioate bond between nucleotides
  modified_base 18^19: mod_base = OTHER; note = phosphorothioate bond between nucleotides
tccagagagattttggcac

SEQ ID NO: 983 - RNA, 19 nt, synthetic construct
  source 1..19: mol_type = other RNA
  modified_base 1: mod_base = OTHER; note = 2'-deoxy-2'-fluorouridine
  modified_base 2: mod_base = OTHER; note = 2'-deoxy-2'-fluorocytidine
  modified_base 3: mod_base = OTHER; note = cm
  modified_base 4: mod_base = OTHER; note = 2'-deoxy-2'-fluoroadenosine
  modified_base 5: mod_base = OTHER; note = gm
  modified_base 6: mod_base = OTHER; note = 2'-deoxy-2'-fluoroadenosine
  modified_base 7: mod_base = OTHER; note = gm
  modified_base 8: mod_base = OTHER; note = 2'-deoxy-2'-fluoroadenosine
  modified_base 9: mod_base = OTHER; note = gm
  modified_base 10: mod_base = OTHER; note = 2'-deoxy-2'-fluoroadenosine
  modified_base 11: mod_base = OTHER; note = um
  modified_base 12: mod_base = OTHER; note = 2'-deoxy-2'-fluorouridine
  modified_base 13: mod_base = OTHER; note = um
  modified_base 14: mod_base = OTHER; note = 2'-deoxy-2'-fluorouridine
  modified_base 15: mod_base = OTHER; note = gm
  modified_base 16: mod_base = OTHER; note = 2'-deoxy-2'-fluoroguanosine
  modified_base 17: mod_base = OTHER; note = cm
  modified_base 18: mod_base = OTHER; note = 2'-deoxy-2'-fluoroadenosine
  modified_base 19: mod_base = OTHER; note = cm
  modified_base 18^19: mod_base = OTHER; note = phosphorothioate bond between nucleotides
tccagagagattttggcac

SEQ ID NO: 984 - RNA, 19 nt, synthetic construct
  source 1..19: mol_type = other RNA
  modified_base 3: mod_base = OTHER; note = cm
  modified_base 17: mod_base = OTHER; note = cm
  modified_base 18^19: mod_base = OTHER; note = phosphorothioate bond between nucleotides
tccagagagattttggcac

SEQ ID NO: 985 - RNA, 20 nt, synthetic construct
  source 1..20: mol_type = other RNA
  modified_base 1: mod_base = OTHER; note = 5'-E-vinylphosphonate-2'-O-methyl-uridine
  modified_base 2: mod_base = OTHER; note = 2'-deoxy-2'-fluorocytidine
  modified_base 3: mod_base = OTHER; note = cm
  modified_base 7: mod_base = OTHER; note = gm
  modified_base 18: mod_base = OTHER; note = cm
  modified_base 1..3: mod_base = OTHER; note = phosphorothioate bond between nucleotides
  modified_base 18..20: mod_base = OTHER; note = phosphorothioate bond between nucleotides
tccagaggagattttggcac

SEQ ID NO: 986 - RNA, 20 nt, synthetic construct
  source 1..20: mol_type = other RNA
  modified_base 1: mod_base = OTHER; note = 5'-E-vinylphosphonate-2'-O-methyl-uridine
  modified_base 2: mod_base = OTHER; note = 2'-deoxy-2'-fluorocytidine
  modified_base 3: mod_base = OTHER; note = cm
  modified_base 7: mod_base = OTHER; note = gm
  modified_base 18: mod_base = OTHER; note = cm
  modified_base 1^2: mod_base = OTHER; note = phosphorothioate bond between nucleotides
  modified_base 19^20: mod_base = OTHER; note = phosphorothioate bond between nucleotides
tccagaggagattttggcac

SEQ ID NO: 987 - RNA, 20 nt, synthetic construct
  source 1..20: mol_type = other RNA
  modified_base 1: mod_base = OTHER; note = 5'-E-vinylphosphonate-2'-O-methyl-uridine
  modified_base 2: mod_base = OTHER; note = 2'-deoxy-2'-fluorocytidine
  modified_base 3: mod_base = OTHER; note = cm
  modified_base 7: mod_base = OTHER; note = gm
  modified_base 18: mod_base = OTHER; note = cm
  modified_base 1..3: mod_base = OTHER; note = phosphorothioate bond between nucleotides
  modified_base 18..20: mod_base = OTHER; note = phosphorothioate bond between nucleotides
tccagaggagattttggcac

SEQ ID NO: 988 - RNA, 19 nt, synthetic construct
  source 1..19: mol_type = other RNA
  modified_base 1: mod_base = OTHER; note = 5'-E-vinylphosphonate-2'-O-methyl-uridine
  modified_base 2: mod_base = OTHER; note = 2'-deoxy-2'-fluorocytidine
  modified_base 3: mod_base = OTHER; note = cm
  modified_base 7: mod_base = OTHER; note = gm
  modified_base 17: mod_base = OTHER; note = cm
  modified_base 1^2: mod_base = OTHER; note = phosphorothioate bond between nucleotides
  modified_base 18^19: mod_base = OTHER; note = phosphorothioate bond between nucleotides
tccagagagattttggcac

SEQ ID NO: 989 - RNA, 20 nt, synthetic construct
  source 1..20: mol_type = other RNA
  modified_base 1: mod_base = OTHER; note = 5'-E-vinylphosphonate-2'-O-methyl-uridine
  modified_base 2: mod_base = OTHER; note = 2'-deoxy-2'-fluorocytidine
  modified_base 3: mod_base = OTHER; note = cm
  modified_base 7: mod_base = OTHER; note = gm
  modified_base 18: mod_base = OTHER; note = cm
  modified_base 1..3: mod_base = OTHER; note = phosphorothioate bond between nucleotides
  modified_base 18..20: mod_base = OTHER; note = phosphorothioate bond between nucleotides
tccagaggagattttggcac

SEQ ID NO: 990 - RNA, 20 nt, synthetic construct
  source 1..20: mol_type = other RNA
  modified_base 1: mod_base = OTHER; note = 5'-E-vinylphosphonate-2'-O-methyl-uridine
  modified_base 3: mod_base = OTHER; note = 2'-deoxy-2'-fluorocytidine
  modified_base 4: mod_base = OTHER; note = cm
  modified_base 8: mod_base = OTHER; note = gm
  modified_base 18: mod_base = OTHER; note = cm
  modified_base 1^2: mod_base = OTHER; note = phosphorothioate bond between nucleotides
  modified_base 19^20: mod_base = OTHER; note = phosphorothioate bond between nucleotides
  modified_base 2^3: mod_base = OTHER; note = phosphorothioate bond between nucleotides
ttccagagagattttggcac

SEQ ID NO: 991 - RNA, 19 nt, synthetic construct
  source 1..19: mol_type = other RNA
  modified_base 1: mod_base = OTHER; note = 2'-deoxy-2'-fluorouridine
  modified_base 3: mod_base = OTHER; note = cm
  modified_base 5: mod_base = OTHER; note = gm
  modified_base 6: mod_base = OTHER; note = 2'-deoxy-2'-fluoroadenosine
  modified_base 7: mod_base = OTHER; note = gm
  modified_base 9: mod_base = OTHER; note = gm
  modified_base 10: mod_base = OTHER; note = 2'-deoxy-2'-fluoroadenosine
  modified_base 18^19: mod_base = OTHER; note = phosphorothioate bond between nucleotides
tccagagagattttggcac

SEQ ID NO: 992 - RNA, 19 nt, synthetic construct
  source 1..19: mol_type = other RNA
  modified_base 2: mod_base = OTHER; note = cm
  modified_base 4: mod_base = OTHER; note = 2'-O-methyladenosine
  modified_base 6: mod_base = OTHER; note = 2'-O-methyladenosine
  modified_base 8: mod_base = OTHER; note = 2'-O-methyladenosine
  modified_base 10: mod_base = OTHER; note = 2'-O-methyladenosine
  modified_base 12: mod_base = OTHER; note = um
  modified_base 16: mod_base = OTHER; note = gm
  modified_base 18: mod_base = OTHER; note = 2'-O-methyladenosine
  modified_base 18^19: mod_base = OTHER; note = phosphorothioate bond between nucleotides
tccagagagattttggcac

SEQ ID NO: 993 - RNA, 19 nt, synthetic construct
  source 1..19: mol_type = other RNA
  modified_base 2: mod_base = OTHER; note = 2'-deoxy-2'-fluorouridine
  modified_base 3: mod_base = OTHER; note = 2'-deoxy-2'-fluorouridine
  modified_base 12: mod_base = OTHER; note = 2'-deoxy-2'-fluorouridine
  modified_base 13: mod_base = OTHER; note = 2'-deoxy-2'-fluorouridine
  modified_base 17: mod_base = OTHER; note = 2'-deoxy-2'-fluorocytidine
  modified_base 19: mod_base = OTHER; note = 2'-deoxy-2'-fluorocytidine
  modified_base 18^19: mod_base = OTHER; note = phosphorothioate bond between nucleotides
tttagagagattttggcac

SEQ ID NO: 994 - RNA, 18 nt, synthetic construct
  source 1..18: mol_type = other RNA
  modified_base 4: mod_base = OTHER; note = 2'-O-methyladenosine
  modified_base 5: mod_base = OTHER; note = gm
  modified_base 6: mod_base = OTHER; note = 2'-O-methyladenosine
  modified_base 7: mod_base = OTHER; note = 2'-deoxy-2'-fluoroguanosine
  modified_base 8: mod_base = OTHER; note = 2'-deoxy-2'-fluoroadenosine
  modified_base 15: mod_base = OTHER; note = gm
  modified_base 16: mod_base = OTHER; note = 2'-deoxy-2'-fluorocytidine
  modified_base 17: mod_base = OTHER; note = 2'-O-methyladenosine
  modified_base 18: mod_base = OTHER; note = 2'-deoxy-2'-fluorocytidine
  modified_base 17^18: mod_base = OTHER; note = phosphorothioate bond between nucleotides
tccagagagatttggcac

SEQ ID NO: 995 - RNA, 19 nt, synthetic construct
  source 1..19: mol_type = other RNA
  modified_base 3: mod_base = OTHER; note = cm
  modified_base 18^19: mod_base = OTHER; note = phosphorothioate bond between nucleotides
tccagagagattttggcac

SEQ ID NO: 996 - RNA, 19 nt, synthetic construct
  source 1..19: mol_type = other RNA
  modified_base 3: mod_base = OTHER; note = cm
  modified_base 17: mod_base = OTHER; note = cm
  modified_base 17..19: mod_base = OTHER; note = phosphorothioate bond between nucleotides
tccagagagattttggcac

SEQ ID NO: 997 - RNA, 19 nt, synthetic construct
  source 1..19: mol_type = other RNA
  modified_base 1^2: mod_base = OTHER; note = phosphorothioate bond between nucleotides
  modified_base 18^19: mod_base = OTHER; note = phosphorothioate bond between nucleotides
tccagagagattttggcac

SEQ ID NO: 998 - RNA, 19 nt, synthetic construct
  source 1..19: mol_type = other RNA
  modified_base 1: mod_base = OTHER; note = 5'-E-vinylphosphonate-2'-O-methyl-uridine
  modified_base 2: mod_base = m5c
  modified_base 3: mod_base = m5c
  modified_base 18^19: mod_base = OTHER; note = phosphorothioate bond between nucleotides
tccagagagattttggcac

SEQ ID NO: 999 - RNA, 19 nt, synthetic construct
  source 1..19: mol_type = other RNA
  modified_base 1: mod_base = OTHER; note = 5'-E-vinylphosphonate-2'-O-methyl-uridine
  modified_base 11: mod_base = OTHER; note = m5u
  modified_base 12: mod_base = OTHER; note = m5u
  modified_base 13: mod_base = OTHER; note = m5u
  modified_base 14: mod_base = OTHER; note = m5u
  modified_base 17: mod_base = m5c
  modified_base 19: mod_base = m5c
  modified_base 18^19: mod_base = OTHER; note = phosphorothioate bond between nucleotides
tccagagagattttggcac

SEQ ID NO: 1000 - RNA, 19 nt, synthetic construct
  source 1..19: mol_type = other RNA
  modified_base 1: mod_base = OTHER; note = 2'-deoxy-2'-fluoroadenosine
  modified_base 2: mod_base = OTHER; note = 2'-deoxy-2'-fluoroadenosine
  modified_base 3: mod_base = OTHER; note = um
  modified_base 4: mod_base = OTHER; note = 2'-deoxy-2'-fluorouridine
  modified_base 5: mod_base = OTHER; note = cm
  modified_base 6: mod_base = OTHER; note = 2'-deoxy-2'-fluoroguanosine
  modified_base 7: mod_base = OTHER; note = cm
  modified_base 8: mod_base = OTHER; note = 2'-deoxy-2'-fluoroadenosine
  modified_base 9: mod_base = OTHER; note = cm
  modified_base 10: mod_base = OTHER; note = 2'-deoxy-2'-fluoroadenosine
  modified_base 11: mod_base = OTHER; note = um
  modified_base 12: mod_base = OTHER; note = 2'-deoxy-2'-fluoroguanosine
  modified_base 13: mod_base = OTHER; note = cm
  modified_base 14: mod_base = OTHER; note = 2'-deoxy-2'-fluorouridine
  modified_base 15: mod_base = OTHER; note = cm
  modified_base 16: mod_base = OTHER; note = 2'-deoxy-2'-fluorocytidine
  modified_base 17: mod_base = OTHER; note = 2'-O-methyladenosine
  modified_base 18: mod_base = OTHER; note = 2'-deoxy-2'-fluorouridine
  modified_base 19: mod_base = OTHER; note = cm
aattcgcacatgctccatc

SEQ ID NO: 1001 - RNA, 19 nt, synthetic construct
  source 1..19: mol_type = other RNA
  modified_base 1: mod_base = OTHER; note = 2'-deoxy-2'-fluoroadenosine
  modified_base 2: mod_base = OTHER; note = 2'-deoxy-2'-fluoroadenosine
  modified_base 3: mod_base = OTHER; note = um
  modified_base 4: mod_base = OTHER; note = 2'-deoxy-2'-fluorouridine
  modified_base 5: mod_base = OTHER; note = cm
  modified_base 6: mod_base = OTHER; note = 2'-deoxy-2'-fluoroguanosine
  modified_base 7: mod_base = OTHER; note = cm
  modified_base 8: mod_base = OTHER; note = 2'-deoxy-2'-fluoroadenosine
  modified_base 9: mod_base = OTHER; note = cm
  modified_base 10: mod_base = OTHER; note = 2'-deoxy-2'-fluoroadenosine
  modified_base 11: mod_base = OTHER; note = um
  modified_base 12: mod_base = OTHER; note = 2'-deoxy-2'-fluoroguanosine
  modified_base 13: mod_base = OTHER; note = cm
  modified_base 14: mod_base = OTHER; note = 2'-deoxy-2'-fluorouridine
  modified_base 15: mod_base = OTHER; note = cm
  modified_base 16: mod_base = OTHER; note = 2'-deoxy-2'-fluorocytidine
  modified_base 17: mod_base = OTHER; note = 2'-O-methyladenosine
  modified_base 18: mod_base = OTHER; note = 2'-deoxy-2'-fluorouridine
  modified_base 19: mod_base = OTHER; note = cm
  modified_base 18^19: mod_base = OTHER; note = phosphorothioate bond between nucleotides
aattcgcacatgctccatc

SEQ ID NO: 1002 - RNA, 19 nt, synthetic construct
  source 1..19: mol_type = other RNA
  modified_base 1: mod_base = OTHER; note = 2'-deoxy-2'-fluoroadenosine
  modified_base 2: mod_base = OTHER; note = 2'-deoxy-2'-fluoroadenosine
  modified_base 3: mod_base = OTHER; note = um
  modified_base 4: mod_base = OTHER; note = 2'-deoxy-2'-fluorouridine
  modified_base 5: mod_base = OTHER; note = cm
  modified_base 6: mod_base = OTHER; note = 2'-deoxy-2'-fluoroguanosine
  modified_base 7: mod_base = OTHER; note = cm
  modified_base 8: mod_base = OTHER; note = 2'-deoxy-2'-fluoroadenosine
  modified_base 9: mod_base = OTHER; note = cm
  modified_base 10: mod_base = OTHER; note = 2'-deoxy-2'-fluoroadenosine
  modified_base 11: mod_base = OTHER; note = um
  modified_base 12: mod_base = OTHER; note = 2'-deoxy-2'-fluoroguanosine
  modified_base 13: mod_base = OTHER; note = cm
  modified_base 14: mod_base = OTHER; note = 2'-deoxy-2'-fluorouridine
  modified_base 15: mod_base = OTHER; note = cm
  modified_base 16: mod_base = OTHER; note = 2'-deoxy-2'-fluorocytidine
  modified_base 17: mod_base = OTHER; note = 2'-O-methyladenosine
  modified_base 18: mod_base = OTHER; note = 2'-deoxy-2'-fluorouridine
  modified_base 19: mod_base = OTHER; note = cm
  modified_base 1..3: mod_base = OTHER; note = phosphorothioate bond between nucleotides
  modified_base 18^19: mod_base = OTHER; note = phosphorothioate bond between nucleotides
aattcgcacatgctccatc

SEQ ID NO: 1003 - RNA, 19 nt, synthetic construct
  source 1..19: mol_type = other RNA
  modified_base 1: mod_base = OTHER; note = 2'-deoxy-2'-fluoroadenosine
  modified_base 2: mod_base = OTHER; note = 2'-deoxy-2'-fluoroadenosine
  modified_base 3: mod_base = OTHER; note = um
  modified_base 4: mod_base = OTHER; note = 2'-deoxy-2'-fluorouridine
  modified_base 5: mod_base = OTHER; note = cm
  modified_base 6: mod_base = OTHER; note = 2'-deoxy-2'-fluoroguanosine
  modified_base 7: mod_base = OTHER; note = cm
  modified_base 8: mod_base = OTHER; note = 2'-deoxy-2'-fluoroadenosine
  modified_base 9: mod_base = OTHER; note = cm
  modified_base 10: mod_base = OTHER; note = 2'-deoxy-2'-fluoroadenosine
  modified_base 11: mod_base = OTHER; note = um
  modified_base 12: mod_base = OTHER; note = 2'-deoxy-2'-fluoroguanosine
  modified_base 13: mod_base = OTHER; note = cm
  modified_base 14: mod_base = OTHER; note = 2'-deoxy-2'-fluorouridine
  modified_base 15: mod_base = OTHER; note = cm
  modified_base 16: mod_base = OTHER; note = 2'-deoxy-2'-fluorocytidine
  modified_base 17: mod_base = OTHER; note = 2'-O-methyladenosine
  modified_base 18: mod_base = OTHER; note = 2'-deoxy-2'-fluorouridine
  modified_base 19: mod_base = OTHER; note = cm
  modified_base 1^2: mod_base = OTHER; note = phosphorothioate bond between nucleotides
  modified_base 18^19: mod_base = OTHER; note = phosphorothioate bond between nucleotides
aattcgcacatgctccatc

SEQ ID NO: 1004 - RNA, 19 nt, synthetic construct
  source 1..19: mol_type = other RNA
  modified_base 7: mod_base = OTHER; note = cm
  modified_base 9: mod_base = OTHER; note = cm
  modified_base 16: mod_base = OTHER; note = cm
  modified_base 18^19: mod_base = OTHER; note = phosphorothioate bond between nucleotides
aattcgcacatgctccatc

SEQ ID NO: 1005 - RNA, 19 nt, synthetic construct
  source 1..19: mol_type = other RNA
  modified_base 1: mod_base = OTHER; note = 5'-E-vinylphosphonate-2'-O-methyl-adenosine
  modified_base 7: mod_base = OTHER; note = cm
  modified_base 8: mod_base = OTHER; note = Glycol nucleic acid (GNA) monomer
  modified_base 9: mod_base = OTHER; note = cm
  modified_base 16: mod_base = OTHER; note = cm
  modified_base 1..3: mod_base = OTHER; note = phosphorothioate bond between nucleotides
  modified_base 17..19: mod_base = OTHER; note = phosphorothioate bond between nucleotides
aattcgcacatgctccatc

SEQ ID NO: 1006 - RNA, 19 nt, synthetic construct
  source 1..19: mol_type = other RNA
  modified_base 1: mod_base = OTHER; note = 5'-E-vinylphosphonate-2'-O-methyl-adenosine
  modified_base 7: mod_base = OTHER; note = cm
  modified_base 8: mod_base = OTHER; note = Glycol nucleic acid (GNA) monomer
  modified_base 9: mod_base = OTHER; note = cm
  modified_base 16: mod_base = OTHER; note = cm
  modified_base 1^2: mod_base = OTHER; note = phosphorothioate bond between nucleotides
  modified_base 18^19: mod_base = OTHER; note = phosphorothioate bond between nucleotides
aattcgcacatgctccatc

SEQ ID NO: 1007 - RNA, 19 nt, synthetic construct
  source 1..19: mol_type = other RNA
  modified_base 1: mod_base = OTHER; note = 5'-E-vinylphosphonate-2'-O-methyl-adenosine
  modified_base 7: mod_base = OTHER; note = cm
  modified_base 8: mod_base = OTHER; note = Glycol nucleic acid (GNA) monomer
  modified_base 9: mod_base = OTHER; note = cm
  modified_base 16: mod_base = OTHER; note = cm
  modified_base 1..3: mod_base = OTHER; note = phosphorothioate bond between nucleotides
  modified_base 17..19: mod_base = OTHER; note = phosphorothioate bond between nucleotides
aattcgcacatgctccatc

SEQ ID NO: 1008 - RNA, 19 nt, synthetic construct
  source 1..19: mol_type = other RNA
  modified_base 1: mod_base = OTHER; note = 5'-E-vinylphosphonate-2'-O-methyl-adenosine
  modified_base 7: mod_base = OTHER; note = cm
  modified_base 8: mod_base = OTHER; note = Glycol nucleic acid (GNA) monomer
  modified_base 9: mod_base = OTHER; note = cm
  modified_base 16: mod_base = OTHER; note = cm
  modified_base 1^2: mod_base = OTHER; note = phosphorothioate bond between nucleotides
  modified_base 18^19: mod_base = OTHER; note = phosphorothioate bond between nucleotides
aattcgcacatgctccatc

SEQ ID NO: 1009 - RNA, 19 nt, synthetic construct
  source 1..19: mol_type = other RNA
  modified_base 1: mod_base = OTHER; note = 5'-E-vinylphosphonate-2'-O-methyl-adenosine
  modified_base 7: mod_base = OTHER; note = cm
  modified_base 8: mod_base = OTHER; note = Glycol nucleic acid (GNA) monomer
  modified_base 9: mod_base = OTHER; note = cm
  modified_base 16: mod_base = OTHER; note = cm
  modified_base 1..3: mod_base = OTHER; note = phosphorothioate bond between nucleotides
  modified_base 17..19: mod_base = OTHER; note = phosphorothioate bond between nucleotides
aattcgcacatgctccatc

SEQ ID NO: 1010 - RNA, 19 nt, synthetic construct
  source 1..19: mol_type = other RNA
  modified_base 1: mod_base = OTHER; note = 5'-E-vinylphosphonate-2'-O-methyl-adenosine
  modified_base 7: mod_base = OTHER; note = cm
  modified_base 8: mod_base = OTHER; note = Glycol nucleic acid (GNA) monomer
  modified_base 9: mod_base = OTHER; note = cm
  modified_base 16: mod_base = OTHER; note = cm
  modified_base 1^2: mod_base = OTHER; note = phosphorothioate bond between nucleotides
  modified_base 18^19: mod_base = OTHER; note = phosphorothioate bond between nucleotides
aattcgcacatgctccatc

SEQ ID NO: 1011 - RNA, 19 nt, synthetic construct
  source 1..19: mol_type = other RNA
  modified_base 2: mod_base = OTHER; note = 2'-deoxy-2'-fluoroadenosine
  modified_base 4: mod_base = OTHER; note = 2'-deoxy-2'-fluorouridine
  modified_base 5: mod_base = OTHER; note = cm
  modified_base 7: mod_base = OTHER; note = cm
  modified_base 11: mod_base = OTHER; note = um
  modified_base 16: mod_base = OTHER; note = cm
  modified_base 18^19: mod_base = OTHER; note = phosphorothioate bond between nucleotides
aattcgcacatgctccatc

SEQ ID NO: 1012 - RNA, 19 nt, synthetic construct
  source 1..19: mol_type = other RNA
  modified_base 2: mod_base = OTHER; note = 2'-O-methyladenosine
  modified_base 4: mod_base = OTHER; note = um
  modified_base 6: mod_base = OTHER; note = gm
  modified_base 8: mod_base = OTHER; note = 2'-O-methyladenosine
  modified_base 10: mod_base = OTHER; note = 2'-O-methyladenosine
  modified_base 12: mod_base = OTHER; note = gm
  modified_base 14: mod_base = OTHER; note = um
  modified_base 16: mod_base = OTHER; note = cm
  modified_base 18: mod_base = OTHER; note = um
  modified_base 18^19: mod_base = OTHER; note = phosphorothioate bond between nucleotides
aattcgcacatgctccatc

SEQ ID NO: 1013 - RNA, 19 nt, synthetic construct
  source 1..19: mol_type = other RNA
  modified_base 4: mod_base = OTHER; note = 2'-deoxy-2'-fluorouridine
  modified_base 5: mod_base = OTHER; note = 2'-deoxy-2'-fluorocytidine
  modified_base 7: mod_base = OTHER; note = 2'-deoxy-2'-fluorocytidine
  modified_base 11: mod_base = OTHER; note = 2'-deoxy-2'-fluorouridine
  modified_base 16: mod_base = OTHER; note = 2'-deoxy-2'-fluorocytidine
  modified_base 18: mod_base = OTHER; note = 2'-deoxy-2'-fluorouridine
  modified_base 18^19: mod_base = OTHER; note = phosphorothioate bond between nucleotides
aattcgcacatgctccatc

SEQ ID NO: 1014 - RNA, 19 nt, synthetic construct
  source 1..19: mol_type = other RNA
  modified_base 6: mod_base = OTHER; note = gm
  modified_base 7: mod_base = OTHER; note = 2'-deoxy-2'-fluorocytidine
  modified_base 8: mod_base = OTHER; note = 2'-deoxy-2'-fluoroadenosine
  modified_base 9: mod_base = OTHER; note = cm
  modified_base 12: mod_base = OTHER; note = gm
  modified_base 16: mod_base = OTHER; note = cm
  modified_base 17: mod_base = OTHER; note = 2'-O-methyladenosine
  modified_base 18^19: mod_base = OTHER; note = phosphorothioate bond between nucleotides
aattcgcacatgctccatc

SEQ ID NO: 1015 - RNA, 19 nt, synthetic construct
  source 1..19: mol_type = other RNA
  modified_base 7: mod_base = OTHER; note = cm
  modified_base 16: mod_base = OTHER; note = cm
  modified_base 18^19: mod_base = OTHER; note = phosphorothioate bond between nucleotides
aattcgcacatgctccatc

SEQ ID NO: 1016 - RNA, 19 nt, synthetic construct
  source 1..19: mol_type = other RNA
  modified_base 1: mod_base = OTHER; note = 2'-deoxy-2'-fluoroadenosine
  modified_base 2: mod_base = OTHER; note = 2'-deoxy-2'-fluoroadenosine
  modified_base 4: mod_base = OTHER; note = 2'-deoxy-2'-fluorouridine
  modified_base 5: mod_base = OTHER; note = 2'-deoxy-2'-fluorocytidine
  modified_base 13: mod_base = OTHER; note = cm
  modified_base 2^3: mod_base = OTHER; note = phosphorothioate bond between nucleotides
  modified_base 17..19: mod_base = OTHER; note = phosphorothioate bond between nucleotides
aattcgcacatgcgccatc

SEQ ID NO: 1017 - RNA, 19 nt, synthetic construct
  source 1..19: mol_type = other RNA
  modified_base 18^19: mod_base = OTHER; note = phosphorothioate bond between nucleotides
aattcgcacatgctccatc

SEQ ID NO: 1018 - RNA, 19 nt, synthetic construct
  source 1..19: mol_type = other RNA
  modified_base 1: mod_base = OTHER; note = 5'-E-vinylphosphonate-2'-O-methyl-adenosine
  modified_base 7: mod_base = m5c
  modified_base 9: mod_base = m5c
  modified_base 16: mod_base = m5c
  modified_base 18^19: mod_base = OTHER; note = phosphorothioate bond between nucleotides
aattcgcacatgctccatc

SEQ ID NO: 1019 - RNA, 19 nt, synthetic construct
  source 1..19: mol_type = other RNA
  modified_base 1: mod_base = OTHER; note = 5'-E-vinylphosphonate-2'-O-methyl-adenosine
  modified_base 3: mod_base = OTHER; note = m5u
  modified_base 4: mod_base = OTHER; note = m5u
  modified_base 5: mod_base = m5c
  modified_base 7: mod_base = m5c
  modified_base 9: mod_base = m5c
  modified_base 16: mod_base = m5c
  modified_base 18^19: mod_base = OTHER; note = phosphorothioate bond between nucleotides
aattcgcacatgctccatc

SEQ ID NO: 1020 - RNA, 19 nt, synthetic construct
  source 1..19: mol_type = other RNA
  modified_base 1: mod_base = OTHER; note = 5'-E-vinylphosphonate-2'-O-methyl-adenosine
  modified_base 13: mod_base = m5c
  modified_base 14: mod_base = OTHER; note = m5u
  modified_base 15: mod_base = m5c
  modified_base 16: mod_base = m5c
  modified_base 18: mod_base = OTHER; note = m5u
  modified_base 19: mod_base = m5c
  modified_base 18^19: mod_base = OTHER; note = phosphorothioate bond between nucleotides
aattcgcacatgctccatc

SEQ ID NO: 1021 - RNA, 19 nt, synthetic construct
  source 1..19: mol_type = other RNA
  modified_base 7: mod_base = OTHER; note = cm
  modified_base 9: mod_base = OTHER; note = cm
  modified_base 16: mod_base = OTHER; note = cm
aattcgcacatgctccatc

SEQ ID NO: 1022 - RNA, 19 nt, synthetic construct
  source 1..19: mol_type = other RNA
  modified_base 1: mod_base = OTHER; note = 2'-deoxy-2'-fluorouridine
  modified_base 2: mod_base = OTHER; note = 2'-deoxy-2'-fluoroguanosine
  modified_base 3: mod_base = OTHER; note = um
  modified_base 4: mod_base = OTHER; note = 2'-deoxy-2'-fluorocytidine
  modified_base 5: mod_base = OTHER; note = 2'-O-methyladenosine
  modified_base 6: mod_base = OTHER; note = 2'-deoxy-2'-fluorocytidine
  modified_base 7: mod_base = OTHER; note = 2'-O-methyladenosine
  modified_base 8: mod_base = OTHER; note = 2'-deoxy-2'-fluoroguanosine
  modified_base 9: mod_base = OTHER; note = um
  modified_base 10: mod_base = OTHER; note = 2'-deoxy-2'-fluoroguanosine
  modified_base 11: mod_base = OTHER; note = 2'-O-methyladenosine
  modified_base 12: mod_base = OTHER; note = 2'-deoxy-2'-fluorocytidine
  modified_base 13: mod_base = OTHER; note = 2'-O-methyladenosine
  modified_base 14: mod_base = OTHER; note = 2'-deoxy-2'-fluoroadenosine
  modified_base 15: mod_base = OTHER; note = gm
  modified_base 16: mod_base = OTHER; note = 2'-deoxy-2'-fluorocytidine
  modified_base 17: mod_base = OTHER; note = um
  modified_base 18: mod_base = OTHER; note = 2'-deoxy-2'-fluorouridine
  modified_base 19: mod_base = OTHER; note = gm
tgtcacagtgacaagcttg

SEQ ID NO: 1023 - RNA, 19 nt, synthetic construct
  source 1..19: mol_type = other RNA
  modified_base 1: mod_base = OTHER; note = 2'-deoxy-2'-fluorouridine
  modified_base 2: mod_base = OTHER; note = 2'-deoxy-2'-fluoroguanosine
  modified_base 3: mod_base = OTHER; note = um
  modified_base 4: mod_base = OTHER; note = 2'-deoxy-2'-fluorocytidine
  modified_base 5: mod_base = OTHER; note = 2'-O-methyladenosine
  modified_base 6: mod_base = OTHER; note = 2'-deoxy-2'-fluorocytidine
  modified_base 7: mod_base = OTHER; note = 2'-O-methyladenosine
  modified_base 8: mod_base = OTHER; note = 2'-deoxy-2'-fluoroguanosine
  modified_base 9: mod_base = OTHER; note = um
  modified_base 10: mod_base = OTHER; note = 2'-deoxy-2'-fluoroguanosine
  modified_base 11: mod_base = OTHER; note = 2'-O-methyladenosine
  modified_base 12: mod_base = OTHER; note = 2'-deoxy-2'-fluorocytidine
  modified_base 13: mod_base = OTHER; note = 2'-O-methyladenosine
  modified_base 14: mod_base = OTHER; note = 2'-deoxy-2'-fluoroadenosine
  modified_base 15: mod_base = OTHER; note = gm
  modified_base 16: mod_base = OTHER; note = 2'-deoxy-2'-fluorocytidine
  modified_base 17: mod_base = OTHER; note = um
  modified_base 18: mod_base = OTHER; note = 2'-deoxy-2'-fluorouridine
  modified_base 19: mod_base = OTHER; note = gm
  modified_base 1..3: mod_base = OTHER; note = phosphorothioate bond between nucleotides
  modified_base 18^19: mod_base = OTHER; note = phosphorothioate bond between nucleotides
tgtcacagtgacaagcttg

SEQ ID NO: 1024 - RNA, 19 nt, synthetic construct
  source 1..19: mol_type = other RNA
  modified_base 1: mod_base = OTHER; note = 2'-deoxy-2'-fluorouridine
  modified_base 2: mod_base = OTHER; note = 2'-deoxy-2'-fluoroguanosine
  modified_base 3: mod_base = OTHER; note = um
  modified_base 4: mod_base = OTHER; note = 2'-deoxy-2'-fluorocytidine
  modified_base 5: mod_base = OTHER; note = 2'-O-methyladenosine
  modified_base 6: mod_base = OTHER; note = 2'-deoxy-2'-fluorocytidine
  modified_base 7: mod_base = OTHER; note = 2'-O-methyladenosine
  modified_base 8: mod_base = OTHER; note = 2'-deoxy-2'-fluoroguanosine
  modified_base 9: mod_base = OTHER; note = um
  modified_base 10: mod_base = OTHER; note = 2'-deoxy-2'-fluoroguanosine
  modified_base 11: mod_base = OTHER; note = 2'-O-methyladenosine
  modified_base 12: mod_base = OTHER; note = 2'-deoxy-2'-fluorocytidine
  modified_base 13: mod_base = OTHER; note = 2'-O-methyladenosine
  modified_base 14: mod_base = OTHER; note = 2'-deoxy-2'-fluoroadenosine
  modified_base 15: mod_base = OTHER; note = gm
  modified_base 16: mod_base = OTHER; note = 2'-deoxy-2'-fluorocytidine
  modified_base 17: mod_base = OTHER; note = um
  modified_base 18: mod_base = OTHER; note = 2'-deoxy-2'-fluorouridine
  modified_base 19: mod_base = OTHER; note = gm
  modified_base 1^2: mod_base = OTHER; note = phosphorothioate bond between nucleotides
  modified_base 18^19: mod_base = OTHER; note = phosphorothioate bond between nucleotides
tgtcacagtgacaagcttg

SEQ ID NO: 1025 - RNA, 19 nt, synthetic construct
  source 1..19: mol_type = other RNA
  modified_base 1: mod_base = OTHER; note = 2'-deoxy-2'-fluorouridine
  modified_base 2: mod_base = OTHER; note = 2'-deoxy-2'-fluoroguanosine
  modified_base 3: mod_base = OTHER; note = um
  modified_base 4: mod_base = OTHER; note = 2'-deoxy-2'-fluorocytidine
  modified_base 5: mod_base = OTHER; note = 2'-O-methyladenosine
  modified_base 6: mod_base = OTHER; note = 2'-deoxy-2'-fluorocytidine
  modified_base 7: mod_base = OTHER; note = 2'-O-methyladenosine
  modified_base 8: mod_base = OTHER; note = 2'-deoxy-2'-fluoroguanosine
  modified_base 9: mod_base = OTHER; note = um
  modified_base 10: mod_base = OTHER; note = 2'-deoxy-2'-fluoroguanosine
  modified_base 11: mod_base = OTHER; note = 2'-O-methyladenosine
  modified_base 12: mod_base = OTHER; note = 2'-deoxy-2'-fluorocytidine
  modified_base 13: mod_base = OTHER; note = 2'-O-methyladenosine
  modified_base 14: mod_base = OTHER; note = 2'-deoxy-2'-fluoroadenosine
  modified_base 15: mod_base = OTHER; note = gm
  modified_base 16: mod_base = OTHER; note = 2'-deoxy-2'-fluorocytidine
  modified_base 17: mod_base = OTHER; note = um
  modified_base 18: mod_base = OTHER; note = 2'-deoxy-2'-fluorouridine
  modified_base 19: mod_base = OTHER; note = gm
  modified_base 18^19: mod_base = OTHER; note = phosphorothioate bond between nucleotides
tgtcacagtgacaagcttg

SEQ ID NO: 1026 - RNA, 19 nt, synthetic construct
  source 1..19: mol_type = other RNA
  modified_base 4: mod_base = OTHER; note = cm
  modified_base 6: mod_base = OTHER; note = cm
  modified_base 12: mod_base = OTHER; note = cm
  modified_base 18^19: mod_base = OTHER; note = phosphorothioate bond between nucleotides
tgtcacagtgacaagcttg

SEQ ID NO: 1027 - RNA, 19 nt, synthetic construct
  source 1..19: mol_type = other RNA
  modified_base 1: mod_base = OTHER; note = 5'-E-vinylphosphonate-2'-O-methyl-uridine
  modified_base 4: mod_base = OTHER; note = cm
  modified_base 6: mod_base = OTHER; note = cm
  modified_base 7: mod_base = OTHER; note = Glycol nucleic acid (GNA) monomer
  modified_base 12: mod_base = OTHER; note = cm
  modified_base 1..3: mod_base = OTHER; note = phosphorothioate bond between nucleotides
  modified_base 17..19: mod_base = OTHER; note = phosphorothioate bond between nucleotides
tgtcacagtgacaagcttg

SEQ ID NO: 1028 - RNA, 19 nt, synthetic construct
  source 1..19: mol_type = other RNA
  modified_base 1: mod_base = OTHER; note = 5'-E-vinylphosphonate-2'-O-methyl-uridine
  modified_base 4: mod_base = OTHER; note = cm
  modified_base 6: mod_base = OTHER; note = cm
  modified_base 7: mod_base = OTHER; note = Glycol nucleic acid (GNA) monomer
  modified_base 12: mod_base = OTHER; note = cm
  modified_base 1^2: mod_base = OTHER; note = phosphorothioate bond between nucleotides
  modified_base 18^19: mod_base = OTHER; note = phosphorothioate bond between nucleotides
tgtcacagtgacaagcttg

SEQ ID NO: 1029 - RNA, 19 nt, synthetic construct
  source 1..19: mol_type = other RNA
  modified_base 1: mod_base = OTHER; note = 5'-E-vinylphosphonate-2'-O-methyl-uridine
  modified_base 4: mod_base = OTHER; note = cm
  modified_base 6: mod_base = OTHER; note = cm
  modified_base 7: mod_base = OTHER; note = Glycol nucleic acid (GNA) monomer
  modified_base 12: mod_base = OTHER; note = cm
  modified_base 1..3: mod_base = OTHER; note = phosphorothioate bond between nucleotides
  modified_base 17..19: mod_base = OTHER; note = phosphorothioate bond between nucleotides
tgtcacagtgacaagcttg

SEQ ID NO: 1030 - RNA, 19 nt, synthetic construct
  source 1..19: mol_type = other RNA
  modified_base 1: mod_base = OTHER; note = 5'-E-vinylphosphonate-2'-O-methyl-uridine
  modified_base 4: mod_base = OTHER; note = cm
  modified_base 6: mod_base = OTHER; note = cm
  modified_base 7: mod_base = OTHER; note = Glycol nucleic acid (GNA) monomer
  modified_base 12: mod_base = OTHER; note = cm
  modified_base 1^2: mod_base = OTHER; note = phosphorothioate bond between nucleotides
  modified_base 18^19: mod_base = OTHER; note = phosphorothioate bond between nucleotides
tgtcacagtgacaagcttg

SEQ ID NO: 1031 - RNA, 19 nt, synthetic construct
  source 1..19: mol_type = other RNA
  modified_base 1: mod_base = OTHER; note = 5'-E-vinylphosphonate-2'-O-methyl-uridine
  modified_base 4: mod_base = OTHER; note = cm
  modified_base 6: mod_base = OTHER; note = cm
  modified_base 7: mod_base = OTHER; note = Glycol nucleic acid (GNA) monomer
  modified_base 12: mod_base = OTHER; note = cm
  modified_base 1..3: mod_base = OTHER; note = phosphorothioate bond between nucleotides
  modified_base 17..19: mod_base = OTHER; note = phosphorothioate bond between nucleotides
tgtcacagtgacaagcttg

SEQ ID NO: 1032 - RNA, 19 nt, synthetic construct
  source 1..19: mol_type = other RNA
  modified_base 1: mod_base = OTHER; note = 5'-E-vinylphosphonate-2'-O-methyl-uridine
  modified_base 4: mod_base = OTHER; note = cm
  modified_base 6: mod_base = OTHER; note = cm
  modified_base 7: mod_base = OTHER; note = Glycol nucleic acid (GNA) monomer
  modified_base 12: mod_base = OTHER; note = cm
  modified_base 1^2: mod_base = OTHER; note = phosphorothioate bond between nucleotides
  modified_base 18^19: mod_base = OTHER; note = phosphorothioate bond between nucleotides
tgtcacagtgacaagcttg

SEQ ID NO: 1033 - RNA, 19 nt, synthetic construct
  source 1..19: mol_type = other RNA
  modified_base 1: mod_base = OTHER; note = 2'-deoxy-2'-fluorouridine
  modified_base 2: mod_base = OTHER; note = gm
  modified_base 3: mod_base = OTHER; note = um
  modified_base 4: mod_base = OTHER; note = 2'-deoxy-2'-fluorocytidine
  modified_base 5: mod_base = OTHER; note = 2'-O-methyladenosine
  modified_base 6: mod_base = OTHER; note = 2'-deoxy-2'-fluorocytidine
  modified_base 7: mod_base = OTHER; note = 2'-O-methyladenosine
  modified_base 12: mod_base = OTHER; note = cm
  modified_base 18^19: mod_base = OTHER; note = phosphorothioate bond between nucleotides
tgtcacagtgacaagcttg

SEQ ID NO: 1034 - RNA, 19 nt, synthetic construct
  source 1..19: mol_type = other RNA
  modified_base 2: mod_base = OTHER; note = gm
  modified_base 4: mod_base = OTHER; note = cm
  modified_base 6: mod_base = OTHER; note = cm
  modified_base 8: mod_base = OTHER; note = gm
  modified_base 10: mod_base = OTHER; note = gm
  modified_base 12: mod_base = OTHER; note = cm
  modified_base 14: mod_base = OTHER; note = 2'-O-methyladenosine
  modified_base 16: mod_base = OTHER; note = cm
  modified_base 18: mod_base = OTHER; note = um
  modified_base 18^19: mod_base = OTHER; note = phosphorothioate bond between nucleotides
tgtcacagtgacaagcttg

SEQ ID NO: 1035 - RNA, 19 nt, synthetic construct
  source 1..19: mol_type = other RNA
  modified_base 1: mod_base = OTHER; note = 2'-deoxy-2'-fluorouridine
  modified_base 4: mod_base = OTHER; note = 2'-deoxy-2'-fluorocytidine
  modified_base 6: mod_base = OTHER; note = 2'-deoxy-2'-fluorocytidine
  modified_base 12: mod_base = OTHER; note = 2'-deoxy-2'-fluorocytidine
  modified_base 17: mod_base = OTHER; note = 2'-deoxy-2'-fluorouridine
  modified_base 18: mod_base = OTHER; note = 2'-deoxy-2'-fluorouridine
  modified_base 18^19: mod_base = OTHER; note = phosphorothioate bond between nucleotides
tgtcacagtgacaagcttg

SEQ ID NO: 1036 - RNA, 19 nt, synthetic construct
  source 1..19: mol_type = other RNA
  modified_base 5: mod_base = OTHER; note = 2'-O-methyladenosine
  modified_base 7: mod_base = OTHER; note = 2'-deoxy-2'-fluoroadenosine
  modified_base 8: mod_base = OTHER; note = 2'-deoxy-2'-fluoroguanosine
  modified_base 13: mod_base = OTHER; note = 2'-O-methyladenosine
  modified_base 15: mod_base = OTHER; note = gm
  modified_base 19: mod_base = OTHER; note = gm
  modified_base 18^19: mod_base = OTHER; note = phosphorothioate bond between nucleotides
tgtcacagtgacaagcttg

SEQ ID NO: 1037 - RNA, 19 nt, synthetic construct
  source 1..19: mol_type = other RNA
  modified_base 3: mod_base = OTHER; note = um
  modified_base 4: mod_base = OTHER; note = cm
  modified_base 18^19: mod_base = OTHER; note = phosphorothioate bond between nucleotides
tgtcacagtgacaagcttg

SEQ ID NO: 1038 - RNA, 19 nt, synthetic construct
  source 1..19: mol_type = other RNA
  modified_base 1: mod_base = OTHER; note = 2'-deoxy-2'-fluorouridine
  modified_base 2: mod_base = OTHER; note = 2'-deoxy-2'-fluoroguanosine
  modified_base 4: mod_base = OTHER; note = 2'-deoxy-2'-fluorocytidine
  modified_base 5: mod_base = OTHER; note = 2'-deoxy-2'-fluoroadenosine
  modified_base 6: mod_base = OTHER; note = cm
  modified_base 12: mod_base = OTHER; note = cm
  modified_base 18: mod_base = OTHER; note = um
  modified_base 2^3: mod_base = OTHER; note = phosphorothioate bond between nucleotides
  modified_base 16..19: mod_base = OTHER; note = phosphorothioate bond between nucleotides
tgtcacagtgacaagcttg

SEQ ID NO: 1039 - RNA, 19 nt, synthetic construct
  source 1..19: mol_type = other RNA
  modified_base 18^19: mod_base = OTHER; note = phosphorothioate bond between nucleotides
tgtcacagtgacaagcttg

SEQ ID NO: 1040 - RNA, 20 nt, synthetic construct
  source 1..20: mol_type = other RNA
  modified_base 1: mod_base = OTHER; note = 5'-E-vinylphosphonate-2'-O-methyl-uridine
  modified_base 7: mod_base = m5c
  modified_base 13: mod_base = m5c
  modified_base 1^2: mod_base = OTHER; note = phosphorothioate bond between nucleotides
ttgtcacagtgacaagcttg

SEQ ID NO: 1041 - RNA, 19 nt, synthetic construct
  source 1..19: mol_type = other RNA
  modified_base 1: mod_base = OTHER; note = 5'-E-vinylphosphonate-2'-O-methyl-5-methyuridine
  modified_base 3: mod_base = OTHER; note = m5u
  modified_base 4: mod_base = m5c
  modified_base 6: mod_base = m5c
  modified_base 12: mod_base = m5c
  modified_base 18^19: mod_base = OTHER; note = phosphorothioate bond between nucleotides
tgtcacagtgacaagcttg

SEQ ID NO: 1042 - RNA, 19 nt, synthetic construct
  source 1..19: mol_type = other RNA
  modified_base 1: mod_base = OTHER; note = 5'-E-vinylphosphonate-2'-O-methyl-uridine
  modified_base 12: mod_base = m5c
  modified_base 17: mod_base = OTHER; note = m5u
  modified_base 18: mod_base = OTHER; note = m5u
  modified_base 18^19: mod_base = OTHER; note = phosphorothioate bond between nucleotides
tgtcacagtgacaagcttg

SEQ ID NO: 1043 - RNA, 19 nt, synthetic construct
  source 1..19: mol_type = other RNA
  modified_base 1: mod_base = OTHER; note = 2'-deoxy-2'-fluorouridine
  modified_base 2: mod_base = OTHER; note = 2'-deoxy-2'-fluoroguanosine
  modified_base 3: mod_base = OTHER; note = um
  modified_base 4: mod_base = OTHER; note = 2'-deoxy-2'-fluorocytidine
  modified_base 5: mod_base = OTHER; note = 2'-O-methyladenosine
  modified_base 6: mod_base = OTHER; note = 2'-deoxy-2'-fluorocytidine
  modified_base 7: mod_base = OTHER; note = 2'-O-methyladenosine
  modified_base 8: mod_base = OTHER; note = 2'-deoxy-2'-fluoroguanosine
  modified_base 9: mod_base = OTHER; note = um
  modified_base 10: mod_base = OTHER; note = 2'-deoxy-2'-fluoroguanosine
  modified_base 11: mod_base = OTHER; note = 2'-O-methyladenosine
  modified_base 12: mod_base = OTHER; note = 2'-deoxy-2'-fluorocytidine
  modified_base 13: mod_base = OTHER; note = 2'-O-methyladenosine
  modified_base 14: mod_base = OTHER; note = 2'-deoxy-2'-fluoroadenosine
  modified_base 15: mod_base = OTHER; note = gm
  modified_base 16: mod_base = OTHER; note = 2'-deoxy-2'-fluorocytidine
  modified_base 17: mod_base = OTHER; note = um
  modified_base 18: mod_base = OTHER; note = 2'-deoxy-2'-fluorouridine
  modified_base 19: mod_base = OTHER; note = gm
tgtcacagtgacaagcttg

SEQ ID NO: 1044 - RNA, 19 nt, synthetic construct
  source 1..19: mol_type = other RNA
  modified_base 1: mod_base = OTHER; note = 2'-deoxy-2'-fluorouridine
  modified_base 2: mod_base = OTHER; note = 2'-deoxy-2'-fluoroguanosine
  modified_base 3: mod_base = OTHER; note = um
  modified_base 4: mod_base = OTHER; note = 2'-deoxy-2'-fluorocytidine
  modified_base 5: mod_base = OTHER; note = 2'-O-methyladenosine
  modified_base 6: mod_base = OTHER; note = 2'-deoxy-2'-fluorocytidine
  modified_base 7: mod_base = OTHER; note = 2'-O-methyladenosine
  modified_base 8: mod_base = OTHER; note = 2'-deoxy-2'-fluoroguanosine
  modified_base 9: mod_base = OTHER; note = um
  modified_base 10: mod_base = OTHER; note = 2'-deoxy-2'-fluoroguanosine
  modified_base 11: mod_base = OTHER; note = 2'-O-methyladenosine
  modified_base 12: mod_base = OTHER; note = 2'-deoxy-2'-fluorocytidine
  modified_base 13: mod_base = OTHER; note = 2'-O-methyladenosine
  modified_base 14: mod_base = OTHER; note = 2'-deoxy-2'-fluoroadenosine
  modified_base 15: mod_base = OTHER; note = gm
  modified_base 16: mod_base = OTHER; note = 2'-deoxy-2'-fluorocytidine
  modified_base 17: mod_base = OTHER; note = um
  modified_base 18: mod_base = OTHER; note = 2'-deoxy-2'-fluorouridine
  modified_base 19: mod_base = OTHER; note = gm
tgtcacagtgacaagcttg

SEQ ID NO: 1045 - RNA, 21 nt, synthetic construct
  source 1..21: mol_type = other RNA
  modified_base 1: mod_base = OTHER; note = 2'-deoxy-2'-fluorocytidine
  modified_base 2: mod_base = OTHER; note = 2'-deoxy-2'-fluoroadenosine
  modified_base 3: mod_base = OTHER; note = 2'-O-methyladenosine
  modified_base 4: mod_base = OTHER; note = 2'-deoxy-2'-fluorocytidine
  modified_base 5: mod_base = OTHER; note = cm
  modified_base 6: mod_base = OTHER; note = 2'-deoxy-2'-fluoroadenosine
  modified_base 7: mod_base = OTHER; note = gm
  modified_base 8: mod_base = OTHER; note = 2'-deoxy-2'-fluorocytidine
  modified_base 9: mod_base = OTHER; note = cm
  modified_base 10: mod_base = OTHER; note = 2'-deoxy-2'-fluoroadenosine
  modified_base 11: mod_base = OTHER; note = gm
  modified_base 12: mod_base = OTHER; note = 2'-deoxy-2'-fluoroguanosine
  modified_base 13: mod_base = OTHER; note = um
  modified_base 14: mod_base = OTHER; note = 2'-deoxy-2'-fluorouridine
  modified_base 15: mod_base = OTHER; note = um
  modified_base 16: mod_base = OTHER; note = 2'-deoxy-2'-fluorouridine
  modified_base 17: mod_base = OTHER; note = gm
  modified_base 18: mod_base = OTHER; note = 2'-deoxy-2'-fluoroguanosine
  modified_base 19: mod_base = OTHER; note = um
  modified_base 20: mod_base = OTHER; note = 2'-deoxy-2'-fluorocytidine
  modified_base 21: mod_base = OTHER; note = cm
caaccagccaggttttggtcc

SEQ ID NO: 1046 - RNA, 21 nt, synthetic construct
  source 1..21: mol_type = other RNA
  modified_base 1: mod_base = OTHER; note = 2'-deoxy-2'-fluorocytidine
  modified_base 2: mod_base = OTHER; note = 2'-deoxy-2'-fluoroadenosine
  modified_base 3: mod_base = OTHER; note = 2'-O-methyladenosine
  modified_base 4: mod_base = OTHER; note = 2'-deoxy-2'-fluorocytidine
  modified_base 5: mod_base = OTHER; note = cm
  modified_base 6: mod_base = OTHER; note = 2'-deoxy-2'-fluoroadenosine
  modified_base 7: mod_base = OTHER; note = gm
  modified_base 8: mod_base = OTHER; note = 2'-deoxy-2'-fluorocytidine
  modified_base 9: mod_base = OTHER; note = cm
  modified_base 10: mod_base = OTHER; note = 2'-deoxy-2'-fluoroadenosine
  modified_base 11: mod_base = OTHER; note = gm
  modified_base 12: mod_base = OTHER; note = 2'-deoxy-2'-fluoroguanosine
  modified_base 13: mod_base = OTHER; note = um
  modified_base 14: mod_base = OTHER; note = 2'-deoxy-2'-fluorouridine
  modified_base 15: mod_base = OTHER; note = um
  modified_base 16: mod_base = OTHER; note = 2'-deoxy-2'-fluorouridine
  modified_base 17: mod_base = OTHER; note = gm
  modified_base 18: mod_base = OTHER; note = 2'-deoxy-2'-fluoroguanosine
  modified_base 19: mod_base = OTHER; note = um
  modified_base 20: mod_base = OTHER; note = 2'-deoxy-2'-fluorocytidine
  modified_base 21: mod_base = OTHER; note = cm
caaccagccaggttttggtcc

SEQ ID NO: 1047 - RNA, 19 nt, synthetic construct
  source 1..19: mol_type = other RNA
  modified_base 1: mod_base = OTHER; note = 2'-deoxy-2'-fluorocytidine
  modified_base 2: mod_base = OTHER; note = 2'-deoxy-2'-fluoroadenosine
  modified_base 3: mod_base = OTHER; note = 2'-O-methyladenosine
  modified_base 4: mod_base = OTHER; note = 2'-deoxy-2'-fluorocytidine
  modified_base 5: mod_base = OTHER; note = cm
  modified_base 6: mod_base = OTHER; note = 2'-deoxy-2'-fluoroadenosine
  modified_base 7: mod_base = OTHER; note = gm
  modified_base 8: mod_base = OTHER; note = 2'-deoxy-2'-fluorocytidine
  modified_base 9: mod_base = OTHER; note = cm
  modified_base 10: mod_base = OTHER; note = 2'-deoxy-2'-fluoroadenosine
  modified_base 11: mod_base = OTHER; note = gm
  modified_base 12: mod_base = OTHER; note = 2'-deoxy-2'-fluoroguanosine
  modified_base 13: mod_base = OTHER; note = um
  modified_base 14: mod_base = OTHER; note = 2'-deoxy-2'-fluorouridine
  modified_base 15: mod_base = OTHER; note = um
  modified_base 16: mod_base = OTHER; note = 2'-deoxy-2'-fluorouridine
  modified_base 17: mod_base = OTHER; note = gm
  modified_base 18: mod_base = OTHER; note = 2'-deoxy-2'-fluoroguanosine
  modified_base 19: mod_base = OTHER; note = um
caaccagccaggttttggt

SEQ ID NO: 1048 - RNA, 19 nt, synthetic construct
  source 1..19: mol_type = other RNA
  modified_base 1: mod_base = OTHER; note = 2'-deoxy-2'-fluorocytidine
  modified_base 2: mod_base = OTHER; note = 2'-deoxy-2'-fluoroadenosine
  modified_base 3: mod_base = OTHER; note = 2'-O-methyladenosine
  modified_base 4: mod_base = OTHER; note = 2'-deoxy-2'-fluorocytidine
  modified_base 5: mod_base = OTHER; note = cm
  modified_base 6: mod_base = OTHER; note = 2'-deoxy-2'-fluoroadenosine
  modified_base 7: mod_base = OTHER; note = gm
  modified_base 8: mod_base = OTHER; note = 2'-deoxy-2'-fluorocytidine
  modified_base 9: mod_base = OTHER; note = cm
  modified_base 10: mod_base = OTHER; note = 2'-deoxy-2'-fluoroadenosine
  modified_base 11: mod_base = OTHER; note = gm
  modified_base 12: mod_base = OTHER; note = 2'-deoxy-2'-fluoroguanosine
  modified_base 13: mod_base = OTHER; note = um
  modified_base 14: mod_base = OTHER; note = 2'-deoxy-2'-fluorouridine
  modified_base 15: mod_base = OTHER; note = um
  modified_base 16: mod_base = OTHER; note = 2'-deoxy-2'-fluorouridine
  modified_base 17: mod_base = OTHER; note = gm
  modified_base 18: mod_base = OTHER; note = 2'-deoxy-2'-fluoroguanosine
  modified_base 19: mod_base = OTHER; note = um
  modified_base 1..3: mod_base = OTHER; note = phosphorothioate bond between nucleotides
  modified_base 17..19: mod_base = OTHER; note = phosphorothioate bond between nucleotides
caaccagccaggttttggt

SEQ ID NO: 1049 - RNA, 19 nt, synthetic construct
  source 1..19: mol_type = other RNA
  modified_base 1: mod_base = OTHER; note = 2'-deoxy-2'-fluorocytidine
  modified_base 2: mod_base = OTHER; note = 2'-deoxy-2'-fluoroadenosine
  modified_base 3: mod_base = OTHER; note = 2'-O-methyladenosine
  modified_base 4: mod_base = OTHER; note = 2'-deoxy-2'-fluorocytidine
  modified_base 5: mod_base = OTHER; note = cm
  modified_base 6: mod_base = OTHER; note = 2'-deoxy-2'-fluoroadenosine
  modified_base 7: mod_base = OTHER; note = gm
  modified_base 8: mod_base = OTHER; note = 2'-deoxy-2'-fluorocytidine
  modified_base 9: mod_base = OTHER; note = cm
  modified_base 10: mod_base = OTHER; note = 2'-deoxy-2'-fluoroadenosine
  modified_base 11: mod_base = OTHER; note = gm
  modified_base 12: mod_base = OTHER; note = 2'-deoxy-2'-fluoroguanosine
  modified_base 13: mod_base = OTHER; note = um
  modified_base 14: mod_base = OTHER; note = 2'-deoxy-2'-fluorouridine
  modified_base 15: mod_base = OTHER; note = um
  modified_base 16: mod_base = OTHER; note = 2'-deoxy-2'-fluorouridine
  modified_base 17: mod_base = OTHER; note = gm
  modified_base 18: mod_base = OTHER; note = 2'-deoxy-2'-fluoroguanosine
  modified_base 19: mod_base = OTHER; note = um
  modified_base 1^2: mod_base = OTHER; note = phosphorothioate bond between nucleotides
  modified_base 18^19: mod_base = OTHER; note = phosphorothioate bond between nucleotides
caaccagccaggttttggt

SEQ ID NO: 1050 - RNA, 19 nt, synthetic construct
  source 1..19: mol_type = other RNA
  modified_base 1: mod_base = OTHER; note = 2'-deoxy-2'-fluorocytidine
  modified_base 2: mod_base = OTHER; note = 2'-deoxy-2'-fluoroadenosine
  modified_base 3: mod_base = OTHER; note = 2'-O-methyladenosine
  modified_base 4: mod_base = OTHER; note = 2'-deoxy-2'-fluorocytidine
  modified_base 5: mod_base = OTHER; note = cm
  modified_base 6: mod_base = OTHER; note = 2'-deoxy-2'-fluoroadenosine
  modified_base 7: mod_base = OTHER; note = gm
  modified_base 8: mod_base = OTHER; note = 2'-deoxy-2'-fluorocytidine
  modified_base 9: mod_base = OTHER; note = cm
  modified_base 10: mod_base = OTHER; note = 2'-deoxy-2'-fluoroadenosine
  modified_base 11: mod_base = OTHER; note = gm
  modified_base 12: mod_base = OTHER; note = 2'-deoxy-2'-fluoroguanosine
  modified_base 13: mod_base = OTHER; note = um
  modified_base 14: mod_base = OTHER; note = 2'-deoxy-2'-fluorouridine
  modified_base 15: mod_base = OTHER; note = um
  modified_base 16: mod_base = OTHER; note = 2'-deoxy-2'-fluorouridine
  modified_base 17: mod_base = OTHER; note = gm
  modified_base 18: mod_base = OTHER; note = 2'-deoxy-2'-fluoroguanosine
  modified_base 19: mod_base = OTHER; note = um
  modified_base 18^19: mod_base = OTHER; note = phosphorothioate bond between nucleotides
caaccagccaggttttggt

SEQ ID NO: 1051 - RNA, 19 nt, synthetic construct
  source 1..19: mol_type = other RNA
  modified_base 1: mod_base = OTHER; note = cm
  modified_base 5: mod_base = OTHER; note = cm
  modified_base 9: mod_base = OTHER; note = cm
  modified_base 18^19: mod_base = OTHER; note = phosphorothioate bond between nucleotides
caaccagccaggttttggt

SEQ ID NO: 1052 - RNA, 18 nt, synthetic construct
  source 1..18: mol_type = other RNA
  modified_base 1: mod_base = OTHER; note = 5'-E-vinylphosphonate-2'-O-methyl-adenosine
  modified_base 4: mod_base = OTHER; note = cm
  modified_base 7: mod_base = OTHER; note = Glycol nucleic acid (GNA) monomer
  modified_base 1..3: mod_base = OTHER; note = phosphorothioate bond between nucleotides
  modified_base 16..18: mod_base = OTHER; note = phosphorothioate bond between nucleotides
aaccagccaggttttggt

SEQ ID NO: 1053 - RNA, 18 nt, synthetic construct
  source 1..18: mol_type = other RNA
  modified_base 1: mod_base = OTHER; note = 5'-E-vinylphosphonate-2'-O-methyl-adenosine
  modified_base 4: mod_base = OTHER; note = cm
  modified_base 7: mod_base = OTHER; note = Glycol nucleic acid (GNA) monomer
  modified_base 1^2: mod_base = OTHER; note = phosphorothioate bond between nucleotides
  modified_base 17^18: mod_base = OTHER; note = phosphorothioate bond between nucleotides
aaccagccaggttttggt

SEQ ID NO: 1054 - RNA, 18 nt, synthetic construct
  source 1..18: mol_type = other RNA
  modified_base 1: mod_base = OTHER; note = 5'-E-vinylphosphonate-2'-O-methyl-adenosine
  modified_base 4: mod_base = OTHER; note = cm
  modified_base 7: mod_base = OTHER; note = Glycol nucleic acid (GNA) monomer
  modified_base 1..3: mod_base = OTHER; note = phosphorothioate bond between nucleotides
  modified_base 16..18: mod_base = OTHER; note = phosphorothioate bond between nucleotides
aaccagccaggttttggt

SEQ ID NO: 1055 - RNA, 18 nt, synthetic construct
  source 1..18: mol_type = other RNA
  modified_base 1: mod_base = OTHER; note = 5'-E-vinylphosphonate-2'-O-methyl-adenosine
  modified_base 4: mod_base = OTHER; note = cm
  modified_base 7: mod_base = OTHER; note = Glycol nucleic acid (GNA) monomer
  modified_base 1^2: mod_base = OTHER; note = phosphorothioate bond between nucleotides
  modified_base 17^18: mod_base = OTHER; note = phosphorothioate bond between nucleotides
aaccagccaggttttggt

SEQ ID NO: 1056 - RNA, 18 nt, synthetic construct
  source 1..18: mol_type = other RNA
  modified_base 1: mod_base = OTHER; note = 5'-E-vinylphosphonate-2'-O-methyl-adenosine
  modified_base 4: mod_base = OTHER; note = cm
  modified_base 7: mod_base = OTHER; note = Glycol nucleic acid (GNA) monomer
  modified_base 1..3: mod_base = OTHER; note = phosphorothioate bond between nucleotides
  modified_base 16..18: mod_base = OTHER; note = phosphorothioate bond between nucleotides
aaccagccaggttttggt

SEQ ID NO: 1057 - RNA, 18 nt, synthetic construct
  source 1..18: mol_type = other RNA
  modified_base 1: mod_base = OTHER; note = 5'-E-vinylphosphonate-2'-O-methyl-adenosine
  modified_base 4: mod_base = OTHER; note = cm
  modified_base 7: mod_base = OTHER; note = Glycol nucleic acid (GNA) monomer
  modified_base 1^2: mod_base = OTHER; note = phosphorothioate bond between nucleotides
  modified_base 17^18: mod_base = OTHER; note = phosphorothioate bond between nucleotides
aaccagccaggttttggt

SEQ ID NO: 1058 - RNA, 19 nt, synthetic construct
  source 1..19: mol_type = other RNA
  modified_base 1: mod_base = OTHER; note = 2'-deoxy-2'-fluorocytidine
  modified_base 2: mod_base = OTHER; note = 2'-O-methyladenosine
  modified_base 3: mod_base = OTHER; note = 2'-deoxy-2'-fluoroadenosine
  modified_base 4: mod_base = OTHER; note = cm
  modified_base 5: mod_base = OTHER; note = 2'-deoxy-2'-fluorocytidine
  modified_base 6: mod_base = OTHER; note = 2'-O-methyladenosine
  modified_base 7: mod_base = OTHER; note = gm
  modified_base 16: mod_base = OTHER; note = um
  modified_base 19: mod_base = OTHER; note = um
  modified_base 18^19: mod_base = OTHER; note = phosphorothioate bond between nucleotides
caaccagccaggttttggt

SEQ ID NO: 1059 - RNA, 19 nt, synthetic construct
  source 1..19: mol_type = other RNA
  modified_base 2: mod_base = OTHER; note = 2'-O-methyladenosine
  modified_base 4: mod_base = OTHER; note = cm
  modified_base 6: mod_base = OTHER; note = 2'-O-methyladenosine
  modified_base 8: mod_base = OTHER; note = cm
  modified_base 10: mod_base = OTHER; note = 2'-O-methyladenosine
  modified_base 12: mod_base = OTHER; note = gm
  modified_base 14: mod_base = OTHER; note = um
  modified_base 16: mod_base = OTHER; note = um
  modified_base 18: mod_base = OTHER; note = gm
  modified_base 18^19: mod_base = OTHER; note = phosphorothioate bond between nucleotides
caaccagccaggttttggt

SEQ ID NO: 1060 - RNA, 19 nt, synthetic construct
  source 1..19: mol_type = other RNA
  modified_base 1: mod_base = OTHER; note = 2'-deoxy-2'-fluorocytidine
  modified_base 5: mod_base = OTHER; note = 2'-deoxy-2'-fluorocytidine
  modified_base 8: mod_base = OTHER; note = 2'-deoxy-2'-fluorocytidine
  modified_base 15: mod_base = OTHER; note = 2'-deoxy-2'-fluorouridine
  modified_base 16: mod_base = OTHER; note = 2'-deoxy-2'-fluorouridine
  modified_base 19: mod_base = OTHER; note = 2'-deoxy-2'-fluorouridine
  modified_base 18^19: mod_base = OTHER; note = phosphorothioate bond between nucleotides
caaccagccaggttttggt

SEQ ID NO: 1061 - RNA, 19 nt, synthetic construct
  source 1..19: mol_type = other RNA
caaccagccaggttttggt

SEQ ID NO: 1062 - RNA, 19 nt, synthetic construct
  source 1..19: mol_type = other RNA
  modified_base 5: mod_base = OTHER; note = cm
  modified_base 16: mod_base = OTHER; note = um
  modified_base 18^19: mod_base = OTHER; note = phosphorothioate bond between nucleotides
caaccagccaggttttggt

SEQ ID NO: 1063 - RNA, 19 nt, synthetic construct
  source 1..19: mol_type = other RNA
  modified_base 1: mod_base = OTHER; note = 2'-deoxy-2'-fluorocytidine
  modified_base 2: mod_base = OTHER; note = 2'-deoxy-2'-fluoroadenosine
  modified_base 4: mod_base = OTHER; note = 2'-deoxy-2'-fluorocytidine
  modified_base 5: mod_base = OTHER; note = 2'-deoxy-2'-fluorocytidine
  modified_base 9: mod_base = OTHER; note = cm
  modified_base 16: mod_base = OTHER; note = um
  modified_base 2..4: mod_base = OTHER; note = phosphorothioate bond between nucleotides
  modified_base 5^6: mod_base = OTHER; note = phosphorothioate bond between nucleotides
  modified_base 17..19: mod_base = OTHER; note = phosphorothioate bond between nucleotides
caaccagccaggttttggt

SEQ ID NO: 1064 - RNA, 19 nt, synthetic construct
  source 1..19: mol_type = other RNA
  modified_base 18^19: mod_base = OTHER; note = phosphorothioate bond between nucleotides
caaccagccaggttttggt

SEQ ID NO: 1065 - RNA, 19 nt, synthetic construct
  source 1..19: mol_type = other RNA
  modified_base 1: mod_base = OTHER; note = 5'-E-vinylphosphonate-2'-O-methyl-cytidine
  modified_base 8: mod_base = m5c
  modified_base 9: mod_base = m5c
  modified_base 18^19: mod_base = OTHER; note = phosphorothioate bond between nucleotides
caaccagccaggttttggt

SEQ ID NO: 1066 - RNA, 19 nt, synthetic construct
  source 1..19: mol_type = other RNA
  modified_base 1: mod_base = OTHER; note = 5'-E-vinylphosphonate-2'-O-methyl-cytidine
  modified_base 4: mod_base = m5c
  modified_base 5: mod_base = m5c
  modified_base 8: mod_base = m5c
  modified_base 18^19: mod_base = OTHER; note = phosphorothioate bond between nucleotides
caaccagccaggttttggt

SEQ ID NO: 1067 - RNA, 19 nt, synthetic construct
  source 1..19: mol_type = other RNA
  modified_base 1: mod_base = OTHER; note = cm
  modified_base 5: mod_base = OTHER; note = cm
  modified_base 9: mod_base = OTHER; note = cm
  modified_base 18^19: mod_base = OTHER; note = phosphorothioate bond between nucleotides
caaccagccaggttttggt

SEQ ID NO: 1068 - RNA, 19 nt, synthetic construct
  source 1..19: mol_type = other RNA
  modified_base 1: mod_base = OTHER; note = 2'-deoxy-2'-fluorocytidine
  modified_base 2: mod_base = OTHER; note = 2'-deoxy-2'-fluoroadenosine
  modified_base 3: mod_base = OTHER; note = 2'-O-methyladenosine
  modified_base 4: mod_base = OTHER; note = 2'-deoxy-2'-fluorocytidine
  modified_base 5: mod_base = OTHER; note = cm
  modified_base 6: mod_base = OTHER; note = 2'-deoxy-2'-fluoroadenosine
  modified_base 7: mod_base = OTHER; note = gm
  modified_base 8: mod_base = OTHER; note = 2'-deoxy-2'-fluorocytidine
  modified_base 9: mod_base = OTHER; note = cm
  modified_base 10: mod_base = OTHER; note = 2'-deoxy-2'-fluoroadenosine
  modified_base 11: mod_base = OTHER; note = gm
  modified_base 12: mod_base = OTHER; note = 2'-deoxy-2'-fluoroguanosine
  modified_base 13: mod_base = OTHER; note = um
  modified_base 14: mod_base = OTHER; note = 2'-deoxy-2'-fluorouridine
  modified_base 15: mod_base = OTHER; note = um
  modified_base 16: mod_base = OTHER; note = 2'-deoxy-2'-fluorouridine
  modified_base 17: mod_base = OTHER; note = gm
  modified_base 18: mod_base = OTHER; note = 2'-deoxy-2'-fluoroguanosine
  modified_base 19: mod_base = OTHER; note = um
caaccagccaggttttggt

SEQ ID NO: 1069 - RNA, 19 nt, synthetic construct
  source 1..19: mol_type = other RNA
  modified_base 1: mod_base = OTHER; note = 2'-deoxy-2'-fluorocytidine
  modified_base 2: mod_base = OTHER; note = 2'-deoxy-2'-fluoroadenosine
  modified_base 3: mod_base = OTHER; note = 2'-O-methyladenosine
  modified_base 4: mod_base = OTHER; note = 2'-deoxy-2'-fluorocytidine
  modified_base 5: mod_base = OTHER; note = cm
  modified_base 6: mod_base = OTHER; note = 2'-deoxy-2'-fluoroadenosine
  modified_base 7: mod_base = OTHER; note = gm
  modified_base 8: mod_base = OTHER; note = 2'-deoxy-2'-fluorocytidine
  modified_base 9: mod_base = OTHER; note = cm
  modified_base 10: mod_base = OTHER; note = 2'-deoxy-2'-fluoroadenosine
  modified_base 11: mod_base = OTHER; note = gm
  modified_base 12: mod_base = OTHER; note = 2'-deoxy-2'-fluoroguanosine
  modified_base 13: mod_base = OTHER; note = um
  modified_base 14: mod_base = OTHER; note = 2'-deoxy-2'-fluorouridine
  modified_base 15: mod_base = OTHER; note = um
  modified_base 16: mod_base = OTHER; note = 2'-deoxy-2'-fluorouridine
  modified_base 17: mod_base = OTHER; note = gm
  modified_base 18: mod_base = OTHER; note = 2'-deoxy-2'-fluoroguanosine
  modified_base 19: mod_base = OTHER; note = um
caaccagccaggttttggt

SEQ ID NO: 1070 - RNA, 19 nt, synthetic construct
  source 1..19: mol_type = other RNA
  modified_base 1: mod_base = OTHER; note = 2'-deoxy-2'-fluorouridine
  modified_base 2: mod_base = OTHER; note = 2'-deoxy-2'-fluoroguanosine
  modified_base 3: mod_base = OTHER; note = um
  modified_base 4: mod_base = OTHER; note = 2'-deoxy-2'-fluorocytidine
  modified_base 5: mod_base = OTHER; note = um
  modified_base 6: mod_base = OTHER; note = 2'-deoxy-2'-fluorouridine
  modified_base 7: mod_base = OTHER; note = um
  modified_base 8: mod_base = OTHER; note = 2'-deoxy-2'-fluorocytidine
  modified_base 9: mod_base = OTHER; note = cm
  modified_base 10: mod_base = OTHER; note = 2'-deoxy-2'-fluorouridine
  modified_base 11: mod_base = OTHER; note = gm
  modified_base 12: mod_base = OTHER; note = 2'-deoxy-2'-fluorocytidine
  modified_base 13: mod_base = OTHER; note = 2'-O-methyladenosine
  modified_base 14: mod_base = OTHER; note = 2'-deoxy-2'-fluorocytidine
  modified_base 15: mod_base = OTHER; note = um
  modified_base 16: mod_base = OTHER; note = 2'-deoxy-2'-fluoroguanosine
  modified_base 17: mod_base = OTHER; note = cm
  modified_base 18: mod_base = OTHER; note = 2'-deoxy-2'-fluoroadenosine
  modified_base 19: mod_base = OTHER; note = gm
tgtctttcctgcactgcag

SEQ ID NO: 1071 - RNA, 19 nt, synthetic construct
  source 1..19: mol_type = other RNA
  modified_base 1: mod_base = OTHER; note = 2'-deoxy-2'-fluorouridine
  modified_base 2: mod_base = OTHER; note = 2'-deoxy-2'-fluoroguanosine
  modified_base 3: mod_base = OTHER; note = um
  modified_base 4: mod_base = OTHER; note = 2'-deoxy-2'-fluorocytidine
  modified_base 5: mod_base = OTHER; note = um
  modified_base 6: mod_base = OTHER; note = 2'-deoxy-2'-fluorouridine
  modified_base 7: mod_base = OTHER; note = um
  modified_base 8: mod_base = OTHER; note = 2'-deoxy-2'-fluorocytidine
  modified_base 9: mod_base = OTHER; note = cm
  modified_base 10: mod_base = OTHER; note = 2'-deoxy-2'-fluorouridine
  modified_base 11: mod_base = OTHER; note = gm
  modified_base 12: mod_base = OTHER; note = 2'-deoxy-2'-fluorocytidine
  modified_base 13: mod_base = OTHER; note = 2'-O-methyladenosine
  modified_base 14: mod_base = OTHER; note = 2'-deoxy-2'-fluorocytidine
  modified_base 15: mod_base = OTHER; note = um
  modified_base 16: mod_base = OTHER; note = 2'-deoxy-2'-fluoroguanosine
  modified_base 17: mod_base = OTHER; note = cm
  modified_base 18: mod_base = OTHER; note = 2'-deoxy-2'-fluoroadenosine
  modified_base 19: mod_base = OTHER; note = gm
tgtctttcctgcactgcag

SEQ ID NO: 1072 - RNA, 19 nt, synthetic construct
  source 1..19: mol_type = other RNA
  modified_base 1: mod_base = OTHER; note = 2'-deoxy-2'-fluorouridine
  modified_base 2: mod_base = OTHER; note = 2'-deoxy-2'-fluoroguanosine
  modified_base 3: mod_base = OTHER; note = 2'-O-methyladenosine
  modified_base 4: mod_base = OTHER; note = 2'-deoxy-2'-fluoroadenosine
  modified_base 5: mod_base = OTHER; note = cm
  modified_base 6: mod_base = OTHER; note = 2'-deoxy-2'-fluorocytidine
  modified_base 7: mod_base = OTHER; note = 2'-O-methyladenosine
  modified_base 8: mod_base = OTHER; note = 2'-deoxy-2'-fluorocytidine
  modified_base 9: mod_base = OTHER; note = 2'-O-methyladenosine
  modified_base 10: mod_base = OTHER; note = 2'-deoxy-2'-fluorouridine
  modified_base 11: mod_base = OTHER; note = gm
  modified_base 12: mod_base = OTHER; note = 2'-deoxy-2'-fluoroguanosine
  modified_base 13: mod_base = OTHER; note = cm
  modified_base 14: mod_base = OTHER; note = 2'-deoxy-2'-fluorouridine
  modified_base 15: mod_base = OTHER; note = 2'-O-methyladenosine
  modified_base 16: mod_base = OTHER; note = 2'-deoxy-2'-fluorouridine
  modified_base 17: mod_base = OTHER; note = gm
  modified_base 18: mod_base = OTHER; note = 2'-deoxy-2'-fluoroadenosine
  modified_base 19: mod_base = OTHER; note = cm
tgaaccacatggctatgac

SEQ ID NO: 1073 - RNA, 19 nt, synthetic construct
  source 1..19: mol_type = other RNA
  modified_base 1: mod_base = OTHER; note = 2'-deoxy-2'-fluorouridine
  modified_base 2: mod_base = OTHER; note = 2'-deoxy-2'-fluoroguanosine
  modified_base 3: mod_base = OTHER; note = 2'-O-methyladenosine
  modified_base 4: mod_base = OTHER; note = 2'-deoxy-2'-fluoroadenosine
  modified_base 5: mod_base = OTHER; note = cm
  modified_base 6: mod_base = OTHER; note = 2'-deoxy-2'-fluorocytidine
  modified_base 7: mod_base = OTHER; note = 2'-O-methyladenosine
  modified_base 8: mod_base = OTHER; note = 2'-deoxy-2'-fluorocytidine
  modified_base 9: mod_base = OTHER; note = 2'-O-methyladenosine
  modified_base 10: mod_base = OTHER; note = 2'-deoxy-2'-fluorouridine
  modified_base 11: mod_base = OTHER; note = gm
  modified_base 12: mod_base = OTHER; note = 2'-deoxy-2'-fluoroguanosine
  modified_base 13: mod_base = OTHER; note = cm
  modified_base 14: mod_base = OTHER; note = 2'-deoxy-2'-fluorouridine
  modified_base 15: mod_base = OTHER; note = 2'-O-methyladenosine
  modified_base 16: mod_base = OTHER; note = 2'-deoxy-2'-fluorouridine
  modified_base 17: mod_base = OTHER; note = gm
  modified_base 18: mod_base = OTHER; note = 2'-deoxy-2'-fluoroadenosine
  modified_base 19: mod_base = OTHER; note = cm
tgaaccacatggctatgac

SEQ ID NO: 1074 - RNA, 21 nt, synthetic construct
  source 1..21: mol_type = other RNA
  modified_base 1: mod_base = OTHER; note = 2'-deoxy-2'-fluorocytidine
  modified_base 2: mod_base = OTHER; note = 2'-deoxy-2'-fluoroadenosine
  modified_base 3: mod_base = OTHER; note = 2'-O-methyladenosine
  modified_base 4: mod_base = OTHER; note = 2'-deoxy-2'-fluorocytidine
  modified_base 5: mod_base = OTHER; note = cm
  modified_base 6: mod_base = OTHER; note = 2'-deoxy-2'-fluoroadenosine
  modified_base 7: mod_base = OTHER; note = gm
  modified_base 8: mod_base = OTHER; note = 2'-deoxy-2'-fluorocytidine
  modified_base 9: mod_base = OTHER; note = cm
  modified_base 10: mod_base = OTHER; note = 2'-deoxy-2'-fluoroadenosine
  modified_base 11: mod_base = OTHER; note = gm
  modified_base 12: mod_base = OTHER; note = 2'-deoxy-2'-fluoroguanosine
  modified_base 13: mod_base = OTHER; note = um
  modified_base 14: mod_base = OTHER; note = 2'-deoxy-2'-fluorouridine
  modified_base 15: mod_base = OTHER; note = um
  modified_base 16: mod_base = OTHER; note = 2'-deoxy-2'-fluorouridine
  modified_base 17: mod_base = OTHER; note = gm
  modified_base 18: mod_base = OTHER; note = 2'-deoxy-2'-fluoroguanosine
  modified_base 19: mod_base = OTHER; note = um
  modified_base 20: mod_base = OTHER; note = 2'-deoxy-2'-fluorocytidine
  modified_base 21: mod_base = OTHER; note = cm
caaccagccaggttttggtcc

SEQ ID NO: 1075 - RNA, 21 nt, synthetic construct
  source 1..21: mol_type = other RNA
  modified_base 1: mod_base = OTHER; note = 2'-deoxy-2'-fluorocytidine
  modified_base 2: mod_base = OTHER; note = 2'-deoxy-2'-fluoroadenosine
  modified_base 3: mod_base = OTHER; note = 2'-O-methyladenosine
  modified_base 4: mod_base = OTHER; note = 2'-deoxy-2'-fluorocytidine
  modified_base 5: mod_base = OTHER; note = cm
  modified_base 6: mod_base = OTHER; note = 2'-deoxy-2'-fluoroadenosine
  modified_base 7: mod_base = OTHER; note = gm
  modified_base 8: mod_base = OTHER; note = 2'-deoxy-2'-fluorocytidine
  modified_base 9: mod_base = OTHER; note = cm
  modified_base 10: mod_base = OTHER; note = 2'-deoxy-2'-fluoroadenosine
  modified_base 11: mod_base = OTHER; note = gm
  modified_base 12: mod_base = OTHER; note = 2'-deoxy-2'-fluoroguanosine
  modified_base 13: mod_base = OTHER; note = um
  modified_base 14: mod_base = OTHER; note = 2'-deoxy-2'-fluorouridine
  modified_base 15: mod_base = OTHER; note = um
  modified_base 16: mod_base = OTHER; note = 2'-deoxy-2'-fluorouridine
  modified_base 17: mod_base = OTHER; note = gm
  modified_base 18: mod_base = OTHER; note = 2'-deoxy-2'-fluoroguanosine
  modified_base 19: mod_base = OTHER; note = um
  modified_base 20: mod_base = OTHER; note = 2'-deoxy-2'-fluorocytidine
  modified_base 21: mod_base = OTHER; note = cm
  modified_base 1..3: mod_base = OTHER; note = phosphorothioate bond between nucleotides
  modified_base 20^21: mod_base = OTHER; note = phosphorothioate bond between nucleotides
caaccagccaggttttggtcc

SEQ ID NO: 1076 - RNA, 21 nt, synthetic construct
  source 1..21: mol_type = other RNA
  modified_base 1: mod_base = OTHER; note = 2'-deoxy-2'-fluorocytidine
  modified_base 2: mod_base = OTHER; note = 2'-deoxy-2'-fluoroadenosine
  modified_base 3: mod_base = OTHER; note = 2'-O-methyladenosine
  modified_base 4: mod_base = OTHER; note = 2'-deoxy-2'-fluorocytidine
  modified_base 5: mod_base = OTHER; note = cm
  modified_base 6: mod_base = OTHER; note = 2'-deoxy-2'-fluoroadenosine
  modified_base 7: mod_base = OTHER; note = gm
  modified_base 8: mod_base = OTHER; note = 2'-deoxy-2'-fluorocytidine
  modified_base 9: mod_base = OTHER; note = cm
  modified_base 10: mod_base = OTHER; note = 2'-deoxy-2'-fluoroadenosine
  modified_base 11: mod_base = OTHER; note = gm
  modified_base 12: mod_base = OTHER; note = 2'-deoxy-2'-fluoroguanosine
  modified_base 13: mod_base = OTHER; note = um
  modified_base 14: mod_base = OTHER; note = 2'-deoxy-2'-fluorouridine
  modified_base 15: mod_base = OTHER; note = um
  modified_base 16: mod_base = OTHER; note = 2'-deoxy-2'-fluorouridine
  modified_base 17: mod_base = OTHER; note = gm
  modified_base 18: mod_base = OTHER; note = 2'-deoxy-2'-fluoroguanosine
  modified_base 19: mod_base = OTHER; note = um
  modified_base 20: mod_base = OTHER; note = 2'-deoxy-2'-fluorocytidine
  modified_base 21: mod_base = OTHER; note = cm
  modified_base 1^2: mod_base = OTHER; note = phosphorothioate bond between nucleotides
  modified_base 20^21: mod_base = OTHER; note = phosphorothioate bond between nucleotides
caaccagccaggttttggtcc

SEQ ID NO: 1077 - RNA, 21 nt, synthetic construct
  source 1..21: mol_type = other RNA
  modified_base 1: mod_base = OTHER; note = 2'-deoxy-2'-fluorocytidine
  modified_base 2: mod_base = OTHER; note = 2'-deoxy-2'-fluoroadenosine
  modified_base 3: mod_base = OTHER; note = 2'-O-methyladenosine
  modified_base 4: mod_base = OTHER; note = 2'-deoxy-2'-fluorocytidine
  modified_base 5: mod_base = OTHER; note = cm
  modified_base 6: mod_base = OTHER; note = 2'-deoxy-2'-fluoroadenosine
  modified_base 7: mod_base = OTHER; note = gm
  modified_base 8: mod_base = OTHER; note = 2'-deoxy-2'-fluorocytidine
  modified_base 9: mod_base = OTHER; note = cm
  modified_base 10: mod_base = OTHER; note = 2'-deoxy-2'-fluoroadenosine
  modified_base 11: mod_base = OTHER; note = gm
  modified_base 12: mod_base = OTHER; note = 2'-deoxy-2'-fluoroguanosine
  modified_base 13: mod_base = OTHER; note = um
  modified_base 14: mod_base = OTHER; note = 2'-deoxy-2'-fluorouridine
  modified_base 15: mod_base = OTHER; note = um
  modified_base 16: mod_base = OTHER; note = 2'-deoxy-2'-fluorouridine
  modified_base 17: mod_base = OTHER; note = gm
  modified_base 18: mod_base = OTHER; note = 2'-deoxy-2'-fluoroguanosine
  modified_base 19: mod_base = OTHER; note = um
  modified_base 20: mod_base = OTHER; note = 2'-deoxy-2'-fluorocytidine
  modified_base 21: mod_base = OTHER; note = cm
  modified_base 20^21: mod_base = OTHER; note = phosphorothioate bond between nucleotides
caaccagccaggttttggtcc

SEQ ID NO: 1078 - RNA, 21 nt, synthetic construct
  source 1..21: mol_type = other RNA
  modified_base 1: mod_base = OTHER; note = cm
  modified_base 5: mod_base = OTHER; note = cm
  modified_base 9: mod_base = OTHER; note = cm
  modified_base 20^21: mod_base = OTHER; note = phosphorothioate bond between nucleotides
caaccagccaggttttggtcc

SEQ ID NO: 1079 - RNA, 21 nt, synthetic construct
  source 1..21: mol_type = other RNA
  modified_base 1: mod_base = OTHER; note = 5'-E-vinylphosphonate-2'-O-methyl-cytidine
  modified_base 7: mod_base = OTHER; note = gm
  modified_base 1..3: mod_base = OTHER; note = phosphorothioate bond between nucleotides
  modified_base 19..21: mod_base = OTHER; note = phosphorothioate bond between nucleotides
caaccagccaggttttggtcc

SEQ ID NO: 1080 - RNA, 21 nt, synthetic construct
  source 1..21: mol_type = other RNA
  modified_base 1: mod_base = OTHER; note = 5'-E-vinylphosphonate-2'-O-methyl-cytidine
  modified_base 7: mod_base = OTHER; note = gm
  modified_base 1^2: mod_base = OTHER; note = phosphorothioate bond between nucleotides
  modified_base 20^21: mod_base = OTHER; note = phosphorothioate bond between nucleotides
caaccagccaggttttggtcc

SEQ ID NO: 1081 - RNA, 21 nt, synthetic construct
  source 1..21: mol_type = other RNA
  modified_base 1: mod_base = OTHER; note = 5'-E-vinylphosphonate-2'-O-methyl-cytidine
  modified_base 7: mod_base = OTHER; note = gm
  modified_base 1..3: mod_base = OTHER; note = phosphorothioate bond between nucleotides
  modified_base 19..21: mod_base = OTHER; note = phosphorothioate bond between nucleotides
caaccagccaggttttggtcc

SEQ ID NO: 1082 - RNA, 21 nt, synthetic construct
  source 1..21: mol_type = other RNA
  modified_base 1: mod_base = OTHER; note = 5'-E-vinylphosphonate-2'-O-methyl-cytidine
  modified_base 7: mod_base = OTHER; note = gm
  modified_base 1^2: mod_base = OTHER; note = phosphorothioate bond between nucleotides
  modified_base 20^21: mod_base = OTHER; note = phosphorothioate bond between nucleotides
caaccagccaggttttggtcc

SEQ ID NO: 1083 - RNA, 21 nt, synthetic construct
  source 1..21: mol_type = other RNA
  modified_base 1: mod_base = OTHER; note = 5'-E-vinylphosphonate-2'-O-methyl-cytidine
  modified_base 7: mod_base = OTHER; note = gm
  modified_base 1..3: mod_base = OTHER; note = phosphorothioate bond between nucleotides
  modified_base 19..21: mod_base = OTHER; note = phosphorothioate bond between nucleotides
caaccagccaggttttggtcc

SEQ ID NO: 1084 - RNA, 21 nt, synthetic construct
  source 1..21: mol_type = other RNA
  modified_base 1: mod_base = OTHER; note = 5'-E-vinylphosphonate-2'-O-methyl-cytidine
  modified_base 7: mod_base = OTHER; note = gm
  modified_base 1^2: mod_base = OTHER; note = phosphorothioate bond between nucleotides
  modified_base 20^21: mod_base = OTHER; note = phosphorothioate bond between nucleotides
caaccagccaggttttggtcc

SEQ ID NO: 1085 - RNA, 21 nt, synthetic construct
  source 1..21: mol_type = other RNA
  modified_base 1: mod_base = OTHER; note = 2'-deoxy-2'-fluorocytidine
  modified_base 2: mod_base = OTHER; note = 2'-O-methyladenosine
  modified_base 5: mod_base = OTHER; note = 2'-deoxy-2'-fluorocytidine
  modified_base 9: mod_base = OTHER; note = 2'-deoxy-2'-fluorocytidine
  modified_base 16: mod_base = OTHER; note = um
  modified_base 20^21: mod_base = OTHER; note = phosphorothioate bond between nucleotides
caaccagccaggttttggtcc

SEQ ID NO: 1086 - RNA, 21 nt, synthetic construct
  source 1..21: mol_type = other RNA
  modified_base 2: mod_base = OTHER; note = 2'-O-methyladenosine
  modified_base 4: mod_base = OTHER; note = cm
  modified_base 6: mod_base = OTHER; note = 2'-O-methyladenosine
  modified_base 8: mod_base = OTHER; note = cm
  modified_base 10: mod_base = OTHER; note = 2'-O-methyladenosine
  modified_base 12: mod_base = OTHER; note = gm
  modified_base 14: mod_base = OTHER; note = um
  modified_base 16: mod_base = OTHER; note = um
  modified_base 18: mod_base = OTHER; note = gm
  modified_base 20: mod_base = OTHER; note = cm
  modified_base 20^21: mod_base = OTHER; note = phosphorothioate bond between nucleotides
caaccagccaggttttggtcc

SEQ ID NO: 1087 - RNA, 21 nt, synthetic construct
  source 1..21: mol_type = other RNA
  modified_base 1: mod_base = OTHER; note = 2'-deoxy-2'-fluorocytidine
  modified_base 4: mod_base = OTHER; note = 2'-deoxy-2'-fluorocytidine
  modified_base 5: mod_base = OTHER; note = 2'-deoxy-2'-fluorocytidine
  modified_base 9: mod_base = OTHER; note = 2'-deoxy-2'-fluorocytidine
  modified_base 16: mod_base = OTHER; note = 2'-deoxy-2'-fluorouridine
  modified_base 19: mod_base = OTHER; note = 2'-deoxy-2'-fluorouridine
  modified_base 20^21: mod_base = OTHER; note = phosphorothioate bond between nucleotides
caaccagccaggttttggtcc

SEQ ID NO: 1088 - RNA, 21 nt, synthetic construct
  source 1..21: mol_type = other RNA
  modified_base 2: mod_base = OTHER; note = 2'-O-methyladenosine
  modified_base 3: mod_base = OTHER; note = 2'-O-methyladenosine
  modified_base 6: mod_base = OTHER; note = 2'-O-methyladenosine
  modified_base 17: mod_base = OTHER; note = gm
  modified_base 18: mod_base = OTHER; note = gm
  modified_base 20^21: mod_base = OTHER; note = phosphorothioate bond between nucleotides
caaccagccaggttttggtcc

SEQ ID NO: 1089 - RNA, 21 nt, synthetic construct
  source 1..21: mol_type = other RNA
  modified_base 2: mod_base = OTHER; note = 2'-O-methyladenosine
  modified_base 6: mod_base = OTHER; note = 2'-O-methyladenosine
  modified_base 20^21: mod_base = OTHER; note = phosphorothioate bond between nucleotides
caaccagccaggttttggtcc

SEQ ID NO: 1090 - RNA, 21 nt, synthetic construct
  source 1..21: mol_type = other RNA
  modified_base 1: mod_base = OTHER; note = 2'-deoxy-2'-fluorocytidine
  modified_base 2: mod_base = OTHER; note = 2'-deoxy-2'-fluoroadenosine
  modified_base 4: mod_base = OTHER; note = 2'-deoxy-2'-fluorocytidine
  modified_base 5: mod_base = OTHER; note = 2'-deoxy-2'-fluorocytidine
  modified_base 16: mod_base = OTHER; note = um
  modified_base 2..4: mod_base = OTHER; note = phosphorothioate bond between nucleotides
  modified_base 18..21: mod_base = OTHER; note = phosphorothioate bond between nucleotides
caaccagccaggttttggtcc

SEQ ID NO: 1091 - RNA, 21 nt, synthetic construct
  source 1..21: mol_type = other RNA
  modified_base 1: mod_base = OTHER; note = 2'-deoxy-2'-fluorocytidine
  modified_base 20^21: mod_base = OTHER; note = phosphorothioate bond between nucleotides
caaccagccaggttttggtcc

SEQ ID NO: 1092 - RNA, 21 nt, synthetic construct
  source 1..21: mol_type = other RNA
  modified_base 1: mod_base = OTHER; note = 5'-E-vinylphosphonate-2'-O-methyl-cytidine
  modified_base 8: mod_base = m5c
  modified_base 9: mod_base = m5c
  modified_base 20^21: mod_base = OTHER; note = phosphorothioate bond between nucleotides
caaccagccaggttttggtcc

SEQ ID NO: 1093 - RNA, 21 nt, synthetic construct
  source 1..21: mol_type = other RNA
  modified_base 1: mod_base = OTHER; note = 5'-E-vinylphosphonate-2'-O-methyl-cytidine
  modified_base 4: mod_base = m5c
  modified_base 5: mod_base = m5c
  modified_base 20^21: mod_base = OTHER; note = phosphorothioate bond between nucleotides
caaccagccaggttttggtcc

SEQ ID NO: 1094 - RNA, 21 nt, synthetic construct
  source 1..21: mol_type = other RNA
  modified_base 1: mod_base = OTHER; note = 5'-E-vinylphosphonate-2'-O-methyl-cytidine
  modified_base 13: mod_base = OTHER; note = m5u
  modified_base 15: mod_base = OTHER; note = m5u
  modified_base 16: mod_base = OTHER; note = m5u
  modified_base 19: mod_base = OTHER; note = m5u
  modified_base 20: mod_base = m5c
  modified_base 21: mod_base = m5c
  modified_base 20^21: mod_base = OTHER; note = phosphorothioate bond between nucleotides
caaccagccaggttttggtcc

SEQ ID NO: 1095 - RNA, 19 nt, synthetic construct
  source 1..19: mol_type = other RNA
  modified_base 1: mod_base = OTHER; note = 2'-deoxy-2'-fluorouridine
  modified_base 2: mod_base = OTHER; note = 2'-deoxy-2'-fluoroguanosine
  modified_base 3: mod_base = OTHER; note = 2'-O-methyladenosine
  modified_base 4: mod_base = OTHER; note = 2'-deoxy-2'-fluoroadenosine
  modified_base 5: mod_base = OTHER; note = cm
  modified_base 6: mod_base = OTHER; note = 2'-deoxy-2'-fluorocytidine
  modified_base 7: mod_base = OTHER; note = 2'-O-methyladenosine
  modified_base 8: mod_base = OTHER; note = 2'-deoxy-2'-fluorocytidine
  modified_base 9: mod_base = OTHER; note = 2'-O-methyladenosine
  modified_base 10: mod_base = OTHER; note = 2'-deoxy-2'-fluorouridine
  modified_base 11: mod_base = OTHER; note = gm
  modified_base 12: mod_base = OTHER; note = 2'-deoxy-2'-fluoroguanosine
  modified_base 13: mod_base = OTHER; note = cm
  modified_base 14: mod_base = OTHER; note = 2'-deoxy-2'-fluorouridine
  modified_base 15: mod_base = OTHER; note = 2'-O-methyladenosine
  modified_base 16: mod_base = OTHER; note = 2'-deoxy-2'-fluorouridine
  modified_base 17: mod_base = OTHER; note = gm
  modified_base 18: mod_base = OTHER; note = 2'-deoxy-2'-fluoroadenosine
  modified_base 19: mod_base = OTHER; note = cm
tgaaccacatggctatgac

SEQ ID NO: 1096 - RNA, 19 nt, synthetic construct
  source 1..19: mol_type = other RNA
  modified_base 1: mod_base = OTHER; note = 2'-deoxy-2'-fluorouridine
  modified_base 2: mod_base = OTHER; note = 2'-deoxy-2'-fluoroguanosine
  modified_base 3: mod_base = OTHER; note = um
  modified_base 4: mod_base = OTHER; note = 2'-deoxy-2'-fluorocytidine
  modified_base 5: mod_base = OTHER; note = um
  modified_base 6: mod_base = OTHER; note = 2'-deoxy-2'-fluorouridine
  modified_base 7: mod_base = OTHER; note = um
  modified_base 8: mod_base = OTHER; note = 2'-deoxy-2'-fluorocytidine
  modified_base 9: mod_base = OTHER; note = cm
  modified_base 10: mod_base = OTHER; note = 2'-deoxy-2'-fluorouridine
  modified_base 11: mod_base = OTHER; note = gm
  modified_base 12: mod_base = OTHER; note = 2'-deoxy-2'-fluorocytidine
  modified_base 13: mod_base = OTHER; note = 2'-O-methyladenosine
  modified_base 14: mod_base = OTHER; note = 2'-deoxy-2'-fluorocytidine
  modified_base 15: mod_base = OTHER; note = um
  modified_base 16: mod_base = OTHER; note = 2'-deoxy-2'-fluoroguanosine
  modified_base 17: mod_base = OTHER; note = cm
  modified_base 18: mod_base = OTHER; note = 2'-deoxy-2'-fluoroadenosine
  modified_base 19: mod_base = OTHER; note = gm
tgtctttcctgcactgcag

SEQ ID NO: 1097 - RNA, 19 nt, synthetic construct
  source 1..19: mol_type = other RNA
  modified_base 1: mod_base = OTHER; note = 2'-deoxy-2'-fluorouridine
  modified_base 2: mod_base = OTHER; note = 2'-deoxy-2'-fluoroguanosine
  modified_base 3: mod_base = OTHER; note = 2'-O-methyladenosine
  modified_base 4: mod_base = OTHER; note = 2'-deoxy-2'-fluoroadenosine
  modified_base 5: mod_base = OTHER; note = cm
  modified_base 6: mod_base = OTHER; note = 2'-deoxy-2'-fluorocytidine
  modified_base 7: mod_base = OTHER; note = 2'-O-methyladenosine
  modified_base 8: mod_base = OTHER; note = 2'-deoxy-2'-fluorocytidine
  modified_base 9: mod_base = OTHER; note = 2'-O-methyladenosine
  modified_base 10: mod_base = OTHER; note = 2'-deoxy-2'-fluorouridine
  modified_base 11: mod_base = OTHER; note = gm
  modified_base 12: mod_base = OTHER; note = 2'-deoxy-2'-fluoroguanosine
  modified_base 13: mod_base = OTHER; note = cm
  modified_base 14: mod_base = OTHER; note = 2'-deoxy-2'-fluorouridine
  modified_base 15: mod_base = OTHER; note = 2'-O-methyladenosine
  modified_base 16: mod_base = OTHER; note = 2'-deoxy-2'-fluorouridine
  modified_base 17: mod_base = OTHER; note = gm
  modified_base 18: mod_base = OTHER; note = 2'-deoxy-2'-fluoroadenosine
  modified_base 19: mod_base = OTHER; note = cm
tgaaccacatggctatgac

SEQ ID NO: 1098 - RNA, 19 nt, synthetic construct
  source 1..19: mol_type = other RNA
  modified_base 1: mod_base = OTHER; note = cm
  modified_base 2: mod_base = OTHER; note = gm
  modified_base 3: mod_base = OTHER; note = 2'-deoxy-2'-fluoroguanosine
  modified_base 4: mod_base = OTHER; note = 2'-O-methyladenosine
  modified_base 5: mod_base = OTHER; note = 2'-deoxy-2'-fluoroadenosine
  modified_base 6: mod_base = OTHER; note = um
  modified_base 7: mod_base = OTHER; note = 2'-deoxy-2'-fluorouridine
  modified_base 8: mod_base = OTHER; note = 2'-O-methyladenosine
  modified_base 9: mod_base = OTHER; note = 2'-deoxy-2'-fluoroguanosine
  modified_base 10: mod_base = OTHER; note = um
  modified_base 11: mod_base = OTHER; note = 2'-deoxy-2'-fluoroguanosine
  modified_base 12: mod_base = OTHER; note = 2'-O-methyladenosine
  modified_base 13: mod_base = OTHER; note = 2'-deoxy-2'-fluorocytidine
  modified_base 14: mod_base = OTHER; note = um
  modified_base 15: mod_base = OTHER; note = 2'-deoxy-2'-fluoroguanosine
  modified_base 16: mod_base = OTHER; note = gm
  modified_base 17: mod_base = OTHER; note = 2'-deoxy-2'-fluoroadenosine
  modified_base 18: mod_base = OTHER; note = um
  modified_base 19: mod_base = OTHER; note = 2'-deoxy-2'-fluorocytidine
cggaattagtgactggatc

SEQ ID NO: 1099 - RNA, 19 nt, synthetic construct
  source 1..19: mol_type = other RNA
  modified_base 1: mod_base = OTHER; note = cm
  modified_base 2: mod_base = OTHER; note = gm
  modified_base 3: mod_base = OTHER; note = 2'-deoxy-2'-fluoroguanosine
  modified_base 4: mod_base = OTHER; note = 2'-O-methyladenosine
  modified_base 5: mod_base = OTHER; note = 2'-deoxy-2'-fluoroadenosine
  modified_base 6: mod_base = OTHER; note = um
  modified_base 7: mod_base = OTHER; note = 2'-deoxy-2'-fluorouridine
  modified_base 8: mod_base = OTHER; note = 2'-O-methyladenosine
  modified_base 9: mod_base = OTHER; note = 2'-deoxy-2'-fluoroguanosine
  modified_base 10: mod_base = OTHER; note = um
  modified_base 11: mod_base = OTHER; note = 2'-deoxy-2'-fluoroguanosine
  modified_base 12: mod_base = OTHER; note = 2'-O-methyladenosine
  modified_base 13: mod_base = OTHER; note = 2'-deoxy-2'-fluorocytidine
  modified_base 14: mod_base = OTHER; note = um
  modified_base 15: mod_base = OTHER; note = 2'-deoxy-2'-fluoroguanosine
  modified_base 16: mod_base = OTHER; note = gm
  modified_base 17: mod_base = OTHER; note = 2'-deoxy-2'-fluoroadenosine
  modified_base 18: mod_base = OTHER; note = um
  modified_base 19: mod_base = OTHER; note = 2'-deoxy-2'-fluorocytidine
  modified_base 1..3: mod_base = OTHER; note = phosphorothioate bond between nucleotides
cggaattagtgactggatc

SEQ ID NO: 1100 - RNA, 19 nt, synthetic construct
  source 1..19: mol_type = other RNA
  modified_base 1: mod_base = OTHER; note = cm
  modified_base 2: mod_base = OTHER; note = gm
  modified_base 3: mod_base = OTHER; note = 2'-deoxy-2'-fluoroguanosine
  modified_base 4: mod_base = OTHER; note = 2'-O-methyladenosine
  modified_base 5: mod_base = OTHER; note = 2'-deoxy-2'-fluoroadenosine
  modified_base 6: mod_base = OTHER; note = um
  modified_base 7: mod_base = OTHER; note = 2'-deoxy-2'-fluorouridine
  modified_base 8: mod_base = OTHER; note = 2'-O-methyladenosine
  modified_base 9: mod_base = OTHER; note = 2'-deoxy-2'-fluoroguanosine
  modified_base 10: mod_base = OTHER; note = um
  modified_base 11: mod_base = OTHER; note = 2'-deoxy-2'-fluoroguanosine
  modified_base 12: mod_base = OTHER; note = 2'-O-methyladenosine
  modified_base 13: mod_base = OTHER; note = 2'-deoxy-2'-fluorocytidine
  modified_base 14: mod_base = OTHER; note = um
  modified_base 15: mod_base = OTHER; note = 2'-deoxy-2'-fluoroguanosine
  modified_base 16: mod_base = OTHER; note = gm
  modified_base 17: mod_base = OTHER; note = 2'-deoxy-2'-fluoroadenosine
  modified_base 18: mod_base = OTHER; note = um
  modified_base 19: mod_base = OTHER; note = 2'-deoxy-2'-fluorocytidine
  modified_base 1^2: mod_base = OTHER; note = phosphorothioate bond between nucleotides
cggaattagtgactggatc

SEQ ID NO: 1101 - RNA, 19 nt, synthetic construct
  source 1..19: mol_type = other RNA
  modified_base 1: mod_base = OTHER; note = cm
  modified_base 6: mod_base = OTHER; note = um
  modified_base 7: mod_base = OTHER; note = um
  modified_base 10: mod_base = OTHER; note = um
  modified_base 13: mod_base = OTHER; note = cm
  modified_base 14: mod_base = OTHER; note = um
  modified_base 18: mod_base = OTHER; note = um
  modified_base 19: mod_base = OTHER; note = cm
  modified_base 1^2: mod_base = OTHER; note = phosphorothioate bond between nucleotides
cggaattagtgactggatc

SEQ ID NO: 1102 - RNA, 19 nt, synthetic construct
  source 1..19: mol_type = other RNA
  modified_base 1: mod_base = OTHER; note = cm
  modified_base 6: mod_base = OTHER; note = um
  modified_base 7: mod_base = OTHER; note = um
  modified_base 10: mod_base = OTHER; note = um
  modified_base 13: mod_base = OTHER; note = cm
  modified_base 14: mod_base = OTHER; note = 2'-deoxy-2'-fluorouridine
  modified_base 18: mod_base = OTHER; note = um
  modified_base 19: mod_base = OTHER; note = cm
  modified_base 1^2: mod_base = OTHER; note = phosphorothioate bond between nucleotides
cggaattagtgactggatc

SEQ ID NO: 1103 - RNA, 19 nt, synthetic construct
  source 1..19: mol_type = other RNA
  modified_base 1: mod_base = OTHER; note = cm
  modified_base 6: mod_base = OTHER; note = um
  modified_base 7: mod_base = OTHER; note = um
  modified_base 10: mod_base = OTHER; note = um
  modified_base 13: mod_base = OTHER; note = cm
  modified_base 14: mod_base = OTHER; note = um
  modified_base 18: mod_base = OTHER; note = um
  modified_base 19: mod_base = OTHER; note = cm
  modified_base 1^2: mod_base = OTHER; note = phosphorothioate bond between nucleotides
cggaattagtgactggatc

SEQ ID NO: 1104 - RNA, 19 nt, synthetic construct
  source 1..19: mol_type = other RNA
  modified_base 1: mod_base = OTHER; note = Unlocked nucleic acid (UNA) monomer
  modified_base 6: mod_base = OTHER; note = um
  modified_base 7: mod_base = OTHER; note = um
  modified_base 10: mod_base = OTHER; note = um
  modified_base 13: mod_base = OTHER; note = cm
  modified_base 14: mod_base = OTHER; note = um
  modified_base 18: mod_base = OTHER; note = um
  modified_base 19: mod_base = OTHER; note = cm
  modified_base 1^2: mod_base = OTHER; note = phosphorothioate bond between nucleotides
cggaattagtgactggatc

SEQ ID NO: 1105 - RNA, 19 nt, synthetic construct
  source 1..19: mol_type = other RNA
  modified_base 1: mod_base = OTHER; note = Unlocked nucleic acid (UNA) monomer
  modified_base 6: mod_base = OTHER; note = um
  modified_base 7: mod_base = OTHER; note = um
  modified_base 10: mod_base = OTHER; note = um
  modified_base 13: mod_base = OTHER; note = cm
  modified_base 14: mod_base = OTHER; note = um
  modified_base 18: mod_base = OTHER; note = um
  modified_base 19: mod_base = OTHER; note = cm
  modified_base 1^2: mod_base = OTHER; note = phosphorothioate bond between nucleotides
cggaattagtgactggatc

SEQ ID NO: 1106 - RNA, 19 nt, synthetic construct
  source 1..19: mol_type = other RNA
  modified_base 1: mod_base = OTHER; note = 5'-O-methyl modified 2'-deoxycytidine
  modified_base 6: mod_base = OTHER; note = um
  modified_base 7: mod_base = OTHER; note = um
  modified_base 10: mod_base = OTHER; note = um
  modified_base 13: mod_base = OTHER; note = cm
  modified_base 14: mod_base = OTHER; note = um
  modified_base 18: mod_base = OTHER; note = um
  modified_base 19: mod_base = OTHER; note = cm
  modified_base 1^2: mod_base = OTHER; note = phosphorothioate bond between nucleotides
cggaattagtgactggatc

SEQ ID NO: 1107 - RNA, 19 nt, synthetic construct
  source 1..19: mol_type = other RNA
  modified_base 1: mod_base = OTHER; note = 5'-O-methyl modified 2'-deoxycytidine
  modified_base 6: mod_base = OTHER; note = um
  modified_base 7: mod_base = OTHER; note = um
  modified_base 10: mod_base = OTHER; note = um
  modified_base 13: mod_base = OTHER; note = cm
  modified_base 14: mod_base = OTHER; note = um
  modified_base 18: mod_base = OTHER; note = um
  modified_base 19: mod_base = OTHER; note = cm
  modified_base 1^2: mod_base = OTHER; note = phosphorothioate bond between nucleotides
cggaattagtgactggatc

SEQ ID NO: 1108 - RNA, 19 nt, synthetic construct
  source 1..19: mol_type = other RNA
  modified_base 1: mod_base = OTHER; note = 2'-deoxy-2'-fluorocytidine
  modified_base 2: mod_base = OTHER; note = gm
  modified_base 3: mod_base = OTHER; note = 2'-deoxy-2'-fluoroguanosine
  modified_base 4: mod_base = OTHER; note = 2'-O-methyladenosine
  modified_base 5: mod_base = OTHER; note = 2'-deoxy-2'-fluoroadenosine
  modified_base 6: mod_base = OTHER; note = um
  modified_base 7: mod_base = OTHER; note = 2'-deoxy-2'-fluorouridine
  modified_base 8: mod_base = OTHER; note = 2'-O-methyladenosine
  modified_base 1^2: mod_base = OTHER; note = phosphorothioate bond between nucleotides
cggaattagtgactggatc

SEQ ID NO: 1109 - RNA, 19 nt, synthetic construct
  source 1..19: mol_type = other RNA
  modified_base 1: mod_base = OTHER; note = cm
  modified_base 3: mod_base = OTHER; note = gm
  modified_base 5: mod_base = OTHER; note = 2'-O-methyladenosine
  modified_base 7: mod_base = OTHER; note = um
  modified_base 9: mod_base = OTHER; note = gm
  modified_base 11: mod_base = OTHER; note = gm
  modified_base 13: mod_base = OTHER; note = cm
  modified_base 15: mod_base = OTHER; note = gm
  modified_base 17: mod_base = OTHER; note = um
  modified_base 19: mod_base = OTHER; note = 2'-deoxy-2'-fluorocytidine
  modified_base 1^2: mod_base = OTHER; note = phosphorothioate bond between nucleotides
cggaattagtgactggttc

SEQ ID NO: 1110 - RNA, 19 nt, synthetic construct
  source 1..19: mol_type = other RNA
  modified_base 3: mod_base = OTHER; note = 2'-deoxy-2'-fluoroguanosine
  modified_base 5: mod_base = OTHER; note = 2'-deoxy-2'-fluoroadenosine
  modified_base 7: mod_base = OTHER; note = 2'-deoxy-2'-fluorouridine
  modified_base 9: mod_base = OTHER; note = 2'-deoxy-2'-fluoroguanosine
  modified_base 11: mod_base = OTHER; note = 2'-deoxy-2'-fluoroguanosine
  modified_base 13: mod_base = OTHER; note = 2'-deoxy-2'-fluorocytidine
  modified_base 15: mod_base = OTHER; note = 2'-deoxy-2'-fluoroguanosine
  modified_base 17: mod_base = OTHER; note = 2'-deoxy-2'-fluorouridine
  modified_base 19: mod_base = OTHER; note = 2'-deoxy-2'-fluorocytidine
  modified_base 1^2: mod_base = OTHER; note = phosphorothioate bond between nucleotides
cggaattagtgactggttc

SEQ ID NO: 1111 - RNA, 21 nt, synthetic construct
  source 1..21: mol_type = other RNA
  modified_base 1: mod_base = OTHER; note = abasic site of inverted abasic deoxyribose
  modified_base 2: mod_base = OTHER; note = 2'-deoxy-2'-fluorocytidine
  modified_base 7: mod_base = OTHER; note = 2'-deoxy-2'-fluorouridine
  modified_base 8: mod_base = OTHER; note = 2'-deoxy-2'-fluorouridine
  modified_base 15: mod_base = OTHER; note = 2'-deoxy-2'-fluorouridine
  modified_base 19: mod_base = OTHER; note = 2'-deoxy-2'-fluorouridine
  modified_base 20: mod_base = OTHER; note = 2'-deoxy-2'-fluorocytidine
  modified_base 21: mod_base = OTHER; note = abasic site of inverted abasic deoxyribose
  modified_base 2^3: mod_base = OTHER; note = phosphorothioate bond between nucleotides
ncggaattagtgactggatcn

SEQ ID NO: 1112 - RNA, 19 nt, synthetic construct
  source 1..19: mol_type = other RNA
  modified_base 2: mod_base = OTHER; note = gm
  modified_base 3: mod_base = OTHER; note = gm
  modified_base 4: mod_base = OTHER; note = 2'-O-methyladenosine
  modified_base 5: mod_base = OTHER; note = 2'-O-methyladenosine
  modified_base 8: mod_base = OTHER; note = 2'-O-methyladenosine
  modified_base 11: mod_base = OTHER; note = gm
  modified_base 12: mod_base = OTHER; note = 2'-O-methyladenosine
  modified_base 15: mod_base = OTHER; note = gm
  modified_base 16: mod_base = OTHER; note = gm
  modified_base 17: mod_base = OTHER; note = 2'-O-methyladenosine
  modified_base 1^2: mod_base = OTHER; note = phosphorothioate bond between nucleotides
cggaattagtgactggatc

SEQ ID NO: 1113 - RNA, 19 nt, synthetic construct
  source 1..19: mol_type = other RNA
  modified_base 1: mod_base = OTHER; note = cm
  modified_base 6: mod_base = OTHER; note = um
  modified_base 7: mod_base = OTHER; note = um
  modified_base 10: mod_base = OTHER; note = um
  modified_base 13: mod_base = OTHER; note = cm
  modified_base 19: mod_base = OTHER; note = cm
  modified_base 1^2: mod_base = OTHER; note = phosphorothioate bond between nucleotides
cggaattagtgactggatc

SEQ ID NO: 1114 - DNA, 19 bp, synthetic construct
  source 1..19: mol_type = other DNA
  misc_feature 1..5: note = DNA
  misc_feature 6..13: note = RNA
  misc_feature 14..19: note = DNA
  modified_base 6: mod_base = OTHER; note = 2'-deoxy-2'-fluorouridine
  modified_base 7: mod_base = OTHER; note = 2'-deoxy-2'-fluorouridine
  modified_base 8: mod_base = OTHER; note = 2'-deoxy-2'-fluoroadenosine
  modified_base 9: mod_base = OTHER; note = 2'-deoxy-2'-fluoroguanosine
  modified_base 10: mod_base = OTHER; note = 2'-deoxy-2'-fluorouridine
  modified_base 11: mod_base = OTHER; note = 2'-deoxy-2'-fluoroguanosine
  modified_base 12: mod_base = OTHER; note = 2'-deoxy-2'-fluoroadenosine
  modified_base 14: mod_base = i
  modified_base 18: mod_base = i
  modified_base 1^2: mod_base = OTHER; note = phosphorothioate bond between nucleotides
cggaattagtgacnggant

SEQ ID NO: 1115 - RNA, 19 nt, synthetic construct
  source 1..19: mol_type = other RNA
  modified_base 1: mod_base = OTHER; note = cm
  modified_base 6: mod_base = OTHER; note = um
  modified_base 7: mod_base = OTHER; note = um
  modified_base 10: mod_base = OTHER; note = um
  modified_base 13: mod_base = OTHER; note = cm
  modified_base 14: mod_base = OTHER; note = um
  modified_base 18: mod_base = OTHER; note = um
  modified_base 19: mod_base = OTHER; note = cm
  modified_base 1^2: mod_base = OTHER; note = phosphorothioate bond between nucleotides
cggaattagtgactggatc

SEQ ID NO: 1116 - RNA, 19 nt, synthetic construct
  source 1..19: mol_type = other RNA
  modified_base 1: mod_base = OTHER; note = cm
  modified_base 6: mod_base = OTHER; note = um
  modified_base 7: mod_base = OTHER; note = um
  modified_base 10: mod_base = OTHER; note = um
  modified_base 13: mod_base = OTHER; note = cm
  modified_base 14: mod_base = OTHER; note = um
  modified_base 18: mod_base = OTHER; note = um
  modified_base 19: mod_base = OTHER; note = cm
  modified_base 1^2: mod_base = OTHER; note = phosphorothioate bond between nucleotides
cggaattagtgactggatc

SEQ ID NO: 1117 - RNA, 19 nt, synthetic construct
  source 1..19: mol_type = other RNA
  modified_base 1: mod_base = OTHER; note = gm
  modified_base 2: mod_base = OTHER; note = um
  modified_base 3: mod_base = OTHER; note = 2'-deoxy-2'-fluoroguanosine
  modified_base 4: mod_base = OTHER; note = cm
  modified_base 5: mod_base = OTHER; note = 2'-deoxy-2'-fluorocytidine
  modified_base 6: mod_base = OTHER; note = 2'-O-methyladenosine
  modified_base 7: mod_base = OTHER; note = 2'-deoxy-2'-fluoroadenosine
  modified_base 8: mod_base = OTHER; note = 2'-O-methyladenosine
  modified_base 9: mod_base = OTHER; note = 2'-deoxy-2'-fluoroadenosine
  modified_base 10: mod_base = OTHER; note = um
  modified_base 11: mod_base = OTHER; note = 2'-deoxy-2'-fluorocytidine
  modified_base 12: mod_base = OTHER; note = um
  modified_base 13: mod_base = OTHER; note = 2'-deoxy-2'-fluorocytidine
  modified_base 14: mod_base = OTHER; note = um
  modified_base 15: mod_base = OTHER; note = 2'-deoxy-2'-fluorocytidine
  modified_base 16: mod_base = OTHER; note = um
  modified_base 17: mod_base = OTHER; note = 2'-deoxy-2'-fluoroguanosine
  modified_base 18: mod_base = OTHER; note = gm
  modified_base 19: mod_base = OTHER; note = 2'-deoxy-2'-fluoroadenosine
gtgccaaaatctctctgga

SEQ ID NO: 1118 - RNA, 19 nt, synthetic construct
  source 1..19: mol_type = other RNA
  modified_base 1: mod_base = OTHER; note = gm
  modified_base 2: mod_base = OTHER; note = um
  modified_base 3: mod_base = OTHER; note = 2'-deoxy-2'-fluoroguanosine
  modified_base 4: mod_base = OTHER; note = cm
  modified_base 5: mod_base = OTHER; note = 2'-deoxy-2'-fluorocytidine
  modified_base 6: mod_base = OTHER; note = 2'-O-methyladenosine
  modified_base 7: mod_base = OTHER; note = 2'-deoxy-2'-fluoroadenosine
  modified_base 8: mod_base = OTHER; note = 2'-O-methyladenosine
  modified_base 9: mod_base = OTHER; note = 2'-deoxy-2'-fluoroadenosine
  modified_base 10: mod_base = OTHER; note = um
  modified_base 11: mod_base = OTHER; note = 2'-deoxy-2'-fluorocytidine
  modified_base 12: mod_base = OTHER; note = um
  modified_base 13: mod_base = OTHER; note = 2'-deoxy-2'-fluorocytidine
  modified_base 14: mod_base = OTHER; note = um
  modified_base 15: mod_base = OTHER; note = 2'-deoxy-2'-fluorocytidine
  modified_base 16: mod_base = OTHER; note = um
  modified_base 17: mod_base = OTHER; note = 2'-deoxy-2'-fluoroguanosine
  modified_base 18: mod_base = OTHER; note = gm
  modified_base 19: mod_base = OTHER; note = 2'-deoxy-2'-fluoroadenosine
  modified_base 1^2: mod_base = OTHER; note = phosphorothioate bond between nucleotides
gtgccaaaatctctctgga

SEQ ID NO: 1119 - RNA, 19 nt, synthetic construct
  source 1..19: mol_type = other RNA
  modified_base 1: mod_base = OTHER; note = gm
  modified_base 2: mod_base = OTHER; note = um
  modified_base 3: mod_base = OTHER; note = 2'-deoxy-2'-fluoroguanosine
  modified_base 4: mod_base = OTHER; note = cm
  modified_base 5: mod_base = OTHER; note = 2'-deoxy-2'-fluorocytidine
  modified_base 6: mod_base = OTHER; note = 2'-O-methyladenosine
  modified_base 7: mod_base = OTHER; note = 2'-deoxy-2'-fluoroadenosine
  modified_base 8: mod_base = OTHER; note = 2'-O-methyladenosine
  modified_base 9: mod_base = OTHER; note = 2'-deoxy-2'-fluoroadenosine
  modified_base 10: mod_base = OTHER; note = um
  modified_base 11: mod_base = OTHER; note = 2'-deoxy-2'-fluorocytidine
  modified_base 12: mod_base = OTHER; note = um
  modified_base 13: mod_base = OTHER; note = 2'-deoxy-2'-fluorocytidine
  modified_base 14: mod_base = OTHER; note = um
  modified_base 15: mod_base = OTHER; note = 2'-deoxy-2'-fluorocytidine
  modified_base 16: mod_base = OTHER; note = um
  modified_base 17: mod_base = OTHER; note = 2'-deoxy-2'-fluoroguanosine
  modified_base 18: mod_base = OTHER; note = gm
  modified_base 19: mod_base = OTHER; note = 2'-deoxy-2'-fluoroadenosine
  modified_base 1^2: mod_base = OTHER; note = phosphorothioate bond between nucleotides
gtgccaaaatctctctgga

SEQ ID NO: 1120 - RNA, 19 nt, synthetic construct
  source 1..19: mol_type = other RNA
  modified_base 1: mod_base = OTHER; note = gm
  modified_base 2: mod_base = OTHER; note = um
  modified_base 3: mod_base = OTHER; note = 2'-deoxy-2'-fluoroguanosine
  modified_base 4: mod_base = OTHER; note = cm
  modified_base 5: mod_base = OTHER; note = 2'-deoxy-2'-fluorocytidine
  modified_base 6: mod_base = OTHER; note = 2'-O-methyladenosine
  modified_base 7: mod_base = OTHER; note = 2'-deoxy-2'-fluoroadenosine
  modified_base 8: mod_base = OTHER; note = 2'-O-methyladenosine
  modified_base 9: mod_base = OTHER; note = 2'-deoxy-2'-fluoroadenosine
  modified_base 10: mod_base = OTHER; note = um
  modified_base 11: mod_base = OTHER; note = 2'-deoxy-2'-fluorocytidine
  modified_base 12: mod_base = OTHER; note = um
  modified_base 13: mod_base = OTHER; note = 2'-deoxy-2'-fluorocytidine
  modified_base 14: mod_base = OTHER; note = um
  modified_base 15: mod_base = OTHER; note = 2'-deoxy-2'-fluorocytidine
  modified_base 16: mod_base = OTHER; note = um
  modified_base 17: mod_base = OTHER; note = 2'-deoxy-2'-fluoroguanosine
  modified_base 18: mod_base = OTHER; note = gm
  modified_base 19: mod_base = OTHER; note = 2'-deoxy-2'-fluoroadenosine
  modified_base 1^2: mod_base = OTHER; note = phosphorothioate bond between nucleotides
gtgccaaaatctctctgga

SEQ ID NO: 1121 - RNA, 19 nt, synthetic construct
  source 1..19: mol_type = other RNA
  modified_base 1: mod_base = OTHER; note = gm
  modified_base 2: mod_base = OTHER; note = um
  modified_base 4: mod_base = OTHER; note = cm
  modified_base 5: mod_base = OTHER; note = cm
  modified_base 10: mod_base = OTHER; note = um
  modified_base 11: mod_base = OTHER; note = cm
  modified_base 12: mod_base = OTHER; note = um
  modified_base 13: mod_base = OTHER; note = cm
  modified_base 14: mod_base = OTHER; note = um
  modified_base 15: mod_base = OTHER; note = cm
  modified_base 16: mod_base = OTHER; note = um
  modified_base 1^2: mod_base = OTHER; note = phosphorothioate bond between nucleotides
gtgccaaaatctctctgga

SEQ ID NO: 1122 - RNA, 19 nt, synthetic construct
  source 1..19: mol_type = other RNA
  modified_base 1: mod_base = OTHER; note = gm
  modified_base 2: mod_base = OTHER; note = um
  modified_base 4: mod_base = OTHER; note = cm
  modified_base 5: mod_base = OTHER; note = cm
  modified_base 10: mod_base = OTHER; note = um
  modified_base 11: mod_base = OTHER; note = cm
  modified_base 12: mod_base = OTHER; note = um
  modified_base 13: mod_base = OTHER; note = cm
  modified_base 14: mod_base = OTHER; note = um
  modified_base 15: mod_base = OTHER; note = cm
  modified_base 16: mod_base = OTHER; note = um
  modified_base 1^2: mod_base = OTHER; note = phosphorothioate bond between nucleotides
gtgccaaaatctctctgga

SEQ ID NO: 1123 - RNA, 19 nt, synthetic construct
  source 1..19: mol_type = other RNA
  modified_base 1: mod_base = OTHER; note = gm
  modified_base 2: mod_base = OTHER; note = um
  modified_base 4: mod_base = OTHER; note = cm
  modified_base 5: mod_base = OTHER; note = cm
  modified_base 10: mod_base = OTHER; note = um
  modified_base 11: mod_base = OTHER; note = cm
  modified_base 12: mod_base = OTHER; note = um
  modified_base 13: mod_base = OTHER; note = cm
  modified_base 14: mod_base = OTHER; note = um
  modified_base 15: mod_base = OTHER; note = cm
  modified_base 16: mod_base = OTHER; note = um
  modified_base 1^2: mod_base = OTHER; note = phosphorothioate bond between nucleotides
gtgccaaaatctctctgga

SEQ ID NO: 1124 - RNA, 19 nt, synthetic construct
  source 1..19: mol_type = other RNA
  modified_base 1: mod_base = OTHER; note = Unlocked nucleic acid (UNA) monomer
  modified_base 2: mod_base = OTHER; note = um
  modified_base 4: mod_base = OTHER; note = cm
  modified_base 5: mod_base = OTHER; note = cm
  modified_base 10: mod_base = OTHER; note = um
  modified_base 11: mod_base = OTHER; note = cm
  modified_base 12: mod_base = OTHER; note = um
  modified_base 13: mod_base = OTHER; note = cm
  modified_base 14: mod_base = OTHER; note = um
  modified_base 15: mod_base = OTHER; note = cm
  modified_base 16: mod_base = OTHER; note = um
  modified_base 1^2: mod_base = OTHER; note = phosphorothioate bond between nucleotides
gtgccaaaatctctctgga

SEQ ID NO: 1125 - RNA, 19 nt, synthetic construct
  source 1..19: mol_type = other RNA
  modified_base 1: mod_base = OTHER; note = Unlocked nucleic acid (UNA) monomer
  modified_base 2: mod_base = OTHER; note = um
  modified_base 4: mod_base = OTHER; note = cm
  modified_base 5: mod_base = OTHER; note = cm
  modified_base 10: mod_base = OTHER; note = um
  modified_base 11: mod_base = OTHER; note = cm
  modified_base 12: mod_base = OTHER; note = um
  modified_base 13: mod_base = OTHER; note = cm
  modified_base 14: mod_base = OTHER; note = um
  modified_base 15: mod_base = OTHER; note = cm
  modified_base 16: mod_base = OTHER; note = um
  modified_base 1^2: mod_base = OTHER; note = phosphorothioate bond between nucleotides
gtgccaaaatctctctgga

SEQ ID NO: 1126 - RNA, 19 nt, synthetic construct
  source 1..19: mol_type = other RNA
  modified_base 1: mod_base = OTHER; note = 5'-O-methyl modified 2'-deoxyguanosine
  modified_base 2: mod_base = OTHER; note = um
  modified_base 4: mod_base = OTHER; note = cm
  modified_base 5: mod_base = OTHER; note = cm
  modified_base 10: mod_base = OTHER; note = um
  modified_base 11: mod_base = OTHER; note = cm
  modified_base 12: mod_base = OTHER; note = um
  modified_base 13: mod_base = OTHER; note = cm
  modified_base 14: mod_base = OTHER; note = um
  modified_base 15: mod_base = OTHER; note = cm
  modified_base 16: mod_base = OTHER; note = um
  modified_base 1^2: mod_base = OTHER; note = phosphorothioate bond between nucleotides
gtgccaaaatctctctgga

SEQ ID NO: 1127 - RNA, 19 nt, synthetic construct
  source 1..19: mol_type = other RNA
  modified_base 1: mod_base = OTHER; note = 5'-O-methyl modified 2'-deoxyguanosine
  modified_base 2: mod_base = OTHER; note = um
  modified_base 4: mod_base = OTHER; note = cm
  modified_base 5: mod_base = OTHER; note = cm
  modified_base 10: mod_base = OTHER; note = um
  modified_base 11: mod_base = OTHER; note = cm
  modified_base 12: mod_base = OTHER; note = um
  modified_base 13: mod_base = OTHER; note = cm
  modified_base 14: mod_base = OTHER; note = um
  modified_base 15: mod_base = OTHER; note = cm
  modified_base 16: mod_base = OTHER; note = um
  modified_base 1^2: mod_base = OTHER; note = phosphorothioate bond between nucleotides
gtgccaaaatctctctgga

SEQ ID NO: 1128 - RNA, 19 nt, synthetic construct
  source 1..19: mol_type = other RNA
  modified_base 1: mod_base = OTHER; note = gm
  modified_base 3: mod_base = OTHER; note = 2'-deoxy-2'-fluoroguanosine
  modified_base 4: mod_base = OTHER; note = 2'-deoxy-2'-fluorocytidine
  modified_base 5: mod_base = OTHER; note = 2'-deoxy-2'-fluorocytidine
  modified_base 7: mod_base = OTHER; note = 2'-deoxy-2'-fluoroadenosine
  modified_base 8: mod_base = OTHER; note = 2'-O-methyladenosine
  modified_base 1^2: mod_base = OTHER; note = phosphorothioate bond between nucleotides
gtgccaaaatctctctgga

SEQ ID NO: 1129 - RNA, 19 nt, synthetic construct
  source 1..19: mol_type = other RNA
  modified_base 1: mod_base = OTHER; note = gm
  modified_base 3: mod_base = OTHER; note = gm
  modified_base 5: mod_base = OTHER; note = cm
  modified_base 7: mod_base = OTHER; note = 2'-deoxy-2'-fluoroadenosine
  modified_base 9: mod_base = OTHER; note = 2'-deoxy-2'-fluoroadenosine
  modified_base 11: mod_base = OTHER; note = cm
  modified_base 13: mod_base = OTHER; note = cm
  modified_base 15: mod_base = OTHER; note = cm
  modified_base 17: mod_base = OTHER; note = gm
  modified_base 19: mod_base = OTHER; note = 2'-O-methyladenosine
  modified_base 1^2: mod_base = OTHER; note = phosphorothioate bond between nucleotides
gtgccaaaatctctctgga

SEQ ID NO: 1130 - RNA, 19 nt, synthetic construct
  source 1..19: mol_type = other RNA
  modified_base 2: mod_base = OTHER; note = 2'-deoxy-2'-fluorouridine
  modified_base 5: mod_base = OTHER; note = 2'-deoxy-2'-fluorocytidine
  modified_base 14: mod_base = OTHER; note = 2'-deoxy-2'-fluorouridine
  modified_base 16: mod_base = OTHER; note = um
  modified_base 1^2: mod_base = OTHER; note = phosphorothioate bond between nucleotides
gtgccaaaatctctctgga

SEQ ID NO: 1131 - RNA, 21 nt, synthetic construct
  source 1..21: mol_type = other RNA
  modified_base 1: mod_base = OTHER; note = abasic site of inverted abasic deoxyribose
  modified_base 3: mod_base = OTHER; note = 2'-deoxy-2'-fluorouridine
  modified_base 5: mod_base = OTHER; note = 2'-deoxy-2'-fluorocytidine
  modified_base 6: mod_base = OTHER; note = 2'-deoxy-2'-fluorocytidine
  modified_base 11: mod_base = OTHER; note = 2'-deoxy-2'-fluorouridine
  modified_base 12: mod_base = OTHER; note = 2'-deoxy-2'-fluorocytidine
  modified_base 13: mod_base = OTHER; note = um
  modified_base 14: mod_base = OTHER; note = cm
  modified_base 15: mod_base = OTHER; note = 2'-deoxy-2'-fluorouridine
  modified_base 16: mod_base = OTHER; note = 2'-deoxy-2'-fluorocytidine
  modified_base 17: mod_base = OTHER; note = 2'-deoxy-2'-fluorouridine
  modified_base 21: mod_base = OTHER; note = abasic site of inverted abasic deoxyribose
  modified_base 2^3: mod_base = OTHER; note = phosphorothioate bond between nucleotides
ngtgccaaaatctctctggan

SEQ ID NO: 1132 - RNA, 19 nt, synthetic construct
  source 1..19: mol_type = other RNA
  modified_base 2: mod_base = OTHER; note = um
  modified_base 4: mod_base = OTHER; note = um
  modified_base 5: mod_base = OTHER; note = um
  modified_base 11: mod_base = OTHER; note = um
  modified_base 13: mod_base = OTHER; note = um
  modified_base 15: mod_base = OTHER; note = um
  modified_base 1^2: mod_base = OTHER; note = phosphorothioate bond between nucleotides
gtgttaaaatttttttgga

SEQ ID NO: 1133 - RNA, 19 nt, synthetic construct
  source 1..19: mol_type = other RNA
  modified_base 2: mod_base = OTHER; note = um
  modified_base 4: mod_base = OTHER; note = cm
  modified_base 5: mod_base = OTHER; note = cm
  modified_base 16: mod_base = OTHER; note = um
  modified_base 1..4: mod_base = OTHER; note = phosphorothioate bond between nucleotides
gtgccaaaatctctctgga

SEQ ID NO: 1134 - DNA, 19 bp, synthetic construct
  source 1..19: mol_type = other DNA
  misc_feature 1..5: note = DNA
  misc_feature 6..14: note = RNA
  misc_feature 15..19: note = DNA
  modified_base 4: mod_base = i
  modified_base 5: mod_base = i
  modified_base 6: mod_base = OTHER; note = 2'-O-methyladenosine
  modified_base 7: mod_base = OTHER; note = 2'-O-methyladenosine
  modified_base 8: mod_base = OTHER; note = 2'-O-methyladenosine
  modified_base 9: mod_base = OTHER; note = 2'-O-methyladenosine
  modified_base 11: mod_base = OTHER; note = cm
  modified_base 12: mod_base = OTHER; note = um
  modified_base 13: mod_base = OTHER; note = cm
  modified_base 14: mod_base = OTHER; note = um
  modified_base 15: mod_base = i
  modified_base 16: mod_base = i
  modified_base 1^2: mod_base = OTHER; note = phosphorothioate bond between nucleotides
gtgnnaaaatctctnngga

SEQ ID NO: 1135 - RNA, 19 nt, synthetic construct
  source 1..19: mol_type = other RNA
  modified_base 1: mod_base = OTHER; note = gm
  modified_base 2: mod_base = OTHER; note = um
  modified_base 4: mod_base = OTHER; note = cm
  modified_base 5: mod_base = OTHER; note = cm
  modified_base 10: mod_base = OTHER; note = um
  modified_base 11: mod_base = OTHER; note = cm
  modified_base 12: mod_base = OTHER; note = um
  modified_base 13: mod_base = OTHER; note = cm
  modified_base 14: mod_base = OTHER; note = um
  modified_base 15: mod_base = OTHER; note = cm
  modified_base 16: mod_base = OTHER; note = um
  modified_base 18^19: mod_base = OTHER; note = phosphorothioate bond between nucleotides
gtgccaaaatctctctgga

SEQ ID NO: 1136 - RNA, 19 nt, synthetic construct
  source 1..19: mol_type = other RNA
  modified_base 1: mod_base = OTHER; note = gm
  modified_base 2: mod_base = OTHER; note = um
  modified_base 4: mod_base = OTHER; note = cm
  modified_base 5: mod_base = OTHER; note = cm
  modified_base 10: mod_base = OTHER; note = um
  modified_base 11: mod_base = OTHER; note = cm
  modified_base 12: mod_base = OTHER; note = um
  modified_base 13: mod_base = OTHER; note = cm
  modified_base 14: mod_base = OTHER; note = um
  modified_base 15: mod_base = OTHER; note = cm
  modified_base 16: mod_base = OTHER; note = um
  modified_base 18^19: mod_base = OTHER; note = phosphorothioate bond between nucleotides
gtgccaaaatctctctgga

SEQ ID NO: 1137 - RNA, 19 nt, synthetic construct
  source 1..19: mol_type = other RNA
  modified_base 1: mod_base = OTHER; note = gm
  modified_base 2: mod_base = OTHER; note = 2'-O-methyladenosine
  modified_base 3: mod_base = OTHER; note = 2'-deoxy-2'-fluorouridine
  modified_base 4: mod_base = OTHER; note = gm
  modified_base 5: mod_base = OTHER; note = 2'-deoxy-2'-fluoroguanosine
  modified_base 6: mod_base = OTHER; note = 2'-O-methyladenosine
  modified_base 7: mod_base = OTHER; note = 2'-deoxy-2'-fluoroguanosine
  modified_base 8: mod_base = OTHER; note = cm
  modified_base 9: mod_base = OTHER; note = 2'-deoxy-2'-fluoroadenosine
  modified_base 10: mod_base = OTHER; note = um
  modified_base 11: mod_base = OTHER; note = 2'-deoxy-2'-fluoroguanosine
  modified_base 12: mod_base = OTHER; note = um
  modified_base 13: mod_base = OTHER; note = 2'-deoxy-2'-fluoroguanosine
  modified_base 14: mod_base = OTHER; note = cm
  modified_base 15: mod_base = OTHER; note = 2'-deoxy-2'-fluoroguanosine
  modified_base 16: mod_base = OTHER; note = 2'-O-methyladenosine
  modified_base 17: mod_base = OTHER; note = 2'-deoxy-2'-fluoroadenosine
  modified_base 18: mod_base = OTHER; note = um
  modified_base 19: mod_base = OTHER; note = 2'-deoxy-2'-fluorouridine
gatggagcatgtgcgaatt

SEQ ID NO: 1138 - RNA, 19 nt, synthetic construct
  source 1..19: mol_type = other RNA
  modified_base 1: mod_base = OTHER; note = gm
  modified_base 2: mod_base = OTHER; note = 2'-O-methyladenosine
  modified_base 3: mod_base = OTHER; note = 2'-deoxy-2'-fluorouridine
  modified_base 4: mod_base = OTHER; note = gm
  modified_base 5: mod_base = OTHER; note = 2'-deoxy-2'-fluoroguanosine
  modified_base 6: mod_base = OTHER; note = 2'-O-methyladenosine
  modified_base 7: mod_base = OTHER; note = 2'-deoxy-2'-fluoroguanosine
  modified_base 8: mod_base = OTHER; note = cm
  modified_base 9: mod_base = OTHER; note = 2'-deoxy-2'-fluoroadenosine
  modified_base 10: mod_base = OTHER; note = um
  modified_base 11: mod_base = OTHER; note = 2'-deoxy-2'-fluoroguanosine
  modified_base 12: mod_base = OTHER; note = um
  modified_base 13: mod_base = OTHER; note = 2'-deoxy-2'-fluoroguanosine
  modified_base 14: mod_base = OTHER; note = cm
  modified_base 15: mod_base = OTHER; note = 2'-deoxy-2'-fluoroguanosine
  modified_base 16: mod_base = OTHER; note = 2'-O-methyladenosine
  modified_base 17: mod_base = OTHER; note = 2'-deoxy-2'-fluoroadenosine
  modified_base 18: mod_base = OTHER; note = um
  modified_base 19: mod_base = OTHER; note = 2'-deoxy-2'-fluorouridine
  modified_base 1^2: mod_base = OTHER; note = phosphorothioate bond between nucleotides
gatggagcatgtgcgaatt

SEQ ID NO: 1139 - RNA, 19 nt, synthetic construct
  source 1..19: mol_type = other RNA
  modified_base 1: mod_base = OTHER; note = gm
  modified_base 2: mod_base = OTHER; note = 2'-O-methyladenosine
  modified_base 3: mod_base = OTHER; note = 2'-deoxy-2'-fluorouridine
  modified_base 4: mod_base = OTHER; note = gm
  modified_base 5: mod_base = OTHER; note = 2'-deoxy-2'-fluoroguanosine
  modified_base 6: mod_base = OTHER; note = 2'-O-methyladenosine
  modified_base 7: mod_base = OTHER; note = 2'-deoxy-2'-fluoroguanosine
  modified_base 8: mod_base = OTHER; note = cm
  modified_base 9: mod_base = OTHER; note = 2'-deoxy-2'-fluoroadenosine
  modified_base 10: mod_base = OTHER; note = um
  modified_base 11: mod_base = OTHER; note = 2'-deoxy-2'-fluoroguanosine
  modified_base 12: mod_base = OTHER; note = um
  modified_base 13: mod_base = OTHER; note = 2'-deoxy-2'-fluoroguanosine
  modified_base 14: mod_base = OTHER; note = cm
  modified_base 15: mod_base = OTHER; note = 2'-deoxy-2'-fluoroguanosine
  modified_base 16: mod_base = OTHER; note = 2'-O-methyladenosine
  modified_base 17: mod_base = OTHER; note = 2'-deoxy-2'-fluoroadenosine
  modified_base 18: mod_base = OTHER; note = um
  modified_base 19: mod_base = OTHER; note = 2'-deoxy-2'-fluorouridine
  modified_base 1^2: mod_base = OTHER; note = phosphorothioate bond between nucleotides
gatggagcatgtgcgaatt

SEQ ID NO: 1140 - RNA, 19 nt, synthetic construct
  source 1..19: mol_type = other RNA
  modified_base 1: mod_base = OTHER; note = gm
  modified_base 2: mod_base = OTHER; note = 2'-O-methyladenosine
  modified_base 3: mod_base = OTHER; note = 2'-deoxy-2'-fluorouridine
  modified_base 4: mod_base = OTHER; note = gm
  modified_base 5: mod_base = OTHER; note = 2'-deoxy-2'-fluoroguanosine
  modified_base 6: mod_base = OTHER; note = 2'-O-methyladenosine
  modified_base 7: mod_base = OTHER; note = 2'-deoxy-2'-fluoroguanosine
  modified_base 8: mod_base = OTHER; note = cm
  modified_base 9: mod_base = OTHER; note = 2'-deoxy-2'-fluoroadenosine
  modified_base 10: mod_base = OTHER; note = um
  modified_base 11: mod_base = OTHER; note = 2'-deoxy-2'-fluoroguanosine
  modified_base 12: mod_base = OTHER; note = um
  modified_base 13: mod_base = OTHER; note = 2'-deoxy-2'-fluoroguanosine
  modified_base 14: mod_base = OTHER; note = cm
  modified_base 15: mod_base = OTHER; note = 2'-deoxy-2'-fluoroguanosine
  modified_base 16: mod_base = OTHER; note = 2'-O-methyladenosine
  modified_base 17: mod_base = OTHER; note = 2'-deoxy-2'-fluoroadenosine
  modified_base 18: mod_base = OTHER; note = um
  modified_base 19: mod_base = OTHER; note = 2'-deoxy-2'-fluorouridine
  modified_base 1^2: mod_base = OTHER; note = phosphorothioate bond between nucleotides
gatggagcatgtgcgaatt

SEQ ID NO: 1141 - RNA, 19 nt, synthetic construct
  source 1..19: mol_type = other RNA
  modified_base 1: mod_base = OTHER; note = gm
  modified_base 3: mod_base = OTHER; note = um
  modified_base 8: mod_base = OTHER; note = cm
  modified_base 10: mod_base = OTHER; note = um
  modified_base 12: mod_base = OTHER; note = um
  modified_base 14: mod_base = OTHER; note = cm
  modified_base 18: mod_base = OTHER; note = um
  modified_base 19: mod_base = OTHER; note = um
  modified_base 1^2: mod_base = OTHER; note = phosphorothioate bond between nucleotides
gatggagcatgtgcgaatt

SEQ ID NO: 1142 - RNA, 19 nt, synthetic construct
  source 1..19: mol_type = other RNA
  modified_base 1: mod_base = OTHER; note = gm
  modified_base 3: mod_base = OTHER; note = um
  modified_base 8: mod_base = OTHER; note = cm
  modified_base 10: mod_base = OTHER; note = um
  modified_base 12: mod_base = OTHER; note = um
  modified_base 14: mod_base = OTHER; note = cm
  modified_base 18: mod_base = OTHER; note = um
  modified_base 19: mod_base = OTHER; note = um
  modified_base 1^2: mod_base = OTHER; note = phosphorothioate bond between nucleotides
gatggagcatgtgcgaatt

SEQ ID NO: 1143 - RNA, 19 nt, synthetic construct
  source 1..19: mol_type = other RNA
  modified_base 1: mod_base = OTHER; note = gm
  modified_base 3: mod_base = OTHER; note = um
  modified_base 8: mod_base = OTHER; note = cm
  modified_base 10: mod_base = OTHER; note = um
  modified_base 12: mod_base = OTHER; note = um
  modified_base 14: mod_base = OTHER; note = cm
  modified_base 18: mod_base = OTHER; note = um
  modified_base 19: mod_base = OTHER; note = um
  modified_base 1^2: mod_base = OTHER; note = phosphorothioate bond between nucleotides
gatggagcatgtgcgaatt

SEQ ID NO: 1144 - RNA, 19 nt, synthetic construct
  source 1..19: mol_type = other RNA
  modified_base 1: mod_base = OTHER; note = Unlocked nucleic acid (UNA) monomer
  modified_base 3: mod_base = OTHER; note = um
  modified_base 8: mod_base = OTHER; note = cm
  modified_base 10: mod_base = OTHER; note = um
  modified_base 12: mod_base = OTHER; note = um
  modified_base 14: mod_base = OTHER; note = cm
  modified_base 18: mod_base = OTHER; note = um
  modified_base 19: mod_base = OTHER; note = um
  modified_base 1^2: mod_base = OTHER; note = phosphorothioate bond between nucleotides
gatggagcatgtgcgaatt

SEQ ID NO: 1145 - RNA, 19 nt, synthetic construct
  source 1..19: mol_type = other RNA
  modified_base 1: mod_base = OTHER; note = Unlocked nucleic acid (UNA) monomer
  modified_base 3: mod_base = OTHER; note = um
  modified_base 8: mod_base = OTHER; note = cm
  modified_base 10: mod_base = OTHER; note = um
  modified_base 12: mod_base = OTHER; note = um
  modified_base 14: mod_base = OTHER; note = cm
  modified_base 18: mod_base = OTHER; note = um
  modified_base 19: mod_base = OTHER; note = um
  modified_base 1^2: mod_base = OTHER; note = phosphorothioate bond between nucleotides
gatggagcatgtgcgaatt

SEQ ID NO: 1146 - RNA, 19 nt, synthetic construct
  source 1..19: mol_type = other RNA
  modified_base 1: mod_base = OTHER; note = 5'-O-methyl modified 2'-deoxyguanosine
  modified_base 3: mod_base = OTHER; note = um
  modified_base 8: mod_base = OTHER; note = cm
  modified_base 10: mod_base = OTHER; note = um
  modified_base 12: mod_base = OTHER; note = um
  modified_base 14: mod_base = OTHER; note = cm
  modified_base 18: mod_base = OTHER; note = um
  modified_base 19: mod_base = OTHER; note = um
  modified_base 1^2: mod_base = OTHER; note = phosphorothioate bond between nucleotides
gatggagcatgtgcgaatt

SEQ ID NO: 1147 - RNA, 19 nt, synthetic construct
  source 1..19: mol_type = other RNA
  modified_base 1: mod_base = OTHER; note = 5'-O-methyl modified 2'-deoxyguanosine
  modified_base 3: mod_base = OTHER; note = um
  modified_base 8: mod_base = OTHER; note = cm
  modified_base 10: mod_base = OTHER; note = um
  modified_base 12: mod_base = OTHER; note = um
  modified_base 14: mod_base = OTHER; note = cm
  modified_base 18: mod_base = OTHER; note = um
  modified_base 19: mod_base = OTHER; note = um
  modified_base 1^2: mod_base = OTHER; note = phosphorothioate bond between nucleotides
gatggagcatgtgcgaatt

SEQ ID NO: 1148 - RNA, 19 nt, synthetic construct
  source 1..19: mol_type = other RNA
  modified_base 1: mod_base = OTHER; note = gm
  modified_base 2: mod_base = OTHER; note = 2'-O-methyladenosine
  modified_base 3: mod_base = OTHER; note = um
  modified_base 4: mod_base = OTHER; note = gm
  modified_base 5: mod_base = OTHER; note = gm
  modified_base 6: mod_base = OTHER; note = 2'-deoxy-2'-fluorouridine
  modified_base 8: mod_base = OTHER; note = cm
  modified_base 10: mod_base = OTHER; note = um
  modified_base 12: mod_base = OTHER; note = um
  modified_base 14: mod_base = OTHER; note = cm
  modified_base 18: mod_base = OTHER; note = um
  modified_base 19: mod_base = OTHER; note = um
  modified_base 1^2: mod_base = OTHER; note = phosphorothioate bond between nucleotides
gatggtgcatgtgcgaatt

SEQ ID NO: 1149 - RNA, 19 nt, synthetic construct
  source 1..19: mol_type = other RNA
  modified_base 1: mod_base = OTHER; note = gm
  modified_base 3: mod_base = OTHER; note = um
  modified_base 5: mod_base = OTHER; note = gm
  modified_base 7: mod_base = OTHER; note = gm
  modified_base 8: mod_base = OTHER; note = cm
  modified_base 9: mod_base = OTHER; note = 2'-O-methyladenosine
  modified_base 10: mod_base = OTHER; note = um
  modified_base 11: mod_base = OTHER; note = gm
  modified_base 12: mod_base = OTHER; note = um
  modified_base 13: mod_base = OTHER; note = gm
  modified_base 14: mod_base = OTHER; note = cm
  modified_base 15: mod_base = OTHER; note = gm
  modified_base 17: mod_base = OTHER; note = 2'-O-methyladenosine
  modified_base 19: mod_base = OTHER; note = um
  modified_base 1^2: mod_base = OTHER; note = phosphorothioate bond between nucleotides
  modified_base 18^19: mod_base = OTHER; note = phosphorothioate bond between nucleotides
gatggagcatgtgcgaatt

SEQ ID NO: 1150 - RNA, 19 nt, synthetic construct
  source 1..19: mol_type = other RNA
  modified_base 3: mod_base = OTHER; note = 2'-deoxy-2'-fluorouridine
  modified_base 8: mod_base = OTHER; note = 2'-deoxy-2'-fluorocytidine
  modified_base 12: mod_base = OTHER; note = 2'-deoxy-2'-fluorouridine
  modified_base 18: mod_base = OTHER; note = 2'-deoxy-2'-fluorouridine
  modified_base 1^2: mod_base = OTHER; note = phosphorothioate bond between nucleotides
gatggagcatgtgcgaatt

SEQ ID NO: 1151 - RNA, 21 nt, synthetic construct
  source 1..21: mol_type = other RNA
  modified_base 1: mod_base = OTHER; note = abasic site of inverted abasic deoxyribose
  modified_base 4: mod_base = OTHER; note = 2'-deoxy-2'-fluorouridine
  modified_base 9: mod_base = OTHER; note = 2'-deoxy-2'-fluorocytidine
  modified_base 15: mod_base = OTHER; note = 2'-deoxy-2'-fluorocytidine
  modified_base 19: mod_base = OTHER; note = 2'-deoxy-2'-fluorouridine
  modified_base 20: mod_base = OTHER; note = 2'-deoxy-2'-fluorouridine
  modified_base 21: mod_base = OTHER; note = abasic site of inverted abasic deoxyribose
  modified_base 2^3: mod_base = OTHER; note = phosphorothioate bond between nucleotides
ngatggagcatgtgcgaattn

SEQ ID NO: 1152 - RNA, 19 nt, synthetic construct
  source 1..19: mol_type = other RNA
  modified_base 1: mod_base = OTHER; note = gm
  modified_base 3: mod_base = OTHER; note = um
  modified_base 8: mod_base = OTHER; note = cm
  modified_base 10: mod_base = OTHER; note = um
  modified_base 12: mod_base = OTHER; note = um
  modified_base 14: mod_base = OTHER; note = cm
  modified_base 18: mod_base = OTHER; note = um
  modified_base 19: mod_base = OTHER; note = um
  modified_base 1^2: mod_base = OTHER; note = phosphorothioate bond between nucleotides
gatggagcatgtgcgaatt

SEQ ID NO: 1153 - RNA, 19 nt, synthetic construct
  source 1..19: mol_type = other RNA
  modified_base 3: mod_base = OTHER; note = um
  modified_base 4: mod_base = OTHER; note = gm
  modified_base 8: mod_base = OTHER; note = cm
  modified_base 12: mod_base = OTHER; note = um
  modified_base 13: mod_base = OTHER; note = gm
  modified_base 1^2: mod_base = OTHER; note = phosphorothioate bond between nucleotides
gatggagcatgtgcgaatt

SEQ ID NO: 1154 - DNA, 19 bp, synthetic construct
  source 1..19: mol_type = other DNA
  misc_feature 1..5: note = DNA
  misc_feature 6..15: note = RNA
  misc_feature 16..19: note = DNA
  modified_base 2: mod_base = OTHER; note = uracil
  modified_base 3: mod_base = i
  modified_base 7: mod_base = OTHER; note = gm
  modified_base 8: mod_base = OTHER; note = cm
  modified_base 9: mod_base = OTHER; note = 2'-O-methyladenosine
  modified_base 12: mod_base = OTHER; note = um
  modified_base 13: mod_base = OTHER; note = gm
  modified_base 14: mod_base = OTHER; note = cm
  modified_base 15: mod_base = OTHER; note = gm
  modified_base 18: mod_base = i
  modified_base 19: mod_base = i
  modified_base 1^2: mod_base = OTHER; note = phosphorothioate bond between nucleotides
gtnggagcatgtgcgaann

SEQ ID NO: 1155 - RNA, 19 nt, synthetic construct
  source 1..19: mol_type = other RNA
  modified_base 1: mod_base = OTHER; note = Unlocked nucleic acid (UNA) monomer
  modified_base 1^2: mod_base = OTHER; note = phosphorothioate bond between nucleotides
gatggagcatgtgcgaatt

SEQ ID NO: 1156 - RNA, 19 nt, synthetic construct
  source 1..19: mol_type = other RNA
  modified_base 1: mod_base = OTHER; note = Unlocked nucleic acid (UNA) monomer
  modified_base 1^2: mod_base = OTHER; note = phosphorothioate bond between nucleotides
gatggagcatgtgcgaatt

SEQ ID NO: 1157 - RNA, 19 nt, synthetic construct
  source 1..19: mol_type = other RNA
  modified_base 1: mod_base = OTHER; note = Unlocked nucleic acid (UNA) monomer
  modified_base 1^2: mod_base = OTHER; note = phosphorothioate bond between nucleotides
gatggagcatgtgcgaatt

SEQ ID NO: 1158 - RNA, 19 nt, synthetic construct
  source 1..19: mol_type = other RNA
  modified_base 1: mod_base = OTHER; note = gm
  modified_base 3: mod_base = OTHER; note = um
  modified_base 8: mod_base = OTHER; note = cm
  modified_base 10: mod_base = OTHER; note = um
  modified_base 12: mod_base = OTHER; note = um
  modified_base 14: mod_base = OTHER; note = cm
  modified_base 18: mod_base = OTHER; note = um
  modified_base 19: mod_base = OTHER; note = um
gatggagcatgtgcgaatt

SEQ ID NO: 1159 - RNA, 19 nt, synthetic construct
  source 1..19: mol_type = other RNA
  modified_base 1: mod_base = OTHER; note = cm
  modified_base 2: mod_base = OTHER; note = 2'-O-methyladenosine
  modified_base 3: mod_base = OTHER; note = 2'-deoxy-2'-fluoroadenosine
  modified_base 4: mod_base = OTHER; note = gm
  modified_base 5: mod_base = OTHER; note = 2'-deoxy-2'-fluorocytidine
  modified_base 6: mod_base = OTHER; note = um
  modified_base 7: mod_base = OTHER; note = 2'-deoxy-2'-fluorouridine
  modified_base 8: mod_base = OTHER; note = gm
  modified_base 9: mod_base = OTHER; note = 2'-deoxy-2'-fluorouridine
  modified_base 10: mod_base = OTHER; note = cm
  modified_base 11: mod_base = OTHER; note = 2'-deoxy-2'-fluoroadenosine
  modified_base 12: mod_base = OTHER; note = cm
  modified_base 13: mod_base = OTHER; note = 2'-deoxy-2'-fluorouridine
  modified_base 14: mod_base = OTHER; note = gm
  modified_base 15: mod_base = OTHER; note = 2'-deoxy-2'-fluorouridine
  modified_base 16: mod_base = OTHER; note = gm
  modified_base 17: mod_base = OTHER; note = 2'-deoxy-2'-fluoroadenosine
  modified_base 18: mod_base = OTHER; note = cm
  modified_base 19: mod_base = OTHER; note = 2'-deoxy-2'-fluoroadenosine
caagcttgtcactgtgaca

SEQ ID NO: 1160 - RNA, 19 nt, synthetic construct
  source 1..19: mol_type = other RNA
  modified_base 1: mod_base = OTHER; note = cm
  modified_base 2: mod_base = OTHER; note = 2'-O-methyladenosine
  modified_base 3: mod_base = OTHER; note = 2'-deoxy-2'-fluoroadenosine
  modified_base 4: mod_base = OTHER; note = gm
  modified_base 5: mod_base = OTHER; note = 2'-deoxy-2'-fluorocytidine
  modified_base 6: mod_base = OTHER; note = um
  modified_base 7: mod_base = OTHER; note = 2'-deoxy-2'-fluorouridine
  modified_base 8: mod_base = OTHER; note = gm
  modified_base 9: mod_base = OTHER; note = 2'-deoxy-2'-fluorouridine
  modified_base 10: mod_base = OTHER; note = cm
  modified_base 11: mod_base = OTHER; note = 2'-deoxy-2'-fluoroadenosine
  modified_base 12: mod_base = OTHER; note = cm
  modified_base 13: mod_base = OTHER; note = 2'-deoxy-2'-fluorouridine
  modified_base 14: mod_base = OTHER; note = gm
  modified_base 15: mod_base = OTHER; note = 2'-deoxy-2'-fluorouridine
  modified_base 16: mod_base = OTHER; note = gm
  modified_base 17: mod_base = OTHER; note = 2'-deoxy-2'-fluoroadenosine
  modified_base 18: mod_base = OTHER; note = cm
  modified_base 19: mod_base = OTHER; note = 2'-deoxy-2'-fluoroadenosine
  modified_base 1^2: mod_base = OTHER; note = phosphorothioate bond between nucleotides
caagcttgtcactgtgaca

SEQ ID NO: 1161 - RNA, 19 nt, synthetic construct
  source 1..19: mol_type = other RNA
  modified_base 1: mod_base = OTHER; note = cm
  modified_base 2: mod_base = OTHER; note = 2'-O-methyladenosine
  modified_base 3: mod_base = OTHER; note = 2'-deoxy-2'-fluoroadenosine
  modified_base 4: mod_base = OTHER; note = gm
  modified_base 5: mod_base = OTHER; note = 2'-deoxy-2'-fluorocytidine
  modified_base 6: mod_base = OTHER; note = um
  modified_base 7: mod_base = OTHER; note = 2'-deoxy-2'-fluorouridine
  modified_base 8: mod_base = OTHER; note = gm
  modified_base 9: mod_base = OTHER; note = 2'-deoxy-2'-fluorouridine
  modified_base 10: mod_base = OTHER; note = cm
  modified_base 11: mod_base = OTHER; note = 2'-deoxy-2'-fluoroadenosine
  modified_base 12: mod_base = OTHER; note = cm
  modified_base 13: mod_base = OTHER; note = 2'-deoxy-2'-fluorouridine
  modified_base 14: mod_base = OTHER; note = gm
  modified_base 15: mod_base = OTHER; note = 2'-deoxy-2'-fluorouridine
  modified_base 16: mod_base = OTHER; note = gm
  modified_base 17: mod_base = OTHER; note = 2'-deoxy-2'-fluoroadenosine
  modified_base 18: mod_base = OTHER; note = cm
  modified_base 19: mod_base = OTHER; note = 2'-deoxy-2'-fluoroadenosine
  modified_base 1^2: mod_base = OTHER; note = phosphorothioate bond between nucleotides
caagcttgtcactgtgaca

SEQ ID NO: 1162 - RNA, 19 nt, synthetic construct
  source 1..19: mol_type = other RNA
  modified_base 1: mod_base = OTHER; note = cm
  modified_base 2: mod_base = OTHER; note = 2'-O-methyladenosine
  modified_base 3: mod_base = OTHER; note = 2'-deoxy-2'-fluoroadenosine
  modified_base 4: mod_base = OTHER; note = gm
  modified_base 5: mod_base = OTHER; note = 2'-deoxy-2'-fluorocytidine
  modified_base 6: mod_base = OTHER; note = um
  modified_base 7: mod_base = OTHER; note = 2'-deoxy-2'-fluorouridine
  modified_base 8: mod_base = OTHER; note = gm
  modified_base 9: mod_base = OTHER; note = 2'-deoxy-2'-fluorouridine
  modified_base 10: mod_base = OTHER; note = cm
  modified_base 11: mod_base = OTHER; note = 2'-deoxy-2'-fluoroadenosine
  modified_base 12: mod_base = OTHER; note = cm
  modified_base 13: mod_base = OTHER; note = 2'-deoxy-2'-fluorouridine
  modified_base 14: mod_base = OTHER; note = gm
  modified_base 15: mod_base = OTHER; note = 2'-deoxy-2'-fluorouridine
  modified_base 16: mod_base = OTHER; note = gm
  modified_base 17: mod_base = OTHER; note = 2'-deoxy-2'-fluoroadenosine
  modified_base 18: mod_base = OTHER; note = cm
  modified_base 19: mod_base = OTHER; note = 2'-deoxy-2'-fluoroadenosine
  modified_base 1^2: mod_base = OTHER; note = phosphorothioate bond between nucleotides
caagcttgtcactgtgaca

SEQ ID NO: 1163 - RNA, 19 nt, synthetic construct
  source 1..19: mol_type = other RNA
  modified_base 1: mod_base = OTHER; note = cm
  modified_base 5: mod_base = OTHER; note = cm
  modified_base 6: mod_base = OTHER; note = um
  modified_base 7: mod_base = OTHER; note = um
  modified_base 9: mod_base = OTHER; note = um
  modified_base 10: mod_base = OTHER; note = cm
  modified_base 12: mod_base = OTHER; note = cm
  modified_base 13: mod_base = OTHER; note = um
  modified_base 14: mod_base = OTHER; note = gm
  modified_base 15: mod_base = OTHER; note = um
  modified_base 18: mod_base = OTHER; note = cm
  modified_base 1^2: mod_base = OTHER; note = phosphorothioate bond between nucleotides
caagcttgtcactgtgaca

SEQ ID NO: 1164 - RNA, 19 nt, synthetic construct
  source 1..19: mol_type = other RNA
  modified_base 1: mod_base = OTHER; note = cm
  modified_base 5: mod_base = OTHER; note = cm
  modified_base 6: mod_base = OTHER; note = um
  modified_base 7: mod_base = OTHER; note = um
  modified_base 9: mod_base = OTHER; note = um
  modified_base 10: mod_base = OTHER; note = cm
  modified_base 12: mod_base = OTHER; note = cm
  modified_base 13: mod_base = OTHER; note = um
  modified_base 14: mod_base = OTHER; note = gm
  modified_base 15: mod_base = OTHER; note = um
  modified_base 18: mod_base = OTHER; note = cm
  modified_base 1^2: mod_base = OTHER; note = phosphorothioate bond between nucleotides
caagcttgtcactgtgaca

SEQ ID NO: 1165 - RNA, 19 nt, synthetic construct
  source 1..19: mol_type = other RNA
  modified_base 1: mod_base = OTHER; note = cm
  modified_base 5: mod_base = OTHER; note = cm
  modified_base 6: mod_base = OTHER; note = um
  modified_base 7: mod_base = OTHER; note = um
  modified_base 9: mod_base = OTHER; note = um
  modified_base 10: mod_base = OTHER; note = cm
  modified_base 12: mod_base = OTHER; note = cm
  modified_base 13: mod_base = OTHER; note = um
  modified_base 14: mod_base = OTHER; note = gm
  modified_base 15: mod_base = OTHER; note = um
  modified_base 18: mod_base = OTHER; note = cm
  modified_base 1^2: mod_base = OTHER; note = phosphorothioate bond between nucleotides
caagcttgtcactgtgaca

SEQ ID NO: 1166 - RNA, 19 nt, synthetic construct
  source 1..19: mol_type = other RNA
  modified_base 1: mod_base = OTHER; note = Unlocked nucleic acid (UNA) monomer
  modified_base 5: mod_base = OTHER; note = cm
  modified_base 6: mod_base = OTHER; note = um
  modified_base 7: mod_base = OTHER; note = um
  modified_base 9: mod_base = OTHER; note = um
  modified_base 10: mod_base = OTHER; note = cm
  modified_base 12: mod_base = OTHER; note = cm
  modified_base 13: mod_base = OTHER; note = um
  modified_base 14: mod_base = OTHER; note = gm
  modified_base 15: mod_base = OTHER; note = um
  modified_base 18: mod_base = OTHER; note = cm
  modified_base 1^2: mod_base = OTHER; note = phosphorothioate bond between nucleotides
caagcttgtcactgtgaca

SEQ ID NO: 1167 - RNA, 19 nt, synthetic construct
  source 1..19: mol_type = other RNA
  modified_base 1: mod_base = OTHER; note = Unlocked nucleic acid (UNA) monomer
  modified_base 5: mod_base = OTHER; note = cm
  modified_base 6: mod_base = OTHER; note = um
  modified_base 7: mod_base = OTHER; note = um
  modified_base 9: mod_base = OTHER; note = um
  modified_base 10: mod_base = OTHER; note = cm
  modified_base 12: mod_base = OTHER; note = cm
  modified_base 13: mod_base = OTHER; note = um
  modified_base 14: mod_base = OTHER; note = gm
  modified_base 15: mod_base = OTHER; note = um
  modified_base 18: mod_base = OTHER; note = cm
  modified_base 1^2: mod_base = OTHER; note = phosphorothioate bond between nucleotides
caagcttgtcactgtgaca

SEQ ID NO: 1168 - RNA, 19 nt, synthetic construct
  source 1..19: mol_type = other RNA
  modified_base 1: mod_base = OTHER; note = 5'-O-methyl modified 2'-deoxycytidine
  modified_base 5: mod_base = OTHER; note = cm
  modified_base 6: mod_base = OTHER; note = um
  modified_base 7: mod_base = OTHER; note = um
  modified_base 9: mod_base = OTHER; note = um
  modified_base 10: mod_base = OTHER; note = cm
  modified_base 12: mod_base = OTHER; note = cm
  modified_base 13: mod_base = OTHER; note = um
  modified_base 14: mod_base = OTHER; note = gm
  modified_base 15: mod_base = OTHER; note = um
  modified_base 18: mod_base = OTHER; note = cm
  modified_base 1^2: mod_base = OTHER; note = phosphorothioate bond between nucleotides
caagcttgtcactgtgaca

SEQ ID NO: 1169 - RNA, 19 nt, synthetic construct
  source 1..19: mol_type = other RNA
  modified_base 1: mod_base = OTHER; note = 5'-O-methyl modified 2'-deoxycytidine
  modified_base 5: mod_base = OTHER; note = cm
  modified_base 6: mod_base = OTHER; note = um
  modified_base 7: mod_base = OTHER; note = um
  modified_base 9: mod_base = OTHER; note = um
  modified_base 10: mod_base = OTHER; note = cm
  modified_base 12: mod_base = OTHER; note = cm
  modified_base 13: mod_base = OTHER; note = um
  modified_base 14: mod_base = OTHER; note = gm
  modified_base 15: mod_base = OTHER; note = um
  modified_base 18: mod_base = OTHER; note = cm
  modified_base 1^2: mod_base = OTHER; note = phosphorothioate bond between nucleotides
caagcttgtcactgtgaca

SEQ ID NO: 1170 - RNA, 19 nt, synthetic construct
  source 1..19: mol_type = other RNA
  modified_base 1: mod_base = OTHER; note = cm
  modified_base 2: mod_base = OTHER; note = 2'-deoxy-2'-fluoroadenosine
  modified_base 3: mod_base = OTHER; note = 2'-O-methyladenosine
  modified_base 4: mod_base = OTHER; note = 2'-deoxy-2'-fluoroguanosine
  modified_base 5: mod_base = OTHER; note = cm
  modified_base 6: mod_base = OTHER; note = 2'-deoxy-2'-fluorouridine
  modified_base 7: mod_base = OTHER; note = 2'-deoxy-2'-fluorouridine
  modified_base 1^2: mod_base = OTHER; note = phosphorothioate bond between nucleotides
caagcttgtcactgtgaca

SEQ ID NO: 1171 - RNA, 19 nt, synthetic construct
  source 1..19: mol_type = other RNA
  modified_base 1: mod_base = OTHER; note = cm
  modified_base 3: mod_base = OTHER; note = 2'-O-methyladenosine
  modified_base 5: mod_base = OTHER; note = cm
  modified_base 7: mod_base = OTHER; note = um
  modified_base 9: mod_base = OTHER; note = um
  modified_base 11: mod_base = OTHER; note = 2'-O-methyladenosine
  modified_base 13: mod_base = OTHER; note = um
  modified_base 15: mod_base = OTHER; note = um
  modified_base 17: mod_base = OTHER; note = 2'-O-methyladenosine
  modified_base 19: mod_base = OTHER; note = 2'-O-methyladenosine
  modified_base 1^2: mod_base = OTHER; note = phosphorothioate bond between nucleotides
caagcttgtcactgtgaca

SEQ ID NO: 1172 - RNA, 19 nt, synthetic construct
  source 1..19: mol_type = other RNA
  modified_base 1: mod_base = OTHER; note = 2'-deoxy-2'-fluorocytidine
  modified_base 5: mod_base = OTHER; note = 2'-deoxy-2'-fluorocytidine
  modified_base 7: mod_base = OTHER; note = 2'-deoxy-2'-fluorouridine
  modified_base 15: mod_base = OTHER; note = 2'-deoxy-2'-fluorouridine
  modified_base 18^19: mod_base = OTHER; note = phosphorothioate bond between nucleotides
caagcttgtcactgtgaca

SEQ ID NO: 1173 - RNA, 21 nt, synthetic construct
  source 1..21: mol_type = other RNA
  modified_base 1: mod_base = OTHER; note = abasic site of inverted abasic deoxyribose
  modified_base 21: mod_base = OTHER; note = abasic site of inverted abasic deoxyribose
  modified_base 2^3: mod_base = OTHER; note = phosphorothioate bond between nucleotides
ncaagcttgtcactgtgacan

SEQ ID NO: 1174 - RNA, 19 nt, synthetic construct
  source 1..19: mol_type = other RNA
  modified_base 1: mod_base = OTHER; note = cm
  modified_base 6: mod_base = OTHER; note = um
  modified_base 7: mod_base = OTHER; note = um
  modified_base 9: mod_base = OTHER; note = um
  modified_base 13: mod_base = OTHER; note = um
  modified_base 15: mod_base = OTHER; note = um
  modified_base 18: mod_base = OTHER; note = cm
  modified_base 1^2: mod_base = OTHER; note = phosphorothioate bond between nucleotides
caagcttgtcactgtgaca

SEQ ID NO: 1175 - RNA, 19 nt, synthetic construct
  source 1..19: mol_type = other RNA
  modified_base 1: mod_base = OTHER; note = cm
  modified_base 7: mod_base = OTHER; note = um
  modified_base 13: mod_base = OTHER; note = um
  modified_base 15: mod_base = OTHER; note = um
  modified_base 18: mod_base = OTHER; note = cm
  modified_base 18^19: mod_base = OTHER; note = phosphorothioate bond between nucleotides
caagcttgtcactgtgaca

SEQ ID NO: 1176 - DNA, 19 bp, synthetic construct
  source 1..19: mol_type = other DNA
  misc_feature 1..6: note = DNA
  misc_feature 7..15: note = RNA
  misc_feature 16..19: note = DNA
  modified_base 6: mod_base = i
  modified_base 7: mod_base = OTHER; note = um
  modified_base 8: mod_base = OTHER; note = gm
  modified_base 9: mod_base = OTHER; note = um
  modified_base 10: mod_base = OTHER; note = cm
  modified_base 11: mod_base = OTHER; note = 2'-O-methyladenosine
  modified_base 12: mod_base = OTHER; note = cm
  modified_base 13: mod_base = OTHER; note = um
  modified_base 14: mod_base = OTHER; note = 2'-deoxy-2'-fluoroguanosine
  modified_base 15: mod_base = OTHER; note = 2'-deoxy-2'-fluorouridine
  modified_base 1^2: mod_base = OTHER; note = phosphorothioate bond between nucleotides
caagcntgtcactgtgaca

SEQ ID NO: 1177 - RNA, 19 nt, synthetic construct
  source 1..19: mol_type = other RNA
  modified_base 1: mod_base = OTHER; note = Unlocked nucleic acid (UNA) monomer
  modified_base 5: mod_base = OTHER; note = cm
  modified_base 6: mod_base = OTHER; note = um
  modified_base 7: mod_base = OTHER; note = um
  modified_base 9: mod_base = OTHER; note = um
  modified_base 10: mod_base = OTHER; note = cm
  modified_base 12: mod_base = OTHER; note = cm
  modified_base 13: mod_base = OTHER; note = um
  modified_base 14: mod_base = OTHER; note = gm
  modified_base 15: mod_base = OTHER; note = um
  modified_base 18: mod_base = OTHER; note = cm
  modified_base 1^2: mod_base = OTHER; note = phosphorothioate bond between nucleotides
caagcttgtcactgtgaca

SEQ ID NO: 1178 - RNA, 19 nt, synthetic construct
  source 1..19: mol_type = other RNA
  modified_base 1: mod_base = OTHER; note = Unlocked nucleic acid (UNA) monomer
  modified_base 5: mod_base = OTHER; note = cm
  modified_base 6: mod_base = OTHER; note = um
  modified_base 7: mod_base = OTHER; note = um
  modified_base 9: mod_base = OTHER; note = um
  modified_base 10: mod_base = OTHER; note = cm
  modified_base 12: mod_base = OTHER; note = cm
  modified_base 13: mod_base = OTHER; note = um
  modified_base 14: mod_base = OTHER; note = gm
  modified_base 15: mod_base = OTHER; note = um
  modified_base 18: mod_base = OTHER; note = cm
  modified_base 1^2: mod_base = OTHER; note = phosphorothioate bond between nucleotides
caagcttgtcactgtgaca

SEQ ID NO: 1179 - RNA, 19 nt, synthetic construct
  source 1..19: mol_type = other RNA
  modified_base 1: mod_base = OTHER; note = Unlocked nucleic acid (UNA) monomer
  modified_base 5: mod_base = OTHER; note = cm
  modified_base 6: mod_base = OTHER; note = um
  modified_base 7: mod_base = OTHER; note = um
  modified_base 9: mod_base = OTHER; note = um
  modified_base 10: mod_base = OTHER; note = cm
  modified_base 12: mod_base = OTHER; note = cm
  modified_base 13: mod_base = OTHER; note = um
  modified_base 14: mod_base = OTHER; note = gm
  modified_base 15: mod_base = OTHER; note = um
  modified_base 18: mod_base = OTHER; note = cm
  modified_base 1^2: mod_base = OTHER; note = phosphorothioate bond between nucleotides
caagcttgtcactgtgaca

SEQ ID NO: 1180 - RNA, 17 nt, synthetic construct
  source 1..17: mol_type = other RNA
  modified_base 1: mod_base = OTHER; note = cm
  modified_base 2: mod_base = OTHER; note = 2'-O-methyladenosine
  modified_base 3: mod_base = OTHER; note = 2'-deoxy-2'-fluoroadenosine
  modified_base 4: mod_base = OTHER; note = gm
  modified_base 5: mod_base = OTHER; note = 2'-deoxy-2'-fluorocytidine
  modified_base 6: mod_base = OTHER; note = um
  modified_base 7: mod_base = OTHER; note = 2'-deoxy-2'-fluorouridine
  modified_base 8: mod_base = OTHER; note = gm
  modified_base 9: mod_base = OTHER; note = 2'-deoxy-2'-fluorouridine
  modified_base 10: mod_base = OTHER; note = cm
  modified_base 11: mod_base = OTHER; note = 2'-deoxy-2'-fluoroadenosine
  modified_base 12: mod_base = OTHER; note = cm
  modified_base 13: mod_base = OTHER; note = 2'-deoxy-2'-fluorouridine
  modified_base 14: mod_base = OTHER; note = gm
  modified_base 15: mod_base = OTHER; note = 2'-deoxy-2'-fluorouridine
  modified_base 16: mod_base = OTHER; note = gm
  modified_base 17: mod_base = OTHER; note = 2'-deoxy-2'-fluoroadenosine
caagcttgtcactgtga

SEQ ID NO: 1181 - RNA, 15 nt, synthetic construct
  source 1..15: mol_type = other RNA
  modified_base 1: mod_base = OTHER; note = cm
  modified_base 2: mod_base = OTHER; note = 2'-O-methyladenosine
  modified_base 3: mod_base = OTHER; note = 2'-deoxy-2'-fluoroadenosine
  modified_base 4: mod_base = OTHER; note = gm
  modified_base 5: mod_base = OTHER; note = 2'-deoxy-2'-fluorocytidine
  modified_base 6: mod_base = OTHER; note = um
  modified_base 7: mod_base = OTHER; note = 2'-deoxy-2'-fluorouridine
  modified_base 8: mod_base = OTHER; note = gm
  modified_base 9: mod_base = OTHER; note = 2'-deoxy-2'-fluorouridine
  modified_base 10: mod_base = OTHER; note = cm
  modified_base 11: mod_base = OTHER; note = 2'-deoxy-2'-fluoroadenosine
  modified_base 12: mod_base = OTHER; note = cm
  modified_base 13: mod_base = OTHER; note = 2'-deoxy-2'-fluorouridine
  modified_base 14: mod_base = OTHER; note = gm
  modified_base 15: mod_base = OTHER; note = 2'-deoxy-2'-fluorouridine
caagcttgtcactgt

SEQ ID NO: 1182 - RNA, 19 nt, synthetic construct
  source 1..19: mol_type = other RNA
  modified_base 1: mod_base = OTHER; note = 2'-O-methyladenosine
  modified_base 2: mod_base = OTHER; note = cm
  modified_base 3: mod_base = OTHER; note = 2'-deoxy-2'-fluorocytidine
  modified_base 4: mod_base = OTHER; note = 2'-O-methyladenosine
  modified_base 5: mod_base = OTHER; note = 2'-deoxy-2'-fluoroadenosine
  modified_base 6: mod_base = OTHER; note = 2'-O-methyladenosine
  modified_base 7: mod_base = OTHER; note = 2'-deoxy-2'-fluoroadenosine
  modified_base 8: mod_base = OTHER; note = cm
  modified_base 9: mod_base = OTHER; note = 2'-deoxy-2'-fluorocytidine
  modified_base 10: mod_base = OTHER; note = um
  modified_base 11: mod_base = OTHER; note = 2'-deoxy-2'-fluoroguanosine
  modified_base 12: mod_base = OTHER; note = gm
  modified_base 13: mod_base = OTHER; note = 2'-deoxy-2'-fluorocytidine
  modified_base 14: mod_base = OTHER; note = um
  modified_base 15: mod_base = OTHER; note = 2'-deoxy-2'-fluoroguanosine
  modified_base 16: mod_base = OTHER; note = gm
  modified_base 17: mod_base = OTHER; note = 2'-deoxy-2'-fluorouridine
  modified_base 18: mod_base = OTHER; note = gm
  modified_base 19: mod_base = OTHER; note = 2'-deoxy-2'-fluoroadenosine
accaaaacctggctggtga

SEQ ID NO: 1183 - RNA, 17 nt, synthetic construct
  source 1..17: mol_type = other RNA
  modified_base 1: mod_base = OTHER; note = 2'-O-methyladenosine
  modified_base 2: mod_base = OTHER; note = cm
  modified_base 3: mod_base = OTHER; note = 2'-deoxy-2'-fluorocytidine
  modified_base 4: mod_base = OTHER; note = 2'-O-methyladenosine
  modified_base 5: mod_base = OTHER; note = 2'-deoxy-2'-fluoroadenosine
  modified_base 6: mod_base = OTHER; note = 2'-O-methyladenosine
  modified_base 7: mod_base = OTHER; note = 2'-deoxy-2'-fluoroadenosine
  modified_base 8: mod_base = OTHER; note = cm
  modified_base 9: mod_base = OTHER; note = 2'-deoxy-2'-fluorocytidine
  modified_base 10: mod_base = OTHER; note = um
  modified_base 11: mod_base = OTHER; note = 2'-deoxy-2'-fluoroguanosine
  modified_base 12: mod_base = OTHER; note = gm
  modified_base 13: mod_base = OTHER; note = 2'-deoxy-2'-fluorocytidine
  modified_base 14: mod_base = OTHER; note = um
  modified_base 15: mod_base = OTHER; note = 2'-deoxy-2'-fluoroguanosine
  modified_base 16: mod_base = OTHER; note = gm
  modified_base 17: mod_base = OTHER; note = 2'-deoxy-2'-fluoroadenosine
accaaaacctggctgga

SEQ ID NO: 1184 - RNA, 19 nt, synthetic construct
  source 1..19: mol_type = other RNA
  modified_base 1: mod_base = OTHER; note = 2'-O-methyladenosine
  modified_base 2: mod_base = OTHER; note = cm
  modified_base 3: mod_base = OTHER; note = 2'-deoxy-2'-fluorocytidine
  modified_base 4: mod_base = OTHER; note = 2'-O-methyladenosine
  modified_base 5: mod_base = OTHER; note = 2'-deoxy-2'-fluoroadenosine
  modified_base 6: mod_base = OTHER; note = 2'-O-methyladenosine
  modified_base 7: mod_base = OTHER; note = 2'-deoxy-2'-fluoroadenosine
  modified_base 8: mod_base = OTHER; note = cm
  modified_base 9: mod_base = OTHER; note = 2'-deoxy-2'-fluorocytidine
  modified_base 10: mod_base = OTHER; note = um
  modified_base 11: mod_base = OTHER; note = 2'-deoxy-2'-fluoroguanosine
  modified_base 12: mod_base = OTHER; note = gm
  modified_base 13: mod_base = OTHER; note = 2'-deoxy-2'-fluorocytidine
  modified_base 14: mod_base = OTHER; note = um
  modified_base 15: mod_base = OTHER; note = 2'-deoxy-2'-fluoroguanosine
  modified_base 16: mod_base = OTHER; note = gm
  modified_base 17: mod_base = OTHER; note = 2'-deoxy-2'-fluorouridine
  modified_base 18: mod_base = OTHER; note = um
  modified_base 19: mod_base = OTHER; note = 2'-deoxy-2'-fluoroguanosine
accaaaacctggctggttg

SEQ ID NO: 1185 - RNA, 19 nt, synthetic construct
  source 1..19: mol_type = other RNA
  modified_base 1: mod_base = OTHER; note = 2'-O-methyladenosine
  modified_base 2: mod_base = OTHER; note = cm
  modified_base 3: mod_base = OTHER; note = 2'-deoxy-2'-fluorocytidine
  modified_base 4: mod_base = OTHER; note = 2'-O-methyladenosine
  modified_base 5: mod_base = OTHER; note = 2'-deoxy-2'-fluoroadenosine
  modified_base 6: mod_base = OTHER; note = 2'-O-methyladenosine
  modified_base 7: mod_base = OTHER; note = 2'-deoxy-2'-fluoroadenosine
  modified_base 8: mod_base = OTHER; note = cm
  modified_base 9: mod_base = OTHER; note = 2'-deoxy-2'-fluorocytidine
  modified_base 10: mod_base = OTHER; note = um
  modified_base 11: mod_base = OTHER; note = 2'-deoxy-2'-fluoroguanosine
  modified_base 12: mod_base = OTHER; note = gm
  modified_base 13: mod_base = OTHER; note = 2'-deoxy-2'-fluorocytidine
  modified_base 14: mod_base = OTHER; note = um
  modified_base 15: mod_base = OTHER; note = 2'-deoxy-2'-fluoroguanosine
  modified_base 16: mod_base = OTHER; note = gm
  modified_base 17: mod_base = OTHER; note = 2'-deoxy-2'-fluorouridine
  modified_base 18: mod_base = OTHER; note = um
  modified_base 19: mod_base = OTHER; note = 2'-deoxy-2'-fluoroguanosine
  modified_base 1..3: mod_base = OTHER; note = phosphorothioate bond between nucleotides
accaaaacctggctggttg

SEQ ID NO: 1186 - RNA, 19 nt, synthetic construct
  source 1..19: mol_type = other RNA
  modified_base 1: mod_base = OTHER; note = 2'-O-methyladenosine
  modified_base 2: mod_base = OTHER; note = cm
  modified_base 3: mod_base = OTHER; note = 2'-deoxy-2'-fluorocytidine
  modified_base 4: mod_base = OTHER; note = 2'-O-methyladenosine
  modified_base 5: mod_base = OTHER; note = 2'-deoxy-2'-fluoroadenosine
  modified_base 6: mod_base = OTHER; note = 2'-O-methyladenosine
  modified_base 7: mod_base = OTHER; note = 2'-deoxy-2'-fluoroadenosine
  modified_base 8: mod_base = OTHER; note = cm
  modified_base 9: mod_base = OTHER; note = 2'-deoxy-2'-fluorocytidine
  modified_base 10: mod_base = OTHER; note = um
  modified_base 11: mod_base = OTHER; note = 2'-deoxy-2'-fluoroguanosine
  modified_base 12: mod_base = OTHER; note = gm
  modified_base 13: mod_base = OTHER; note = 2'-deoxy-2'-fluorocytidine
  modified_base 14: mod_base = OTHER; note = um
  modified_base 15: mod_base = OTHER; note = 2'-deoxy-2'-fluoroguanosine
  modified_base 16: mod_base = OTHER; note = gm
  modified_base 17: mod_base = OTHER; note = 2'-deoxy-2'-fluorouridine
  modified_base 18: mod_base = OTHER; note = um
  modified_base 19: mod_base = OTHER; note = 2'-deoxy-2'-fluoroguanosine
  modified_base 1^2: mod_base = OTHER; note = phosphorothioate bond between nucleotides
accaaaacctggctggttg

SEQ ID NO: 1187 - RNA, 19 nt, synthetic construct
  source 1..19: mol_type = other RNA
  modified_base 1: mod_base = OTHER; note = 2'-O-methyladenosine
  modified_base 2: mod_base = OTHER; note = cm
  modified_base 3: mod_base = OTHER; note = 2'-deoxy-2'-fluorocytidine
  modified_base 4: mod_base = OTHER; note = 2'-O-methyladenosine
  modified_base 5: mod_base = OTHER; note = 2'-deoxy-2'-fluoroadenosine
  modified_base 6: mod_base = OTHER; note = 2'-O-methyladenosine
  modified_base 7: mod_base = OTHER; note = 2'-deoxy-2'-fluoroadenosine
  modified_base 8: mod_base = OTHER; note = cm
  modified_base 9: mod_base = OTHER; note = 2'-deoxy-2'-fluorocytidine
  modified_base 10: mod_base = OTHER; note = um
  modified_base 11: mod_base = OTHER; note = 2'-deoxy-2'-fluoroguanosine
  modified_base 12: mod_base = OTHER; note = gm
  modified_base 13: mod_base = OTHER; note = 2'-deoxy-2'-fluorocytidine
  modified_base 14: mod_base = OTHER; note = um
  modified_base 15: mod_base = OTHER; note = 2'-deoxy-2'-fluoroguanosine
  modified_base 16: mod_base = OTHER; note = gm
  modified_base 17: mod_base = OTHER; note = 2'-deoxy-2'-fluorouridine
  modified_base 18: mod_base = OTHER; note = um
  modified_base 19: mod_base = OTHER; note = 2'-deoxy-2'-fluoroguanosine
  modified_base 1^2: mod_base = OTHER; note = phosphorothioate bond between nucleotides
accaaaacctggctggttg

SEQ ID NO: 1188 - RNA, 19 nt, synthetic construct
  source 1..19: mol_type = other RNA
  modified_base 1: mod_base = OTHER; note = 2'-O-methyladenosine
  modified_base 2: mod_base = OTHER; note = cm
  modified_base 3: mod_base = OTHER; note = cm
  modified_base 8: mod_base = OTHER; note = cm
  modified_base 9: mod_base = OTHER; note = cm
  modified_base 10: mod_base = OTHER; note = um
  modified_base 13: mod_base = OTHER; note = cm
  modified_base 14: mod_base = OTHER; note = um
  modified_base 17: mod_base = OTHER; note = um
  modified_base 18: mod_base = OTHER; note = um
  modified_base 1^2: mod_base = OTHER; note = phosphorothioate bond between nucleotides
accaaaacctggctggttg

SEQ ID NO: 1189 - RNA, 19 nt, synthetic construct
  source 1..19: mol_type = other RNA
  modified_base 1: mod_base = OTHER; note = 2'-O-methyladenosine
  modified_base 2: mod_base = OTHER; note = cm
  modified_base 3: mod_base = OTHER; note = cm
  modified_base 8: mod_base = OTHER; note = cm
  modified_base 9: mod_base = OTHER; note = cm
  modified_base 10: mod_base = OTHER; note = um
  modified_base 13: mod_base = OTHER; note = cm
  modified_base 14: mod_base = OTHER; note = um
  modified_base 17: mod_base = OTHER; note = um
  modified_base 18: mod_base = OTHER; note = um
  modified_base 1^2: mod_base = OTHER; note = phosphorothioate bond between nucleotides
accaaaacctggctggttg

SEQ ID NO: 1190 - RNA, 19 nt, synthetic construct
  source 1..19: mol_type = other RNA
  modified_base 1: mod_base = OTHER; note = 2'-O-methyladenosine
  modified_base 2: mod_base = OTHER; note = cm
  modified_base 3: mod_base = OTHER; note = cm
  modified_base 8: mod_base = OTHER; note = cm
  modified_base 9: mod_base = OTHER; note = cm
  modified_base 10: mod_base = OTHER; note = um
  modified_base 13: mod_base = OTHER; note = cm
  modified_base 14: mod_base = OTHER; note = um
  modified_base 17: mod_base = OTHER; note = um
  modified_base 18: mod_base = OTHER; note = um
  modified_base 1^2: mod_base = OTHER; note = phosphorothioate bond between nucleotides
accaaaacctggctggttg

SEQ ID NO: 1191 - RNA, 19 nt, synthetic construct
  source 1..19: mol_type = other RNA
  modified_base 1: mod_base = OTHER; note = Unlocked nucleic acid (UNA) monomer
  modified_base 2: mod_base = OTHER; note = cm
  modified_base 3: mod_base = OTHER; note = cm
  modified_base 8: mod_base = OTHER; note = cm
  modified_base 9: mod_base = OTHER; note = cm
  modified_base 10: mod_base = OTHER; note = um
  modified_base 13: mod_base = OTHER; note = cm
  modified_base 14: mod_base = OTHER; note = um
  modified_base 17: mod_base = OTHER; note = um
  modified_base 18: mod_base = OTHER; note = um
  modified_base 1^2: mod_base = OTHER; note = phosphorothioate bond between nucleotides
accaaaacctggctggttg

SEQ ID NO: 1192 - RNA, 19 nt, synthetic construct
  source 1..19: mol_type = other RNA
  modified_base 1: mod_base = OTHER; note = Unlocked nucleic acid (UNA) monomer
  modified_base 2: mod_base = OTHER; note = cm
  modified_base 3: mod_base = OTHER; note = cm
  modified_base 8: mod_base = OTHER; note = cm
  modified_base 9: mod_base = OTHER; note = cm
  modified_base 10: mod_base = OTHER; note = um
  modified_base 13: mod_base = OTHER; note = cm
  modified_base 14: mod_base = OTHER; note = um
  modified_base 17: mod_base = OTHER; note = um
  modified_base 18: mod_base = OTHER; note = um
  modified_base 1^2: mod_base = OTHER; note = phosphorothioate bond between nucleotides
accaaaacctggctggttg

SEQ ID NO: 1193 - RNA, 19 nt, synthetic construct
  source 1..19: mol_type = other RNA
  modified_base 1: mod_base = OTHER; note = 5'-O-methyladenosine
  modified_base 2: mod_base = OTHER; note = cm
  modified_base 3: mod_base = OTHER; note = cm
  modified_base 8: mod_base = OTHER; note = cm
  modified_base 9: mod_base = OTHER; note = cm
  modified_base 10: mod_base = OTHER; note = um
  modified_base 13: mod_base = OTHER; note = cm
  modified_base 14: mod_base = OTHER; note = um
  modified_base 17: mod_base = OTHER; note = um
  modified_base 18: mod_base = OTHER; note = um
  modified_base 1^2: mod_base = OTHER; note = phosphorothioate bond between nucleotides
accaaaacctggctggttg

SEQ ID NO: 1194 - RNA, 19 nt, synthetic construct
  source 1..19: mol_type = other RNA
  modified_base 1: mod_base = OTHER; note = 5'-O-methyladenosine
  modified_base 2: mod_base = OTHER; note = cm
  modified_base 3: mod_base = OTHER; note = cm
  modified_base 8: mod_base = OTHER; note = cm
  modified_base 9: mod_base = OTHER; note = cm
  modified_base 10: mod_base = OTHER; note = um
  modified_base 13: mod_base = OTHER; note = cm
  modified_base 14: mod_base = OTHER; note = um
  modified_base 17: mod_base = OTHER; note = um
  modified_base 18: mod_base = OTHER; note = um
  modified_base 1^2: mod_base = OTHER; note = phosphorothioate bond between nucleotides
accaaaacctggctggttg

SEQ ID NO: 1195 - RNA, 19 nt, synthetic construct
  source 1..19: mol_type = other RNA
  modified_base 1: mod_base = OTHER; note = 2'-O-methyladenosine
  modified_base 2: mod_base = OTHER; note = cm
  modified_base 3: mod_base = OTHER; note = 2'-deoxy-2'-fluorocytidine
  modified_base 4: mod_base = OTHER; note = 2'-O-methyladenosine
  modified_base 5: mod_base = OTHER; note = 2'-deoxy-2'-fluoroadenosine
  modified_base 6: mod_base = OTHER; note = 2'-O-methyladenosine
  modified_base 7: mod_base = OTHER; note = 2'-deoxy-2'-fluoroadenosine
  modified_base 1^2: mod_base = OTHER; note = phosphorothioate bond between nucleotides
accaaaacctggctggttg

SEQ ID NO: 1196 - RNA, 19 nt, synthetic construct
  source 1..19: mol_type = other RNA
  modified_base 1: mod_base = OTHER; note = 2'-O-methyladenosine
  modified_base 3: mod_base = OTHER; note = cm
  modified_base 5: mod_base = OTHER; note = 2'-O-methyladenosine
  modified_base 7: mod_base = OTHER; note = 2'-O-methyladenosine
  modified_base 11: mod_base = OTHER; note = gm
  modified_base 13: mod_base = OTHER; note = cm
  modified_base 15: mod_base = OTHER; note = gm
  modified_base 17: mod_base = OTHER; note = um
  modified_base 19: mod_base = OTHER; note = gm
  modified_base 1^2: mod_base = OTHER; note = phosphorothioate bond between nucleotides
accaaaacctggctggttg

SEQ ID NO: 1197 - RNA, 19 nt, synthetic construct
  source 1..19: mol_type = other RNA
  modified_base 2: mod_base = OTHER; note = 2'-deoxy-2'-fluorocytidine
  modified_base 3: mod_base = OTHER; note = 2'-deoxy-2'-fluorocytidine
  modified_base 14: mod_base = OTHER; note = 2'-deoxy-2'-fluorouridine
  modified_base 18: mod_base = OTHER; note = 2'-deoxy-2'-fluorouridine
  modified_base 18^19: mod_base = OTHER; note = phosphorothioate bond between nucleotides
accaaaacctggctggttg

SEQ ID NO: 1198 - RNA, 21 nt, synthetic construct
  source 1..21: mol_type = other RNA
  modified_base 1: mod_base = OTHER; note = abasic site of inverted abasic deoxyribose
  modified_base 3: mod_base = OTHER; note = 2'-deoxy-2'-fluorocytidine
  modified_base 4: mod_base = OTHER; note = 2'-deoxy-2'-fluorocytidine
  modified_base 9: mod_base = OTHER; note = 2'-deoxy-2'-fluorocytidine
  modified_base 15: mod_base = OTHER; note = 2'-deoxy-2'-fluorouridine
  modified_base 18: mod_base = OTHER; note = 2'-deoxy-2'-fluorouridine
  modified_base 19: mod_base = OTHER; note = 2'-deoxy-2'-fluorouridine
  modified_base 21: mod_base = OTHER; note = abasic site of inverted abasic deoxyribose
  modified_base 2^3: mod_base = OTHER; note = phosphorothioate bond between nucleotides
naccaaaacctggctggttgn

SEQ ID NO: 1199 - RNA, 19 nt, synthetic construct
  source 1..19: mol_type = other RNA
  modified_base 2: mod_base = OTHER; note = cm
  modified_base 3: mod_base = OTHER; note = cm
  modified_base 8: mod_base = OTHER; note = cm
  modified_base 9: mod_base = OTHER; note = cm
  modified_base 13: mod_base = OTHER; note = cm
  modified_base 14: mod_base = OTHER; note = um
  modified_base 17: mod_base = OTHER; note = um
  modified_base 18: mod_base = OTHER; note = um
  modified_base 1^2: mod_base = OTHER; note = phosphorothioate bond between nucleotides
accaaaacctggctggttg

SEQ ID NO: 1200 - RNA, 19 nt, synthetic construct
  source 1..19: mol_type = other RNA
  modified_base 3: mod_base = OTHER; note = cm
  modified_base 10: mod_base = OTHER; note = um
  modified_base 14: mod_base = OTHER; note = um
  modified_base 18: mod_base = OTHER; note = um
  modified_base 1^2: mod_base = OTHER; note = phosphorothioate bond between nucleotides
accaaaacctggctggttg

SEQ ID NO: 1201 - DNA, 19 bp, synthetic construct
  source 1..19: mol_type = other DNA
  misc_feature 1..7: note = DNA
  misc_feature 8..15: note = RNA
  misc_feature 16..19: note = DNA
  modified_base 8: mod_base = OTHER; note = cm
  modified_base 9: mod_base = OTHER; note = cm
  modified_base 10: mod_base = OTHER; note = um
  modified_base 11: mod_base = OTHER; note = gm
  modified_base 12: mod_base = OTHER; note = gm
  modified_base 13: mod_base = OTHER; note = cm
  modified_base 14: mod_base = OTHER; note = um
  modified_base 15: mod_base = OTHER; note = gm
  modified_base 17: mod_base = i
  modified_base 18: mod_base = i
  modified_base 1^2: mod_base = OTHER; note = phosphorothioate bond between nucleotides
accaaaacctggctggnng

SEQ ID NO: 1202 - RNA, 19 nt, synthetic construct
  source 1..19: mol_type = other RNA
  modified_base 1: mod_base = OTHER; note = Unlocked nucleic acid (UNA) monomer
  modified_base 2: mod_base = OTHER; note = cm
  modified_base 3: mod_base = OTHER; note = cm
  modified_base 8: mod_base = OTHER; note = cm
  modified_base 9: mod_base = OTHER; note = cm
  modified_base 10: mod_base = OTHER; note = um
  modified_base 13: mod_base = OTHER; note = cm
  modified_base 14: mod_base = OTHER; note = um
  modified_base 17: mod_base = OTHER; note = um
  modified_base 18: mod_base = OTHER; note = um
  modified_base 1^2: mod_base = OTHER; note = phosphorothioate bond between nucleotides
accaaaacctggctggttg

SEQ ID NO: 1203 - RNA, 19 nt, synthetic construct
  source 1..19: mol_type = other RNA
  modified_base 1: mod_base = OTHER; note = Unlocked nucleic acid (UNA) monomer
  modified_base 2: mod_base = OTHER; note = cm
  modified_base 3: mod_base = OTHER; note = cm
  modified_base 8: mod_base = OTHER; note = cm
  modified_base 9: mod_base = OTHER; note = cm
  modified_base 10: mod_base = OTHER; note = um
  modified_base 13: mod_base = OTHER; note = cm
  modified_base 14: mod_base = OTHER; note = um
  modified_base 17: mod_base = OTHER; note = um
  modified_base 18: mod_base = OTHER; note = um
accaaaacctggctggttg

SEQ ID NO: 1204 - RNA, 16 nt, synthetic construct
  source 1..16: mol_type = other RNA
  modified_base 1: mod_base = OTHER; note = 2'-O-methyladenosine
  modified_base 2: mod_base = OTHER; note = cm
  modified_base 3: mod_base = OTHER; note = cm
  modified_base 5: mod_base = OTHER; note = cm
  modified_base 6: mod_base = OTHER; note = cm
  modified_base 7: mod_base = OTHER; note = um
  modified_base 10: mod_base = OTHER; note = cm
  modified_base 11: mod_base = OTHER; note = um
  modified_base 14: mod_base = OTHER; note = um
  modified_base 15: mod_base = OTHER; note = um
  modified_base 1^2: mod_base = OTHER; note = phosphorothioate bond between nucleotides
accacctggctggttg

SEQ ID NO: 1205 - RNA, 17 nt, synthetic construct
  source 1..17: mol_type = other RNA
  modified_base 1: mod_base = OTHER; note = 2'-O-methyladenosine
  modified_base 2: mod_base = OTHER; note = cm
  modified_base 3: mod_base = OTHER; note = 2'-deoxy-2'-fluorocytidine
  modified_base 4: mod_base = OTHER; note = 2'-O-methyladenosine
  modified_base 5: mod_base = OTHER; note = 2'-deoxy-2'-fluoroadenosine
  modified_base 6: mod_base = OTHER; note = 2'-O-methyladenosine
  modified_base 7: mod_base = OTHER; note = 2'-deoxy-2'-fluoroadenosine
  modified_base 8: mod_base = OTHER; note = cm
  modified_base 9: mod_base = OTHER; note = 2'-deoxy-2'-fluorocytidine
  modified_base 10: mod_base = OTHER; note = um
  modified_base 11: mod_base = OTHER; note = 2'-deoxy-2'-fluoroguanosine
  modified_base 12: mod_base = OTHER; note = gm
  modified_base 13: mod_base = OTHER; note = 2'-deoxy-2'-fluorocytidine
  modified_base 14: mod_base = OTHER; note = um
  modified_base 15: mod_base = OTHER; note = 2'-deoxy-2'-fluoroguanosine
  modified_base 16: mod_base = OTHER; note = gm
  modified_base 17: mod_base = OTHER; note = 2'-deoxy-2'-fluorouridine
accaaaacctggctggt

SEQ ID NO: 1206 - RNA, 15 nt, synthetic construct
  source 1..15: mol_type = other RNA
  modified_base 1: mod_base = OTHER; note = 2'-O-methyladenosine
  modified_base 2: mod_base = OTHER; note = cm
  modified_base 3: mod_base = OTHER; note = 2'-deoxy-2'-fluorocytidine
  modified_base 4: mod_base = OTHER; note = 2'-O-methyladenosine
  modified_base 5: mod_base = OTHER; note = 2'-deoxy-2'-fluoroadenosine
  modified_base 6: mod_base = OTHER; note = 2'-O-methyladenosine
  modified_base 7: mod_base = OTHER; note = 2'-deoxy-2'-fluoroadenosine
  modified_base 8: mod_base = OTHER; note = cm
  modified_base 9: mod_base = OTHER; note = 2'-deoxy-2'-fluorocytidine
  modified_base 10: mod_base = OTHER; note = um
  modified_base 11: mod_base = OTHER; note = 2'-deoxy-2'-fluoroguanosine
  modified_base 12: mod_base = OTHER; note = gm
  modified_base 13: mod_base = OTHER; note = 2'-deoxy-2'-fluorocytidine
  modified_base 14: mod_base = OTHER; note = um
  modified_base 15: mod_base = OTHER; note = 2'-deoxy-2'-fluoroguanosine
accaaaacctggctg

SEQ ID NO: 1207 - RNA, 17 nt, synthetic construct
  source 1..17: mol_type = other RNA
  modified_base 1: mod_base = OTHER; note = cm
  modified_base 2: mod_base = OTHER; note = um
  modified_base 3: mod_base = OTHER; note = 2'-deoxy-2'-fluoroguanosine
  modified_base 4: mod_base = OTHER; note = cm
  modified_base 5: mod_base = OTHER; note = 2'-deoxy-2'-fluoroadenosine
  modified_base 6: mod_base = OTHER; note = gm
  modified_base 7: mod_base = OTHER; note = 2'-deoxy-2'-fluorouridine
  modified_base 8: mod_base = OTHER; note = gm
  modified_base 9: mod_base = OTHER; note = 2'-deoxy-2'-fluorocytidine
  modified_base 10: mod_base = OTHER; note = 2'-O-methyladenosine
  modified_base 11: mod_base = OTHER; note = 2'-deoxy-2'-fluoroguanosine
  modified_base 12: mod_base = OTHER; note = gm
  modified_base 13: mod_base = OTHER; note = 2'-deoxy-2'-fluoroadenosine
  modified_base 14: mod_base = OTHER; note = 2'-O-methyladenosine
  modified_base 15: mod_base = OTHER; note = 2'-deoxy-2'-fluoroadenosine
  modified_base 16: mod_base = OTHER; note = gm
  modified_base 17: mod_base = OTHER; note = 2'-deoxy-2'-fluoroadenosine
ctgcagtgcaggaaaga

SEQ ID NO: 1208 - RNA, 15 nt, synthetic construct
  source 1..15: mol_type = other RNA
  modified_base 1: mod_base = OTHER; note = cm
  modified_base 2: mod_base = OTHER; note = um
  modified_base 3: mod_base = OTHER; note = 2'-deoxy-2'-fluoroguanosine
  modified_base 4: mod_base = OTHER; note = cm
  modified_base 5: mod_base = OTHER; note = 2'-deoxy-2'-fluoroadenosine
  modified_base 6: mod_base = OTHER; note = gm
  modified_base 7: mod_base = OTHER; note = 2'-deoxy-2'-fluorouridine
  modified_base 8: mod_base = OTHER; note = gm
  modified_base 9: mod_base = OTHER; note = 2'-deoxy-2'-fluorocytidine
  modified_base 10: mod_base = OTHER; note = 2'-O-methyladenosine
  modified_base 11: mod_base = OTHER; note = 2'-deoxy-2'-fluoroguanosine
  modified_base 12: mod_base = OTHER; note = gm
  modified_base 13: mod_base = OTHER; note = 2'-deoxy-2'-fluoroadenosine
  modified_base 14: mod_base = OTHER; note = 2'-O-methyladenosine
  modified_base 15: mod_base = OTHER; note = 2'-deoxy-2'-fluoroadenosine
ctgcagtgcaggaaa

SEQ ID NO: 1209 - RNA, 17 nt, synthetic construct
  source 1..17: mol_type = other RNA
  modified_base 1: mod_base = OTHER; note = gm
  modified_base 2: mod_base = OTHER; note = um
  modified_base 3: mod_base = OTHER; note = 2'-deoxy-2'-fluorocytidine
  modified_base 4: mod_base = OTHER; note = 2'-O-methyladenosine
  modified_base 5: mod_base = OTHER; note = 2'-deoxy-2'-fluorouridine
  modified_base 6: mod_base = OTHER; note = 2'-O-methyladenosine
  modified_base 7: mod_base = OTHER; note = 2'-deoxy-2'-fluoroguanosine
  modified_base 8: mod_base = OTHER; note = cm
  modified_base 9: mod_base = OTHER; note = 2'-deoxy-2'-fluorocytidine
  modified_base 10: mod_base = OTHER; note = 2'-O-methyladenosine
  modified_base 11: mod_base = OTHER; note = 2'-deoxy-2'-fluorouridine
  modified_base 12: mod_base = OTHER; note = gm
  modified_base 13: mod_base = OTHER; note = 2'-deoxy-2'-fluorouridine
  modified_base 14: mod_base = OTHER; note = gm
  modified_base 15: mod_base = OTHER; note = 2'-deoxy-2'-fluoroguanosine
  modified_base 16: mod_base = OTHER; note = um
  modified_base 17: mod_base = OTHER; note = 2'-deoxy-2'-fluorouridine
gtcatagccatgtggtt

SEQ ID NO: 1210 - RNA, 15 nt, synthetic construct
  source 1..15: mol_type = other RNA
  modified_base 1: mod_base = OTHER; note = gm
  modified_base 2: mod_base = OTHER; note = um
  modified_base 3: mod_base = OTHER; note = 2'-deoxy-2'-fluorocytidine
  modified_base 4: mod_base = OTHER; note = 2'-O-methyladenosine
  modified_base 5: mod_base = OTHER; note = 2'-deoxy-2'-fluorouridine
  modified_base 6: mod_base = OTHER; note = 2'-O-methyladenosine
  modified_base 7: mod_base = OTHER; note = 2'-deoxy-2'-fluoroguanosine
  modified_base 8: mod_base = OTHER; note = cm
  modified_base 9: mod_base = OTHER; note = 2'-deoxy-2'-fluorocytidine
  modified_base 10: mod_base = OTHER; note = 2'-O-methyladenosine
  modified_base 11: mod_base = OTHER; note = 2'-deoxy-2'-fluorouridine
  modified_base 12: mod_base = OTHER; note = gm
  modified_base 13: mod_base = OTHER; note = 2'-deoxy-2'-fluorouridine
  modified_base 14: mod_base = OTHER; note = gm
  modified_base 15: mod_base = OTHER; note = 2'-deoxy-2'-fluoroguanosine
gtcatagccatgtgg

SEQ ID NO: 1211 - RNA, 21 nt, synthetic construct
  source 1..21: mol_type = other RNA
  modified_base 1: mod_base = OTHER; note = 2'-O-methyladenosine
  modified_base 2: mod_base = OTHER; note = cm
  modified_base 3: mod_base = OTHER; note = 2'-deoxy-2'-fluorocytidine
  modified_base 4: mod_base = OTHER; note = 2'-O-methyladenosine
  modified_base 5: mod_base = OTHER; note = 2'-deoxy-2'-fluoroadenosine
  modified_base 6: mod_base = OTHER; note = 2'-O-methyladenosine
  modified_base 7: mod_base = OTHER; note = 2'-deoxy-2'-fluoroadenosine
  modified_base 8: mod_base = OTHER; note = cm
  modified_base 9: mod_base = OTHER; note = 2'-deoxy-2'-fluorocytidine
  modified_base 10: mod_base = OTHER; note = um
  modified_base 11: mod_base = OTHER; note = 2'-deoxy-2'-fluoroguanosine
  modified_base 12: mod_base = OTHER; note = gm
  modified_base 13: mod_base = OTHER; note = 2'-deoxy-2'-fluorocytidine
  modified_base 14: mod_base = OTHER; note = um
  modified_base 15: mod_base = OTHER; note = 2'-deoxy-2'-fluoroguanosine
  modified_base 16: mod_base = OTHER; note = gm
  modified_base 17: mod_base = OTHER; note = 2'-deoxy-2'-fluorouridine
  modified_base 18: mod_base = OTHER; note = um
  modified_base 19: mod_base = OTHER; note = 2'-deoxy-2'-fluoroguanosine
  modified_base 20: mod_base = OTHER; note = gm
  modified_base 21: mod_base = OTHER; note = 2'-deoxy-2'-fluoroadenosine
accaaaacctggctggttgga

SEQ ID NO: 1212 - RNA, 21 nt, synthetic construct
  source 1..21: mol_type = other RNA
  modified_base 1: mod_base = OTHER; note = 2'-O-methyladenosine
  modified_base 2: mod_base = OTHER; note = cm
  modified_base 3: mod_base = OTHER; note = 2'-deoxy-2'-fluorocytidine
  modified_base 4: mod_base = OTHER; note = 2'-O-methyladenosine
  modified_base 5: mod_base = OTHER; note = 2'-deoxy-2'-fluoroadenosine
  modified_base 6: mod_base = OTHER; note = 2'-O-methyladenosine
  modified_base 7: mod_base = OTHER; note = 2'-deoxy-2'-fluoroadenosine
  modified_base 8: mod_base = OTHER; note = cm
  modified_base 9: mod_base = OTHER; note = 2'-deoxy-2'-fluorocytidine
  modified_base 10: mod_base = OTHER; note = um
  modified_base 11: mod_base = OTHER; note = 2'-deoxy-2'-fluoroguanosine
  modified_base 12: mod_base = OTHER; note = gm
  modified_base 13: mod_base = OTHER; note = 2'-deoxy-2'-fluorocytidine
  modified_base 14: mod_base = OTHER; note = um
  modified_base 15: mod_base = OTHER; note = 2'-deoxy-2'-fluoroguanosine
  modified_base 16: mod_base = OTHER; note = gm
  modified_base 17: mod_base = OTHER; note = 2'-deoxy-2'-fluorouridine
  modified_base 18: mod_base = OTHER; note = um
  modified_base 19: mod_base = OTHER; note = 2'-deoxy-2'-fluoroguanosine
  modified_base 20: mod_base = OTHER; note = gm
  modified_base 21: mod_base = OTHER; note = 2'-deoxy-2'-fluoroadenosine
  modified_base 1^2: mod_base = OTHER; note = phosphorothioate bond between nucleotides
accaaaacctggctggttgga

SEQ ID NO: 1213 - RNA, 21 nt, synthetic construct
  source 1..21: mol_type = other RNA
  modified_base 1: mod_base = OTHER; note = 2'-O-methyladenosine
  modified_base 2: mod_base = OTHER; note = cm
  modified_base 3: mod_base = OTHER; note = 2'-deoxy-2'-fluorocytidine
  modified_base 4: mod_base = OTHER; note = 2'-O-methyladenosine
  modified_base 5: mod_base = OTHER; note = 2'-deoxy-2'-fluoroadenosine
  modified_base 6: mod_base = OTHER; note = 2'-O-methyladenosine
  modified_base 7: mod_base = OTHER; note = 2'-deoxy-2'-fluoroadenosine
  modified_base 8: mod_base = OTHER; note = cm
  modified_base 9: mod_base = OTHER; note = 2'-deoxy-2'-fluorocytidine
  modified_base 10: mod_base = OTHER; note = um
  modified_base 11: mod_base = OTHER; note = 2'-deoxy-2'-fluoroguanosine
  modified_base 12: mod_base = OTHER; note = gm
  modified_base 13: mod_base = OTHER; note = 2'-deoxy-2'-fluorocytidine
  modified_base 14: mod_base = OTHER; note = um
  modified_base 15: mod_base = OTHER; note = 2'-deoxy-2'-fluoroguanosine
  modified_base 16: mod_base = OTHER; note = gm
  modified_base 17: mod_base = OTHER; note = 2'-deoxy-2'-fluorouridine
  modified_base 18: mod_base = OTHER; note = um
  modified_base 19: mod_base = OTHER; note = 2'-deoxy-2'-fluoroguanosine
  modified_base 20: mod_base = OTHER; note = gm
  modified_base 21: mod_base = OTHER; note = 2'-deoxy-2'-fluoroadenosine
  modified_base 1^2: mod_base = OTHER; note = phosphorothioate bond between nucleotides
accaaaacctggctggttgga

SEQ ID NO: 1214 - RNA, 21 nt, synthetic construct
  source 1..21: mol_type = other RNA
  modified_base 1: mod_base = OTHER; note = 2'-O-methyladenosine
  modified_base 2: mod_base = OTHER; note = cm
  modified_base 3: mod_base = OTHER; note = 2'-deoxy-2'-fluorocytidine
  modified_base 4: mod_base = OTHER; note = 2'-O-methyladenosine
  modified_base 5: mod_base = OTHER; note = 2'-deoxy-2'-fluoroadenosine
  modified_base 6: mod_base = OTHER; note = 2'-O-methyladenosine
  modified_base 7: mod_base = OTHER; note = 2'-deoxy-2'-fluoroadenosine
  modified_base 8: mod_base = OTHER; note = cm
  modified_base 9: mod_base = OTHER; note = 2'-deoxy-2'-fluorocytidine
  modified_base 10: mod_base = OTHER; note = um
  modified_base 11: mod_base = OTHER; note = 2'-deoxy-2'-fluoroguanosine
  modified_base 12: mod_base = OTHER; note = gm
  modified_base 13: mod_base = OTHER; note = 2'-deoxy-2'-fluorocytidine
  modified_base 14: mod_base = OTHER; note = um
  modified_base 15: mod_base = OTHER; note = 2'-deoxy-2'-fluoroguanosine
  modified_base 16: mod_base = OTHER; note = gm
  modified_base 17: mod_base = OTHER; note = 2'-deoxy-2'-fluorouridine
  modified_base 18: mod_base = OTHER; note = um
  modified_base 19: mod_base = OTHER; note = 2'-deoxy-2'-fluoroguanosine
  modified_base 20: mod_base = OTHER; note = gm
  modified_base 21: mod_base = OTHER; note = 2'-deoxy-2'-fluoroadenosine
  modified_base 1^2: mod_base = OTHER; note = phosphorothioate bond between nucleotides
accaaaacctggctggttgga

SEQ ID NO: 1215 - RNA, 21 nt, synthetic construct
  source 1..21: mol_type = other RNA
  modified_base 1: mod_base = OTHER; note = 2'-O-methyladenosine
  modified_base 2: mod_base = OTHER; note = cm
  modified_base 3: mod_base = OTHER; note = cm
  modified_base 8: mod_base = OTHER; note = cm
  modified_base 9: mod_base = OTHER; note = cm
  modified_base 10: mod_base = OTHER; note = um
  modified_base 13: mod_base = OTHER; note = cm
  modified_base 14: mod_base = OTHER; note = um
  modified_base 17: mod_base = OTHER; note = um
  modified_base 18: mod_base = OTHER; note = um
  modified_base 1^2: mod_base = OTHER; note = phosphorothioate bond between nucleotides
accaaaacctggctggttgga

SEQ ID NO: 1216 - RNA, 21 nt, synthetic construct
  source 1..21: mol_type = other RNA
  modified_base 1: mod_base = OTHER; note = 2'-O-methyladenosine
  modified_base 2: mod_base = OTHER; note = cm
  modified_base 3: mod_base = OTHER; note = cm
  modified_base 8: mod_base = OTHER; note = cm
  modified_base 9: mod_base = OTHER; note = cm
  modified_base 10: mod_base = OTHER; note = um
  modified_base 13: mod_base = OTHER; note = cm
  modified_base 14: mod_base = OTHER; note = um
  modified_base 17: mod_base = OTHER; note = um
  modified_base 18: mod_base = OTHER; note = um
  modified_base 1^2: mod_base = OTHER; note = phosphorothioate bond between nucleotides
accaaaacctggctggttgga

SEQ ID NO: 1217 - RNA, 21 nt, synthetic construct
  source 1..21: mol_type = other RNA
  modified_base 1: mod_base = OTHER; note = 2'-O-methyladenosine
  modified_base 2: mod_base = OTHER; note = cm
  modified_base 3: mod_base = OTHER; note = cm
  modified_base 8: mod_base = OTHER; note = cm
  modified_base 9: mod_base = OTHER; note = cm
  modified_base 10: mod_base = OTHER; note = um
  modified_base 13: mod_base = OTHER; note = cm
  modified_base 14: mod_base = OTHER; note = um
  modified_base 17: mod_base = OTHER; note = um
  modified_base 18: mod_base = OTHER; note = um
  modified_base 1^2: mod_base = OTHER; note = phosphorothioate bond between nucleotides
accaaaacctggctggttgga

SEQ ID NO: 1218 - RNA, 21 nt, synthetic construct
  source 1..21: mol_type = other RNA
  modified_base 1: mod_base = OTHER; note = Unlocked nucleic acid (UNA) monomer
  modified_base 2: mod_base = OTHER; note = cm
  modified_base 3: mod_base = OTHER; note = cm
  modified_base 8: mod_base = OTHER; note = cm
  modified_base 9: mod_base = OTHER; note = cm
  modified_base 10: mod_base = OTHER; note = um
  modified_base 13: mod_base = OTHER; note = cm
  modified_base 14: mod_base = OTHER; note = um
  modified_base 17: mod_base = OTHER; note = um
  modified_base 18: mod_base = OTHER; note = um
  modified_base 1^2: mod_base = OTHER; note = phosphorothioate bond between nucleotides
accaaaacctggctggttgga

SEQ ID NO: 1219 - RNA, 21 nt, synthetic construct
  source 1..21: mol_type = other RNA
  modified_base 1: mod_base = OTHER; note = Unlocked nucleic acid (UNA) monomer
  modified_base 2: mod_base = OTHER; note = cm
  modified_base 3: mod_base = OTHER; note = cm
  modified_base 8: mod_base = OTHER; note = cm
  modified_base 9: mod_base = OTHER; note = cm
  modified_base 10: mod_base = OTHER; note = um
  modified_base 13: mod_base = OTHER; note = cm
  modified_base 14: mod_base = OTHER; note = um
  modified_base 17: mod_base = OTHER; note = um
  modified_base 18: mod_base = OTHER; note = um
  modified_base 1^2: mod_base = OTHER; note = phosphorothioate bond between nucleotides
accaaaacctggctggttgga

SEQ ID NO: 1220 - RNA, 21 nt, synthetic construct
  source 1..21: mol_type = other RNA
  modified_base 1: mod_base = OTHER; note = 5'-O-methyladenosine
  modified_base 2: mod_base = OTHER; note = cm
  modified_base 3: mod_base = OTHER; note = cm
  modified_base 8: mod_base = OTHER; note = cm
  modified_base 9: mod_base = OTHER; note = cm
  modified_base 10: mod_base = OTHER; note = um
  modified_base 13: mod_base = OTHER; note = cm
  modified_base 14: mod_base = OTHER; note = um
  modified_base 17: mod_base = OTHER; note = um
  modified_base 18: mod_base = OTHER; note = um
  modified_base 1^2: mod_base = OTHER; note = phosphorothioate bond between nucleotides
accaaaacctggctggttgga

SEQ ID NO: 1221 - RNA, 21 nt, synthetic construct
  source 1..21: mol_type = other RNA
  modified_base 1: mod_base = OTHER; note = 5'-O-methyladenosine
  modified_base 2: mod_base = OTHER; note = cm
  modified_base 3: mod_base = OTHER; note = cm
  modified_base 8: mod_base = OTHER; note = cm
  modified_base 9: mod_base = OTHER; note = cm
  modified_base 10: mod_base = OTHER; note = um
  modified_base 13: mod_base = OTHER; note = cm
  modified_base 14: mod_base = OTHER; note = um
  modified_base 17: mod_base = OTHER; note = um
  modified_base 18: mod_base = OTHER; note = um
  modified_base 1^2: mod_base = OTHER; note = phosphorothioate bond between nucleotides
accaaaacctggctggttgga

SEQ ID NO: 1222 - RNA, 21 nt, synthetic construct
  source 1..21: mol_type = other RNA
  modified_base 1: mod_base = OTHER; note = 2'-O-methyladenosine
  modified_base 2: mod_base = OTHER; note = 2'-deoxy-2'-fluorocytidine
  modified_base 3: mod_base = OTHER; note = cm
  modified_base 4: mod_base = OTHER; note = 2'-deoxy-2'-fluoroadenosine
  modified_base 5: mod_base = OTHER; note = 2'-O-methyladenosine
  modified_base 6: mod_base = OTHER; note = 2'-deoxy-2'-fluoroadenosine
  modified_base 8: mod_base = OTHER; note = 2'-deoxy-2'-fluorocytidine
  modified_base 1^2: mod_base = OTHER; note = phosphorothioate bond between nucleotides
accaaaacctggctggttgga

SEQ ID NO: 1223 - RNA, 21 nt, synthetic construct
  source 1..21: mol_type = other RNA
  modified_base 1: mod_base = OTHER; note = 2'-O-methyladenosine
  modified_base 3: mod_base = OTHER; note = cm
  modified_base 5: mod_base = OTHER; note = 2'-O-methyladenosine
  modified_base 7: mod_base = OTHER; note = 2'-O-methyladenosine
  modified_base 9: mod_base = OTHER; note = cm
  modified_base 11: mod_base = OTHER; note = gm
  modified_base 13: mod_base = OTHER; note = cm
  modified_base 15: mod_base = OTHER; note = gm
  modified_base 17: mod_base = OTHER; note = um
  modified_base 19: mod_base = OTHER; note = gm
  modified_base 21: mod_base = OTHER; note = 2'-O-methyladenosine
  modified_base 1^2: mod_base = OTHER; note = phosphorothioate bond between nucleotides
accaaaacctggctggttgga

SEQ ID NO: 1224 - RNA, 21 nt, synthetic construct
  source 1..21: mol_type = other RNA
  modified_base 3: mod_base = OTHER; note = 2'-deoxy-2'-fluorocytidine
  modified_base 14: mod_base = OTHER; note = 2'-deoxy-2'-fluorouridine
  modified_base 17: mod_base = OTHER; note = 2'-deoxy-2'-fluorouridine
  modified_base 18: mod_base = OTHER; note = 2'-deoxy-2'-fluorouridine
  modified_base 1^2: mod_base = OTHER; note = phosphorothioate bond between nucleotides
accaaaacctggctggttgga

SEQ ID NO: 1225 - RNA, 23 nt, synthetic construct
  source 1..23: mol_type = other RNA
  modified_base 1: mod_base = OTHER; note = abasic site of inverted abasic deoxyribose
  modified_base 4: mod_base = OTHER; note = 2'-deoxy-2'-fluorocytidine
  modified_base 15: mod_base = OTHER; note = 2'-deoxy-2'-fluorouridine
  modified_base 18: mod_base = OTHER; note = 2'-deoxy-2'-fluorouridine
  modified_base 19: mod_base = OTHER; note = 2'-deoxy-2'-fluorouridine
  modified_base 23: mod_base = OTHER; note = abasic site of inverted abasic deoxyribose
  modified_base 2^3: mod_base = OTHER; note = phosphorothioate bond between nucleotides
naccaaaacctggctggttggan

SEQ ID NO: 1226 - RNA, 21 nt, synthetic construct
  source 1..21: mol_type = other RNA
  modified_base 2: mod_base = OTHER; note = cm
  modified_base 3: mod_base = OTHER; note = cm
  modified_base 8: mod_base = OTHER; note = cm
  modified_base 9: mod_base = OTHER; note = cm
  modified_base 10: mod_base = OTHER; note = um
  modified_base 17: mod_base = OTHER; note = um
  modified_base 18: mod_base = OTHER; note = um
  modified_base 1^2: mod_base = OTHER; note = phosphorothioate bond between nucleotides
accaaaacctggctggttgga

SEQ ID NO: 1227 - RNA, 21 nt, synthetic construct
  source 1..21: mol_type = other RNA
  modified_base 3: mod_base = OTHER; note = cm
  modified_base 14: mod_base = OTHER; note = um
  modified_base 18: mod_base = OTHER; note = um
  modified_base 20^21: mod_base = OTHER; note = phosphorothioate bond between nucleotides
accaaaacctggctggttgga

SEQ ID NO: 1228 - DNA, 21 bp, synthetic construct
  source 1..21: mol_type = other DNA
  misc_feature 1..6: note = DNA
  misc_feature 7..17: note = RNA
  misc_feature 18..21: note = DNA
  modified_base 7: mod_base = OTHER; note = 2'-O-methyladenosine
  modified_base 8: mod_base = OTHER; note = cm
  modified_base 9: mod_base = OTHER; note = cm
  modified_base 10: mod_base = OTHER; note = um
  modified_base 11: mod_base = OTHER; note = gm
  modified_base 12: mod_base = OTHER; note = gm
  modified_base 13: mod_base = OTHER; note = cm
  modified_base 14: mod_base = OTHER; note = um
  modified_base 15: mod_base = OTHER; note = gm
  modified_base 16: mod_base = OTHER; note = gm
  modified_base 17: mod_base = OTHER; note = um
  modified_base 18: mod_base = i
  modified_base 1^2: mod_base = OTHER; note = phosphorothioate bond between nucleotides
accaaaacctggctggtngga

SEQ ID NO: 1229 - RNA, 21 nt, synthetic construct
  source 1..21: mol_type = other RNA
  modified_base 1: mod_base = OTHER; note = Unlocked nucleic acid (UNA) monomer
  modified_base 2: mod_base = OTHER; note = cm
  modified_base 3: mod_base = OTHER; note = cm
  modified_base 8: mod_base = OTHER; note = cm
  modified_base 9: mod_base = OTHER; note = cm
  modified_base 10: mod_base = OTHER; note = um
  modified_base 13: mod_base = OTHER; note = cm
  modified_base 14: mod_base = OTHER; note = um
  modified_base 17: mod_base = OTHER; note = um
  modified_base 18: mod_base = OTHER; note = um
  modified_base 1^2: mod_base = OTHER; note = phosphorothioate bond between nucleotides
accaaaacctggctggttgga

SEQ ID NO: 1230 - RNA, 21 nt, synthetic construct
  source 1..21: mol_type = other RNA
  modified_base 1: mod_base = OTHER; note = Unlocked nucleic acid (UNA) monomer
  modified_base 2: mod_base = OTHER; note = cm
  modified_base 3: mod_base = OTHER; note = cm
  modified_base 8: mod_base = OTHER; note = cm
  modified_base 9: mod_base = OTHER; note = cm
  modified_base 10: mod_base = OTHER; note = um
  modified_base 13: mod_base = OTHER; note = cm
  modified_base 14: mod_base = OTHER; note = um
  modified_base 17: mod_base = OTHER; note = um
  modified_base 18: mod_base = OTHER; note = um
  modified_base 1^2: mod_base = OTHER; note = phosphorothioate bond between nucleotides
accaaaacctggctggttgga

SEQ ID NO: 1231 - RNA, 21 nt, synthetic construct
  source 1..21: mol_type = other RNA
  modified_base 1: mod_base = OTHER; note = Unlocked nucleic acid (UNA) monomer
  modified_base 2: mod_base = OTHER; note = cm
  modified_base 3: mod_base = OTHER; note = cm
  modified_base 8: mod_base = OTHER; note = cm
  modified_base 9: mod_base = OTHER; note = cm
  modified_base 10: mod_base = OTHER; note = um
  modified_base 13: mod_base = OTHER; note = cm
  modified_base 14: mod_base = OTHER; note = um
  modified_base 17: mod_base = OTHER; note = um
  modified_base 18: mod_base = OTHER; note = um
  modified_base 1^2: mod_base = OTHER; note = phosphorothioate bond between nucleotides
accaaaacctggctggttgga

SEQ ID NO: 1232 - RNA, 17 nt, synthetic construct
  source 1..17: mol_type = other RNA
  modified_base 1: mod_base = OTHER; note = gm
  modified_base 2: mod_base = OTHER; note = um
  modified_base 3: mod_base = OTHER; note = 2'-deoxy-2'-fluorocytidine
  modified_base 4: mod_base = OTHER; note = 2'-O-methyladenosine
  modified_base 5: mod_base = OTHER; note = 2'-deoxy-2'-fluorouridine
  modified_base 6: mod_base = OTHER; note = 2'-O-methyladenosine
  modified_base 7: mod_base = OTHER; note = 2'-deoxy-2'-fluoroguanosine
  modified_base 8: mod_base = OTHER; note = cm
  modified_base 9: mod_base = OTHER; note = 2'-deoxy-2'-fluorocytidine
  modified_base 10: mod_base = OTHER; note = 2'-O-methyladenosine
  modified_base 11: mod_base = OTHER; note = 2'-deoxy-2'-fluorouridine
  modified_base 12: mod_base = OTHER; note = gm
  modified_base 13: mod_base = OTHER; note = 2'-deoxy-2'-fluorouridine
  modified_base 14: mod_base = OTHER; note = gm
  modified_base 15: mod_base = OTHER; note = 2'-deoxy-2'-fluoroguanosine
  modified_base 16: mod_base = OTHER; note = um
  modified_base 17: mod_base = OTHER; note = 2'-deoxy-2'-fluorouridine
gtcatagccatgtggtt

SEQ ID NO: 1233 - RNA, 15 nt, synthetic construct
  source 1..15: mol_type = other RNA
  modified_base 1: mod_base = OTHER; note = cm
  modified_base 2: mod_base = OTHER; note = um
  modified_base 3: mod_base = OTHER; note = 2'-deoxy-2'-fluoroguanosine
  modified_base 4: mod_base = OTHER; note = cm
  modified_base 5: mod_base = OTHER; note = 2'-deoxy-2'-fluoroadenosine
  modified_base 6: mod_base = OTHER; note = gm
  modified_base 7: mod_base = OTHER; note = 2'-deoxy-2'-fluorouridine
  modified_base 8: mod_base = OTHER; note = gm
  modified_base 9: mod_base = OTHER; note = 2'-deoxy-2'-fluorocytidine
  modified_base 10: mod_base = OTHER; note = 2'-O-methyladenosine
  modified_base 11: mod_base = OTHER; note = 2'-deoxy-2'-fluoroguanosine
  modified_base 12: mod_base = OTHER; note = gm
  modified_base 13: mod_base = OTHER; note = 2'-deoxy-2'-fluoroadenosine
  modified_base 14: mod_base = OTHER; note = 2'-O-methyladenosine
  modified_base 15: mod_base = OTHER; note = 2'-deoxy-2'-fluoroadenosine
ctgcagtgcaggaaa

SEQ ID NO: 1234 - RNA, 15 nt, synthetic construct
  source 1..15: mol_type = other RNA
  modified_base 1: mod_base = OTHER; note = gm
  modified_base 2: mod_base = OTHER; note = um
  modified_base 3: mod_base = OTHER; note = 2'-deoxy-2'-fluorocytidine
  modified_base 4: mod_base = OTHER; note = 2'-O-methyladenosine
  modified_base 5: mod_base = OTHER; note = 2'-deoxy-2'-fluorouridine
  modified_base 6: mod_base = OTHER; note = 2'-O-methyladenosine
  modified_base 7: mod_base = OTHER; note = 2'-deoxy-2'-fluoroguanosine
  modified_base 8: mod_base = OTHER; note = cm
  modified_base 9: mod_base = OTHER; note = 2'-deoxy-2'-fluorocytidine
  modified_base 10: mod_base = OTHER; note = 2'-O-methyladenosine
  modified_base 11: mod_base = OTHER; note = 2'-deoxy-2'-fluorouridine
  modified_base 12: mod_base = OTHER; note = gm
  modified_base 13: mod_base = OTHER; note = 2'-deoxy-2'-fluorouridine
  modified_base 14: mod_base = OTHER; note = gm
  modified_base 15: mod_base = OTHER; note = 2'-deoxy-2'-fluoroguanosine
gtcatagccatgtgg

SEQ ID NO: 1235 - RNA, 19 nt, synthetic construct
  source 1..19: mol_type = other RNA
  modified_base 1: mod_base = OTHER; note = 2'-deoxy-2'-fluoroadenosine
  modified_base 2: mod_base = OTHER; note = 2'-deoxy-2'-fluoroadenosine
  modified_base 3: mod_base = OTHER; note = cm
  modified_base 4: mod_base = OTHER; note = 2'-deoxy-2'-fluorouridine
  modified_base 5: mod_base = OTHER; note = um
  modified_base 6: mod_base = OTHER; note = 2'-deoxy-2'-fluoroguanosine
  modified_base 7: mod_base = OTHER; note = gm
  modified_base 8: mod_base = OTHER; note = 2'-deoxy-2'-fluoroadenosine
  modified_base 9: mod_base = OTHER; note = gm
  modified_base 10: mod_base = OTHER; note = 2'-deoxy-2'-fluoroguanosine
  modified_base 11: mod_base = OTHER; note = gm
  modified_base 12: mod_base = OTHER; note = 2'-deoxy-2'-fluoroguanosine
  modified_base 13: mod_base = OTHER; note = um
  modified_base 14: mod_base = OTHER; note = 2'-deoxy-2'-fluorouridine
  modified_base 15: mod_base = OTHER; note = gm
  modified_base 16: mod_base = OTHER; note = 2'-deoxy-2'-fluoroguanosine
  modified_base 17: mod_base = OTHER; note = um
  modified_base 18: mod_base = OTHER; note = 2'-deoxy-2'-fluoroguanosine
  modified_base 19: mod_base = OTHER; note = um
aacttggaggggttggtgt

SEQ ID NO: 1236 - RNA, 19 nt, synthetic construct
  source 1..19: mol_type = other RNA
  modified_base 3: mod_base = OTHER; note = cm
  modified_base 4: mod_base = OTHER; note = um
  modified_base 5: mod_base = OTHER; note = um
  modified_base 13: mod_base = OTHER; note = um
  modified_base 14: mod_base = OTHER; note = um
  modified_base 17: mod_base = OTHER; note = um
  modified_base 19: mod_base = OTHER; note = um
aacttggaggggttggtgt

SEQ ID NO: 1237 - RNA, 19 nt, synthetic construct
  source 1..19: mol_type = other RNA
  modified_base 1: mod_base = OTHER; note = 2'-O-methyladenosine
  modified_base 2: mod_base = OTHER; note = cm
  modified_base 3: mod_base = OTHER; note = 2'-deoxy-2'-fluoroadenosine
  modified_base 4: mod_base = OTHER; note = cm
  modified_base 5: mod_base = OTHER; note = 2'-deoxy-2'-fluorocytidine
  modified_base 6: mod_base = OTHER; note = 2'-O-methyladenosine
  modified_base 7: mod_base = OTHER; note = 2'-deoxy-2'-fluoroadenosine
  modified_base 8: mod_base = OTHER; note = cm
  modified_base 9: mod_base = OTHER; note = 2'-deoxy-2'-fluorocytidine
  modified_base 10: mod_base = OTHER; note = cm
  modified_base 11: mod_base = OTHER; note = 2'-deoxy-2'-fluorocytidine
  modified_base 12: mod_base = OTHER; note = um
  modified_base 13: mod_base = OTHER; note = 2'-deoxy-2'-fluorocytidine
  modified_base 14: mod_base = OTHER; note = cm
  modified_base 15: mod_base = OTHER; note = 2'-deoxy-2'-fluoroadenosine
  modified_base 16: mod_base = OTHER; note = 2'-O-methyladenosine
  modified_base 17: mod_base = OTHER; note = 2'-deoxy-2'-fluoroguanosine
  modified_base 18: mod_base = OTHER; note = um
  modified_base 19: mod_base = OTHER; note = 2'-deoxy-2'-fluorouridine
acaccaacccctccaagtt

SEQ ID NO: 1238 - RNA, 19 nt, synthetic construct
  source 1..19: mol_type = other RNA
  modified_base 1: mod_base = OTHER; note = 2'-O-methyladenosine
  modified_base 2: mod_base = OTHER; note = cm
  modified_base 4: mod_base = OTHER; note = cm
  modified_base 5: mod_base = OTHER; note = cm
  modified_base 8: mod_base = OTHER; note = cm
  modified_base 9: mod_base = OTHER; note = cm
  modified_base 10: mod_base = OTHER; note = cm
  modified_base 11: mod_base = OTHER; note = cm
  modified_base 12: mod_base = OTHER; note = um
  modified_base 13: mod_base = OTHER; note = cm
  modified_base 14: mod_base = OTHER; note = cm
  modified_base 18: mod_base = OTHER; note = um
  modified_base 19: mod_base = OTHER; note = um
acaccaacccctccaagtt

SEQ ID NO: 1239 - RNA, 19 nt, synthetic construct
  source 1..19: mol_type = other RNA
  modified_base 1: mod_base = OTHER; note = 5'-E-vinylphosphonate-2'-O-methyl-uridine
  modified_base 6: mod_base = m5c
  modified_base 12: mod_base = m5c
tgtcacagtgacaagcttg

SEQ ID NO: 1240 - RNA, 20 nt, synthetic construct
  source 1..20: mol_type = other RNA
  modified_base 1: mod_base = OTHER; note = 5'-E-vinylphosphonate-2'-O-methyl-uridine
  modified_base 7: mod_base = m5c
  modified_base 13: mod_base = m5c
ttgtcacagtgacaagcttg

SEQ ID NO: 1241 - RNA, 19 nt, synthetic construct
  source 1..19: mol_type = other RNA
  modified_base 1: mod_base = OTHER; note = Unlocked nucleic acid (UNA) monomer
  modified_base 5: mod_base = cm
  modified_base 6: mod_base = um
  modified_base 7: mod_base = um
  modified_base 9: mod_base = um
  modified_base 10: mod_base = cm
  modified_base 12: mod_base = cm
  modified_base 13: mod_base = um
  modified_base 14: mod_base = gm
  modified_base 15: mod_base = um
  modified_base 18: mod_base = cm
  modified_base 1^2: mod_base = OTHER; note = phosphorothioate bond between nucleotides
caagcttgtcactgtgaca

SEQ ID NO: 1242 - RNA, 19 nt, synthetic construct
  source 1..19: mol_type = other RNA
  modified_base 1: mod_base = OTHER; note = Unlocked nucleic acid (UNA) monomer
  modified_base 5: mod_base = cm
  modified_base 6: mod_base = um
  modified_base 7: mod_base = um
  modified_base 9: mod_base = um
  modified_base 10: mod_base = cm
  modified_base 12: mod_base = cm
  modified_base 13: mod_base = um
  modified_base 14: mod_base = gm
  modified_base 15: mod_base = um
  modified_base 18: mod_base = cm
  modified_base 1^2: mod_base = OTHER; note = phosphorothioate bond between nucleotides
caagcttgtcactgtgaca

SEQ ID NO: 1243 - RNA, 19 nt, synthetic construct
  source 1..19: mol_type = other RNA
  modified_base 1: mod_base = OTHER; note = 5'-E-vinylphosphonate-2'-O-methyl-uridine
  modified_base 2: mod_base = OTHER; note = 2'-deoxy-2'-fluorocytidine
  modified_base 3: mod_base = cm
  modified_base 7: mod_base = gm
  modified_base 17: mod_base = cm
  modified_base 1^2: mod_base = OTHER; note = phosphorothioate bond between nucleotides
  modified_base 18^19: mod_base = OTHER; note = phosphorothioate bond between nucleotides
tccagagagattttggcac

SEQ ID NO: 1244 - RNA, 19 nt, synthetic construct
  source 1..19: mol_type = other RNA
  modified_base 1: mod_base = OTHER; note = 5'-O-methyl modified 2'-deoxyguanosine
  modified_base 2: mod_base = um
  modified_base 4: mod_base = cm
  modified_base 5: mod_base = cm
  modified_base 10: mod_base = um
  modified_base 11: mod_base = cm
  modified_base 12: mod_base = um
  modified_base 13: mod_base = cm
  modified_base 14: mod_base = um
  modified_base 15: mod_base = cm
  modified_base 16: mod_base = um
  modified_base 1^2: mod_base = OTHER; note = phosphorothioate bond between nucleotides
gtgccaaaatctctctgga

SEQ ID NO: 1245 - RNA, 21 nt, synthetic construct
  source 1..21: mol_type = other RNA
  modified_base 1: mod_base = OTHER; note = 2'-deoxy-2'-fluorocytidine
  modified_base 2: mod_base = OTHER; note = 2'-deoxy-2'-fluoroadenosine
  modified_base 3: mod_base = OTHER; note = 2'-O-methyladenosine
  modified_base 4: mod_base = OTHER; note = 2'-deoxy-2'-fluorocytidine
  modified_base 5: mod_base = OTHER; note = cm
  modified_base 6: mod_base = OTHER; note = 2'-deoxy-2'-fluoroadenosine
  modified_base 7: mod_base = OTHER; note = gm
  modified_base 8: mod_base = OTHER; note = 2'-deoxy-2'-fluorocytidine
  modified_base 9: mod_base = OTHER; note = cm
  modified_base 10: mod_base = OTHER; note = 2'-deoxy-2'-fluoroadenosine
  modified_base 11: mod_base = OTHER; note = gm
  modified_base 12: mod_base = OTHER; note = 2'-deoxy-2'-fluoroguanosine
  modified_base 13: mod_base = OTHER; note = um
  modified_base 14: mod_base = OTHER; note = 2'-deoxy-2'-fluorouridine
  modified_base 15: mod_base = OTHER; note = um
  modified_base 16: mod_base = OTHER; note = 2'-deoxy-2'-fluorouridine
  modified_base 17: mod_base = OTHER; note = gm
  modified_base 18: mod_base = OTHER; note = 2'-deoxy-2'-fluoroguanosine
  modified_base 19: mod_base = OTHER; note = um
  modified_base 20: mod_base = OTHER; note = 2'-deoxy-2'-fluorouridine
  modified_base 21: mod_base = OTHER; note = um
caaccagccaggttttggttt

SEQ ID NO: 1246 - RNA, 21 nt, synthetic construct
  source 1..21: mol_type = other RNA
  modified_base 1: mod_base = OTHER; note = 2'-deoxy-2'-fluorocytidine
  modified_base 2: mod_base = OTHER; note = 2'-deoxy-2'-fluoroadenosine
  modified_base 3: mod_base = OTHER; note = 2'-O-methyladenosine
  modified_base 4: mod_base = OTHER; note = 2'-deoxy-2'-fluorocytidine
  modified_base 5: mod_base = OTHER; note = cm
  modified_base 6: mod_base = OTHER; note = 2'-deoxy-2'-fluoroadenosine
  modified_base 7: mod_base = OTHER; note = gm
  modified_base 8: mod_base = OTHER; note = 2'-deoxy-2'-fluorocytidine
  modified_base 9: mod_base = OTHER; note = cm
  modified_base 10: mod_base = OTHER; note = 2'-deoxy-2'-fluoroadenosine
  modified_base 11: mod_base = OTHER; note = gm
  modified_base 12: mod_base = OTHER; note = 2'-deoxy-2'-fluoroguanosine
  modified_base 13: mod_base = OTHER; note = um
  modified_base 14: mod_base = OTHER; note = 2'-deoxy-2'-fluorouridine
  modified_base 15: mod_base = OTHER; note = um
  modified_base 16: mod_base = OTHER; note = 2'-deoxy-2'-fluorouridine
  modified_base 17: mod_base = OTHER; note = gm
  modified_base 18: mod_base = OTHER; note = 2'-deoxy-2'-fluoroguanosine
  modified_base 19: mod_base = OTHER; note = um
  modified_base 20: mod_base = OTHER; note = 2'-deoxy-2'-fluorouridine
  modified_base 21: mod_base = OTHER; note = um
  modified_base 1..3: mod_base = OTHER; note = phosphorothioate bond between nucleotides
  modified_base 19..21: mod_base = OTHER; note = phosphorothioate bond between nucleotides
caaccagccaggttttggttt

SEQ ID NO: 1247 - RNA, 21 nt, synthetic construct
  source 1..21: mol_type = other RNA
  modified_base 1: mod_base = OTHER; note = 2'-deoxy-2'-fluorocytidine
  modified_base 2: mod_base = OTHER; note = 2'-deoxy-2'-fluoroadenosine
  modified_base 3: mod_base = OTHER; note = 2'-O-methyladenosine
  modified_base 4: mod_base = OTHER; note = 2'-deoxy-2'-fluorocytidine
  modified_base 5: mod_base = OTHER; note = cm
  modified_base 6: mod_base = OTHER; note = 2'-deoxy-2'-fluoroadenosine
  modified_base 7: mod_base = OTHER; note = gm
  modified_base 8: mod_base = OTHER; note = 2'-deoxy-2'-fluorocytidine
  modified_base 9: mod_base = OTHER; note = cm
  modified_base 10: mod_base = OTHER; note = 2'-deoxy-2'-fluoroadenosine
  modified_base 11: mod_base = OTHER; note = gm
  modified_base 12: mod_base = OTHER; note = 2'-deoxy-2'-fluoroguanosine
  modified_base 13: mod_base = OTHER; note = um
  modified_base 14: mod_base = OTHER; note = 2'-deoxy-2'-fluorouridine
  modified_base 15: mod_base = OTHER; note = um
  modified_base 16: mod_base = OTHER; note = 2'-deoxy-2'-fluorouridine
  modified_base 17: mod_base = OTHER; note = gm
  modified_base 18: mod_base = OTHER; note = 2'-deoxy-2'-fluoroguanosine
  modified_base 19: mod_base = OTHER; note = um
  modified_base 20: mod_base = OTHER; note = 2'-deoxy-2'-fluorouridine
  modified_base 21: mod_base = OTHER; note = um
  modified_base 1^2: mod_base = OTHER; note = phosphorothioate bond between nucleotides
  modified_base 20^21: mod_base = OTHER; note = phosphorothioate bond between nucleotides
caaccagccaggttttggttt

SEQ ID NO: 1248 - RNA, 21 nt, synthetic construct
  source 1..21: mol_type = other RNA
  modified_base 1: mod_base = OTHER; note = 2'-deoxy-2'-fluorocytidine
  modified_base 2: mod_base = OTHER; note = 2'-deoxy-2'-fluoroadenosine
  modified_base 3: mod_base = OTHER; note = 2'-O-methyladenosine
  modified_base 4: mod_base = OTHER; note = 2'-deoxy-2'-fluorocytidine
  modified_base 5: mod_base = OTHER; note = cm
  modified_base 6: mod_base = OTHER; note = 2'-deoxy-2'-fluoroadenosine
  modified_base 7: mod_base = OTHER; note = gm
  modified_base 8: mod_base = OTHER; note = 2'-deoxy-2'-fluorocytidine
  modified_base 9: mod_base = OTHER; note = cm
  modified_base 10: mod_base = OTHER; note = 2'-deoxy-2'-fluoroadenosine
  modified_base 11: mod_base = OTHER; note = gm
  modified_base 12: mod_base = OTHER; note = 2'-deoxy-2'-fluoroguanosine
  modified_base 13: mod_base = OTHER; note = um
  modified_base 14: mod_base = OTHER; note = 2'-deoxy-2'-fluorouridine
  modified_base 15: mod_base = OTHER; note = um
  modified_base 16: mod_base = OTHER; note = 2'-deoxy-2'-fluorouridine
  modified_base 17: mod_base = OTHER; note = gm
  modified_base 18: mod_base = OTHER; note = 2'-deoxy-2'-fluoroguanosine
  modified_base 19: mod_base = OTHER; note = um
  modified_base 20: mod_base = OTHER; note = 2'-deoxy-2'-fluorouridine
  modified_base 21: mod_base = OTHER; note = um
  modified_base 20^21: mod_base = OTHER; note = phosphorothioate bond between nucleotides
caaccagccaggttttggttt

SEQ ID NO: 1249 - RNA, 21 nt, synthetic construct
  source 1..21: mol_type = other RNA
  modified_base 1: mod_base = OTHER; note = cm
  modified_base 5: mod_base = OTHER; note = cm
  modified_base 9: mod_base = OTHER; note = cm
  modified_base 20^21: mod_base = OTHER; note = phosphorothioate bond between nucleotides
caaccagccaggttttggttt

SEQ ID NO: 1250 - RNA, 21 nt, synthetic construct
  source 1..21: mol_type = other RNA
  modified_base 1: mod_base = OTHER; note = 5'-E-vinylphosphonate-2'-O-methyl-cytidine
  modified_base 5: mod_base = OTHER; note = cm
  modified_base 7: mod_base = OTHER; note = gm
  modified_base 9: mod_base = OTHER; note = cm
  modified_base 1..3: mod_base = OTHER; note = phosphorothioate bond between nucleotides
  modified_base 19..21: mod_base = OTHER; note = phosphorothioate bond between nucleotides
caaccagccaggttttggttt

SEQ ID NO: 1251 - RNA, 21 nt, synthetic construct
  source 1..21: mol_type = other RNA
  modified_base 1: mod_base = OTHER; note = 5'-E-vinylphosphonate-2'-O-methyl-cytidine
  modified_base 5: mod_base = OTHER; note = cm
  modified_base 7: mod_base = OTHER; note = gm
  modified_base 9: mod_base = OTHER; note = cm
  modified_base 1^2: mod_base = OTHER; note = phosphorothioate bond between nucleotides
  modified_base 20^21: mod_base = OTHER; note = phosphorothioate bond between nucleotides
caaccagccaggttttggttt

SEQ ID NO: 1252 - RNA, 21 nt, synthetic construct
  source 1..21: mol_type = other RNA
  modified_base 1: mod_base = OTHER; note = 5'-E-vinylphosphonate-2'-O-methyl-cytidine
  modified_base 5: mod_base = OTHER; note = cm
  modified_base 7: mod_base = OTHER; note = gm
  modified_base 9: mod_base = OTHER; note = cm
  modified_base 1..3: mod_base = OTHER; note = phosphorothioate bond between nucleotides
  modified_base 19..21: mod_base = OTHER; note = phosphorothioate bond between nucleotides
caaccagccaggttttggttt

SEQ ID NO: 1253 - RNA, 21 nt, synthetic construct
  source 1..21: mol_type = other RNA
  modified_base 1: mod_base = OTHER; note = 5'-E-vinylphosphonate-2'-O-methyl-cytidine
  modified_base 5: mod_base = OTHER; note = cm
  modified_base 7: mod_base = OTHER; note = gm
  modified_base 9: mod_base = OTHER; note = cm
  modified_base 1^2: mod_base = OTHER; note = phosphorothioate bond between nucleotides
  modified_base 20^21: mod_base = OTHER; note = phosphorothioate bond between nucleotides
caaccagccaggttttggttt

SEQ ID NO: 1254 - RNA, 21 nt, synthetic construct
  source 1..21: mol_type = other RNA
  modified_base 1: mod_base = OTHER; note = 5'-E-vinylphosphonate-2'-O-methyl-cytidine
  modified_base 5: mod_base = OTHER; note = cm
  modified_base 7: mod_base = OTHER; note = gm
  modified_base 9: mod_base = OTHER; note = cm
  modified_base 1..3: mod_base = OTHER; note = phosphorothioate bond between nucleotides
  modified_base 19..21: mod_base = OTHER; note = phosphorothioate bond between nucleotides
caaccagccaggttttggttt

SEQ ID NO: 1255 - RNA, 21 nt, synthetic construct
  source 1..21: mol_type = other RNA
  modified_base 1: mod_base = OTHER; note = 5'-E-vinylphosphonate-2'-O-methyl-cytidine
  modified_base 5: mod_base = OTHER; note = cm
  modified_base 7: mod_base = OTHER; note = gm
  modified_base 9: mod_base = OTHER; note = cm
  modified_base 1^2: mod_base = OTHER; note = phosphorothioate bond between nucleotides
  modified_base 20^21: mod_base = OTHER; note = phosphorothioate bond between nucleotides
caaccagccaggttttggttt

SEQ ID NO: 1256 - RNA, 21 nt, synthetic construct
  source 1..21: mol_type = other RNA
  modified_base 1: mod_base = OTHER; note = 2'-deoxy-2'-fluorocytidine
  modified_base 2: mod_base = OTHER; note = 2'-O-methyladenosine
  modified_base 5: mod_base = OTHER; note = 2'-deoxy-2'-fluorocytidine
  modified_base 6: mod_base = OTHER; note = 2'-O-methyladenosine
  modified_base 9: mod_base = OTHER; note = cm
  modified_base 16: mod_base = OTHER; note = um
  modified_base 19: mod_base = OTHER; note = um
  modified_base 21: mod_base = OTHER; note = um
  modified_base 20^21: mod_base = OTHER; note = phosphorothioate bond between nucleotides
caaccagccaggttttggttt

SEQ ID NO: 1257 - RNA, 21 nt, synthetic construct
  source 1..21: mol_type = other RNA
  modified_base 2: mod_base = OTHER; note = 2'-O-methyladenosine
  modified_base 4: mod_base = OTHER; note = cm
  modified_base 6: mod_base = OTHER; note = 2'-O-methyladenosine
  modified_base 8: mod_base = OTHER; note = cm
  modified_base 10: mod_base = OTHER; note = 2'-O-methyladenosine
  modified_base 12: mod_base = OTHER; note = gm
  modified_base 14: mod_base = OTHER; note = um
  modified_base 16: mod_base = OTHER; note = um
  modified_base 18: mod_base = OTHER; note = gm
  modified_base 20: mod_base = OTHER; note = um
  modified_base 20^21: mod_base = OTHER; note = phosphorothioate bond between nucleotides
caaccagccaggttttggttt

SEQ ID NO: 1258 - RNA, 21 nt, synthetic construct
  source 1..21: mol_type = other RNA
  modified_base 1: mod_base = OTHER; note = 2'-deoxy-2'-fluorocytidine
  modified_base 5: mod_base = OTHER; note = 2'-deoxy-2'-fluorocytidine
  modified_base 15: mod_base = OTHER; note = 2'-deoxy-2'-fluorouridine
  modified_base 16: mod_base = OTHER; note = 2'-deoxy-2'-fluorouridine
  modified_base 19: mod_base = OTHER; note = 2'-deoxy-2'-fluorouridine
  modified_base 21: mod_base = OTHER; note = 2'-deoxy-2'-fluorouridine
  modified_base 20^21: mod_base = OTHER; note = phosphorothioate bond between nucleotides
caaccagccaggttttggttt

SEQ ID NO: 1259 - RNA, 21 nt, synthetic construct
  source 1..21: mol_type = other RNA
  modified_base 6: mod_base = OTHER; note = 2'-O-methyladenosine
  modified_base 7: mod_base = OTHER; note = 2'-deoxy-2'-fluoroguanosine
  modified_base 8: mod_base = OTHER; note = 2'-deoxy-2'-fluorocytidine
  modified_base 12: mod_base = OTHER; note = gm
  modified_base 20^21: mod_base = OTHER; note = phosphorothioate bond between nucleotides
caaccagccaggttttggttt

SEQ ID NO: 1260 - RNA, 21 nt, synthetic construct
  source 1..21: mol_type = other RNA
  modified_base 2: mod_base = OTHER; note = 2'-O-methyladenosine
  modified_base 5: mod_base = OTHER; note = cm
  modified_base 20^21: mod_base = OTHER; note = phosphorothioate bond between nucleotides
caaccagccaggttttggttt

SEQ ID NO: 1261 - RNA, 21 nt, synthetic construct
  source 1..21: mol_type = other RNA
  modified_base 1: mod_base = OTHER; note = 2'-deoxy-2'-fluorocytidine
  modified_base 2: mod_base = OTHER; note = 2'-deoxy-2'-fluoroadenosine
  modified_base 4: mod_base = OTHER; note = 2'-deoxy-2'-fluorocytidine
  modified_base 5: mod_base = OTHER; note = 2'-deoxy-2'-fluorocytidine
  modified_base 9: mod_base = OTHER; note = cm
  modified_base 16: mod_base = OTHER; note = um
  modified_base 2^3: mod_base = OTHER; note = phosphorothioate bond between nucleotides
  modified_base 4..6: mod_base = OTHER; note = phosphorothioate bond between nucleotides
  modified_base 19..21: mod_base = OTHER; note = phosphorothioate bond between nucleotides
caaccagccaggttttggttt

SEQ ID NO: 1262 - RNA, 21 nt, synthetic construct
  source 1..21: mol_type = other RNA
  modified_base 1: mod_base = OTHER; note = 2'-deoxy-2'-fluorocytidine
  modified_base 20^21: mod_base = OTHER; note = phosphorothioate bond between nucleotides
caaccagccaggttttggttt

SEQ ID NO: 1263 - RNA, 21 nt, synthetic construct
  source 1..21: mol_type = other RNA
  modified_base 1: mod_base = OTHER; note = 5'-E-vinylphosphonate-2'-O-methyl-cytidine
  modified_base 8: mod_base = m5c
  modified_base 9: mod_base = m5c
  modified_base 20^21: mod_base = OTHER; note = phosphorothioate bond between nucleotides
caaccagccaggttttggttt

SEQ ID NO: 1264 - RNA, 21 nt, synthetic construct
  source 1..21: mol_type = other RNA
  modified_base 1: mod_base = OTHER; note = 5'-E-vinylphosphonate-2'-O-methyl-5-methylcytidine
  modified_base 4: mod_base = m5c
  modified_base 5: mod_base = m5c
  modified_base 8: mod_base = m5c
  modified_base 9: mod_base = m5c
  modified_base 20^21: mod_base = OTHER; note = phosphorothioate bond between nucleotides
caaccagccaggttttggttt

SEQ ID NO: 1265 - RNA, 21 nt, synthetic construct
  source 1..21: mol_type = other RNA
  modified_base 1: mod_base = OTHER; note = 5'-E-vinylphosphonate-2'-O-methyl-cytidine
  modified_base 13: mod_base = OTHER; note = m5u
  modified_base 15: mod_base = OTHER; note = m5u
  modified_base 16: mod_base = OTHER; note = m5u
  modified_base 19: mod_base = OTHER; note = m5u
  modified_base 20: mod_base = OTHER; note = m5u
  modified_base 21: mod_base = OTHER; note = m5u
  modified_base 20^21: mod_base = OTHER; note = phosphorothioate bond between nucleotides
caaccagccaggttttggttt

SEQ ID NO: 1266 - RNA, 19 nt, synthetic construct
  source 1..19: mol_type = other RNA
  modified_base 1: mod_base = OTHER; note = 2'-O-methyladenosine
  modified_base 2: mod_base = OTHER; note = cm
  modified_base 3: mod_base = OTHER; note = 2'-deoxy-2'-fluorocytidine
  modified_base 4: mod_base = OTHER; note = 2'-O-methyladenosine
  modified_base 5: mod_base = OTHER; note = 2'-deoxy-2'-fluoroadenosine
  modified_base 6: mod_base = OTHER; note = 2'-O-methyladenosine
  modified_base 7: mod_base = OTHER; note = 2'-deoxy-2'-fluoroadenosine
  modified_base 8: mod_base = OTHER; note = cm
  modified_base 9: mod_base = OTHER; note = 2'-deoxy-2'-fluorocytidine
  modified_base 10: mod_base = OTHER; note = um
  modified_base 11: mod_base = OTHER; note = 2'-deoxy-2'-fluoroguanosine
  modified_base 12: mod_base = OTHER; note = gm
  modified_base 13: mod_base = OTHER; note = 2'-deoxy-2'-fluorocytidine
  modified_base 14: mod_base = OTHER; note = um
  modified_base 15: mod_base = OTHER; note = 2'-deoxy-2'-fluoroguanosine
  modified_base 16: mod_base = OTHER; note = cm
  modified_base 17: mod_base = OTHER; note = 2'-deoxy-2'-fluoroadenosine
  modified_base 18: mod_base = OTHER; note = 2'-O-methyladenosine
  modified_base 19: mod_base = OTHER; note = 2'-deoxy-2'-fluorocytidine
accaaaacctggctgcaac

SEQ ID NO: 1267 - RNA, 19 nt, synthetic construct
  source 1..19: mol_type = other RNA
  modified_base 1: mod_base = OTHER; note = 2'-O-methyladenosine
  modified_base 2: mod_base = OTHER; note = cm
  modified_base 3: mod_base = OTHER; note = 2'-deoxy-2'-fluorocytidine
  modified_base 4: mod_base = OTHER; note = 2'-O-methyladenosine
  modified_base 5: mod_base = OTHER; note = 2'-deoxy-2'-fluoroadenosine
  modified_base 6: mod_base = OTHER; note = 2'-O-methyladenosine
  modified_base 7: mod_base = OTHER; note = 2'-deoxy-2'-fluoroadenosine
  modified_base 8: mod_base = OTHER; note = cm
  modified_base 9: mod_base = OTHER; note = 2'-deoxy-2'-fluorocytidine
  modified_base 10: mod_base = OTHER; note = um
  modified_base 11: mod_base = OTHER; note = 2'-deoxy-2'-fluoroguanosine
  modified_base 12: mod_base = OTHER; note = gm
  modified_base 13: mod_base = OTHER; note = 2'-deoxy-2'-fluorocytidine
  modified_base 14: mod_base = OTHER; note = um
  modified_base 15: mod_base = OTHER; note = 2'-deoxy-2'-fluoroguanosine
  modified_base 16: mod_base = OTHER; note = cm
  modified_base 17: mod_base = OTHER; note = 2'-deoxy-2'-fluoroadenosine
  modified_base 18: mod_base = OTHER; note = 2'-O-methyladenosine
  modified_base 19: mod_base = OTHER; note = 2'-deoxy-2'-fluorocytidine
  modified_base 1^2: mod_base = OTHER; note = phosphorothioate bond between nucleotides
accaaaacctggctgcaac

SEQ ID NO: 1268 - RNA, 19 nt, synthetic construct
  source 1..19: mol_type = other RNA
  modified_base 1: mod_base = OTHER; note = 2'-O-methyladenosine
  modified_base 2: mod_base = OTHER; note = cm
  modified_base 3: mod_base = OTHER; note = 2'-deoxy-2'-fluorocytidine
  modified_base 4: mod_base = OTHER; note = 2'-O-methyladenosine
  modified_base 5: mod_base = OTHER; note = 2'-deoxy-2'-fluoroadenosine
  modified_base 6: mod_base = OTHER; note = 2'-O-methyladenosine
  modified_base 7: mod_base = OTHER; note = 2'-deoxy-2'-fluoroadenosine
  modified_base 8: mod_base = OTHER; note = cm
  modified_base 9: mod_base = OTHER; note = 2'-deoxy-2'-fluorocytidine
  modified_base 10: mod_base = OTHER; note = um
  modified_base 11: mod_base = OTHER; note = 2'-deoxy-2'-fluoroguanosine
  modified_base 12: mod_base = OTHER; note = gm
  modified_base 13: mod_base = OTHER; note = 2'-deoxy-2'-fluorocytidine
  modified_base 14: mod_base = OTHER; note = um
  modified_base 15: mod_base = OTHER; note = 2'-deoxy-2'-fluoroguanosine
  modified_base 16: mod_base = OTHER; note = cm
  modified_base 17: mod_base = OTHER; note = 2'-deoxy-2'-fluoroadenosine
  modified_base 18: mod_base = OTHER; note = 2'-O-methyladenosine
  modified_base 19: mod_base = OTHER; note = 2'-deoxy-2'-fluorocytidine
  modified_base 1^2: mod_base = OTHER; note = phosphorothioate bond between nucleotides
accaaaacctggctgcaac

SEQ ID NO: 1269 - RNA, 19 nt, synthetic construct
  source 1..19: mol_type = other RNA
  modified_base 1: mod_base = OTHER; note = 2'-O-methyladenosine
  modified_base 2: mod_base = OTHER; note = cm
  modified_base 3: mod_base = OTHER; note = 2'-deoxy-2'-fluorocytidine
  modified_base 4: mod_base = OTHER; note = 2'-O-methyladenosine
  modified_base 5: mod_base = OTHER; note = 2'-deoxy-2'-fluoroadenosine
  modified_base 6: mod_base = OTHER; note = 2'-O-methyladenosine
  modified_base 7: mod_base = OTHER; note = 2'-deoxy-2'-fluoroadenosine
  modified_base 8: mod_base = OTHER; note = cm
  modified_base 9: mod_base = OTHER; note = 2'-deoxy-2'-fluorocytidine
  modified_base 10: mod_base = OTHER; note = um
  modified_base 11: mod_base = OTHER; note = 2'-deoxy-2'-fluoroguanosine
  modified_base 12: mod_base = OTHER; note = gm
  modified_base 13: mod_base = OTHER; note = 2'-deoxy-2'-fluorocytidine
  modified_base 14: mod_base = OTHER; note = um
  modified_base 15: mod_base = OTHER; note = 2'-deoxy-2'-fluoroguanosine
  modified_base 16: mod_base = OTHER; note = cm
  modified_base 17: mod_base = OTHER; note = 2'-deoxy-2'-fluoroadenosine
  modified_base 18: mod_base = OTHER; note = 2'-O-methyladenosine
  modified_base 19: mod_base = OTHER; note = 2'-deoxy-2'-fluorocytidine
  modified_base 1^2: mod_base = OTHER; note = phosphorothioate bond between nucleotides
accaaaacctggctgcaac

SEQ ID NO: 1270 - RNA, 19 nt, synthetic construct
  source 1..19: mol_type = other RNA
  modified_base 1: mod_base = OTHER; note = 2'-O-methyladenosine
  modified_base 2: mod_base = OTHER; note = cm
  modified_base 3: mod_base = OTHER; note = cm
  modified_base 8: mod_base = OTHER; note = cm
  modified_base 9: mod_base = OTHER; note = cm
  modified_base 10: mod_base = OTHER; note = um
  modified_base 13: mod_base = OTHER; note = cm
  modified_base 14: mod_base = OTHER; note = um
  modified_base 16: mod_base = OTHER; note = cm
  modified_base 19: mod_base = OTHER; note = cm
  modified_base 1^2: mod_base = OTHER; note = phosphorothioate bond between nucleotides
accaaaacctggctgcaac

SEQ ID NO: 1271 - RNA, 19 nt, synthetic construct
  source 1..19: mol_type = other RNA
  modified_base 1: mod_base = OTHER; note = 2'-O-methyladenosine
  modified_base 2: mod_base = OTHER; note = cm
  modified_base 3: mod_base = OTHER; note = cm
  modified_base 8: mod_base = OTHER; note = cm
  modified_base 9: mod_base = OTHER; note = cm
  modified_base 10: mod_base = OTHER; note = um
  modified_base 13: mod_base = OTHER; note = cm
  modified_base 14: mod_base = OTHER; note = um
  modified_base 16: mod_base = OTHER; note = cm
  modified_base 19: mod_base = OTHER; note = cm
  modified_base 1^2: mod_base = OTHER; note = phosphorothioate bond between nucleotides
accaaaacctggctgcaac

SEQ ID NO: 1272 - RNA, 19 nt, synthetic construct
  source 1..19: mol_type = other RNA
  modified_base 1: mod_base = OTHER; note = 2'-O-methyladenosine
  modified_base 2: mod_base = OTHER; note = cm
  modified_base 3: mod_base = OTHER; note = cm
  modified_base 8: mod_base = OTHER; note = cm
  modified_base 9: mod_base = OTHER; note = cm
  modified_base 10: mod_base = OTHER; note = um
  modified_base 13: mod_base = OTHER; note = cm
  modified_base 14: mod_base = OTHER; note = um
  modified_base 16: mod_base = OTHER; note = cm
  modified_base 19: mod_base = OTHER; note = cm
  modified_base 1^2: mod_base = OTHER; note = phosphorothioate bond between nucleotides
accaaaacctggctgcaac

SEQ ID NO: 1273 - RNA, 19 nt, synthetic construct
  source 1..19: mol_type = other RNA
  modified_base 1: mod_base = OTHER; note = Unlocked nucleic acid (UNA) monomer
  modified_base 2: mod_base = OTHER; note = cm
  modified_base 3: mod_base = OTHER; note = cm
  modified_base 8: mod_base = OTHER; note = cm
  modified_base 9: mod_base = OTHER; note = cm
  modified_base 10: mod_base = OTHER; note = um
  modified_base 13: mod_base = OTHER; note = cm
  modified_base 14: mod_base = OTHER; note = um
  modified_base 16: mod_base = OTHER; note = cm
  modified_base 19: mod_base = OTHER; note = cm
  modified_base 1^2: mod_base = OTHER; note = phosphorothioate bond between nucleotides
accaaaacctggctgcaac

SEQ ID NO: 1274 - RNA, 19 nt, synthetic construct
  source 1..19: mol_type = other RNA
  modified_base 1: mod_base = OTHER; note = Unlocked nucleic acid (UNA) monomer
  modified_base 2: mod_base = OTHER; note = cm
  modified_base 3: mod_base = OTHER; note = cm
  modified_base 8: mod_base = OTHER; note = cm
  modified_base 9: mod_base = OTHER; note = cm
  modified_base 10: mod_base = OTHER; note = um
  modified_base 13: mod_base = OTHER; note = cm
  modified_base 14: mod_base = OTHER; note = um
  modified_base 16: mod_base = OTHER; note = cm
  modified_base 19: mod_base = OTHER; note = cm
  modified_base 1^2: mod_base = OTHER; note = phosphorothioate bond between nucleotides
accaaaacctggctgcaac

SEQ ID NO: 1275 - RNA, 19 nt, synthetic construct
  source 1..19: mol_type = other RNA
  modified_base 1: mod_base = OTHER; note = 5'-O-methyladenosine
  modified_base 2: mod_base = OTHER; note = cm
  modified_base 3: mod_base = OTHER; note = cm
  modified_base 8: mod_base = OTHER; note = cm
  modified_base 9: mod_base = OTHER; note = cm
  modified_base 10: mod_base = OTHER; note = um
  modified_base 13: mod_base = OTHER; note = cm
  modified_base 14: mod_base = OTHER; note = um
  modified_base 16: mod_base = OTHER; note = cm
  modified_base 19: mod_base = OTHER; note = cm
  modified_base 1^2: mod_base = OTHER; note = phosphorothioate bond between nucleotides
accaaaacctggctgcaac

SEQ ID NO: 1276 - RNA, 19 nt, synthetic construct
  source 1..19: mol_type = other RNA
  modified_base 1: mod_base = OTHER; note = 5'-O-methyladenosine
  modified_base 2: mod_base = OTHER; note = cm
  modified_base 3: mod_base = OTHER; note = cm
  modified_base 8: mod_base = OTHER; note = cm
  modified_base 9: mod_base = OTHER; note = cm
  modified_base 10: mod_base = OTHER; note = um
  modified_base 13: mod_base = OTHER; note = cm
  modified_base 14: mod_base = OTHER; note = um
  modified_base 16: mod_base = OTHER; note = cm
  modified_base 19: mod_base = OTHER; note = cm
  modified_base 1^2: mod_base = OTHER; note = phosphorothioate bond between nucleotides
accaaaacctggctgcaac

SEQ ID NO: 1277 - RNA, 19 nt, synthetic construct
  source 1..19: mol_type = other RNA
  modified_base 1: mod_base = OTHER; note = 2'-O-methyladenosine
  modified_base 2: mod_base = OTHER; note = 2'-deoxy-2'-fluorocytidine
  modified_base 3: mod_base = OTHER; note = cm
  modified_base 4: mod_base = OTHER; note = 2'-deoxy-2'-fluoroadenosine
  modified_base 5: mod_base = OTHER; note = 2'-O-methyladenosine
  modified_base 6: mod_base = OTHER; note = 2'-deoxy-2'-fluoroadenosine
  modified_base 8: mod_base = OTHER; note = 2'-deoxy-2'-fluorocytidine
  modified_base 1^2: mod_base = OTHER; note = phosphorothioate bond between nucleotides
accaaaacctggctgcaac

SEQ ID NO: 1278 - RNA, 19 nt, synthetic construct
  source 1..19: mol_type = other RNA
  modified_base 1: mod_base = OTHER; note = 2'-O-methyladenosine
  modified_base 3: mod_base = OTHER; note = cm
  modified_base 5: mod_base = OTHER; note = 2'-deoxy-2'-fluoroadenosine
  modified_base 7: mod_base = OTHER; note = 2'-deoxy-2'-fluoroadenosine
  modified_base 9: mod_base = OTHER; note = cm
  modified_base 11: mod_base = OTHER; note = gm
  modified_base 13: mod_base = OTHER; note = cm
  modified_base 15: mod_base = OTHER; note = gm
  modified_base 17: mod_base = OTHER; note = 2'-O-methyladenosine
  modified_base 19: mod_base = OTHER; note = cm
  modified_base 1^2: mod_base = OTHER; note = phosphorothioate bond between nucleotides
accaaaacctggctgcaac

SEQ ID NO: 1279 - RNA, 19 nt, synthetic construct
  source 1..19: mol_type = other RNA
  modified_base 3: mod_base = OTHER; note = 2'-deoxy-2'-fluorocytidine
  modified_base 5: mod_base = OTHER; note = 2'-deoxy-2'-fluoroadenosine
  modified_base 14: mod_base = OTHER; note = 2'-deoxy-2'-fluorouridine
  modified_base 16: mod_base = OTHER; note = 2'-deoxy-2'-fluorocytidine
  modified_base 1^2: mod_base = OTHER; note = phosphorothioate bond between nucleotides
accaaaacctggctgcaac

SEQ ID NO: 1280 - RNA, 21 nt, synthetic construct
  source 1..21: mol_type = other RNA
  modified_base 1: mod_base = OTHER; note = abasic site of inverted abasic deoxyribose
  modified_base 4: mod_base = OTHER; note = 2'-deoxy-2'-fluorocytidine
  modified_base 15: mod_base = OTHER; note = 2'-deoxy-2'-fluorouridine
  modified_base 17: mod_base = OTHER; note = 2'-deoxy-2'-fluorocytidine
  modified_base 18: mod_base = OTHER; note = 2'-deoxy-2'-fluoroadenosine
  modified_base 21: mod_base = OTHER; note = abasic site of inverted abasic deoxyribose
  modified_base 2^3: mod_base = OTHER; note = phosphorothioate bond between nucleotides
naccaaaacctggctgcaacn

SEQ ID NO: 1281 - RNA, 19 nt, synthetic construct
  source 1..19: mol_type = other RNA
  modified_base 2: mod_base = OTHER; note = cm
  modified_base 3: mod_base = OTHER; note = cm
  modified_base 8: mod_base = OTHER; note = cm
  modified_base 13: mod_base = OTHER; note = cm
  modified_base 16: mod_base = OTHER; note = cm
  modified_base 19: mod_base = OTHER; note = cm
  modified_base 1^2: mod_base = OTHER; note = phosphorothioate bond between nucleotides
accaaaacctggctgcaac

SEQ ID NO: 1282 - RNA, 19 nt, synthetic construct
  source 1..19: mol_type = other RNA
  modified_base 3: mod_base = OTHER; note = cm
  modified_base 13: mod_base = OTHER; note = cm
  modified_base 16: mod_base = OTHER; note = cm
  modified_base 18^19: mod_base = OTHER; note = phosphorothioate bond between nucleotides
accaaaacctggctgcaac

SEQ ID NO: 1283 - DNA, 19 bp, synthetic construct
  source 1..19: mol_type = other DNA
  misc_feature 1..6: note = DNA
  misc_feature 7..14: note = RNA
  misc_feature 15..19: note = DNA
  modified_base 7: mod_base = OTHER; note = 2'-O-methyladenosine
  modified_base 8: mod_base = OTHER; note = cm
  modified_base 9: mod_base = OTHER; note = cm
  modified_base 10: mod_base = OTHER; note = um
  modified_base 11: mod_base = OTHER; note = gm
  modified_base 12: mod_base = OTHER; note = gm
  modified_base 13: mod_base = OTHER; note = cm
  modified_base 14: mod_base = OTHER; note = um
  modified_base 1^2: mod_base = OTHER; note = phosphorothioate bond between nucleotides
accaaaacctggctgcaac

SEQ ID NO: 1284 - RNA, 19 nt, synthetic construct
  source 1..19: mol_type = other RNA
  modified_base 1: mod_base = OTHER; note = Unlocked nucleic acid (UNA) monomer
  modified_base 2: mod_base = OTHER; note = cm
  modified_base 3: mod_base = OTHER; note = cm
  modified_base 8: mod_base = OTHER; note = cm
  modified_base 9: mod_base = OTHER; note = cm
  modified_base 10: mod_base = OTHER; note = um
  modified_base 13: mod_base = OTHER; note = cm
  modified_base 14: mod_base = OTHER; note = um
  modified_base 16: mod_base = OTHER; note = cm
  modified_base 19: mod_base = OTHER; note = cm
  modified_base 1^2: mod_base = OTHER; note = phosphorothioate bond between nucleotides
accaaaacctggctgcaac

SEQ ID NO: 1285 - RNA, 19 nt, synthetic construct
  source 1..19: mol_type = other RNA
  modified_base 1: mod_base = OTHER; note = Unlocked nucleic acid (UNA) monomer
  modified_base 2: mod_base = OTHER; note = cm
  modified_base 3: mod_base = OTHER; note = cm
  modified_base 8: mod_base = OTHER; note = cm
  modified_base 9: mod_base = OTHER; note = cm
  modified_base 10: mod_base = OTHER; note = um
  modified_base 13: mod_base = OTHER; note = cm
  modified_base 14: mod_base = OTHER; note = um
  modified_base 16: mod_base = OTHER; note = cm
  modified_base 19: mod_base = OTHER; note = cm
  modified_base 1^2: mod_base = OTHER; note = phosphorothioate bond between nucleotides
accaaaacctggctgcaac

SEQ ID NO: 1286 - RNA, 19 nt, synthetic construct
  source 1..19: mol_type = other RNA
  modified_base 1: mod_base = OTHER; note = Unlocked nucleic acid (UNA) monomer
  modified_base 2: mod_base = OTHER; note = cm
  modified_base 3: mod_base = OTHER; note = cm
  modified_base 8: mod_base = OTHER; note = cm
  modified_base 9: mod_base = OTHER; note = cm
  modified_base 10: mod_base = OTHER; note = um
  modified_base 13: mod_base = OTHER; note = cm
  modified_base 14: mod_base = OTHER; note = um
  modified_base 16: mod_base = OTHER; note = cm
  modified_base 19: mod_base = OTHER; note = cm
  modified_base 1^2: mod_base = OTHER; note = phosphorothioate bond between nucleotides
accaaaacctggctgcaac

SEQ ID NO: 1287 - DNA, 19 bp, synthetic construct
  source 1..19: mol_type = other DNA
caagcttgtcactgtgaca

SEQ ID NO: 1288 - DNA, 19 bp, synthetic construct
  source 1..19: mol_type = other DNA
accagctggctgatgagct

SEQ ID NO: 1289 - DNA, 19 bp, synthetic construct
  source 1..19: mol_type = other DNA
caaaacctggctggttgga

SEQ ID NO: 1290 - DNA, 19 bp, synthetic construct
  source 1..19: mol_type = other DNA
caagcttgtcactgtgacg

SEQ ID NO: 1291 - DNA, 19 bp, synthetic construct
  source 1..19: mol_type = other DNA
accagctggctgatgagcc

SEQ ID NO: 1292 - DNA, 19 bp, synthetic construct
  source 1..19: mol_type = other DNA
caaaacctggctggttggg

SEQ ID NO: 1293 - RNA, 19 nt, synthetic construct
  source 1..19: mol_type = other RNA
cgtcacagtgacaagcttg

SEQ ID NO: 1294 - RNA, 19 nt, synthetic construct
  source 1..19: mol_type = other RNA
ggctcatcagccagctggt

SEQ ID NO: 1295 - RNA, 19 nt, synthetic construct
  source 1..19: mol_type = other RNA
cccaaccagccaggttttg

SEQ ID NO: 1296 - RNA, 19 nt, synthetic construct
  source 1..19: mol_type = other RNA
caagcttgtcactgtgacg

SEQ ID NO: 1297 - RNA, 19 nt, synthetic construct
  source 1..19: mol_type = other RNA
accagctggctgatgagcc

SEQ ID NO: 1298 - RNA, 19 nt, synthetic construct
  source 1..19: mol_type = other RNA
caaaacctggctggttggg

SEQ ID NO: 1299 - RNA, 18 nt, synthetic construct
  source 1..18: mol_type = other RNA
gatccagtcactaattcc

SEQ ID NO: 1300 - RNA, 18 nt, synthetic construct
  source 1..18: mol_type = other RNA
tccagagagattttggca

SEQ ID NO: 1301 - RNA, 18 nt, synthetic construct
  source 1..18: mol_type = other RNA
tgaattcgcacatgctcc

SEQ ID NO: 1302 - RNA, 18 nt, synthetic construct
  source 1..18: mol_type = other RNA
agagagattttggcacac

SEQ ID NO: 1303 - RNA, 18 nt, synthetic construct
  source 1..18: mol_type = other RNA
gagagattttggcacact

SEQ ID NO: 1304 - RNA, 18 nt, synthetic construct
  source 1..18: mol_type = other RNA
cagagagattttggcaca

SEQ ID NO: 1305 - RNA, 18 nt, synthetic construct
  source 1..18: mol_type = other RNA
ggtccttggatccagtca

SEQ ID NO: 1306 - RNA, 18 nt, synthetic construct
  source 1..18: mol_type = other RNA
aattcgcacatgctccat

SEQ ID NO: 1307 - RNA, 18 nt, synthetic construct
  source 1..18: mol_type = other RNA
tcttccaccttcgagggt

SEQ ID NO: 1308 - RNA, 18 nt, synthetic construct
  source 1..18: mol_type = other RNA
atccagtcactaattccg

SEQ ID NO: 1309 - RNA, 18 nt, synthetic construct
  source 1..18: mol_type = other RNA
atgagtctcattgtagtc

SEQ ID NO: 1310 - RNA, 18 nt, synthetic construct
  source 1..18: mol_type = other RNA
cacatgctccatcattgg

SEQ ID NO: 1311 - RNA, 18 nt, synthetic construct
  source 1..18: mol_type = other RNA
ggatccagtcactaattc

SEQ ID NO: 1312 - RNA, 18 nt, synthetic construct
  source 1..18: mol_type = other RNA
tgaccacttcttcaaaag

SEQ ID NO: 1313 - RNA, 18 nt, synthetic construct
  source 1..18: mol_type = other RNA
ccagagagattttggcac

SEQ ID NO: 1314 - RNA, 18 nt, synthetic construct
  source 1..18: mol_type = other RNA
ccttggatccagtcacta

SEQ ID NO: 1315 - RNA, 18 nt, synthetic construct
  source 1..18: mol_type = other RNA
cttggatccagtcactaa

SEQ ID NO: 1316 - RNA, 18 nt, synthetic construct
  source 1..18: mol_type = other RNA
aaggtggtctttcttggc

SEQ ID NO: 1317 - RNA, 18 nt, synthetic construct
  source 1..18: mol_type = other RNA
tatgggagtaaaggcttg

SEQ ID NO: 1318 - RNA, 18 nt, synthetic construct
  source 1..18: mol_type = other RNA
agtaaaggcttgctttgg

SEQ ID NO: 1319 - RNA, 18 nt, synthetic construct
  source 1..18: mol_type = other RNA
tctatgggagtaaaggct

SEQ ID NO: 1320 - RNA, 18 nt, synthetic construct
  source 1..18: mol_type = other RNA
ttcaagaactccatctgc

SEQ ID NO: 1321 - RNA, 18 nt, synthetic construct
  source 1..18: mol_type = other RNA
agtctcattgtagtccat

SEQ ID NO: 1322 - RNA, 18 nt, synthetic construct
  source 1..18: mol_type = other RNA
tggatccagtcactaatt

SEQ ID NO: 1323 - RNA, 18 nt, synthetic construct
  source 1..18: mol_type = other RNA
ttggatccagtcactaat

SEQ ID NO: 1324 - RNA, 18 nt, synthetic construct
  source 1..18: mol_type = other RNA
tccttggatccagtcact

SEQ ID NO: 1325 - RNA, 18 nt, synthetic construct
  source 1..18: mol_type = other RNA
gtccttggatccagtcac

SEQ ID NO: 1326 - RNA, 18 nt, synthetic construct
  source 1..18: mol_type = other RNA
tggtccttggatccagtc

SEQ ID NO: 1327 - RNA, 18 nt, synthetic construct
  source 1..18: mol_type = other RNA
gcacatgctccatcattg

SEQ ID NO: 1328 - RNA, 18 nt, synthetic construct
  source 1..18: mol_type = other RNA
cgcacatgctccatcatt

SEQ ID NO: 1329 - RNA, 18 nt, synthetic construct
  source 1..18: mol_type = other RNA
tcgcacatgctccatcat

SEQ ID NO: 1330 - RNA, 18 nt, synthetic construct
  source 1..18: mol_type = other RNA
ttcgcacatgctccatca

SEQ ID NO: 1331 - RNA, 18 nt, synthetic construct
  source 1..18: mol_type = other RNA
attcgcacatgctccatc

SEQ ID NO: 1332 - RNA, 18 nt, synthetic construct
  source 1..18: mol_type = other RNA
gaattcgcacatgctcca

SEQ ID NO: 1333 - RNA, 18 nt, synthetic construct
  source 1..18: mol_type = other RNA
accttcgagggtccagtt

SEQ ID NO: 1334 - RNA, 18 nt, synthetic construct
  source 1..18: mol_type = other RNA
caccttcgagggtccagt

SEQ ID NO: 1335 - RNA, 18 nt, synthetic construct
  source 1..18: mol_type = other RNA
ccaccttcgagggtccag

SEQ ID NO: 1336 - RNA, 18 nt, synthetic construct
  source 1..18: mol_type = other RNA
tccaccttcgagggtcca

SEQ ID NO: 1337 - RNA, 18 nt, synthetic construct
  source 1..18: mol_type = other RNA
ttccaccttcgagggtcc

SEQ ID NO: 1338 - RNA, 18 nt, synthetic construct
  source 1..18: mol_type = other RNA
cttccaccttcgagggtc

SEQ ID NO: 1339 - RNA, 18 nt, synthetic construct
  source 1..18: mol_type = other RNA
ygtcacagtgacaagctt

SEQ ID NO: 1340 - RNA, 18 nt, synthetic construct
  source 1..18: mol_type = other RNA
caaccagccaggttttgg

SEQ ID NO: 1341 - RNA, 18 nt, synthetic construct
  source 1..18: mol_type = other RNA
ctcatcagccagctggtg

SEQ ID NO: 1342 - RNA, 18 nt, synthetic construct
  source 1..18: mol_type = other RNA
tgtctttcctgcactgca

SEQ ID NO: 1343 - RNA, 18 nt, synthetic construct
  source 1..18: mol_type = other RNA
tgaaccacatggctatga

SEQ ID NO: 1344 - RNA, 18 nt, synthetic construct
  source 1..18: mol_type = other RNA
rgctcatcagccagctgg

SEQ ID NO: 1345 - RNA, 18 nt, synthetic construct
  source 1..18: mol_type = other RNA
gtcacagtgacaagcttg

SEQ ID NO: 1346 - RNA, 18 nt, synthetic construct
  source 1..18: mol_type = other RNA
yccaaccagccaggtttt

SEQ ID NO: 1347 - RNA, 18 nt, synthetic construct
  source 1..18: mol_type = other RNA
aacttggaggggttggtg

SEQ ID NO: 1348 - RNA, 18 nt, synthetic construct
  source 1..18: mol_type = other RNA
acgtccagcaccttgatg

SEQ ID NO: 1349 - RNA, 18 nt, synthetic construct
  source 1..18: mol_type = other RNA
atgtctttcctgcactgc

SEQ ID NO: 1350 - RNA, 18 nt, synthetic construct
  source 1..18: mol_type = other RNA
tagaactgcctgttgatg

SEQ ID NO: 1351 - RNA, 18 nt, synthetic construct
  source 1..18: mol_type = other RNA
gctcatcagccagctggt

SEQ ID NO: 1352 - RNA, 18 nt, synthetic construct
  source 1..18: mol_type = other RNA
accagccaggttttggtc

SEQ ID NO: 1353 - RNA, 18 nt, synthetic construct
  source 1..18: mol_type = other RNA
aaccagccaggttttggt

SEQ ID NO: 1354 - RNA, 18 nt, synthetic construct
  source 1..18: mol_type = other RNA
ccaaccagccaggttttg

SEQ ID NO: 1355 - RNA, 18 nt, synthetic construct
  source 1..18: mol_type = other RNA
gacacctgctgcccagcc

SEQ ID NO: 1356 - RNA, 18 nt, synthetic construct
  source 1..18: mol_type = other RNA
tgccagcagtaggtgaac

SEQ ID NO: 1357 - RNA, 18 nt, synthetic construct
  source 1..18: mol_type = other RNA
atgccagcagtaggtgaa

SEQ ID NO: 1358 - RNA, 18 nt, synthetic construct
  source 1..18: mol_type = other RNA
tccttggtgggcatcagg

SEQ ID NO: 1359 - RNA, 18 nt, synthetic construct
  source 1..18: mol_type = other RNA
atccttggtgggcatcag

SEQ ID NO: 1360 - RNA, 18 nt, synthetic construct
  source 1..18: mol_type = other RNA
cggaagagcagggagtag

SEQ ID NO: 1361 - RNA, 18 nt, synthetic construct
  source 1..18: mol_type = other RNA
acggaagagcagggagta

SEQ ID NO: 1362 - RNA, 18 nt, synthetic construct
  source 1..18: mol_type = other RNA
ggggctgagcgggttctc

SEQ ID NO: 1363 - RNA, 18 nt, synthetic construct
  source 1..18: mol_type = other RNA
ggaattagtgactggatc

SEQ ID NO: 1364 - RNA, 18 nt, synthetic construct
  source 1..18: mol_type = other RNA
tgccaaaatctctctgga

SEQ ID NO: 1365 - RNA, 18 nt, synthetic construct
  source 1..18: mol_type = other RNA
ggagcatgtgcgaattca

SEQ ID NO: 1366 - RNA, 18 nt, synthetic construct
  source 1..18: mol_type = other RNA
gtgtgccaaaatctctct

SEQ ID NO: 1367 - RNA, 18 nt, synthetic construct
  source 1..18: mol_type = other RNA
agtgtgccaaaatctctc

SEQ ID NO: 1368 - RNA, 18 nt, synthetic construct
  source 1..18: mol_type = other RNA
tgtgccaaaatctctctg

SEQ ID NO: 1369 - RNA, 18 nt, synthetic construct
  source 1..18: mol_type = other RNA
tgactggatccaaggacc

SEQ ID NO: 1370 - RNA, 18 nt, synthetic construct
  source 1..18: mol_type = other RNA
atggagcatgtgcgaatt

SEQ ID NO: 1371 - RNA, 18 nt, synthetic construct
  source 1..18: mol_type = other RNA
accctcgaaggtggaaga

SEQ ID NO: 1372 - RNA, 18 nt, synthetic construct
  source 1..18: mol_type = other RNA
cggaattagtgactggat

SEQ ID NO: 1373 - RNA, 18 nt, synthetic construct
  source 1..18: mol_type = other RNA
gactacaatgagactcat

SEQ ID NO: 1374 - RNA, 18 nt, synthetic construct
  source 1..18: mol_type = other RNA
ccaatgatggagcatgtg

SEQ ID NO: 1375 - RNA, 18 nt, synthetic construct
  source 1..18: mol_type = other RNA
gaattagtgactggatcc

SEQ ID NO: 1376 - RNA, 18 nt, synthetic construct
  source 1..18: mol_type = other RNA
cttttgaagaagtggtca

SEQ ID NO: 1377 - RNA, 18 nt, synthetic construct
  source 1..18: mol_type = other RNA
gtgccaaaatctctctgg

SEQ ID NO: 1378 - RNA, 18 nt, synthetic construct
  source 1..18: mol_type = other RNA
tagtgactggatccaagg

SEQ ID NO: 1379 - RNA, 18 nt, synthetic construct
  source 1..18: mol_type = other RNA
ttagtgactggatccaag

SEQ ID NO: 1380 - RNA, 18 nt, synthetic construct
  source 1..18: mol_type = other RNA
gccaagaaagaccacctt

SEQ ID NO: 1381 - RNA, 18 nt, synthetic construct
  source 1..18: mol_type = other RNA
caagcctttactcccata

SEQ ID NO: 1382 - RNA, 18 nt, synthetic construct
  source 1..18: mol_type = other RNA
ccaaagcaagcctttact

SEQ ID NO: 1383 - RNA, 18 nt, synthetic construct
  source 1..18: mol_type = other RNA
agcctttactcccataga

SEQ ID NO: 1384 - RNA, 18 nt, synthetic construct
  source 1..18: mol_type = other RNA
gcagatggagttcttgaa

SEQ ID NO: 1385 - RNA, 18 nt, synthetic construct
  source 1..18: mol_type = other RNA
atggactacaatgagact

SEQ ID NO: 1386 - RNA, 18 nt, synthetic construct
  source 1..18: mol_type = other RNA
aattagtgactggatcca

SEQ ID NO: 1387 - RNA, 18 nt, synthetic construct
  source 1..18: mol_type = other RNA
attagtgactggatccaa

SEQ ID NO: 1388 - RNA, 18 nt, synthetic construct
  source 1..18: mol_type = other RNA
agtgactggatccaagga

SEQ ID NO: 1389 - RNA, 18 nt, synthetic construct
  source 1..18: mol_type = other RNA
gtgactggatccaaggac

SEQ ID NO: 1390 - RNA, 18 nt, synthetic construct
  source 1..18: mol_type = other RNA
gactggatccaaggacca

SEQ ID NO: 1391 - RNA, 18 nt, synthetic construct
  source 1..18: mol_type = other RNA
caatgatggagcatgtgc

SEQ ID NO: 1392 - RNA, 18 nt, synthetic construct
  source 1..18: mol_type = other RNA
aatgatggagcatgtgcg

SEQ ID NO: 1393 - RNA, 18 nt, synthetic construct
  source 1..18: mol_type = other RNA
atgatggagcatgtgcga

SEQ ID NO: 1394 - RNA, 18 nt, synthetic construct
  source 1..18: mol_type = other RNA
tgatggagcatgtgcgaa

SEQ ID NO: 1395 - RNA, 18 nt, synthetic construct
  source 1..18: mol_type = other RNA
gatggagcatgtgcgaat

SEQ ID NO: 1396 - RNA, 18 nt, synthetic construct
  source 1..18: mol_type = other RNA
tggagcatgtgcgaattc

SEQ ID NO: 1397 - RNA, 18 nt, synthetic construct
  source 1..18: mol_type = other RNA
aactggaccctcgaaggt

SEQ ID NO: 1398 - RNA, 18 nt, synthetic construct
  source 1..18: mol_type = other RNA
actggaccctcgaaggtg

SEQ ID NO: 1399 - RNA, 18 nt, synthetic construct
  source 1..18: mol_type = other RNA
ctggaccctcgaaggtgg

SEQ ID NO: 1400 - RNA, 18 nt, synthetic construct
  source 1..18: mol_type = other RNA
tggaccctcgaaggtgga

SEQ ID NO: 1401 - RNA, 18 nt, synthetic construct
  source 1..18: mol_type = other RNA
ggaccctcgaaggtggaa

SEQ ID NO: 1402 - RNA, 18 nt, synthetic construct
  source 1..18: mol_type = other RNA
gaccctcgaaggtggaag

SEQ ID NO: 1403 - RNA, 18 nt, synthetic construct
  source 1..18: mol_type = other RNA
aagcttgtcactgtgacr

SEQ ID NO: 1404 - RNA, 18 nt, synthetic construct
  source 1..18: mol_type = other RNA
ccaaaacctggctggttg

SEQ ID NO: 1405 - RNA, 18 nt, synthetic construct
  source 1..18: mol_type = other RNA
caccagctggctgatgag

SEQ ID NO: 1406 - RNA, 18 nt, synthetic construct
  source 1..18: mol_type = other RNA
tgcagtgcaggaaagaca

SEQ ID NO: 1407 - RNA, 18 nt, synthetic construct
  source 1..18: mol_type = other RNA
tcatagccatgtggttca

SEQ ID NO: 1408 - RNA, 18 nt, synthetic construct
  source 1..18: mol_type = other RNA
ccagctggctgatgagcy

SEQ ID NO: 1409 - RNA, 18 nt, synthetic construct
  source 1..18: mol_type = other RNA
caagcttgtcactgtgac

SEQ ID NO: 1410 - RNA, 18 nt, synthetic construct
  source 1..18: mol_type = other RNA
aaaacctggctggttggr

SEQ ID NO: 1411 - RNA, 18 nt, synthetic construct
  source 1..18: mol_type = other RNA
caccaacccctccaagtt

SEQ ID NO: 1412 - RNA, 18 nt, synthetic construct
  source 1..18: mol_type = other RNA
catcaaggtgctggacgt

SEQ ID NO: 1413 - RNA, 18 nt, synthetic construct
  source 1..18: mol_type = other RNA
gcagtgcaggaaagacat

SEQ ID NO: 1414 - RNA, 18 nt, synthetic construct
  source 1..18: mol_type = other RNA
catcaacaggcagttcta

SEQ ID NO: 1415 - RNA, 18 nt, synthetic construct
  source 1..18: mol_type = other RNA
accagctggctgatgagc

SEQ ID NO: 1416 - RNA, 18 nt, synthetic construct
  source 1..18: mol_type = other RNA
gaccaaaacctggctggt

SEQ ID NO: 1417 - RNA, 18 nt, synthetic construct
  source 1..18: mol_type = other RNA
accaaaacctggctggtt

SEQ ID NO: 1418 - RNA, 18 nt, synthetic construct
  source 1..18: mol_type = other RNA
caaaacctggctggttgg

SEQ ID NO: 1419 - RNA, 18 nt, synthetic construct
  source 1..18: mol_type = other RNA
ggctgggcagcaggtgtc

SEQ ID NO: 1420 - RNA, 18 nt, synthetic construct
  source 1..18: mol_type = other RNA
gttcacctactgctggca

SEQ ID NO: 1421 - RNA, 18 nt, synthetic construct
  source 1..18: mol_type = other RNA
ttcacctactgctggcat

SEQ ID NO: 1422 - RNA, 18 nt, synthetic construct
  source 1..18: mol_type = other RNA
cctgatgcccaccaagga

SEQ ID NO: 1423 - RNA, 18 nt, synthetic construct
  source 1..18: mol_type = other RNA
ctgatgcccaccaaggat

SEQ ID NO: 1424 - RNA, 18 nt, synthetic construct
  source 1..18: mol_type = other RNA
ctactccctgctcttccg

SEQ ID NO: 1425 - RNA, 18 nt, synthetic construct
  source 1..18: mol_type = other RNA
tactccctgctcttccgt

SEQ ID NO: 1426 - RNA, 18 nt, synthetic construct
  source 1..18: mol_type = other RNA
gagaacccgctcagcccc

SEQ ID NO: 1427 - RNA, 18 nt, synthetic construct
  source 1..18: mol_type = other RNA
  modified_base 3: mod_base = OTHER; note = cm
  modified_base 5: mod_base = OTHER; note = cm
  modified_base 11: mod_base = OTHER; note = cm
  modified_base 17^18: mod_base = OTHER; note = phosphorothioate bond between nucleotides
gtcacagtgacaagcttg

SEQ ID NO: 1428 - RNA, 18 nt, synthetic construct
  source 1..18: mol_type = other RNA
  modified_base 4: mod_base = OTHER; note = 2'-O-methyladenosine
  modified_base 6: mod_base = OTHER; note = 2'-deoxy-2'-fluoroadenosine
  modified_base 7: mod_base = OTHER; note = 2'-deoxy-2'-fluoroguanosine
  modified_base 12: mod_base = OTHER; note = 2'-O-methyladenosine
  modified_base 14: mod_base = OTHER; note = gm
  modified_base 18: mod_base = OTHER; note = gm
  modified_base 17^18: mod_base = OTHER; note = phosphorothioate bond between nucleotides
gtcacagtgacaagcttg

SEQ ID NO: 1429 - RNA, 18 nt, synthetic construct
  source 1..18: mol_type = other RNA
  modified_base 4: mod_base = OTHER; note = 2'-O-methyladenosine
  modified_base 6: mod_base = OTHER; note = 2'-deoxy-2'-fluoroadenosine
  modified_base 7: mod_base = OTHER; note = 2'-deoxy-2'-fluoroguanosine
  modified_base 12: mod_base = OTHER; note = 2'-O-methyladenosine
  modified_base 14: mod_base = OTHER; note = gm
  modified_base 18: mod_base = OTHER; note = gm
  modified_base 17^18: mod_base = OTHER; note = phosphorothioate bond between nucleotides
gtcacagtgacaagcttg

SEQ ID NO: 1430 - RNA, 19 nt, synthetic construct
  source 1..19: mol_type = other RNA
  modified_base 4: mod_base = OTHER; note = cm
  modified_base 6: mod_base = OTHER; note = cm
  modified_base 12: mod_base = OTHER; note = cm
  modified_base 18^19: mod_base = OTHER; note = phosphorothioate bond between nucleotides
cgtcacagtgacaagcttg

SEQ ID NO: 1431 - RNA, 19 nt, synthetic construct
  source 1..19: mol_type = other RNA
  modified_base 5: mod_base = OTHER; note = 2'-O-methyladenosine
  modified_base 7: mod_base = OTHER; note = 2'-deoxy-2'-fluoroadenosine
  modified_base 8: mod_base = OTHER; note = 2'-deoxy-2'-fluoroguanosine
  modified_base 13: mod_base = OTHER; note = 2'-O-methyladenosine
  modified_base 15: mod_base = OTHER; note = gm
  modified_base 19: mod_base = OTHER; note = gm
  modified_base 18^19: mod_base = OTHER; note = phosphorothioate bond between nucleotides
cgtcacagtgacaagcttg

SEQ ID NO: 1432 - RNA, 18 nt, synthetic construct
  source 1..18: mol_type = other RNA
  modified_base 1: mod_base = OTHER; note = cm
  modified_base 5: mod_base = OTHER; note = cm
  modified_base 6: mod_base = OTHER; note = um
  modified_base 7: mod_base = OTHER; note = um
  modified_base 9: mod_base = OTHER; note = um
  modified_base 10: mod_base = OTHER; note = cm
  modified_base 12: mod_base = OTHER; note = cm
  modified_base 13: mod_base = OTHER; note = um
  modified_base 14: mod_base = OTHER; note = gm
  modified_base 15: mod_base = OTHER; note = um
  modified_base 18: mod_base = OTHER; note = cm
  modified_base 1^2: mod_base = OTHER; note = phosphorothioate bond between nucleotides
caagcttgtcactgtgac

SEQ ID NO: 1433 - RNA, 19 nt, synthetic construct
  source 1..19: mol_type = other RNA
  modified_base 1: mod_base = OTHER; note = abasic site of inverted abasic deoxyribose
  modified_base 2^3: mod_base = OTHER; note = phosphorothioate bond between nucleotides
ncaagcttgtcactgtgac

SEQ ID NO: 1434 - RNA, 20 nt, synthetic construct
  source 1..20: mol_type = other RNA
  modified_base 1: mod_base = OTHER; note = abasic site of inverted abasic deoxyribose
  modified_base 20: mod_base = OTHER; note = abasic site of inverted abasic deoxyribose
  modified_base 2^3: mod_base = OTHER; note = phosphorothioate bond between nucleotides
ncaagcttgtcactgtgacn

SEQ ID NO: 1435 - RNA, 19 nt, synthetic construct
  source 1..19: mol_type = other RNA
  modified_base 1: mod_base = OTHER; note = cm
  modified_base 5: mod_base = OTHER; note = cm
  modified_base 6: mod_base = OTHER; note = um
  modified_base 7: mod_base = OTHER; note = um
  modified_base 9: mod_base = OTHER; note = um
  modified_base 10: mod_base = OTHER; note = cm
  modified_base 12: mod_base = OTHER; note = cm
  modified_base 13: mod_base = OTHER; note = um
  modified_base 14: mod_base = OTHER; note = gm
  modified_base 15: mod_base = OTHER; note = um
  modified_base 18: mod_base = OTHER; note = cm
  modified_base 1^2: mod_base = OTHER; note = phosphorothioate bond between nucleotides
caagcttgtcactgtgacg

SEQ ID NO: 1436 - RNA, 21 nt, synthetic construct
  source 1..21: mol_type = other RNA
  modified_base 1: mod_base = OTHER; note = abasic site of inverted abasic deoxyribose
  modified_base 21: mod_base = OTHER; note = abasic site of inverted abasic deoxyribose
  modified_base 2^3: mod_base = OTHER; note = phosphorothioate bond between nucleotides
ncaagcttgtcactgtgacgn